European Patent Application EP 4 364 808 A2, published May 8, 2024. Title: RNAI AGENTS FOR HEPATITIS B VIRUS INFECTION. Applicant: ARROWHEAD PHARMACEUTICALS, INC. Application EP. The sequence listing filed with the application follows.

SEQUENCE LISTING (334 sequences)

SEQ ID NO: 1 - DNA, 3221 bp, synthetic construct
  misc_feature 1..3221: note = Hepatitis B virus (subtype ADW2), genotype A, complete gene (AM282986.1)
  source 1..3221: mol_type = other DNA
ttccactgccttccaccaagctctgcaggatcccaaagtcaggggtctgtattttcctgctggtggctccagttcaggaacagtaaaccctgctccgaatattgcctctcacatctcgtcaatctccgcgaggactggggaccctgtgacgaatatggagaacatcacatcaggattcctaggacccctgctcgtgttacaggcggggtttttcttgttgacaagaatcctcacaataccgcagagtctagactcgtggtggacttctctcaattttctagggggatcacccgtgtgtcttggccaaaattcgcagtccccaacctccaatcactcaccaacctcctgtcctccaatttgtcctggttatcgctggatgtgtctgcggcgttttatcatattcctcttcatcctgctgctatgcctcatcttcttgttggttcttctggattatcaaggtatgttgcccgtttgtcctctaattccaggaacaacaacaaccagtacgggaccatgcaaaacctgcacgactcctgctcaaggcaactctatgtttccctcatgttgctgtacaaaaccttcggatggaaattgcacctgtattcccatcccatcgtcttgggctttcgcaaaatacctatgggagtgggcctcagtccgtttctcttggctcagtttactagtgccatttgttcagtggttcgtagggctttcccccactgtttggctttcagctatatggatgatgtggtattgggggccaagtctgtacagcatcgtgagtccctttataccgctgttaccaattttcttttgtctctgggtatacatttaaaccctaacaaaacaaaaagatggggttattccctaaacttcatgggttacataattggaagttggggaacgttgccacaggatcatattgtacaaaagatcaaacactgttttagaaaacttcctgttaacaggcctattgattggaaagtatgtcaaagaattgtgggtcttttgggctttgctgctccatttacacaatgtggatatcctgccttaatgcctttgtatgcctgtatacaagctaaacaggctttcactttctcgccaacttacaaggcctttctaagtaaacagtacatgaacctttaccccgttgctcggcaacggcctggtctgtgccaagtgtttgctgacgcaacccccactggctggggcttggccataggccatcagcgcatgcgtggaacctttgtggctcctctgccgatccatactgcggaactcctagccgcttgttttgctcgcagccggtctggggcaaagctcatcggaactgacaattctgtcgtcctctcgcggaaatatacatcgtttccatggctgctaggttgtactgccaactggatccttcgcgggacgtcctttgtttacgtcccgtcggcgctgaatcccgcggacgacccctctcggggccgcttgggactctctcgtccccttctccgtctgccgttccagccgaccacggggcgcacctctctttacgcggtctccccgtctgtgccttctcatctgccggtccgtgtgcacttcgcttcacctctgcacgttgcatggagaccaccgtgaacgcccatcagatcctgcccaaggtcttacataagaggactcttggactcccagcaatgtcaacgaccgaccttgaggcctacttcaaagactgtgtgtttaaggactgggaggagctgggggaggagattaggttaaaggtctttgtattaggaggctgtaggcataaattggtctgcgcaccagcaccatgcaactttttcacctctgcctaatcatctcttgtacatgtcccactgttcaagcctccaagctgtgccttgggtggctttggggcatggacattgacccttataaagaatttggagctactgtggagttactctcgtttttgccttctgacttttttccttccgtcagagatctcctagacaccgcctcagctctgtatcgggaagccttagagtctcctgagcattgctcacctcaccatactgcactcaggcaagcaattctctgctggggggaattgatgactctagctacctgggtgggtaataatttggaagatccagcatccagggatctagtagtcaattatgttaatactaacatgggtttaaagatcaggcaactattgtggtttcatatatcttgccttacttttggaagagagactgtacttgaatatttggtctctttcggagtgtggattcgcactcctccagcctatagaccaccaaatgcccctatcttatcaacacttccggaaactactgttgttagacgacgggaccgaggcaggtcccctagaagaagaactccctcgcctcgcagacgcagatctcaatcgccgcgtcgcagaagatctcaatctcgggaatctcaatgttagtattccttggactcataaggtgggaaactttactgggctttattcctctacagtacctatctttaatcctgaatggcaaactccttcctttcctaagattcatttacaagaggacattattaataggtgtcaacaatttgtgggccctctcactgtaaatgaaaagagaagattgaaattaattatgcctgctagattctatcctacccacactaaatatttgcccttagacaaaggaattaaaccttattatccagatcaggtagttaatcattacttcaaaaccagacattatttacatactctttggaaggctggtattctatataagagggaaaccacacgtagcgcatcattttgcgggtcaccatattcttgggaacaagagctacagcatgggaggttggtcatcgaaacctcgcaaaggcatggggacgaatctttctgttcccaaccctctgggattctttcccgatcatcagttggaccctgcattcggagccaactcaaacaatccagattgggacttcaaccccatcaaggaccactggccagcagccaaccaggtaggagtgggagcattcgggccagggttcacccctccacacggcggtgttttggggtggagccctcaggctcagggcatattgaccacagtgtcaacaattcctcctcctgcctccaccaatcggcagtcaggaaggcagcctactcccatctctccacctctaagagacagtcatcctcaggccatgcagtggaa

SEQ ID NO: 2 - DNA, 19 bp, synthetic construct
  misc_feature 1..19: note = HBV cDNA target sequence
  source 1..19: mol_type = other DNA
gtggtggacttctctcaat

SEQ ID NO: 3 - DNA, 19 bp, synthetic construct
  misc_feature 1..19: note = HBV cDNA target sequence
  source 1..19: mol_type = other DNA
tggtggacttctctcaatt

SEQ ID NO: 4 - DNA, 19 bp, synthetic construct
  misc_feature 1..19: note = HBV cDNA target sequence
  source 1..19: mol_type = other DNA
ggacttctctcaattttct

SEQ ID NO: 5 - DNA, 19 bp, synthetic construct
  misc_feature 1..19: note = HBV cDNA target sequence
  source 1..19: mol_type = other DNA
gctgtaggcataaattggt

SEQ ID NO: 6 - DNA, 19 bp, synthetic construct
  misc_feature 1..19: note = HBV cDNA target sequence
  source 1..19: mol_type = other DNA
ctgtaggcataaattggtc

SEQ ID NO: 7 - RNA, 19 nt, synthetic construct
  misc_feature 1..19: note = HBV RNAi agent antisense strand core stretch sequence
  source 1..19: mol_type = other RNA
attgagagaagtccaccac

SEQ ID NO: 8 - RNA, 19 nt, synthetic construct
  misc_feature 1..19: note = HBV RNAi agent antisense strand core stretch sequence
  source 1..19: mol_type = other RNA
tttgagagaagtccaccac

SEQ ID NO: 9 - RNA, 19 nt, synthetic construct
  misc_feature 1..19: note = HBV RNAi agent antisense strand core stretch sequence
  misc_difference 19: note = n = any nucleotide
  source 1..19: mol_type = other RNA
attgagagaagtccaccan

SEQ ID NO: 10 - RNA, 19 nt, synthetic construct
  misc_feature 1..19: note = HBV RNAi agent antisense strand core stretch sequence
  misc_difference 19: note = n = any nucleotide
  source 1..19: mol_type = other RNA
tttgagagaagtccaccan

SEQ ID NO: 11 - RNA, 19 nt, synthetic construct
  misc_feature 1..19: note = HBV RNAi agent antisense strand core stretch sequence
  misc_difference 1: note = n = any nucleotide
  misc_difference 19: note = n = any nucleotide
  source 1..19: mol_type = other RNA
nttgagagaagtccaccan

SEQ ID NO: 12 - RNA, 19 nt, synthetic construct
  misc_feature 1..19: note = HBV RNAi agent antisense strand core stretch sequence
  source 1..19: mol_type = other RNA
aattgagagaagtccacca

SEQ ID NO: 13 - RNA, 19 nt, synthetic construct
  misc_feature 1..19: note = HBV RNAi agent antisense strand core stretch sequence
  source 1..19: mol_type = other RNA
tattgagagaagtccacca

SEQ ID NO: 14 - RNA, 19 nt, synthetic construct
  misc_feature 1..19: note = HBV RNAi agent antisense strand core stretch sequence
  misc_difference 19: note = n = any nucleotide
  source 1..19: mol_type = other RNA
aattgagagaagtccaccn

SEQ ID NO: 15 - RNA, 19 nt, synthetic construct
  misc_feature 1..19: note = HBV RNAi agent antisense strand core stretch sequence
  misc_difference 19: note = n = any nucleotide
  source 1..19: mol_type = other RNA
tattgagagaagtccaccn

SEQ ID NO: 16 - RNA, 19 nt, synthetic construct
  misc_feature 1..19: note = HBV RNAi agent antisense strand core stretch sequence
  misc_difference 1: note = n = any nucleotide
  misc_difference 19: note = n = any nucleotide
  source 1..19: mol_type = other RNA
nattgagagaagtccaccn

SEQ ID NO: 17 - RNA, 19 nt, synthetic construct
  misc_feature 1..19: note = HBV RNAi agent antisense strand core stretch sequence
  source 1..19: mol_type = other RNA
agaaaattgagagaagtcc

SEQ ID NO: 18 - RNA, 19 nt, synthetic construct
  misc_feature 1..19: note = HBV RNAi agent antisense strand core stretch sequence
  source 1..19: mol_type = other RNA
tgaaaattgagagaagtcc

SEQ ID NO: 19 - RNA, 19 nt, synthetic construct
  misc_feature 1..19: note = HBV RNAi agent antisense strand core stretch sequence
  misc_difference 19: note = n = any nucleotide
  source 1..19: mol_type = other RNA
agaaaattgagagaagtcn

SEQ ID NO: 20 - RNA, 19 nt, synthetic construct
  misc_feature 1..19: note = HBV RNAi agent antisense strand core stretch sequence
  misc_difference 19: note = n = any nucleotide
  source 1..19: mol_type = other RNA
tgaaaattgagagaagtcn

SEQ ID NO: 21 - RNA, 19 nt, synthetic construct
  misc_feature 1..19: note = HBV RNAi agent antisense strand core stretch sequence
  misc_difference 1: note = n = any nucleotide
  misc_difference 19: note = n = any nucleotide
  source 1..19: mol_type = other RNA
ngaaaattgagagaagtcn

SEQ ID NO: 22 - RNA, 19 nt, synthetic construct
  misc_feature 1..19: note = HBV RNAi agent antisense strand core stretch sequence
  source 1..19: mol_type = other RNA
accaatttatgcctacagc

SEQ ID NO: 23 - RNA, 19 nt, synthetic construct
  misc_feature 1..19: note = HBV RNAi agent antisense strand core stretch sequence
  source 1..19: mol_type = other RNA
tccaatttatgcctacagc

SEQ ID NO: 24 - RNA, 19 nt, synthetic construct
  misc_feature 1..19: note = HBV RNAi agent antisense strand core stretch sequence
  misc_difference 19: note = n = any nucleotide
  source 1..19: mol_type = other RNA
accaatttatgcctacagn

SEQ ID NO: 25 - RNA, 19 nt, synthetic construct
  misc_feature 1..19: note = HBV RNAi agent antisense strand core stretch sequence
  misc_difference 19: note = n = any nucleotide
  source 1..19: mol_type = other RNA
tccaatttatgcctacagn

SEQ ID NO: 26 - RNA, 19 nt, synthetic construct
  misc_feature 1..19: note = HBV RNAi agent antisense strand core stretch sequence
  misc_difference 1: note = n = any nucleotide
  misc_difference 19: note = n = any nucleotide
  source 1..19: mol_type = other RNA
nccaatttatgcctacagn

SEQ ID NO: 27 - RNA, 19 nt, synthetic construct
  misc_feature 1..19: note = HBV RNAi agent antisense strand core stretch sequence
  source 1..19: mol_type = other RNA
gaccaatttatgcctacag

SEQ ID NO: 28 - RNA, 19 nt, synthetic construct
  misc_feature 1..19: note = HBV RNAi agent antisense strand core stretch sequence
  source 1..19: mol_type = other RNA
aaccaatttatgcctacag

SEQ ID NO: 29 - RNA, 19 nt, synthetic construct
  misc_feature 1..19: note = HBV RNAi agent antisense strand core stretch sequence
  source 1..19: mol_type = other RNA
taccaatttatgcctacag

SEQ ID NO: 30 - RNA, 19 nt, synthetic construct
  misc_feature 1..19: note = HBV RNAi agent antisense strand core stretch sequence
  misc_difference 19: note = n = any nucleotide
  source 1..19: mol_type = other RNA
gaccaatttatgcctacan

SEQ ID NO: 31 - RNA, 19 nt, synthetic construct
  misc_feature 1..19: note = HBV RNAi agent antisense strand core stretch sequence
  misc_difference 19: note = n = any nucleotide
  source 1..19: mol_type = other RNA
aaccaatttatgcctacan

SEQ ID NO: 32 - RNA, 19 nt, synthetic construct
  misc_feature 1..19: note = HBV RNAi agent antisense strand core stretch sequence
  misc_difference 19: note = n = any nucleotide
  source 1..19: mol_type = other RNA
taccaatttatgcctacan

SEQ ID NO: 33 - RNA, 19 nt, synthetic construct
  misc_feature 1..19: note = HBV RNAi agent antisense strand core stretch sequence
  misc_difference 1: note = n = any nucleotide
  misc_difference 19: note = n = any nucleotide
  source 1..19: mol_type = other RNA
naccaatttatgcctacan

SEQ ID NO: 34 - RNA, 19 nt, synthetic construct
  misc_feature 1..19: note = HBV RNAi agent sense strand core stretch sequence
  source 1..19: mol_type = other RNA
gtggtggacttctctcaat

SEQ ID NO: 35 - RNA, 19 nt, synthetic construct
  misc_feature 1..19: note = HBV RNAi agent sense strand core stretch sequence
  source 1..19: mol_type = other RNA
gtggtggacttctctcaaa

SEQ ID NO: 36 - RNA, 19 nt, synthetic construct
  misc_feature 1..19: note = HBV RNAi agent sense strand core stretch sequence
  misc_difference 1: note = n = any nucleotide
  source 1..19: mol_type = other RNA
ntggtggacttctctcaat

SEQ ID NO: 37 - RNA, 19 nt, synthetic construct
  misc_feature 1..19: note = HBV RNAi agent sense strand core stretch sequence
  misc_difference 1: note = n = any nucleotide
  source 1..19: mol_type = other RNA
ntggtggacttctctcaaa

SEQ ID NO: 38 - RNA, 19 nt, synthetic construct
  misc_feature 1..19: note = HBV RNAi agent sense strand core stretch sequence
  misc_difference 1: note = n = any nucleotide
  misc_difference 19: note = n = any nucleotide
  source 1..19: mol_type = other RNA
ntggtggacttctctcaan

SEQ ID NO: 39 - RNA, 19 nt, synthetic construct
  misc_feature 1..19: note = HBV RNAi agent sense strand core stretch sequence
  source 1..19: mol_type = other RNA
tggtggacttctctcaatt

SEQ ID NO: 40 - RNA, 19 nt, synthetic construct
  misc_feature 1..19: note = HBV RNAi agent sense strand core stretch sequence
  source 1..19: mol_type = other RNA
tggtggacttctctcaata

SEQ ID NO: 41 - RNA, 19 nt, synthetic construct
  misc_feature 1..19: note = HBV RNAi agent sense strand core stretch sequence
  misc_difference 1: note = n = any nucleotide
  source 1..19: mol_type = other RNA
nggtggacttctctcaatt

SEQ ID NO: 42 - RNA, 19 nt, synthetic construct
  misc_feature 1..19: note = HBV RNAi agent sense strand core stretch sequence
  misc_difference 1: note = n = any nucleotide
  source 1..19: mol_type = other RNA
nggtggacttctctcaata

SEQ ID NO: 43 - RNA, 19 nt, synthetic construct
  misc_feature 1..19: note = HBV RNAi agent sense strand core stretch sequence
  misc_difference 1: note = n = any nucleotide
  misc_difference 19: note = n = any nucleotide
  source 1..19: mol_type = other RNA
nggtggacttctctcaatn

SEQ ID NO: 44 - RNA, 19 nt, synthetic construct
  misc_feature 1..19: note = HBV RNAi agent sense strand core stretch sequence
  source 1..19: mol_type = other RNA
ggacttctctcaattttct

SEQ ID NO: 45 - RNA, 19 nt, synthetic construct
  misc_feature 1..19: note = HBV RNAi agent sense strand core stretch sequence
  source 1..19: mol_type = other RNA
ggacttctctcaattttca

SEQ ID NO: 46 - RNA, 19 nt, synthetic construct
  misc_feature 1..19: note = HBV RNAi agent sense strand core stretch sequence
  misc_difference 1: note = n = any nucleotide
  source 1..19: mol_type = other RNA
ngacttctctcaattttct

SEQ ID NO: 47 - RNA, 19 nt, synthetic construct
  misc_feature 1..19: note = HBV RNAi agent sense strand core stretch sequence
  misc_difference 1: note = n = any nucleotide
  source 1..19: mol_type = other RNA
ngacttctctcaattttca

SEQ ID NO: 48 - RNA, 19 nt, synthetic construct
  misc_feature 1..19: note = HBV RNAi agent sense strand core stretch sequence
  misc_difference 1: note = n = any nucleotide
  misc_difference 19: note = n = any nucleotide
  source 1..19: mol_type = other RNA
ngacttctctcaattttcn

SEQ ID NO: 49 - RNA, 19 nt, synthetic construct
  misc_feature 1..19: note = HBV RNAi agent sense strand core stretch sequence
  source 1..19: mol_type = other RNA
gctgtaggcataaattggt

SEQ ID NO: 50 - RNA, 19 nt, synthetic construct
  misc_feature 1..19: note = HBV RNAi agent sense strand core stretch sequence
  source 1..19: mol_type = other RNA
gctgtaggcataaattgga

SEQ ID NO: 51 - RNA, 19 nt, synthetic construct
  misc_feature 1..19: note = HBV RNAi agent sense strand core stretch sequence
  misc_difference 1: note = n = any nucleotide
  source 1..19: mol_type = other RNA
nctgtaggcataaattggt

SEQ ID NO: 52 - RNA, 19 nt, synthetic construct
  misc_feature 1..19: note = HBV RNAi agent sense strand core stretch sequence
  misc_difference 1: note = n = any nucleotide
  source 1..19: mol_type = other RNA
nctgtaggcataaattgga

SEQ ID NO: 53 - RNA, 19 nt, synthetic construct
  misc_feature 1..19: note = HBV RNAi agent sense strand core stretch sequence
  misc_difference 1: note = n = any nucleotide
  misc_difference 19: note = n = any nucleotide
  source 1..19: mol_type = other RNA
nctgtaggcataaattggn

SEQ ID NO: 54 - RNA, 19 nt, synthetic construct
  misc_feature 1..19: note = HBV RNAi agent sense strand core stretch sequence
  source 1..19: mol_type = other RNA
ctgtaggcataaattggtc

SEQ ID NO: 55 - RNA, 19 nt, synthetic construct
  misc_feature 1..19: note = HBV RNAi agent sense strand core stretch sequence
  source 1..19: mol_type = other RNA
ctgtaggcataaattggtt

SEQ ID NO: 56 - RNA, 19 nt, synthetic construct
  misc_feature 1..19: note = HBV RNAi agent sense strand core stretch sequence
  source 1..19: mol_type = other RNA
ctgtaggcataaattggta

SEQ ID NO: 57 - RNA, 19 nt, synthetic construct
  misc_feature 1..19: note = HBV RNAi agent sense strand core stretch sequence
  misc_difference 1: note = n = any nucleotide
  source 1..19: mol_type = other RNA
ntgtaggcataaattggtc

SEQ ID NO: 58 - RNA, 19 nt, synthetic construct
  misc_feature 1..19: note = HBV RNAi agent sense strand core stretch sequence
  misc_difference 1: note = n = any nucleotide
  source 1..19: mol_type = other RNA
ntgtaggcataaattggtt

SEQ ID NO: 59 - RNA, 19 nt, synthetic construct
  misc_feature 1..19: note = HBV RNAi agent sense strand core stretch sequence
  misc_difference 1: note = n = any nucleotide
  source 1..19: mol_type = other RNA
ntgtaggcataaattggta

SEQ ID NO: 60 - RNA, 19 nt, synthetic construct
  misc_feature 1..19: note = HBV RNAi agent sense strand core stretch sequence
  misc_difference 1: note = n = any nucleotide
  misc_difference 19: note = n = any nucleotide
  source 1..19: mol_type = other RNA
ntgtaggcataaattggtn

SEQ ID NO: 61 - RNA, 26 nt, synthetic construct
  modified_base 1: mod_base = OTHER; note = 2'-O-methyluridine-3'-phosphorothioate
  modified_base 2: mod_base = OTHER; note = 2'-fluoroadenosine-3'-phosporothioate
  modified_base 3: mod_base = OTHER; note = 2'-O-methylcytidine-3'-phosphate
  modified_base 4: mod_base = OTHER; note = 2'-fluorocytidine-3'-phosphate
  modified_base 5: mod_base = OTHER; note = 2'-O-methyladenosine-3'-phosphate
  modified_base 6: mod_base = OTHER; note = 2'-fluoroadenosine-3'-phosphate
  modified_base 7: mod_base = OTHER; note = 2'-O-methyluridine-3'-phosphate
  modified_base 8: mod_base = OTHER; note = 2'-fluorouridine-3'-phosphate
  modified_base 9: mod_base = OTHER; note = 2'-O-methyluridine-3'-phosphate
  modified_base 10: mod_base = OTHER; note = 2'-fluoroadenosine-3'-phosphate
  modified_base 11: mod_base = OTHER; note = 2'-O-methyluridine-3'-phosphate
  modified_base 12: mod_base = OTHER; note = 2'-fluoroguanosine-3'-phosphate
  modified_base 13: mod_base = OTHER; note = 2'-O-methylcytidine-3'-phosphate
  modified_base 14: mod_base = OTHER; note = 2'-fluorocytidine-3'-phosphate
  modified_base 15: mod_base = OTHER; note = 2'-O-methyluridine-3'-phosphate
  modified_base 16: mod_base = OTHER; note = 2'-fluoroadenosine-3'-phosphate
  modified_base 17: mod_base = OTHER; note = 2'-O-methylcytidine-3'-phosphate
  modified_base 18: mod_base = OTHER; note = 2'-fluoroadenosine-3'-phosphate
  modified_base 19: mod_base = OTHER; note = 2'-O-methylguanosine-3'-phosphate
  modified_base 20: mod_base = OTHER; note = 2'-fluoroguanosine-3'-phosphate
  modified_base 21: mod_base = OTHER; note = 2'-O-methylcytidine-3'-phosphate
  modified_base 22: mod_base = OTHER; note = 2'-O-methylcytidine-3'-phosphorothioate
  modified_base 23: mod_base = OTHER; note = 2'-O-methyluridine-3'-phosphorothioate
  modified_base 24: mod_base = OTHER; note = 2'-O-methyluridine-3'-phosphate
  modified_base 26: mod_base = OTHER; note = 2'-O-methyluridine-3'-phosphate
  misc_feature 1: note = RNA
  misc_feature 2: note = DNA
  misc_feature 3: note = RNA
  misc_feature 4: note = DNA
  misc_feature 5: note = RNA
  misc_feature 6: note = DNA
  misc_feature 7: note = RNA
  misc_feature 8: note = DNA
  misc_feature 9: note = RNA
  misc_feature 10: note = DNA
  misc_feature 11: note = RNA
  misc_feature 12: note = DNA
  misc_feature 13: note = RNA
  misc_feature 14: note = DNA
  misc_feature 15: note = RNA
  misc_feature 16: note = DNA
  misc_feature 17: note = RNA
  misc_feature 18: note = DNA
  misc_feature 19: note = RNA
  misc_feature 20: note = DNA
  misc_feature 21: note = RNA
  misc_feature 22: note = RNA
  misc_feature 23: note = RNA
  misc_feature 24: note = RNA
  misc_feature 26: note = RNA
  source 1..26: mol_type = other RNA
taccaatttatgcctacaggccttat

SEQ ID NO: 62 - RNA, 23 nt, synthetic construct
  modified_base 1: mod_base = OTHER; note = 2'-O-methyluridine-3'-phosphorothioate
  modified_base 2: mod_base = OTHER; note = 2'-fluoroadenosine-3'-phosporothioate
  modified_base 3: mod_base = OTHER; note = 2'-O-methylcytidine-3'-phosphate
  modified_base 4: mod_base = OTHER; note = 2'-fluorocytidine-3'-phosphate
  modified_base 5: mod_base = OTHER; note = 2'-O-methyladenosine-3'-phosphate
  modified_base 6: mod_base = OTHER; note = 2'-fluoroadenosine-3'-phosphate
  modified_base 7: mod_base = OTHER; note = 2'-O-methyluridine-3'-phosphate
  modified_base 8: mod_base = OTHER; note = 2'-fluorouridine-3'-phosphate
  modified_base 9: mod_base = OTHER; note = 2'-O-methyluridine-3'-phosphate
  modified_base 10: mod_base = OTHER; note = 2'-fluoroadenosine-3'-phosphate
  modified_base 11: mod_base = OTHER; note = 2'-O-methyluridine-3'-phosphate
  modified_base 12: mod_base = OTHER; note = 2'-fluoroguanosine-3'-phosphate
  modified_base 13: mod_base = OTHER; note = 2'-O-methylcytidine-3'-phosphate
  modified_base 14: mod_base = OTHER; note = 2'-fluorocytidine-3'-phosphate
  modified_base 15: mod_base = OTHER; note = 2'-O-methyluridine-3'-phosphate
  modified_base 16: mod_base = OTHER; note = 2'-fluoroadenosine-3'-phosphate
  modified_base 17: mod_base = OTHER; note = 2'-O-methylcytidine-3'-phosphate
  modified_base 18: mod_base = OTHER; note = 2'-fluoroadenosine-3'-phosphate
  modified_base 19: mod_base = OTHER; note = 2'-O-methylguanosine-3'-phosphate
  modified_base 20: mod_base = OTHER; note = 2'-fluoroguanosine-3'-phosphate
  modified_base 21: mod_base = OTHER; note = 2'-O-methylcytidine-3'-phosphorothioate
  modified_base 22: mod_base = OTHER; note = 2'-O-methylcytidine-3'-phosphorothioate
  modified_base 23: mod_base = OTHER; note = 2'-O-methyluridine-3'-phosphate
  misc_feature 1: note = RNA
  misc_feature 2: note = DNA
  misc_feature 3: note = RNA
  misc_feature 4: note = DNA
  misc_feature 5: note = RNA
  misc_feature 6: note = DNA
  misc_feature 7: note = RNA
  misc_feature 8: note = DNA
  misc_feature 9: note = RNA
  misc_feature 10: note = DNA
  misc_feature 11: note = RNA
  misc_feature 12: note = DNA
  misc_feature 13: note = RNA
  misc_feature 14: note = DNA
  misc_feature 15: note = RNA
  misc_feature 16: note = DNA
  misc_feature 17: note = RNA
  misc_feature 18: note = DNA
  misc_feature 19: note = RNA
  misc_feature 20: note = DNA
  misc_feature 21: note = RNA
  misc_feature 22: note = RNA
  misc_feature 23: note = RNA
  source 1..23: mol_type = other RNA
taccaatttatgcctacaggcct

SEQ ID NO: 63 - RNA, 23 nt, synthetic construct
  modified_base 1: mod_base = OTHER; note = 2'-O-methyluridine-3'-phosphorothioate
  modified_base 2: mod_base = OTHER; note = 2'-fluoroadenosine-3'-phosporothioate
  modified_base 3: mod_base = OTHER; note = 2'-O-methylcytidine-3'-phosphorothioate
  modified_base 4: mod_base = OTHER; note = 2'-fluorocytidine-3'-phosphate
  modified_base 5: mod_base = OTHER; note = 2'-O-methyladenosine-3'-phosphate
  modified_base 6: mod_base = OTHER; note = 2'-fluoroadenosine-3'-phosphate
  modified_base 7: mod_base = OTHER; note = 2'-O-methyluridine-3'-phosphate
  modified_base 8: mod_base = OTHER; note = 2'-fluorouridine-3'-phosphate
  modified_base 9: mod_base = OTHER; note = 2'-O-methyluridine-3'-phosphate
  modified_base 10: mod_base = OTHER; note = 2'-fluoroadenosine-3'-phosphate
  modified_base 11: mod_base = OTHER; note = 2'-O-methyluridine-3'-phosphate
  modified_base 12: mod_base = OTHER; note = 2'-fluoroguanosine-3'-phosphate
  modified_base 13: mod_base = OTHER; note = 2'-O-methylcytidine-3'-phosphate
  modified_base 14: mod_base = OTHER; note = 2'-fluorocytidine-3'-phosphate
  modified_base 15: mod_base = OTHER; note = 2'-O-methyluridine-3'-phosphate
  modified_base 16: mod_base = OTHER; note = 2'-fluoroadenosine-3'-phosphate
  modified_base 17: mod_base = OTHER; note = 2'-O-methylcytidine-3'-phosphate
  modified_base 18: mod_base = OTHER; note = 2'-fluoroadenosine-3'-phosphate
  modified_base 19: mod_base = OTHER; note = 2'-O-methylguanosine-3'-phosphate
  modified_base 20: mod_base = OTHER; note = 2'-fluoroguanosine-3'-phosphate
  modified_base 21: mod_base = OTHER; note = 2'-O-methylcytidine-3'-phosphate
  modified_base 22: mod_base = OTHER; note = 2'-O-methylcytidine-3'-phosphorothioate
  modified_base 23: mod_base = OTHER; note = 2'-O-methyluridine-3'-phosphate
  misc_feature 1: note = RNA
  misc_feature 2: note = DNA
  misc_feature 3: note = RNA
  misc_feature 4: note = DNA
  misc_feature 5: note = RNA
  misc_feature 6: note = DNA
  misc_feature 7: note = RNA
  misc_feature 8: note = DNA
  misc_feature 9: note = RNA
  misc_feature 10: note = DNA
  misc_feature 11: note = RNA
  misc_feature 12: note = DNA
  misc_feature 13: note = RNA
  misc_feature 14: note = DNA
  misc_feature 15: note = RNA
  misc_feature 16: note = DNA
  misc_feature 17: note = RNA
  misc_feature 18: note = DNA
  misc_feature 19: note = RNA
  misc_feature 20: note = DNA
  misc_feature 21: note = RNA
  misc_feature 22: note = RNA
  misc_feature 23: note = RNA
  source 1..23: mol_type = other RNA
taccaatttatgcctacaggcct

SEQ ID NO: 64 - RNA, 21 nt, synthetic construct
  modified_base 1: mod_base = OTHER; note = 2'-O-methyluridine-3'-phosphorothioate
  modified_base 2: mod_base = OTHER; note = 2'-fluoroadenosine-3'-phosporothioate
  modified_base 3: mod_base = OTHER; note = 2'-O-methylcytidine-3'-phosphorothioate
  modified_base 4: mod_base = OTHER; note = 2'-fluorocytidine-3'-phosphate
  modified_base 5: mod_base = OTHER; note = 2'-O-methyladenosine-3'-phosphate
  modified_base 6: mod_base = OTHER; note = 2'-fluoroadenosine-3'-phosphate
  modified_base 7: mod_base = OTHER; note = 2'-O-methyluridine-3'-phosphate
  modified_base 8: mod_base = OTHER; note = 2'-fluorouridine-3'-phosphate
  modified_base 9: mod_base = OTHER; note = 2'-O-methyluridine-3'-phosphate
  modified_base 10: mod_base = OTHER; note = 2'-fluoroadenosine-3'-phosphate
  modified_base 11: mod_base = OTHER; note = 2'-O-methyluridine-3'-phosphate
  modified_base 12: mod_base = OTHER; note = 2'-fluoroguanosine-3'-phosphate
  modified_base 13: mod_base = OTHER; note = 2'-O-methylcytidine-3'-phosphate
  modified_base 14: mod_base = OTHER; note = 2'-fluorocytidine-3'-phosphate
  modified_base 15: mod_base = OTHER; note = 2'-O-methyluridine-3'-phosphate
  modified_base 16: mod_base = OTHER; note = 2'-fluoroadenosine-3'-phosphate
  modified_base 17: mod_base = OTHER; note = 2'-O-methylcytidine-3'-phosphate
  modified_base 18: mod_base = OTHER; note = 2'-fluoroadenosine-3'-phosphate
  modified_base 19: mod_base = OTHER; note = 2'-O-methylguanosine-3'-phosphate
  modified_base 20: mod_base = OTHER; note = 2'-fluoroguanosine-3'-phosphorothioate
  modified_base 21: mod_base = OTHER; note = 2'-O-methylcytidine-3'-phosphate
  misc_feature 1: note = RNA
  misc_feature 2: note = DNA
  misc_feature 3: note = RNA
  misc_feature 4: note = DNA
  misc_feature 5: note = RNA
  misc_feature 6: note = DNA
  misc_feature 7: note = RNA
  misc_feature 8: note = DNA
  misc_feature 9: note = RNA
  misc_feature 10: note = DNA
  misc_feature 11: note = RNA
  misc_feature 12: note = DNA
  misc_feature 13: note = RNA
  misc_feature 14: note = DNA
  misc_feature 15: note = RNA
  misc_feature 16: note = DNA
  misc_feature 17: note = RNA
  misc_feature 18: note = DNA
  misc_feature 19: note = RNA
  misc_feature 20: note = DNA
  misc_feature 21: note = RNA
  source 1..21: mol_type = other RNA
taccaatttatgcctacaggc

SEQ ID NO: 65 - RNA, 21 nt, synthetic construct
  modified_base 1: mod_base = OTHER; note = 2'-O-methyluridine-3'-phosphorothioate
  modified_base 2: mod_base = OTHER; note = 2'-fluoroguanosine-3'-phosphorothioate
  modified_base 3: mod_base = OTHER; note = 2'-O-methyluridine-3'-phosphate
  modified_base 4: mod_base = OTHER; note = 2'-O-methylguanosine-3'-phosphate
  modified_base 5: mod_base = OTHER; note = 2'-O-methyladenosine-3'-phosphate
  modified_base 6: mod_base = OTHER; note = 2'-fluoroadenosine-3'-phosphate
  modified_base 7: mod_base = OTHER; note = 2'-O-methylguanosine-3'-phosphate
  modified_base 8: mod_base = OTHER; note = 2'-fluorocytidine-3'-phosphate
  modified_base 9: mod_base = OTHER; note = 2'-fluoroguanosine-3'-phosphate
  modified_base 10: mod_base = OTHER; note = 2'-O-methyladenosine-3'-phosphate
  modified_base 11: mod_base = OTHER; note = 2'-O-methyladenosine-3'-phosphate
  modified_base 12: mod_base = OTHER; note = 2'-O-methylguanosine-3'-phosphate
  modified_base 13: mod_base = OTHER; note = 2'-O-methyluridine-3'-phosphate
  modified_base 14: mod_base = OTHER; note = 2'-fluoroguanosine-3'-phosphate
  modified_base 15: mod_base = OTHER; note = 2'-O-methylcytidine-3'-phosphate
  modified_base 16: mod_base = OTHER; note = 2'-fluoroadenosine-3'-phosphate
  modified_base 17: mod_base = OTHER; note = 2'-O-methylcytidine-3'-phosphate
  modified_base 18: mod_base = OTHER; note = 2'-O-methyladenosine-3'-phosphate
  modified_base 19: mod_base = OTHER; note = 2'-O-methylcytidine-3'-phosphorothioate
  modified_base 20: mod_base = OTHER; note = 2'-O-methyluridine-3'-phosphorothioate
  modified_base 21: mod_base = OTHER; note = 2'-O-methyluridine-3'-phosphate
  misc_feature 1: note = RNA
  misc_feature 2: note = DNA
  misc_feature 3: note = RNA
  misc_feature 4: note = RNA
  misc_feature 5: note = RNA
  misc_feature 6: note = DNA
  misc_feature 7: note = RNA
  misc_feature 8: note = DNA
  misc_feature 9: note = DNA
  misc_feature 10: note = RNA
  misc_feature 11: note = RNA
  misc_feature 12: note = RNA
  misc_feature 13: note = RNA
  misc_feature 14: note = DNA
  misc_feature 15: note = RNA
  misc_feature 16: note = DNA
  misc_feature 17: note = RNA
  misc_feature 18: note = RNA
  misc_feature 19: note = RNA
  misc_feature 20: note = RNA
  misc_feature 21: note = RNA
  source 1..21: mol_type = other RNA
tgtgaagcgaagtgcacactt

SEQ ID NO: 66 - RNA, 26 nt, synthetic construct
  modified_base 1: mod_base = OTHER; note = 2'-O-methyluridine-3'-phosphorothioate
  modified_base 2: mod_base = OTHER; note = 2'-fluoroadenosine-3'-phosporothioate
  modified_base 3: mod_base = OTHER; note = 2'-O-methylcytidine-3'-phosphate
  modified_base 4: mod_base = OTHER; note = 2'-fluorocytidine-3'-phosphate
  modified_base 5: mod_base = OTHER; note = 2'-O-methyladenosine-3'-phosphate
  modified_base 6: mod_base = OTHER; note = 2'-fluoroadenosine-3'-phosphate
  modified_base 7: mod_base = OTHER; note = 2'-O-methyluridine-3'-phosphate
  modified_base 8: mod_base = OTHER; note = 2'-fluorouridine-3'-phosphate
  modified_base 9: mod_base = OTHER; note = 2'-O-methyluridine-3'-phosphate
  modified_base 10: mod_base = OTHER; note = 2'-fluoroadenosine-3'-phosphate
  modified_base 11: mod_base = OTHER; note = 2'-O-methyluridine-3'-phosphate
  modified_base 12: mod_base = OTHER; note = 2'-fluoroguanosine-3'-phosphate
  modified_base 13: mod_base = OTHER; note = 2'-O-methylcytidine-3'-phosphate
  modified_base 14: mod_base = OTHER; note = 2'-fluorocytidine-3'-phosphate
  modified_base 15: mod_base = OTHER; note = 2'-O-methyluridine-3'-phosphate
  modified_base 16: mod_base = OTHER; note = 2'-fluoroadenosine-3'-phosphate
  modified_base 17: mod_base = OTHER; note = 2'-O-methylcytidine-3'-phosphate
  modified_base 18: mod_base = OTHER; note = 2'-fluoroadenosine-3'-phosphate
  modified_base 19: mod_base = OTHER; note = 2'-O-methylguanosine-3'-phosphate
  modified_base 20: mod_base = OTHER; note = 2'-fluorocytidine-3'-phosphate
  modified_base 21: mod_base = OTHER; note = 2'-O-methylcytidine-3'-phosphorothioate
  modified_base 22: mod_base = OTHER; note = 2'-O-methyluridine-3'-phosphorothioate
  modified_base 23: mod_base = OTHER; note = 2'-O-methylcytidine-3'-phosphate
  modified_base 24: mod_base = OTHER; note = 2'-O-methylcytidine-3'-phosphate
  modified_base 25: mod_base = OTHER; note = 2'-O-methylguanosine-3'-phosphate
  modified_base 26: mod_base = OTHER; note = 2'-O-methylcytidine-3'-phosphate
  misc_feature 1: note = RNA
  misc_feature 2: note = DNA
  misc_feature 3: note = RNA
  misc_feature 4: note = DNA
  misc_feature 5: note = RNA
  misc_feature 6: note = DNA
  misc_feature 7: note = RNA
  misc_feature 8: note = DNA
  misc_feature 9: note = RNA
  misc_feature 10: note = DNA
  misc_feature 11: note = RNA
  misc_feature 12: note = DNA
  misc_feature 13: note = RNA
  misc_feature 14: note = DNA
  misc_feature 15: note = RNA
  misc_feature 16: note = DNA
  misc_feature 17: note = RNA
  misc_feature 18: note = DNA
  misc_feature 19: note = RNA
  misc_feature 20: note = DNA
  misc_feature 21: note = RNA
  misc_feature 22: note = RNA
  misc_feature 23: note = RNA
  misc_feature 24: note = RNA
  misc_feature 25: note = RNA
  misc_feature 26: note = RNA
  source 1..26: mol_type = other RNA
taccaatttatgcctacagcctccgc

SEQ ID NO: 67 - RNA, 26 nt, synthetic construct
  modified_base 1: mod_base = OTHER; note = vinyl phosphonate-2'-O-methyluridine-3'-phosphorothioate
  modified_base 2: mod_base = OTHER; note = 2'-fluoroadenosine-3'-phosporothioate
  modified_base 3: mod_base = OTHER; note = 2'-O-methylcytidine-3'-phosphate
  modified_base 4: mod_base = OTHER; note = 2'-fluorocytidine-3'-phosphate
  modified_base 5: mod_base = OTHER; note = 2'-O-methyladenosine-3'-phosphate
  modified_base 6: mod_base = OTHER; note = 2'-fluoroadenosine-3'-phosphate
  modified_base 7: mod_base = OTHER; note = 2'-O-methyluridine-3'-phosphate
  modified_base 8: mod_base = OTHER; note = 2'-fluorouridine-3'-phosphate
  modified_base 9: mod_base = OTHER; note = 2'-O-methyluridine-3'-phosphate
  modified_base 10: mod_base = OTHER; note = 2'-fluoroadenosine-3'-phosphate
  modified_base 11: mod_base = OTHER; note = 2'-O-methyluridine-3'-phosphate
  modified_base 12: mod_base = OTHER; note = 2'-fluoroguanosine-3'-phosphate
  modified_base 13: mod_base = OTHER; note = 2'-O-methylcytidine-3'-phosphate
  modified_base 14: mod_base = OTHER; note = 2'-fluorocytidine-3'-phosphate
  modified_base 15: mod_base = OTHER; note = 2'-O-methyluridine-3'-phosphate
  modified_base 16: mod_base = OTHER; note = 2'-fluoroadenosine-3'-phosphate
  modified_base 17: mod_base = OTHER; note = 2'-O-methylcytidine-3'-phosphate
  modified_base 18: mod_base = OTHER; note = 2'-fluoroadenosine-3'-phosphate
  modified_base 19: mod_base = OTHER; note = 2'-O-methylguanosine-3'-phosphate
  modified_base 20: mod_base = OTHER; note = 2'-fluorocytidine-3'-phosphate
  modified_base 21: mod_base = OTHER; note = 2'-O-methylcytidine-3'-phosphorothioate
  modified_base 22: mod_base = OTHER; note = 2'-O-methyluridine-3'-phosphorothioate
  modified_base 23: mod_base = OTHER; note = 2'-O-methylcytidine-3'-phosphate
  modified_base 24: mod_base = OTHER; note = 2'-O-methylcytidine-3'-phosphate
  modified_base 25: mod_base = OTHER; note = 2'-O-methylguanosine-3'-phosphate
  modified_base 26: mod_base = OTHER; note = 2'-O-methylcytidine-3'-phosphate
  misc_feature 1: note = RNA
  misc_feature 2: note = DNA
  misc_feature 3: note = RNA
  misc_feature 4: note = DNA
  misc_feature 5: note = RNA
  misc_feature 6: note = DNA
  misc_feature 7: note = RNA
  misc_feature 8: note = DNA
  misc_feature 9: note = RNA
  misc_feature 10: note = DNA
  misc_feature 11: note = RNA
  misc_feature 12: note = DNA
  misc_feature 13: note = RNA
  misc_feature 14: note = DNA
  misc_feature 15: note = RNA
  misc_feature 16: note = DNA
  misc_feature 17: note = RNA
  misc_feature 18: note = DNA
  misc_feature 19: note = RNA
  misc_feature 20: note = DNA
  misc_feature 21: note = RNA
  misc_feature 22: note = RNA
  misc_feature 23: note = RNA
  misc_feature 24: note = RNA
  misc_feature 25: note = RNA
  misc_feature 26: note = RNA
  source 1..26: mol_type = other RNA
taccaatttatgcctacagcctccgc

SEQ ID NO: 68 - RNA, 21 nt, synthetic construct
  modified_base 1: mod_base = OTHER; note = 2'-O-methyluridine-3'-phosphorothioate
  modified_base 2: mod_base = OTHER; note = 2'-fluoroadenosine-3'-phosporothioate
  modified_base 3: mod_base = OTHER; note = 2'-O-methylcytidine-3'-phosphorothioate
  modified_base 4: mod_base = OTHER; note = 2'-fluorocytidine-3'-phosphate
  modified_base 5: mod_base = OTHER; note = 2'-O-methyladenosine-3'-phosphate
  modified_base 6: mod_base = OTHER; note = 2'-fluoroadenosine-3'-phosphate
  modified_base 7: mod_base = OTHER; note = 2'-O-methyluridine-3'-phosphate
  modified_base 8: mod_base = OTHER; note = 2'-fluorouridine-3'-phosphate
  modified_base 9: mod_base = OTHER; note = 2'-O-methyluridine-3'-phosphate
  modified_base 10: mod_base = OTHER; note = 2'-fluoroadenosine-3'-phosphate
  modified_base 11: mod_base = OTHER; note = 2'-O-methyluridine-3'-phosphate
  modified_base 12: mod_base = OTHER; note = 2'-fluoroguanosine-3'-phosphate
  modified_base 13: mod_base = OTHER; note = 2'-O-methylcytidine-3'-phosphate
  modified_base 14: mod_base = OTHER; note = 2'-fluorocytidine-3'-phosphate
  modified_base 15: mod_base = OTHER; note = 2'-O-methyluridine-3'-phosphate
  modified_base 16: mod_base = OTHER; note = 2'-fluoroadenosine-3'-phosphate
  modified_base 17: mod_base = OTHER; note = 2'-O-methylcytidine-3'-phosphate
  modified_base 18: mod_base = OTHER; note = 2'-fluoroadenosine-3'-phosphate
  modified_base 19: mod_base = OTHER; note = 2'-O-methylguanosine-3'-phosphate
  modified_base 20: mod_base = OTHER; note = 2'-O-methyluridine-3'-phosphorothioate
  modified_base 21: mod_base = OTHER; note = 2'-O-methyluridine-3'-phosphate
  misc_feature 1: note = RNA
  misc_feature 2: note = DNA
  misc_feature 3: note = RNA
  misc_feature 4: note = DNA
  misc_feature 5: note = RNA
  misc_feature 6: note = DNA
  misc_feature 7: note = RNA
  misc_feature 8: note = DNA
  misc_feature 9: note = RNA
  misc_feature 10: note = DNA
  misc_feature 11: note = RNA
  misc_feature 12: note = DNA
  misc_feature 13: note = RNA
  misc_feature 14: note = DNA
  misc_feature 15: note = RNA
  misc_feature 16: note = DNA
  misc_feature 17: note = RNA
  misc_feature 18: note = DNA
  misc_feature 19: note = RNA
  misc_feature 20: note = RNA
  misc_feature 21: note = RNA
  source 1..21: mol_type = other RNA
taccaatttatgcctacagtt

SEQ ID NO: 69 - RNA, 21 nt, synthetic construct
  modified_base 1: mod_base = OTHER; note = 2'-O-methyluridine-3'-phosphorothioate
  modified_base 2: mod_base = OTHER; note = 2'-fluoroadenosine-3'-phosporothioate
  modified_base 3: mod_base = OTHER; note = 2'-O-methylcytidine-3'-phosphorothioate
  modified_base 4: mod_base = OTHER; note = 2'-fluorocytidine-3'-phosphate
  modified_base 5: mod_base = OTHER; note = 2'-O-methyladenosine-3'-phosphate
  modified_base 6: mod_base = OTHER; note = 2'-fluoroadenosine-3'-phosphate
  modified_base 7: mod_base = OTHER; note = 2'-O-methyluridine-3'-phosphate
  modified_base 8: mod_base = OTHER; note = 2'-fluorouridine-3'-phosphate
  modified_base 9: mod_base = OTHER; note = 2'-O-methyluridine-3'-phosphate
  modified_base 10: mod_base = OTHER; note = 2'-fluoroadenosine-3'-phosphate
  modified_base 11: mod_base = OTHER; note = 2'-O-methyluridine-3'-phosphate
  modified_base 12: mod_base = OTHER; note = 2'-fluoroguanosine-3'-phosphate
  modified_base 13: mod_base = OTHER; note = 2'-O-methylcytidine-3'-phosphate
  modified_base 14: mod_base = OTHER; note = 2'-fluorocytidine-3'-phosphate
  modified_base 15: mod_base = OTHER; note = 2'-O-methyluridine-3'-phosphate
  modified_base 16: mod_base = OTHER; note = 2'-fluoroadenosine-3'-phosphate
  modified_base 17: mod_base = OTHER; note = 2'-O-methylcytidine-3'-phosphate
  modified_base 18: mod_base = OTHER; note = 2'-fluoroadenosine-3'-phosphate
  modified_base 19: mod_base = OTHER; note = 2'-O-methylguanosine-3'-phosphate
  modified_base 20: mod_base = OTHER; note = 2'-O-methylguanosine-3'-phosphorothioate
  modified_base 21: mod_base = OTHER; note = 2'-O-methylcytidine-3'-phosphate
  misc_feature 1: note = RNA
  misc_feature 2: note = DNA
  misc_feature 3: note = RNA
  misc_feature 4: note = DNA
  misc_feature 5: note = RNA
  misc_feature 6: note = DNA
  misc_feature 7: note = RNA
  misc_feature 8: note = DNA
  misc_feature 9: note = RNA
  misc_feature 10: note = DNA
  misc_feature 11: note = RNA
  misc_feature 12: note = DNA
  misc_feature 13: note = RNA
  misc_feature 14: note = DNA
  misc_feature 15: note = RNA
  misc_feature 16: note = DNA
  misc_feature 17: note = RNA
  misc_feature 18: note = DNA
  misc_feature 19: note = RNA
  misc_feature 20: note = RNA
  misc_feature 21: note = RNA
  source 1..21: mol_type = other RNA
taccaatttatgcctacaggc

SEQ ID NO: 70 - RNA, 21 nt, synthetic construct
  modified_base 1: mod_base = OTHER; note = vinyl phosphonate-2'-O-methyluridine-3'-phosphorothioate
  modified_base 2: mod_base = OTHER; note = 2'-fluoroadenosine-3'-phosporothioate
  modified_base 3: mod_base = OTHER; note = 2'-O-methylcytidine-3'-phosphorothioate
  modified_base 4: mod_base = OTHER; note = 2'-fluorocytidine-3'-phosphate
  modified_base 5: mod_base = OTHER; note = 2'-O-methyladenosine-3'-phosphate
  modified_base 6: mod_base = OTHER; note = 2'-fluoroadenosine-3'-phosphate
  modified_base 7: mod_base = OTHER; note = 2'-O-methyluridine-3'-phosphate
  modified_base 8: mod_base = OTHER; note = 2'-fluorouridine-3'-phosphate
  modified_base 9: mod_base = OTHER; note = 2'-O-methyluridine-3'-phosphate
  modified_base 10: mod_base = OTHER; note = 2'-fluoroadenosine-3'-phosphate
  modified_base 11: mod_base = OTHER; note = 2'-O-methyluridine-3'-phosphate
  modified_base 12: mod_base = OTHER; note = 2'-fluoroguanosine-3'-phosphate
  modified_base 13: mod_base = OTHER; note = 2'-O-methylcytidine-3'-phosphate
  modified_base 14: mod_base = OTHER; note = 2'-fluorocytidine-3'-phosphate
  modified_base 15: mod_base = OTHER; note = 2'-O-methyluridine-3'-phosphate
  modified_base 16: mod_base = OTHER; note = 2'-fluoroadenosine-3'-phosphate
  modified_base 17: mod_base = OTHER; note = 2'-O-methylcytidine-3'-phosphate
  modified_base 18: mod_base = OTHER; note = 2'-fluoroadenosine-3'-phosphate
  modified_base 19: mod_base = OTHER; note = 2'-O-methylguanosine-3'-phosphate
  modified_base 20: mod_base = OTHER; note = 2'-fluoroguanosine-3'-phosphorothioate
  modified_base 21: mod_base = OTHER; note = 2'-O-methylcytidine-3'-phosphate
  misc_feature 1: note = RNA
  misc_feature 2: note = DNA
  misc_feature 3: note = RNA
  misc_feature 4: note = DNA
  misc_feature 5: note = RNA
  misc_feature 6: note = DNA
  misc_feature 7: note = RNA
  misc_feature 8: note = DNA
  misc_feature 9: note = RNA
  misc_feature 10: note = DNA
  misc_feature 11: note = RNA
  misc_feature 12: note = DNA
  misc_feature 13: note = RNA
  misc_feature 14: note = DNA
  misc_feature 15: note = RNA
  misc_feature 16: note = DNA
  misc_feature 17: note = RNA
  misc_feature 18: note = DNA
  misc_feature 19: note = RNA
  misc_feature 20: note = DNA
  misc_feature 21: note = RNA
  source 1..21: mol_type = other RNA
taccaatttatgcctacaggc

SEQ ID NO: 71 - RNA, 21 nt, synthetic construct
  modified_base 1: mod_base = OTHER; note = vinyl phosphonate-2'-O-methyluridine-3'-phosphorothioate
  modified_base 2: mod_base = OTHER; note = 2'-fluoroadenosine-3'-phosporothioate
  modified_base 3: mod_base = OTHER; note = 2'-O-methylcytidine-3'-phosphorothioate
  modified_base 4: mod_base = OTHER; note = 2'-fluorocytidine-3'-phosphate
  modified_base 5: mod_base = OTHER; note = 2'-O-methyladenosine-3'-phosphate
  modified_base 6: mod_base = OTHER; note = 2'-fluoroadenosine-3'-phosphate
  modified_base 7: mod_base = OTHER; note = 2'-O-methyluridine-3'-phosphate
  modified_base 8: mod_base = OTHER; note = 2'-fluorouridine-3'-phosphate
  modified_base 9: mod_base = OTHER; note = 2'-O-methyluridine-3'-phosphate
  modified_base 10: mod_base = OTHER; note = 2'-fluoroadenosine-3'-phosphate
  modified_base 11: mod_base = OTHER; note = 2'-O-methyluridine-3'-phosphate
  modified_base 12: mod_base = OTHER; note = 2'-fluoroguanosine-3'-phosphate
  modified_base 13: mod_base = OTHER; note = 2'-O-methylcytidine-3'-phosphate
  modified_base 14: mod_base = OTHER; note = 2'-fluorocytidine-3'-phosphate
  modified_base 15: mod_base = OTHER; note = 2'-O-methyluridine-3'-phosphate
  modified_base 16: mod_base = OTHER; note = 2'-fluoroadenosine-3'-phosphate
  modified_base 17: mod_base = OTHER; note = 2'-O-methylcytidine-3'-phosphate
  modified_base 18: mod_base = OTHER; note = 2'-fluoroadenosine-3'-phosphate
  modified_base 19: mod_base = OTHER; note = 2'-O-methylguanosine-3'-phosphate
  modified_base 20: mod_base = OTHER; note = 2'-O-methyluridine-3'-phosphorothioate
  modified_base 21: mod_base = OTHER; note = 2'-O-methyluridine-3'-phosphate
  misc_feature 1: note = RNA
  misc_feature 2: note = DNA
  misc_feature 3: note = RNA
  misc_feature 4: note = DNA
  misc_feature 5: note = RNA
  misc_feature 6: note = DNA
  misc_feature 7: note = RNA
  misc_feature 8: note = DNA
  misc_feature 9: note = RNA
  misc_feature 10: note = DNA
  misc_feature 11: note = RNA
  misc_feature 12: note = DNA
  misc_feature 13: note = RNA
  misc_feature 14: note = DNA
  misc_feature 15: note = RNA
  misc_feature 16: note = DNA
  misc_feature 17: note = RNA
  misc_feature 18: note = DNA
  misc_feature 19: note = RNA
  misc_feature 20: note = RNA
  misc_feature 21: note = RNA
  source 1..21: mol_type = other RNA
taccaatttatgcctacagtt

SEQ ID NO: 72 - RNA, 21 nt, synthetic construct
  modified_base 1: mod_base = OTHER; note = 2'-O-methyladenosine-3'-phosphorothioate
  modified_base 2: mod_base = OTHER; note = 2'-fluorouridine-3'-phosphorothioate
  modified_base 3: mod_base = OTHER; note = 2'-O-methyluridine-3'-phosphorothioate
  modified_base 4: mod_base = OTHER; note = 2'-fluoroguanosine-3'-phosphate
  modified_base 5: mod_base = OTHER; note = 2'-O-methyladenosine-3'-phosphate
  modified_base 6: mod_base = OTHER; note = 2'-fluoroguanosine-3'-phosphate
  modified_base 7: mod_base = OTHER; note = 2'-O-methyladenosine-3'-phosphate
  modified_base 8: mod_base = OTHER; note = 2'-fluoroguanosine-3'-phosphate
  modified_base 9: mod_base = OTHER; note = 2'-O-methyladenosine-3'-phosphate
  modified_base 10: mod_base = OTHER; note = 2'-fluoroadenosine-3'-phosphate
  modified_base 11: mod_base = OTHER; note = 2'-O-methylguanosine-3'-phosphate
  modified_base 12: mod_base = OTHER; note = 2'-fluorouridine-3'-phosphate
  modified_base 13: mod_base = OTHER; note = 2'-O-methylcytidine-3'-phosphate
  modified_base 14: mod_base = OTHER; note = 2'-fluorocytidine-3'-phosphate
  modified_base 15: mod_base = OTHER; note = 2'-O-methyladenosine-3'-phosphate
  modified_base 16: mod_base = OTHER; note = 2'-fluorocytidine-3'-phosphate
  modified_base 17: mod_base = OTHER; note = 2'-O-methylcytidine-3'-phosphate
  modified_base 18: mod_base = OTHER; note = 2'-fluoroadenosine-3'-phosphate
  modified_base 19: mod_base = OTHER; note = 2'-O-methylcytidine-3'-phosphate
  modified_base 20: mod_base = OTHER; note = 2'-fluoroguanosine-3'-phosphorothioate
  modified_base 21: mod_base = OTHER; note = 2'-O-methyladenosine-3'-phosphate
  misc_feature 1: note = RNA
  misc_feature 2: note = DNA
  misc_feature 3: note = RNA
  misc_feature 4: note = DNA
  misc_feature 5: note = RNA
  misc_feature 6: note = DNA
  misc_feature 7: note = RNA
  misc_feature 8: note = DNA
  misc_feature 9: note = RNA
  misc_feature 10: note = DNA
  misc_feature 11: note = RNA
  misc_feature 12: note = DNA
  misc_feature 13: note = RNA
  misc_feature 14: note = DNA
  misc_feature 15: note = RNA
  misc_feature 16: note = DNA
  misc_feature 17: note = RNA
  misc_feature 18: note = DNA
  misc_feature 19: note = RNA
  misc_feature 20: note = DNA
  misc_feature 21: note = RNA
  source 1..21: mol_type = other RNA
attgagagaagtccaccacga

SEQ ID NO: 73 - RNA, 21 nt, synthetic construct
  modified_base 1: mod_base = OTHER; note = 2'-O-methyladenosine-3'-phosphorothioate
  modified_base 2: mod_base = OTHER; note = 2'-fluorouridine-3'-phosphorothioate
  modified_base 3: mod_base = OTHER; note = 2'-O-methyluridine-3'-phosphorothioate
  modified_base 4: mod_base = OTHER; note = 2'-fluoroguanosine-3'-phosphate
  modified_base 5: mod_base = OTHER; note = 2'-O-methyladenosine-3'-phosphate
  modified_base 6: mod_base = OTHER; note = 2'-fluoroguanosine-3'-phosphate
  modified_base 7: mod_base = OTHER; note = 2'-O-methyladenosine-3'-phosphate
  modified_base 8: mod_base = OTHER; note = 2'-fluoroguanosine-3'-phosphate
  modified_base 9: mod_base = OTHER; note = 2'-O-methyladenosine-3'-phosphate
  modified_base 10: mod_base = OTHER; note = 2'-fluoroadenosine-3'-phosphate
  modified_base 11: mod_base = OTHER; note = 2'-O-methylguanosine-3'-phosphate
  modified_base 12: mod_base = OTHER; note = 2'-fluorouridine-3'-phosphate
  modified_base 13: mod_base = OTHER; note = 2'-O-methylcytidine-3'-phosphate
  modified_base 14: mod_base = OTHER; note = 2'-fluorocytidine-3'-phosphate
  modified_base 15: mod_base = OTHER; note = 2'-O-methyladenosine-3'-phosphate
  modified_base 16: mod_base = OTHER; note = 2'-fluorocytidine-3'-phosphate
  modified_base 17: mod_base = OTHER; note = 2'-O-methylcytidine-3'-phosphate
  modified_base 18: mod_base = OTHER; note = 2'-fluoroadenosine-3'-phosphate
  modified_base 19: mod_base = OTHER; note = 2'-O-methylcytidine-3'-phosphate
  modified_base 20: mod_base = OTHER; note = 2'-O-methylguanosine-3'-phosphorothioate
  modified_base 21: mod_base = OTHER; note = 2'-O-methyladenosine-3'-phosphate
  misc_feature 1: note = RNA
  misc_feature 2: note = DNA
  misc_feature 3: note = RNA
  misc_feature 4: note = DNA
  misc_feature 5: note = RNA
  misc_feature 6: note = DNA
  misc_feature 7: note = RNA
  misc_feature 8: note = DNA
  misc_feature 9: note = RNA
  misc_feature 10: note = DNA
  misc_feature 11: note = RNA
  misc_feature 12: note = DNA
  misc_feature 13: note = RNA
  misc_feature 14: note = DNA
  misc_feature 15: note = RNA
  misc_feature 16: note = DNA
  misc_feature 17: note = RNA
  misc_feature 18: note = DNA
  misc_feature 19: note = RNA
  misc_feature 20: note = RNA
  misc_feature 21: note = RNA
  source 1..21: mol_type = other RNA
attgagagaagtccaccacga

SEQ ID NO: 74 - RNA, 21 nt, synthetic construct
  modified_base 1: mod_base = OTHER; note = 2'-O-methyladenosine-3'-phosphorothioate
  modified_base 2: mod_base = OTHER; note = 2'-fluorouridine-3'-phosphorothioate
  modified_base 3: mod_base = OTHER; note = 2'-O-methyluridine-3'-phosphorothioate
  modified_base 4: mod_base = OTHER; note = 2'-fluoroguanosine-3'-phosphate
  modified_base 5: mod_base = OTHER; note = 2'-O-methyladenosine-3'-phosphate
  modified_base 6: mod_base = OTHER; note = 2'-fluoroguanosine-3'-phosphate
  modified_base 7: mod_base = OTHER; note = 2'-O-methyladenosine-3'-phosphate
  modified_base 8: mod_base = OTHER; note = 2'-fluoroguanosine-3'-phosphate
  modified_base 9: mod_base = OTHER; note = 2'-O-methyladenosine-3'-phosphate
  modified_base 10: mod_base = OTHER; note = 2'-fluoroadenosine-3'-phosphate
  modified_base 11: mod_base = OTHER; note = 2'-O-methylguanosine-3'-phosphate
  modified_base 12: mod_base = OTHER; note = 2'-fluorouridine-3'-phosphate
  modified_base 13: mod_base = OTHER; note = 2'-O-methylcytidine-3'-phosphate
  modified_base 14: mod_base = OTHER; note = 2'-fluorocytidine-3'-phosphate
  modified_base 15: mod_base = OTHER; note = 2'-O-methyladenosine-3'-phosphate
  modified_base 16: mod_base = OTHER; note = 2'-fluorocytidine-3'-phosphate
  modified_base 17: mod_base = OTHER; note = 2'-O-methylcytidine-3'-phosphate
  modified_base 18: mod_base = OTHER; note = 2'-fluoroadenosine-3'-phosphate
  modified_base 19: mod_base = OTHER; note = 2'-O-methylcytidine-3'-phosphate
  modified_base 20: mod_base = OTHER; note = 2'-O-methyluridine-3'-phosphorothioate
  modified_base 21: mod_base = OTHER; note = 2'-O-methyluridine-3'-phosphate
  misc_feature 1: note = RNA
  misc_feature 2: note = DNA
  misc_feature 3: note = RNA
  misc_feature 4: note = DNA
  misc_feature 5: note = RNA
  misc_feature 6: note = DNA
  misc_feature 7: note = RNA
  misc_feature 8: note = DNA
  misc_feature 9: note = RNA
  misc_feature 10: note = DNA
  misc_feature 11: note = RNA
  misc_feature 12: note = DNA
  misc_feature 13: note = RNA
  misc_feature 14: note = DNA
  misc_feature 15: note = RNA
  misc_feature 16: note = DNA
  misc_feature 17: note = RNA
  misc_feature 18: note = DNA
  misc_feature 19: note = RNA
  misc_feature 20: note = RNA
  misc_feature 21: note = RNA
  source 1..21: mol_type = other RNA
attgagagaagtccaccactt

SEQ ID NO: 75 - RNA, 21 nt, synthetic construct
  modified_base 1: mod_base = OTHER; note = vinyl phosphonate-2'-O-methyluridine-3'-phosphorothioate
  modified_base 2: mod_base = OTHER; note = 2'-fluorouridine-3'-phosphorothioate
  modified_base 3: mod_base = OTHER; note = 2'-O-methyluridine-3'-phosphorothioate
  modified_base 4: mod_base = OTHER; note = 2'-fluoroguanosine-3'-phosphate
  modified_base 5: mod_base = OTHER; note = 2'-O-methyladenosine-3'-phosphate
  modified_base 6: mod_base = OTHER; note = 2'-fluoroguanosine-3'-phosphate
  modified_base 7: mod_base = OTHER; note = 2'-O-methyladenosine-3'-phosphate
  modified_base 8: mod_base = OTHER; note = 2'-fluoroguanosine-3'-phosphate
  modified_base 9: mod_base = OTHER; note = 2'-O-methyladenosine-3'-phosphate
  modified_base 10: mod_base = OTHER; note = 2'-fluoroadenosine-3'-phosphate
  modified_base 11: mod_base = OTHER; note = 2'-O-methylguanosine-3'-phosphate
  modified_base 12: mod_base = OTHER; note = 2'-fluorouridine-3'-phosphate
  modified_base 13: mod_base = OTHER; note = 2'-O-methylcytidine-3'-phosphate
  modified_base 14: mod_base = OTHER; note = 2'-fluorocytidine-3'-phosphate
  modified_base 15: mod_base = OTHER; note = 2'-O-methyladenosine-3'-phosphate
  modified_base 16: mod_base = OTHER; note = 2'-fluorocytidine-3'-phosphate
  modified_base 17: mod_base = OTHER; note = 2'-O-methylcytidine-3'-phosphate
  modified_base 18: mod_base = OTHER; note = 2'-fluoroadenosine-3'-phosphate
  modified_base 19: mod_base = OTHER; note = 2'-O-methylcytidine-3'-phosphate
  modified_base 20: mod_base = OTHER; note = 2'-fluoroguanosine-3'-phosphorothioate
  modified_base 21: mod_base = OTHER; note = 2'-O-methyladenosine-3'-phosphate
  misc_feature 1: note = RNA
  misc_feature 2: note = DNA
  misc_feature 3: note = RNA
  misc_feature 4: note = DNA
  misc_feature 5: note = RNA
  misc_feature 6: note = DNA
  misc_feature 7: note = RNA
  misc_feature 8: note = DNA
  misc_feature 9: note = RNA
  misc_feature 10: note = DNA
  misc_feature 11: note = RNA
  misc_feature 12: note = DNA
  misc_feature 13: note = RNA
  misc_feature 14: note = DNA
  misc_feature 15: note = RNA
  misc_feature 16: note = DNA
  misc_feature 17: note = RNA
  misc_feature 18: note = DNA
  misc_feature 19: note = RNA
  misc_feature 20: note = DNA
  misc_feature 21: note = RNA
  source 1..21: mol_type = other RNA
tttgagagaagtccaccacga

SEQ ID NO: 76 - RNA, 21 nt, synthetic construct
  modified_base 1: mod_base = OTHER; note = 2'-O-methyladenosine-3'-phosphorothioate
  modified_base 2: mod_base = OTHER; note = 2'-fluoroadenosine-3'-phosporothioate
  modified_base 3: mod_base = OTHER; note = 2'-O-methyluridine-3'-phosphorothioate
  modified_base 4: mod_base = OTHER; note = 2'-fluorouridine-3'-phosphate
  modified_base 5: mod_base = OTHER; note = 2'-O-methylguanosine-3'-phosphate
  modified_base 6: mod_base = OTHER; note = 2'-fluoroadenosine-3'-phosphate
  modified_base 7: mod_base = OTHER; note = 2'-O-methylguanosine-3'-phosphate
  modified_base 8: mod_base = OTHER; note = 2'-fluoroadenosine-3'-phosphate
  modified_base 9: mod_base = OTHER; note = 2'-O-methylguanosine-3'-phosphate
  modified_base 10: mod_base = OTHER; note = 2'-fluoroadenosine-3'-phosphate
  modified_base 11: mod_base = OTHER; note = 2'-O-methyladenosine-3'-phosphate
  modified_base 12: mod_base = OTHER; note = 2'-fluoroguanosine-3'-phosphate
  modified_base 13: mod_base = OTHER; note = 2'-O-methyluridine-3'-phosphate
  modified_base 14: mod_base = OTHER; note = 2'-fluorocytidine-3'-phosphate
  modified_base 15: mod_base = OTHER; note = 2'-O-methylcytidine-3'-phosphate
  modified_base 16: mod_base = OTHER; note = 2'-fluoroadenosine-3'-phosphate
  modified_base 17: mod_base = OTHER; note = 2'-O-methylcytidine-3'-phosphate
  modified_base 18: mod_base = OTHER; note = 2'-fluorocytidine-3'-phosphate
  modified_base 19: mod_base = OTHER; note = 2'-O-methyladenosine-3'-phosphate
  modified_base 20: mod_base = OTHER; note = 2'-fluorocytidine-3'-phosphorothioate
  modified_base 21: mod_base = OTHER; note = 2'-O-methylguanosine-3'-phosphate
  misc_feature 1: note = RNA
  misc_feature 2: note = DNA
  misc_feature 3: note = RNA
  misc_feature 4: note = DNA
  misc_feature 5: note = RNA
  misc_feature 6: note = DNA
  misc_feature 7: note = RNA
  misc_feature 8: note = DNA
  misc_feature 9: note = RNA
  misc_feature 10: note = DNA
  misc_feature 11: note = RNA
  misc_feature 12: note = DNA
  misc_feature 13: note = RNA
  misc_feature 14: note = DNA
  misc_feature 15: note = RNA
  misc_feature 16: note = DNA
  misc_feature 17: note = RNA
  misc_feature 18: note = DNA
  misc_feature 19: note = RNA
  misc_feature 20: note = DNA
  misc_feature 21: note = RNA
  source 1..21: mol_type = other RNA
aattgagagaagtccaccacg

SEQ ID NO: 77 - RNA, 21 nt, synthetic construct
  modified_base 1: mod_base = OTHER; note = 2'-O-methyladenosine-3'-phosphorothioate
  modified_base 2: mod_base = OTHER; note = 2'-fluoroadenosine-3'-phosporothioate
  modified_base 3: mod_base = OTHER; note = 2'-O-methyluridine-3'-phosphorothioate
  modified_base 4: mod_base = OTHER; note = 2'-fluorouridine-3'-phosphate
  modified_base 5: mod_base = OTHER; note = 2'-O-methylguanosine-3'-phosphate
  modified_base 6: mod_base = OTHER; note = 2'-fluoroadenosine-3'-phosphate
  modified_base 7: mod_base = OTHER; note = 2'-O-methylguanosine-3'-phosphate
  modified_base 8: mod_base = OTHER; note = 2'-fluoroadenosine-3'-phosphate
  modified_base 9: mod_base = OTHER; note = 2'-O-methylguanosine-3'-phosphate
  modified_base 10: mod_base = OTHER; note = 2'-fluoroadenosine-3'-phosphate
  modified_base 11: mod_base = OTHER; note = 2'-O-methyladenosine-3'-phosphate
  modified_base 12: mod_base = OTHER; note = 2'-fluoroguanosine-3'-phosphate
  modified_base 13: mod_base = OTHER; note = 2'-O-methyluridine-3'-phosphate
  modified_base 14: mod_base = OTHER; note = 2'-fluorocytidine-3'-phosphate
  modified_base 15: mod_base = OTHER; note = 2'-O-methylcytidine-3'-phosphate
  modified_base 16: mod_base = OTHER; note = 2'-fluoroadenosine-3'-phosphate
  modified_base 17: mod_base = OTHER; note = 2'-O-methylcytidine-3'-phosphate
  modified_base 18: mod_base = OTHER; note = 2'-fluorocytidine-3'-phosphate
  modified_base 19: mod_base = OTHER; note = 2'-O-methyladenosine-3'-phosphate
  modified_base 20: mod_base = OTHER; note = 2'-O-methylcytidine-3'-phosphorothioate
  modified_base 21: mod_base = OTHER; note = 2'-O-methylguanosine-3'-phosphate
  misc_feature 1: note = RNA
  misc_feature 2: note = DNA
  misc_feature 3: note = RNA
  misc_feature 4: note = DNA
  misc_feature 5: note = RNA
  misc_feature 6: note = DNA
  misc_feature 7: note = RNA
  misc_feature 8: note = DNA
  misc_feature 9: note = RNA
  misc_feature 10: note = DNA
  misc_feature 11: note = RNA
  misc_feature 12: note = DNA
  misc_feature 13: note = RNA
  misc_feature 14: note = DNA
  misc_feature 15: note = RNA
  misc_feature 16: note = DNA
  misc_feature 17: note = RNA
  misc_feature 18: note = DNA
  misc_feature 19: note = RNA
  misc_feature 20: note = RNA
  misc_feature 21: note = RNA
  source 1..21: mol_type = other RNA
aattgagagaagtccaccacg

SEQ ID NO: 78 - RNA, 21 nt, synthetic construct
  modified_base 1: mod_base = OTHER; note = 2'-O-methyladenosine-3'-phosphorothioate
  modified_base 2: mod_base = OTHER; note = 2'-fluoroadenosine-3'-phosporothioate
  modified_base 3: mod_base = OTHER; note = 2'-O-methyluridine-3'-phosphorothioate
  modified_base 4: mod_base = OTHER; note = 2'-fluorouridine-3'-phosphate
  modified_base 5: mod_base = OTHER; note = 2'-O-methylguanosine-3'-phosphate
  modified_base 6: mod_base = OTHER; note = 2'-fluoroadenosine-3'-phosphate
  modified_base 7: mod_base = OTHER; note = 2'-O-methylguanosine-3'-phosphate
  modified_base 8: mod_base = OTHER; note = 2'-fluoroadenosine-3'-phosphate
  modified_base 9: mod_base = OTHER; note = 2'-O-methylguanosine-3'-phosphate
  modified_base 10: mod_base = OTHER; note = 2'-fluoroadenosine-3'-phosphate
  modified_base 11: mod_base = OTHER; note = 2'-O-methyladenosine-3'-phosphate
  modified_base 12: mod_base = OTHER; note = 2'-fluoroguanosine-3'-phosphate
  modified_base 13: mod_base = OTHER; note = 2'-O-methyluridine-3'-phosphate
  modified_base 14: mod_base = OTHER; note = 2'-fluorocytidine-3'-phosphate
  modified_base 15: mod_base = OTHER; note = 2'-O-methylcytidine-3'-phosphate
  modified_base 16: mod_base = OTHER; note = 2'-fluoroadenosine-3'-phosphate
  modified_base 17: mod_base = OTHER; note = 2'-O-methylcytidine-3'-phosphate
  modified_base 18: mod_base = OTHER; note = 2'-fluorocytidine-3'-phosphate
  modified_base 19: mod_base = OTHER; note = 2'-O-methyladenosine-3'-phosphate
  modified_base 20: mod_base = OTHER; note = 2'-O-methyluridine-3'-phosphorothioate
  modified_base 21: mod_base = OTHER; note = 2'-O-methyluridine-3'-phosphate
  misc_feature 1: note = RNA
  misc_feature 2: note = DNA
  misc_feature 3: note = RNA
  misc_feature 4: note = DNA
  misc_feature 5: note = RNA
  misc_feature 6: note = DNA
  misc_feature 7: note = RNA
  misc_feature 8: note = DNA
  misc_feature 9: note = RNA
  misc_feature 10: note = DNA
  misc_feature 11: note = RNA
  misc_feature 12: note = DNA
  misc_feature 13: note = RNA
  misc_feature 14: note = DNA
  misc_feature 15: note = RNA
  misc_feature 16: note = DNA
  misc_feature 17: note = RNA
  misc_feature 18: note = DNA
  misc_feature 19: note = RNA
  misc_feature 20: note = RNA
  misc_feature 21: note = RNA
  source 1..21: mol_type = other RNA
aattgagagaagtccaccatt

SEQ ID NO: 79 - RNA, 21 nt, synthetic construct
  modified_base 1: mod_base = OTHER; note = vinyl phosphonate-2'-O-methyluridine-3'-phosphorothioate
  modified_base 2: mod_base = OTHER; note = 2'-fluoroadenosine-3'-phosporothioate
  modified_base 3: mod_base = OTHER; note = 2'-O-methyluridine-3'-phosphorothioate
  modified_base 4: mod_base = OTHER; note = 2'-fluorouridine-3'-phosphate
  modified_base 5: mod_base = OTHER; note = 2'-O-methylguanosine-3'-phosphate
  modified_base 6: mod_base = OTHER; note = 2'-fluoroadenosine-3'-phosphate
  modified_base 7: mod_base = OTHER; note = 2'-O-methylguanosine-3'-phosphate
  modified_base 8: mod_base = OTHER; note = 2'-fluoroadenosine-3'-phosphate
  modified_base 9: mod_base = OTHER; note = 2'-O-methylguanosine-3'-phosphate
  modified_base 10: mod_base = OTHER; note = 2'-fluoroadenosine-3'-phosphate
  modified_base 11: mod_base = OTHER; note = 2'-O-methyladenosine-3'-phosphate
  modified_base 12: mod_base = OTHER; note = 2'-fluoroguanosine-3'-phosphate
  modified_base 13: mod_base = OTHER; note = 2'-O-methyluridine-3'-phosphate
  modified_base 14: mod_base = OTHER; note = 2'-fluorocytidine-3'-phosphate
  modified_base 15: mod_base = OTHER; note = 2'-O-methylcytidine-3'-phosphate
  modified_base 16: mod_base = OTHER; note = 2'-fluoroadenosine-3'-phosphate
  modified_base 17: mod_base = OTHER; note = 2'-O-methylcytidine-3'-phosphate
  modified_base 18: mod_base = OTHER; note = 2'-fluorocytidine-3'-phosphate
  modified_base 19: mod_base = OTHER; note = 2'-O-methyladenosine-3'-phosphate
  modified_base 20: mod_base = OTHER; note = 2'-fluorocytidine-3'-phosphorothioate
  modified_base 21: mod_base = OTHER; note = 2'-O-methylguanosine-3'-phosphate
  misc_feature 1: note = RNA
  misc_feature 2: note = DNA
  misc_feature 3: note = RNA
  misc_feature 4: note = DNA
  misc_feature 5: note = RNA
  misc_feature 6: note = DNA
  misc_feature 7: note = RNA
  misc_feature 8: note = DNA
  misc_feature 9: note = RNA
  misc_feature 10: note = DNA
  misc_feature 11: note = RNA
  misc_feature 12: note = DNA
  misc_feature 13: note = RNA
  misc_feature 14: note = DNA
  misc_feature 15: note = RNA
  misc_feature 16: note = DNA
  misc_feature 17: note = RNA
  misc_feature 18: note = DNA
  misc_feature 19: note = RNA
  misc_feature 20: note = DNA
  misc_feature 21: note = RNA
  source 1..21: mol_type = other RNA
tattgagagaagtccaccacg

SEQ ID NO: 80 - RNA, 21 nt, synthetic construct
  modified_base 1: mod_base = OTHER; note = 2'-O-methyluridine-3'-phosphorothioate
  modified_base 2: mod_base = OTHER; note = 2'-fluoroadenosine-3'-phosporothioate
  modified_base 3: mod_base = OTHER; note = 2'-O-methylcytidine-3'-phosphorothioate
  modified_base 4: mod_base = OTHER; note = 2'-fluorocytidine-3'-phosphate
  modified_base 5: mod_base = OTHER; note = 2'-O-methyladenosine-3'-phosphate
  modified_base 6: mod_base = OTHER; note = 2'-fluoroadenosine-3'-phosphate
  modified_base 7: mod_base = OTHER; note = 2'-O-methyluridine-3'-phosphate
  modified_base 8: mod_base = OTHER; note = 2'-fluorouridine-3'-phosphate
  modified_base 9: mod_base = OTHER; note = 2'-O-methyluridine-3'-phosphate
  modified_base 10: mod_base = OTHER; note = 2'-fluoroadenosine-3'-phosphate
  modified_base 11: mod_base = OTHER; note = 2'-O-methyluridine-3'-phosphate
  modified_base 12: mod_base = OTHER; note = 2'-fluoroguanosine-3'-phosphate
  modified_base 13: mod_base = OTHER; note = 2'-O-methylcytidine-3'-phosphate
  modified_base 14: mod_base = OTHER; note = 2'-fluorocytidine-3'-phosphate
  modified_base 15: mod_base = OTHER; note = 2'-O-methyluridine-3'-phosphate
  modified_base 16: mod_base = OTHER; note = 2'-fluoroadenosine-3'-phosphate
  modified_base 17: mod_base = OTHER; note = 2'-O-methylcytidine-3'-phosphate
  modified_base 18: mod_base = OTHER; note = 2'-fluoroadenosine-3'-phosphate
  modified_base 19: mod_base = OTHER; note = 2'-O-methylguanosine-3'-phosphate
  modified_base 20: mod_base = OTHER; note = 2'-fluoroguanosine-3'-phosphorothioate
  modified_base 21: mod_base = OTHER; note = 2'-O-methyluridine-3'-phosphate
  misc_feature 1: note = RNA
  misc_feature 2: note = DNA
  misc_feature 3: note = RNA
  misc_feature 4: note = DNA
  misc_feature 5: note = RNA
  misc_feature 6: note = DNA
  misc_feature 7: note = RNA
  misc_feature 8: note = DNA
  misc_feature 9: note = RNA
  misc_feature 10: note = DNA
  misc_feature 11: note = RNA
  misc_feature 12: note = DNA
  misc_feature 13: note = RNA
  misc_feature 14: note = DNA
  misc_feature 15: note = RNA
  misc_feature 16: note = DNA
  misc_feature 17: note = RNA
  misc_feature 18: note = DNA
  misc_feature 19: note = RNA
  misc_feature 20: note = DNA
  misc_feature 21: note = RNA
  source 1..21: mol_type = other RNA
taccaatttatgcctacaggt

SEQ ID NO: 81 - RNA, 21 nt, synthetic construct
  modified_base 1: mod_base = OTHER; note = 2'-O-methyluridine-3'-phosphorothioate
  modified_base 2: mod_base = OTHER; note = 2'-fluoroadenosine-3'-phosporothioate
  modified_base 3: mod_base = OTHER; note = 2'-O-methylcytidine-3'-phosphate
  modified_base 4: mod_base = OTHER; note = 2'-fluorocytidine-3'-phosphate
  modified_base 5: mod_base = OTHER; note = 2'-O-methyladenosine-3'-phosphate
  modified_base 6: mod_base = OTHER; note = 2'-fluoroadenosine-3'-phosphate
  modified_base 7: mod_base = OTHER; note = 2'-O-methyluridine-3'-phosphate
  modified_base 8: mod_base = OTHER; note = 2'-fluorouridine-3'-phosphate
  modified_base 9: mod_base = OTHER; note = 2'-O-methyluridine-3'-phosphate
  modified_base 10: mod_base = OTHER; note = 2'-fluoroadenosine-3'-phosphate
  modified_base 11: mod_base = OTHER; note = 2'-O-methyluridine-3'-phosphate
  modified_base 12: mod_base = OTHER; note = 2'-fluoroguanosine-3'-phosphate
  modified_base 13: mod_base = OTHER; note = 2'-O-methylcytidine-3'-phosphate
  modified_base 14: mod_base = OTHER; note = 2'-fluorocytidine-3'-phosphate
  modified_base 15: mod_base = OTHER; note = 2'-O-methyluridine-3'-phosphate
  modified_base 16: mod_base = OTHER; note = 2'-fluoroadenosine-3'-phosphate
  modified_base 17: mod_base = OTHER; note = 2'-O-methylcytidine-3'-phosphate
  modified_base 18: mod_base = OTHER; note = 2'-fluoroadenosine-3'-phosphate
  modified_base 19: mod_base = OTHER; note = 2'-O-methylguanosine-3'-phosphorothioate
  modified_base 20: mod_base = OTHER; note = 2'-O-methyluridine-3'-phosphorothioate
  modified_base 21: mod_base = OTHER; note = 2'-O-methyluridine-3'-phosphate
  misc_feature 1: note = RNA
  misc_feature 2: note = DNA
  misc_feature 3: note = RNA
  misc_feature 4: note = DNA
  misc_feature 5: note = RNA
  misc_feature 6: note = DNA
  misc_feature 7: note = RNA
  misc_feature 8: note = DNA
  misc_feature 9: note = RNA
  misc_feature 10: note = DNA
  misc_feature 11: note = RNA
  misc_feature 12: note = DNA
  misc_feature 13: note = RNA
  misc_feature 14: note = DNA
  misc_feature 15: note = RNA
  misc_feature 16: note = DNA
  misc_feature 17: note = RNA
  misc_feature 18: note = DNA
  misc_feature 19: note = RNA
  misc_feature 20: note = RNA
  misc_feature 21: note = RNA
  source 1..21: mol_type = other RNA
taccaatttatgcctacagtt

SEQ ID NO: 82 - RNA, 21 nt, synthetic construct
  modified_base 1: mod_base = OTHER; note = 2'-O-methyluridine-3'-phosphorothioate
  modified_base 2: mod_base = OTHER; note = 2'-fluoroadenosine-3'-phosporothioate
  modified_base 3: mod_base = OTHER; note = 2'-O-methylcytidine-3'-phosphorothioate
  modified_base 4: mod_base = OTHER; note = 2'-fluorocytidine-3'-phosphate
  modified_base 5: mod_base = OTHER; note = 2'-O-methyladenosine-3'-phosphate
  modified_base 6: mod_base = OTHER; note = 2'-fluoroadenosine-3'-phosphate
  modified_base 7: mod_base = OTHER; note = 2'-O-methyluridine-3'-phosphate
  modified_base 8: mod_base = OTHER; note = 2'-fluorouridine-3'-phosphate
  modified_base 9: mod_base = OTHER; note = 2'-O-methyluridine-3'-phosphate
  modified_base 10: mod_base = OTHER; note = 2'-fluoroadenosine-3'-phosphate
  modified_base 11: mod_base = OTHER; note = 2'-O-methyluridine-3'-phosphate
  modified_base 12: mod_base = OTHER; note = 2'-fluoroguanosine-3'-phosphate
  modified_base 13: mod_base = OTHER; note = 2'-O-methylcytidine-3'-phosphate
  modified_base 14: mod_base = OTHER; note = 2'-fluorocytidine-3'-phosphate
  modified_base 15: mod_base = OTHER; note = 2'-O-methyluridine-3'-phosphate
  modified_base 16: mod_base = OTHER; note = 2'-fluoroadenosine-3'-phosphate
  modified_base 17: mod_base = OTHER; note = 2'-O-methylcytidine-3'-phosphate
  modified_base 18: mod_base = OTHER; note = 2'-fluoroadenosine-3'-phosphate
  modified_base 19: mod_base = OTHER; note = 2'-O-methylguanosine-3'-phosphate
  modified_base 20: mod_base = OTHER; note = 2'-O-methylcytidine-3'-phosphorothioate
  modified_base 21: mod_base = OTHER; note = 2'-O-methylcytidine-3'-phosphate
  misc_feature 1: note = RNA
  misc_feature 2: note = DNA
  misc_feature 3: note = RNA
  misc_feature 4: note = DNA
  misc_feature 5: note = RNA
  misc_feature 6: note = DNA
  misc_feature 7: note = RNA
  misc_feature 8: note = DNA
  misc_feature 9: note = RNA
  misc_feature 10: note = DNA
  misc_feature 11: note = RNA
  misc_feature 12: note = DNA
  misc_feature 13: note = RNA
  misc_feature 14: note = DNA
  misc_feature 15: note = RNA
  misc_feature 16: note = DNA
  misc_feature 17: note = RNA
  misc_feature 18: note = DNA
  misc_feature 19: note = RNA
  misc_feature 20: note = RNA
  misc_feature 21: note = RNA
  source 1..21: mol_type = other RNA
taccaatttatgcctacagcc

SEQ ID NO: 83 - RNA, 23 nt, synthetic construct
  modified_base 1: mod_base = OTHER; note = 2'-O-methyluridine-3'-phosphorothioate
  modified_base 2: mod_base = OTHER; note = 2'-fluoroadenosine-3'-phosporothioate
  modified_base 3: mod_base = OTHER; note = 2'-O-methylcytidine-3'-phosphorothioate
  modified_base 4: mod_base = OTHER; note = 2'-fluorocytidine-3'-phosphate
  modified_base 5: mod_base = OTHER; note = 2'-O-methyladenosine-3'-phosphate
  modified_base 6: mod_base = OTHER; note = 2'-fluoroadenosine-3'-phosphate
  modified_base 7: mod_base = OTHER; note = 2'-O-methyluridine-3'-phosphate
  modified_base 8: mod_base = OTHER; note = 2'-fluorouridine-3'-phosphate
  modified_base 9: mod_base = OTHER; note = 2'-O-methyluridine-3'-phosphate
  modified_base 10: mod_base = OTHER; note = 2'-fluoroadenosine-3'-phosphate
  modified_base 11: mod_base = OTHER; note = 2'-O-methyluridine-3'-phosphate
  modified_base 12: mod_base = OTHER; note = 2'-fluoroguanosine-3'-phosphate
  modified_base 13: mod_base = OTHER; note = 2'-O-methylcytidine-3'-phosphate
  modified_base 14: mod_base = OTHER; note = 2'-fluorocytidine-3'-phosphate
  modified_base 15: mod_base = OTHER; note = 2'-O-methyluridine-3'-phosphate
  modified_base 16: mod_base = OTHER; note = 2'-fluoroadenosine-3'-phosphate
  modified_base 17: mod_base = OTHER; note = 2'-O-methylcytidine-3'-phosphate
  modified_base 18: mod_base = OTHER; note = 2'-fluoroadenosine-3'-phosphate
  modified_base 19: mod_base = OTHER; note = 2'-O-methylguanosine-3'-phosphate
  modified_base 20: mod_base = OTHER; note = 2'-O-methylcytidine-3'-phosphate
  modified_base 21: mod_base = OTHER; note = 2'-O-methylcytidine-3'-phosphate
  modified_base 22: mod_base = OTHER; note = 2'-O-methyluridine-3'-phosphorothioate
  modified_base 23: mod_base = OTHER; note = 2'-O-methyluridine-3'-phosphate
  misc_feature 1: note = RNA
  misc_feature 2: note = DNA
  misc_feature 3: note = RNA
  misc_feature 4: note = DNA
  misc_feature 5: note = RNA
  misc_feature 6: note = DNA
  misc_feature 7: note = RNA
  misc_feature 8: note = DNA
  misc_feature 9: note = RNA
  misc_feature 10: note = DNA
  misc_feature 11: note = RNA
  misc_feature 12: note = DNA
  misc_feature 13: note = RNA
  misc_feature 14: note = DNA
  misc_feature 15: note = RNA
  misc_feature 16: note = DNA
  misc_feature 17: note = RNA
  misc_feature 18: note = DNA
  misc_feature 19: note = RNA
  misc_feature 20: note = RNA
  misc_feature 21: note = RNA
  misc_feature 22: note = RNA
  misc_feature 23: note = RNA
  source 1..23: mol_type = other RNA
taccaatttatgcctacagcctt

SEQ ID NO: 84 - RNA, 23 nt, synthetic construct
  modified_base 1: mod_base = OTHER; note = 2'-O-methyluridine-3'-phosphorothioate
  modified_base 2: mod_base = OTHER; note = 2'-fluoroadenosine-3'-phosporothioate
  modified_base 3: mod_base = OTHER; note = 2'-O-methylcytidine-3'-phosphorothioate
  modified_base 4: mod_base = OTHER; note = 2'-fluorocytidine-3'-phosphate
  modified_base 5: mod_base = OTHER; note = 2'-O-methyladenosine-3'-phosphate
  modified_base 6: mod_base = OTHER; note = 2'-fluoroadenosine-3'-phosphate
  modified_base 7: mod_base = OTHER; note = 2'-O-methyluridine-3'-phosphate
  modified_base 8: mod_base = OTHER; note = 2'-fluorouridine-3'-phosphate
  modified_base 9: mod_base = OTHER; note = 2'-O-methyluridine-3'-phosphate
  modified_base 10: mod_base = OTHER; note = 2'-fluoroadenosine-3'-phosphate
  modified_base 11: mod_base = OTHER; note = 2'-O-methyluridine-3'-phosphate
  modified_base 12: mod_base = OTHER; note = 2'-fluoroguanosine-3'-phosphate
  modified_base 13: mod_base = OTHER; note = 2'-O-methylcytidine-3'-phosphate
  modified_base 14: mod_base = OTHER; note = 2'-fluorocytidine-3'-phosphate
  modified_base 15: mod_base = OTHER; note = 2'-O-methyluridine-3'-phosphate
  modified_base 16: mod_base = OTHER; note = 2'-fluoroadenosine-3'-phosphate
  modified_base 17: mod_base = OTHER; note = 2'-O-methylcytidine-3'-phosphate
  modified_base 18: mod_base = OTHER; note = 2'-fluoroadenosine-3'-phosphate
  modified_base 19: mod_base = OTHER; note = 2'-O-methylguanosine-3'-phosphate
  modified_base 20: mod_base = OTHER; note = 2'-O-methylcytidine-3'-phosphate
  modified_base 21: mod_base = OTHER; note = 2'-O-methylcytidine-3'-phosphate
  modified_base 22: mod_base = OTHER; note = 2'-O-methyluridine-3'-phosphorothioate
  modified_base 23: mod_base = OTHER; note = 2'-O-methylcytidine-3'-phosphate
  misc_feature 1: note = RNA
  misc_feature 2: note = DNA
  misc_feature 3: note = RNA
  misc_feature 4: note = DNA
  misc_feature 5: note = RNA
  misc_feature 6: note = DNA
  misc_feature 7: note = RNA
  misc_feature 8: note = DNA
  misc_feature 9: note = RNA
  misc_feature 10: note = DNA
  misc_feature 11: note = RNA
  misc_feature 12: note = DNA
  misc_feature 13: note = RNA
  misc_feature 14: note = DNA
  misc_feature 15: note = RNA
  misc_feature 16: note = DNA
  misc_feature 17: note = RNA
  misc_feature 18: note = DNA
  misc_feature 19: note = RNA
  misc_feature 20: note = RNA
  misc_feature 21: note = RNA
  misc_feature 22: note = RNA
  misc_feature 23: note = RNA
  source 1..23: mol_type = other RNA
taccaatttatgcctacagcctc

SEQ ID NO: 85 - RNA, 21 nt, synthetic construct
  modified_base 1: mod_base = OTHER; note = 2'-O-methyluridine-3'-phosphorothioate
  modified_base 2: mod_base = OTHER; note = 2'-fluoroadenosine-3'-phosporothioate
  modified_base 3: mod_base = OTHER; note = 2'-O-methylcytidine-3'-phosphorothioate
  modified_base 4: mod_base = OTHER; note = 2'-O-methylcytidine-3'-phosphate
  modified_base 5: mod_base = OTHER; note = 2'-O-methyladenosine-3'-phosphate
  modified_base 6: mod_base = OTHER; note = 2'-O-methyladenosine-3'-phosphate
  modified_base 7: mod_base = OTHER; note = 2'-O-methyluridine-3'-phosphate
  modified_base 8: mod_base = OTHER; note = 2'-fluorouridine-3'-phosphate
  modified_base 9: mod_base = OTHER; note = 2'-O-methyluridine-3'-phosphate
  modified_base 10: mod_base = OTHER; note = 2'-fluoroadenosine-3'-phosphate
  modified_base 11: mod_base = OTHER; note = 2'-O-methyluridine-3'-phosphate
  modified_base 12: mod_base = OTHER; note = 2'-fluoroguanosine-3'-phosphate
  modified_base 13: mod_base = OTHER; note = 2'-O-methylcytidine-3'-phosphate
  modified_base 14: mod_base = OTHER; note = 2'-fluorocytidine-3'-phosphate
  modified_base 15: mod_base = OTHER; note = 2'-O-methyluridine-3'-phosphate
  modified_base 16: mod_base = OTHER; note = 2'-O-methyladenosine-3'-phosphate
  modified_base 17: mod_base = OTHER; note = 2'-O-methylcytidine-3'-phosphate
  modified_base 18: mod_base = OTHER; note = 2'-O-methyladenosine-3'-phosphate
  modified_base 19: mod_base = OTHER; note = 2'-O-methylguanosine-3'-phosphate
  modified_base 20: mod_base = OTHER; note = 2'-O-methylcytidine-3'-phosphorothioate
  modified_base 21: mod_base = OTHER; note = 2'-O-methylcytidine-3'-phosphate
  misc_feature 1: note = RNA
  misc_feature 2: note = DNA
  misc_feature 3: note = RNA
  misc_feature 4: note = RNA
  misc_feature 5: note = RNA
  misc_feature 6: note = RNA
  misc_feature 7: note = RNA
  misc_feature 8: note = DNA
  misc_feature 9: note = RNA
  misc_feature 10: note = DNA
  misc_feature 11: note = RNA
  misc_feature 12: note = DNA
  misc_feature 13: note = RNA
  misc_feature 14: note = DNA
  misc_feature 15: note = RNA
  misc_feature 16: note = RNA
  misc_feature 17: note = RNA
  misc_feature 18: note = RNA
  misc_feature 19: note = RNA
  misc_feature 20: note = RNA
  misc_feature 21: note = RNA
  source 1..21: mol_type = other RNA
taccaatttatgcctacagcc

SEQ ID NO: 86 - RNA, 23 nt, synthetic construct
  modified_base 1: mod_base = OTHER; note = 2'-O-methyluridine-3'-phosphorothioate
  modified_base 2: mod_base = OTHER; note = 2'-fluoroadenosine-3'-phosporothioate
  modified_base 3: mod_base = OTHER; note = 2'-O-methylcytidine-3'-phosphorothioate
  modified_base 4: mod_base = OTHER; note = 2'-O-methylcytidine-3'-phosphate
  modified_base 5: mod_base = OTHER; note = 2'-O-methyladenosine-3'-phosphate
  modified_base 6: mod_base = OTHER; note = 2'-O-methyladenosine-3'-phosphate
  modified_base 7: mod_base = OTHER; note = 2'-O-methyluridine-3'-phosphate
  modified_base 8: mod_base = OTHER; note = 2'-fluorouridine-3'-phosphate
  modified_base 9: mod_base = OTHER; note = 2'-O-methyluridine-3'-phosphate
  modified_base 10: mod_base = OTHER; note = 2'-fluoroadenosine-3'-phosphate
  modified_base 11: mod_base = OTHER; note = 2'-O-methyluridine-3'-phosphate
  modified_base 12: mod_base = OTHER; note = 2'-fluoroguanosine-3'-phosphate
  modified_base 13: mod_base = OTHER; note = 2'-O-methylcytidine-3'-phosphate
  modified_base 14: mod_base = OTHER; note = 2'-fluorocytidine-3'-phosphate
  modified_base 15: mod_base = OTHER; note = 2'-O-methyluridine-3'-phosphate
  modified_base 16: mod_base = OTHER; note = 2'-O-methyladenosine-3'-phosphate
  modified_base 17: mod_base = OTHER; note = 2'-O-methylcytidine-3'-phosphate
  modified_base 18: mod_base = OTHER; note = 2'-O-methyladenosine-3'-phosphate
  modified_base 19: mod_base = OTHER; note = 2'-O-methylguanosine-3'-phosphate
  modified_base 20: mod_base = OTHER; note = 2'-O-methylcytidine-3'-phosphate
  modified_base 21: mod_base = OTHER; note = 2'-O-methylcytidine-3'-phosphate
  modified_base 22: mod_base = OTHER; note = 2'-O-methyluridine-3'-phosphorothioate
  modified_base 23: mod_base = OTHER; note = 2'-O-methyluridine-3'-phosphate
  misc_feature 1: note = RNA
  misc_feature 2: note = DNA
  misc_feature 3: note = RNA
  misc_feature 4: note = RNA
  misc_feature 5: note = RNA
  misc_feature 6: note = RNA
  misc_feature 7: note = RNA
  misc_feature 8: note = DNA
  misc_feature 9: note = RNA
  misc_feature 10: note = DNA
  misc_feature 11: note = RNA
  misc_feature 12: note = DNA
  misc_feature 13: note = RNA
  misc_feature 14: note = DNA
  misc_feature 15: note = RNA
  misc_feature 16: note = RNA
  misc_feature 17: note = RNA
  misc_feature 18: note = RNA
  misc_feature 19: note = RNA
  misc_feature 20: note = RNA
  misc_feature 21: note = RNA
  misc_feature 22: note = RNA
  misc_feature 23: note = RNA
  source 1..23: mol_type = other RNA
taccaatttatgcctacagcctt

SEQ ID NO: 87 - RNA, 23 nt, synthetic construct
  modified_base 1: mod_base = OTHER; note = 2'-O-methyluridine-3'-phosphorothioate
  modified_base 2: mod_base = OTHER; note = 2'-fluoroadenosine-3'-phosporothioate
  modified_base 3: mod_base = OTHER; note = 2'-O-methylcytidine-3'-phosphorothioate
  modified_base 4: mod_base = OTHER; note = 2'-O-methylcytidine-3'-phosphate
  modified_base 5: mod_base = OTHER; note = 2'-O-methyladenosine-3'-phosphate
  modified_base 6: mod_base = OTHER; note = 2'-O-methyladenosine-3'-phosphate
  modified_base 7: mod_base = OTHER; note = 2'-O-methyluridine-3'-phosphate
  modified_base 8: mod_base = OTHER; note = 2'-fluorouridine-3'-phosphate
  modified_base 9: mod_base = OTHER; note = 2'-O-methyluridine-3'-phosphate
  modified_base 10: mod_base = OTHER; note = 2'-fluoroadenosine-3'-phosphate
  modified_base 11: mod_base = OTHER; note = 2'-O-methyluridine-3'-phosphate
  modified_base 12: mod_base = OTHER; note = 2'-fluoroguanosine-3'-phosphate
  modified_base 13: mod_base = OTHER; note = 2'-O-methylcytidine-3'-phosphate
  modified_base 14: mod_base = OTHER; note = 2'-fluorocytidine-3'-phosphate
  modified_base 15: mod_base = OTHER; note = 2'-O-methyluridine-3'-phosphate
  modified_base 16: mod_base = OTHER; note = 2'-O-methyladenosine-3'-phosphate
  modified_base 17: mod_base = OTHER; note = 2'-O-methylcytidine-3'-phosphate
  modified_base 18: mod_base = OTHER; note = 2'-O-methyladenosine-3'-phosphate
  modified_base 19: mod_base = OTHER; note = 2'-O-methylguanosine-3'-phosphate
  modified_base 20: mod_base = OTHER; note = 2'-O-methylcytidine-3'-phosphate
  modified_base 21: mod_base = OTHER; note = 2'-O-methylcytidine-3'-phosphate
  modified_base 22: mod_base = OTHER; note = 2'-O-methyluridine-3'-phosphorothioate
  modified_base 23: mod_base = OTHER; note = 2'-O-methylcytidine-3'-phosphate
  misc_feature 1: note = RNA
  misc_feature 2: note = DNA
  misc_feature 3: note = RNA
  misc_feature 4: note = RNA
  misc_feature 5: note = RNA
  misc_feature 6: note = RNA
  misc_feature 7: note = RNA
  misc_feature 8: note = DNA
  misc_feature 9: note = RNA
  misc_feature 10: note = DNA
  misc_feature 11: note = RNA
  misc_feature 12: note = DNA
  misc_feature 13: note = RNA
  misc_feature 14: note = DNA
  misc_feature 15: note = RNA
  misc_feature 16: note = RNA
  misc_feature 17: note = RNA
  misc_feature 18: note = RNA
  misc_feature 19: note = RNA
  misc_feature 20: note = RNA
  misc_feature 21: note = RNA
  misc_feature 22: note = RNA
  misc_feature 23: note = RNA
  source 1..23: mol_type = other RNA
taccaatttatgcctacagcctc

SEQ ID NO: 88 - RNA, 21 nt, synthetic construct
  modified_base 1: mod_base = OTHER; note = 2'-O-methyladenosine-3'-phosphorothioate
  modified_base 2: mod_base = OTHER; note = 2'-fluorouridine-3'-phosphorothioate
  modified_base 3: mod_base = OTHER; note = 2'-O-methyluridine-3'-phosphorothioate
  modified_base 4: mod_base = OTHER; note = 2'-O-methylguanosine-3'-phosphate
  modified_base 5: mod_base = OTHER; note = 2'-O-methyladenosine-3'-phosphate
  modified_base 6: mod_base = OTHER; note = 2'-O-methylguanosine-3'-phosphate
  modified_base 7: mod_base = OTHER; note = 2'-O-methyladenosine-3'-phosphate
  modified_base 8: mod_base = OTHER; note = 2'-fluoroguanosine-3'-phosphate
  modified_base 9: mod_base = OTHER; note = 2'-O-methyladenosine-3'-phosphate
  modified_base 10: mod_base = OTHER; note = 2'-fluoroadenosine-3'-phosphate
  modified_base 11: mod_base = OTHER; note = 2'-O-methylguanosine-3'-phosphate
  modified_base 12: mod_base = OTHER; note = 2'-fluorouridine-3'-phosphate
  modified_base 13: mod_base = OTHER; note = 2'-O-methylcytidine-3'-phosphate
  modified_base 14: mod_base = OTHER; note = 2'-fluorocytidine-3'-phosphate
  modified_base 15: mod_base = OTHER; note = 2'-O-methyladenosine-3'-phosphate
  modified_base 16: mod_base = OTHER; note = 2'-O-methylcytidine-3'-phosphate
  modified_base 17: mod_base = OTHER; note = 2'-O-methylcytidine-3'-phosphate
  modified_base 18: mod_base = OTHER; note = 2'-O-methyladenosine-3'-phosphate
  modified_base 19: mod_base = OTHER; note = 2'-O-methylcytidine-3'-phosphate
  modified_base 20: mod_base = OTHER; note = 2'-O-methyluridine-3'-phosphorothioate
  modified_base 21: mod_base = OTHER; note = 2'-O-methyluridine-3'-phosphate
  misc_feature 1: note = RNA
  misc_feature 2: note = DNA
  misc_feature 3: note = RNA
  misc_feature 4: note = RNA
  misc_feature 5: note = RNA
  misc_feature 6: note = RNA
  misc_feature 7: note = RNA
  misc_feature 8: note = DNA
  misc_feature 9: note = RNA
  misc_feature 10: note = DNA
  misc_feature 11: note = RNA
  misc_feature 12: note = DNA
  misc_feature 13: note = RNA
  misc_feature 14: note = DNA
  misc_feature 15: note = RNA
  misc_feature 16: note = RNA
  misc_feature 17: note = RNA
  misc_feature 18: note = RNA
  misc_feature 19: note = RNA
  misc_feature 20: note = RNA
  misc_feature 21: note = RNA
  source 1..21: mol_type = other RNA
attgagagaagtccaccactt

SEQ ID NO: 89 - RNA, 21 nt, synthetic construct
  modified_base 1: mod_base = OTHER; note = 2'-O-methyluridine-3'-phosphorothioate
  modified_base 2: mod_base = OTHER; note = 2'-fluorouridine-3'-phosphorothioate
  modified_base 3: mod_base = OTHER; note = 2'-O-methyluridine-3'-phosphorothioate
  modified_base 4: mod_base = OTHER; note = 2'-fluoroguanosine-3'-phosphate
  modified_base 5: mod_base = OTHER; note = 2'-O-methyladenosine-3'-phosphate
  modified_base 6: mod_base = OTHER; note = 2'-fluoroguanosine-3'-phosphate
  modified_base 7: mod_base = OTHER; note = 2'-O-methyladenosine-3'-phosphate
  modified_base 8: mod_base = OTHER; note = 2'-fluoroguanosine-3'-phosphate
  modified_base 9: mod_base = OTHER; note = 2'-O-methyladenosine-3'-phosphate
  modified_base 10: mod_base = OTHER; note = 2'-fluoroadenosine-3'-phosphate
  modified_base 11: mod_base = OTHER; note = 2'-O-methylguanosine-3'-phosphate
  modified_base 12: mod_base = OTHER; note = 2'-fluorouridine-3'-phosphate
  modified_base 13: mod_base = OTHER; note = 2'-O-methylcytidine-3'-phosphate
  modified_base 14: mod_base = OTHER; note = 2'-fluorocytidine-3'-phosphate
  modified_base 15: mod_base = OTHER; note = 2'-O-methyladenosine-3'-phosphate
  modified_base 16: mod_base = OTHER; note = 2'-fluorocytidine-3'-phosphate
  modified_base 17: mod_base = OTHER; note = 2'-O-methylcytidine-3'-phosphate
  modified_base 18: mod_base = OTHER; note = 2'-fluoroadenosine-3'-phosphate
  modified_base 19: mod_base = OTHER; note = 2'-O-methylcytidine-3'-phosphate
  modified_base 20: mod_base = OTHER; note = 2'-O-methyluridine-3'-phosphorothioate
  modified_base 21: mod_base = OTHER; note = 2'-O-methyluridine-3'-phosphate
  misc_feature 1: note = RNA
  misc_feature 2: note = DNA
  misc_feature 3: note = RNA
  misc_feature 4: note = DNA
  misc_feature 5: note = RNA
  misc_feature 6: note = DNA
  misc_feature 7: note = RNA
  misc_feature 8: note = DNA
  misc_feature 9: note = RNA
  misc_feature 10: note = DNA
  misc_feature 11: note = RNA
  misc_feature 12: note = DNA
  misc_feature 13: note = RNA
  misc_feature 14: note = DNA
  misc_feature 15: note = RNA
  misc_feature 16: note = DNA
  misc_feature 17: note = RNA
  misc_feature 18: note = DNA
  misc_feature 19: note = RNA
  misc_feature 20: note = RNA
  misc_feature 21: note = RNA
  source 1..21: mol_type = other RNA
tttgagagaagtccaccactt

SEQ ID NO: 90 - RNA, 23 nt, synthetic construct
  modified_base 1: mod_base = OTHER; note = 2'-O-methyladenosine-3'-phosphorothioate
  modified_base 2: mod_base = OTHER; note = 2'-fluorouridine-3'-phosphorothioate
  modified_base 3: mod_base = OTHER; note = 2'-O-methyluridine-3'-phosphorothioate
  modified_base 4: mod_base = OTHER; note = 2'-fluoroguanosine-3'-phosphate
  modified_base 5: mod_base = OTHER; note = 2'-O-methyladenosine-3'-phosphate
  modified_base 6: mod_base = OTHER; note = 2'-fluoroguanosine-3'-phosphate
  modified_base 7: mod_base = OTHER; note = 2'-O-methyladenosine-3'-phosphate
  modified_base 8: mod_base = OTHER; note = 2'-fluoroguanosine-3'-phosphate
  modified_base 9: mod_base = OTHER; note = 2'-O-methyladenosine-3'-phosphate
  modified_base 10: mod_base = OTHER; note = 2'-fluoroadenosine-3'-phosphate
  modified_base 11: mod_base = OTHER; note = 2'-O-methylguanosine-3'-phosphate
  modified_base 12: mod_base = OTHER; note = 2'-fluorouridine-3'-phosphate
  modified_base 13: mod_base = OTHER; note = 2'-O-methylcytidine-3'-phosphate
  modified_base 14: mod_base = OTHER; note = 2'-fluorocytidine-3'-phosphate
  modified_base 15: mod_base = OTHER; note = 2'-O-methyladenosine-3'-phosphate
  modified_base 16: mod_base = OTHER; note = 2'-fluorocytidine-3'-phosphate
  modified_base 17: mod_base = OTHER; note = 2'-O-methylcytidine-3'-phosphate
  modified_base 18: mod_base = OTHER; note = 2'-fluoroadenosine-3'-phosphate
  modified_base 19: mod_base = OTHER; note = 2'-O-methylcytidine-3'-phosphate
  modified_base 20: mod_base = OTHER; note = 2'-O-methylguanosine-3'-phosphate
  modified_base 21: mod_base = OTHER; note = 2'-O-methylguanosine-3'-phosphate
  modified_base 22: mod_base = OTHER; note = 2'-O-methyluridine-3'-phosphorothioate
  modified_base 23: mod_base = OTHER; note = 2'-O-methyluridine-3'-phosphate
  misc_feature 1: note = RNA
  misc_feature 2: note = DNA
  misc_feature 3: note = RNA
  misc_feature 4: note = DNA
  misc_feature 5: note = RNA
  misc_feature 6: note = DNA
  misc_feature 7: note = RNA
  misc_feature 8: note = DNA
  misc_feature 9: note = RNA
  misc_feature 10: note = DNA
  misc_feature 11: note = RNA
  misc_feature 12: note = DNA
  misc_feature 13: note = RNA
  misc_feature 14: note = DNA
  misc_feature 15: note = RNA
  misc_feature 16: note = DNA
  misc_feature 17: note = RNA
  misc_feature 18: note = DNA
  misc_feature 19: note = RNA
  misc_feature 20: note = RNA
  misc_feature 21: note = RNA
  misc_feature 22: note = RNA
  misc_feature 23: note = RNA
  source 1..23: mol_type = other RNA
attgagagaagtccaccacggtt

SEQ ID NO: 91 - RNA, 23 nt, synthetic construct
  modified_base 1: mod_base = OTHER; note = 2'-O-methyladenosine-3'-phosphorothioate
  modified_base 2: mod_base = OTHER; note = 2'-fluorouridine-3'-phosphorothioate
  modified_base 3: mod_base = OTHER; note = 2'-O-methyluridine-3'-phosphorothioate
  modified_base 4: mod_base = OTHER; note = 2'-O-methylguanosine-3'-phosphate
  modified_base 5: mod_base = OTHER; note = 2'-O-methyladenosine-3'-phosphate
  modified_base 6: mod_base = OTHER; note = 2'-O-methylguanosine-3'-phosphate
  modified_base 7: mod_base = OTHER; note = 2'-O-methyladenosine-3'-phosphate
  modified_base 8: mod_base = OTHER; note = 2'-fluoroguanosine-3'-phosphate
  modified_base 9: mod_base = OTHER; note = 2'-O-methyladenosine-3'-phosphate
  modified_base 10: mod_base = OTHER; note = 2'-fluoroadenosine-3'-phosphate
  modified_base 11: mod_base = OTHER; note = 2'-O-methylguanosine-3'-phosphate
  modified_base 12: mod_base = OTHER; note = 2'-fluorouridine-3'-phosphate
  modified_base 13: mod_base = OTHER; note = 2'-O-methylcytidine-3'-phosphate
  modified_base 14: mod_base = OTHER; note = 2'-fluorocytidine-3'-phosphate
  modified_base 15: mod_base = OTHER; note = 2'-O-methyladenosine-3'-phosphate
  modified_base 16: mod_base = OTHER; note = 2'-O-methylcytidine-3'-phosphate
  modified_base 17: mod_base = OTHER; note = 2'-O-methylcytidine-3'-phosphate
  modified_base 18: mod_base = OTHER; note = 2'-O-methyladenosine-3'-phosphate
  modified_base 19: mod_base = OTHER; note = 2'-O-methylcytidine-3'-phosphate
  modified_base 20: mod_base = OTHER; note = 2'-O-methylguanosine-3'-phosphate
  modified_base 21: mod_base = OTHER; note = 2'-O-methylguanosine-3'-phosphate
  modified_base 22: mod_base = OTHER; note = 2'-O-methyluridine-3'-phosphorothioate
  modified_base 23: mod_base = OTHER; note = 2'-O-methyluridine-3'-phosphate
  misc_feature 1: note = RNA
  misc_feature 2: note = DNA
  misc_feature 3: note = RNA
  misc_feature 4: note = RNA
  misc_feature 5: note = RNA
  misc_feature 6: note = RNA
  misc_feature 7: note = RNA
  misc_feature 8: note = DNA
  misc_feature 9: note = RNA
  misc_feature 10: note = DNA
  misc_feature 11: note = RNA
  misc_feature 12: note = DNA
  misc_feature 13: note = RNA
  misc_feature 14: note = DNA
  misc_feature 15: note = RNA
  misc_feature 16: note = RNA
  misc_feature 17: note = RNA
  misc_feature 18: note = RNA
  misc_feature 19: note = RNA
  misc_feature 20: note = RNA
  misc_feature 21: note = RNA
  misc_feature 22: note = RNA
  misc_feature 23: note = RNA
  source 1..23: mol_type = other RNA
attgagagaagtccaccacggtt

SEQ ID NO: 92 - RNA, 23 nt, synthetic construct
  modified_base 1: mod_base = OTHER; note = 2'-O-methyladenosine-3'-phosphorothioate
  modified_base 2: mod_base = OTHER; note = 2'-fluorouridine-3'-phosphorothioate
  modified_base 3: mod_base = OTHER; note = 2'-O-methyluridine-3'-phosphorothioate
  modified_base 4: mod_base = OTHER; note = 2'-fluoroguanosine-3'-phosphate
  modified_base 5: mod_base = OTHER; note = 2'-O-methyladenosine-3'-phosphate
  modified_base 6: mod_base = OTHER; note = 2'-fluoroguanosine-3'-phosphate
  modified_base 7: mod_base = OTHER; note = 2'-O-methyladenosine-3'-phosphate
  modified_base 8: mod_base = OTHER; note = 2'-fluoroguanosine-3'-phosphate
  modified_base 9: mod_base = OTHER; note = 2'-O-methyladenosine-3'-phosphate
  modified_base 10: mod_base = OTHER; note = 2'-fluoroadenosine-3'-phosphate
  modified_base 11: mod_base = OTHER; note = 2'-O-methylguanosine-3'-phosphate
  modified_base 12: mod_base = OTHER; note = 2'-fluorouridine-3'-phosphate
  modified_base 13: mod_base = OTHER; note = 2'-O-methylcytidine-3'-phosphate
  modified_base 14: mod_base = OTHER; note = 2'-fluorocytidine-3'-phosphate
  modified_base 15: mod_base = OTHER; note = 2'-O-methyladenosine-3'-phosphate
  modified_base 16: mod_base = OTHER; note = 2'-fluorocytidine-3'-phosphate
  modified_base 17: mod_base = OTHER; note = 2'-O-methylcytidine-3'-phosphate
  modified_base 18: mod_base = OTHER; note = 2'-fluoroadenosine-3'-phosphate
  modified_base 19: mod_base = OTHER; note = 2'-O-methylcytidine-3'-phosphate
  modified_base 20: mod_base = OTHER; note = 2'-O-methylguanosine-3'-phosphate
  modified_base 21: mod_base = OTHER; note = 2'-O-methyladenosine-3'-phosphate
  modified_base 22: mod_base = OTHER; note = 2'-O-methylguanosine-3'-phosphorothioate
  modified_base 23: mod_base = OTHER; note = 2'-O-methyluridine-3'-phosphate
  misc_feature 1: note = RNA
  misc_feature 2: note = DNA
  misc_feature 3: note = RNA
  misc_feature 4: note = DNA
  misc_feature 5: note = RNA
  misc_feature 6: note = DNA
  misc_feature 7: note = RNA
  misc_feature 8: note = DNA
  misc_feature 9: note = RNA
  misc_feature 10: note = DNA
  misc_feature 11: note = RNA
  misc_feature 12: note = DNA
  misc_feature 13: note = RNA
  misc_feature 14: note = DNA
  misc_feature 15: note = RNA
  misc_feature 16: note = DNA
  misc_feature 17: note = RNA
  misc_feature 18: note = DNA
  misc_feature 19: note = RNA
  misc_feature 20: note = RNA
  misc_feature 21: note = RNA
  misc_feature 22: note = RNA
  misc_feature 23: note = RNA
  source 1..23: mol_type = other RNA
attgagagaagtccaccacgagt

SEQ ID NO: 93 - RNA, 21 nt, synthetic construct
  modified_base 1: mod_base = OTHER; note = 2'-O-methyluridine-3'-phosphorothioate
  modified_base 2: mod_base = OTHER; note = 2'-fluoroadenosine-3'-phosporothioate
  modified_base 3: mod_base = OTHER; note = 2'-O-methyluridine-3'-phosphorothioate
  modified_base 4: mod_base = OTHER; note = 2'-fluorouridine-3'-phosphate
  modified_base 5: mod_base = OTHER; note = 2'-O-methylguanosine-3'-phosphate
  modified_base 6: mod_base = OTHER; note = 2'-fluoroadenosine-3'-phosphate
  modified_base 7: mod_base = OTHER; note = 2'-O-methylguanosine-3'-phosphate
  modified_base 8: mod_base = OTHER; note = 2'-fluoroadenosine-3'-phosphate
  modified_base 9: mod_base = OTHER; note = 2'-O-methylguanosine-3'-phosphate
  modified_base 10: mod_base = OTHER; note = 2'-fluoroadenosine-3'-phosphate
  modified_base 11: mod_base = OTHER; note = 2'-O-methyladenosine-3'-phosphate
  modified_base 12: mod_base = OTHER; note = 2'-fluoroguanosine-3'-phosphate
  modified_base 13: mod_base = OTHER; note = 2'-O-methyluridine-3'-phosphate
  modified_base 14: mod_base = OTHER; note = 2'-fluorocytidine-3'-phosphate
  modified_base 15: mod_base = OTHER; note = 2'-O-methylcytidine-3'-phosphate
  modified_base 16: mod_base = OTHER; note = 2'-fluoroadenosine-3'-phosphate
  modified_base 17: mod_base = OTHER; note = 2'-O-methylcytidine-3'-phosphate
  modified_base 18: mod_base = OTHER; note = 2'-fluorocytidine-3'-phosphate
  modified_base 19: mod_base = OTHER; note = 2'-O-methyladenosine-3'-phosphate
  modified_base 20: mod_base = OTHER; note = 2'-fluorocytidine-3'-phosphorothioate
  modified_base 21: mod_base = OTHER; note = 2'-O-methylguanosine-3'-phosphate
  misc_feature 1: note = RNA
  misc_feature 2: note = DNA
  misc_feature 3: note = RNA
  misc_feature 4: note = DNA
  misc_feature 5: note = RNA
  misc_feature 6: note = DNA
  misc_feature 7: note = RNA
  misc_feature 8: note = DNA
  misc_feature 9: note = RNA
  misc_feature 10: note = DNA
  misc_feature 11: note = RNA
  misc_feature 12: note = DNA
  misc_feature 13: note = RNA
  misc_feature 14: note = DNA
  misc_feature 15: note = RNA
  misc_feature 16: note = DNA
  misc_feature 17: note = RNA
  misc_feature 18: note = DNA
  misc_feature 19: note = RNA
  misc_feature 20: note = DNA
  misc_feature 21: note = RNA
  source 1..21: mol_type = other RNA
tattgagagaagtccaccacg

SEQ ID NO: 94 - RNA, 21 nt, synthetic construct
  modified_base 1: mod_base = OTHER; note = 2'-O-methyluridine-3'-phosphorothioate
  modified_base 2: mod_base = OTHER; note = 2'-fluoroadenosine-3'-phosporothioate
  modified_base 3: mod_base = OTHER; note = 2'-O-methyluridine-3'-phosphorothioate
  modified_base 4: mod_base = OTHER; note = 2'-O-methyluridine-3'-phosphate
  modified_base 5: mod_base = OTHER; note = 2'-O-methylguanosine-3'-phosphate
  modified_base 6: mod_base = OTHER; note = 2'-O-methyladenosine-3'-phosphate
  modified_base 7: mod_base = OTHER; note = 2'-O-methylguanosine-3'-phosphate
  modified_base 8: mod_base = OTHER; note = 2'-fluoroadenosine-3'-phosphate
  modified_base 9: mod_base = OTHER; note = 2'-O-methylguanosine-3'-phosphate
  modified_base 10: mod_base = OTHER; note = 2'-fluoroadenosine-3'-phosphate
  modified_base 11: mod_base = OTHER; note = 2'-O-methyladenosine-3'-phosphate
  modified_base 12: mod_base = OTHER; note = 2'-fluoroguanosine-3'-phosphate
  modified_base 13: mod_base = OTHER; note = 2'-O-methyluridine-3'-phosphate
  modified_base 14: mod_base = OTHER; note = 2'-fluorocytidine-3'-phosphate
  modified_base 15: mod_base = OTHER; note = 2'-O-methylcytidine-3'-phosphate
  modified_base 16: mod_base = OTHER; note = 2'-O-methyladenosine-3'-phosphate
  modified_base 17: mod_base = OTHER; note = 2'-O-methylcytidine-3'-phosphate
  modified_base 18: mod_base = OTHER; note = 2'-O-methylcytidine-3'-phosphate
  modified_base 19: mod_base = OTHER; note = 2'-O-methyladenosine-3'-phosphate
  modified_base 20: mod_base = OTHER; note = 2'-O-methylcytidine-3'-phosphorothioate
  modified_base 21: mod_base = OTHER; note = 2'-O-methylguanosine-3'-phosphate
  misc_feature 1: note = RNA
  misc_feature 2: note = DNA
  misc_feature 3: note = RNA
  misc_feature 4: note = RNA
  misc_feature 5: note = RNA
  misc_feature 6: note = RNA
  misc_feature 7: note = RNA
  misc_feature 8: note = DNA
  misc_feature 9: note = RNA
  misc_feature 10: note = DNA
  misc_feature 11: note = RNA
  misc_feature 12: note = DNA
  misc_feature 13: note = RNA
  misc_feature 14: note = DNA
  misc_feature 15: note = RNA
  misc_feature 16: note = RNA
  misc_feature 17: note = RNA
  misc_feature 18: note = RNA
  misc_feature 19: note = RNA
  misc_feature 20: note = RNA
  misc_feature 21: note = RNA
  source 1..21: mol_type = other RNA
tattgagagaagtccaccacg

SEQ ID NO: 95 - RNA, 23 nt, synthetic construct
  modified_base 1: mod_base = OTHER; note = 2'-O-methyluridine-3'-phosphorothioate
  modified_base 2: mod_base = OTHER; note = 2'-fluoroadenosine-3'-phosporothioate
  modified_base 3: mod_base = OTHER; note = 2'-O-methyluridine-3'-phosphorothioate
  modified_base 4: mod_base = OTHER; note = 2'-fluorouridine-3'-phosphate
  modified_base 5: mod_base = OTHER; note = 2'-O-methylguanosine-3'-phosphate
  modified_base 6: mod_base = OTHER; note = 2'-fluoroadenosine-3'-phosphate
  modified_base 7: mod_base = OTHER; note = 2'-O-methylguanosine-3'-phosphate
  modified_base 8: mod_base = OTHER; note = 2'-fluoroadenosine-3'-phosphate
  modified_base 9: mod_base = OTHER; note = 2'-O-methylguanosine-3'-phosphate
  modified_base 10: mod_base = OTHER; note = 2'-fluoroadenosine-3'-phosphate
  modified_base 11: mod_base = OTHER; note = 2'-O-methyladenosine-3'-phosphate
  modified_base 12: mod_base = OTHER; note = 2'-fluoroguanosine-3'-phosphate
  modified_base 13: mod_base = OTHER; note = 2'-O-methyluridine-3'-phosphate
  modified_base 14: mod_base = OTHER; note = 2'-fluorocytidine-3'-phosphate
  modified_base 15: mod_base = OTHER; note = 2'-O-methylcytidine-3'-phosphate
  modified_base 16: mod_base = OTHER; note = 2'-fluoroadenosine-3'-phosphate
  modified_base 17: mod_base = OTHER; note = 2'-O-methylcytidine-3'-phosphate
  modified_base 18: mod_base = OTHER; note = 2'-fluorocytidine-3'-phosphate
  modified_base 19: mod_base = OTHER; note = 2'-O-methyladenosine-3'-phosphate
  modified_base 20: mod_base = OTHER; note = 2'-fluorocytidine-3'-phosphate
  modified_base 21: mod_base = OTHER; note = 2'-O-methylguanosine-3'-phosphate
  modified_base 22: mod_base = OTHER; note = 2'-O-methyluridine-3'-phosphorothioate
  modified_base 23: mod_base = OTHER; note = 2'-O-methyluridine-3'-phosphate
  misc_feature 1: note = RNA
  misc_feature 2: note = DNA
  misc_feature 3: note = RNA
  misc_feature 4: note = DNA
  misc_feature 5: note = RNA
  misc_feature 6: note = DNA
  misc_feature 7: note = RNA
  misc_feature 8: note = DNA
  misc_feature 9: note = RNA
  misc_feature 10: note = DNA
  misc_feature 11: note = RNA
  misc_feature 12: note = DNA
  misc_feature 13: note = RNA
  misc_feature 14: note = DNA
  misc_feature 15: note = RNA
  misc_feature 16: note = DNA
  misc_feature 17: note = RNA
  misc_feature 18: note = DNA
  misc_feature 19: note = RNA
  misc_feature 20: note = DNA
  misc_feature 21: note = RNA
  misc_feature 22: note = RNA
  misc_feature 23: note = RNA
  source 1..23: mol_type = other RNA
tattgagagaagtccaccacgtt

SEQ ID NO: 96 - RNA, 23 nt, synthetic construct
  modified_base 1: mod_base = OTHER; note = 2'-O-methyluridine-3'-phosphorothioate
  modified_base 2: mod_base = OTHER; note = 2'-fluoroadenosine-3'-phosporothioate
  modified_base 3: mod_base = OTHER; note = 2'-O-methyluridine-3'-phosphorothioate
  modified_base 4: mod_base = OTHER; note = 2'-O-methyluridine-3'-phosphate
  modified_base 5: mod_base = OTHER; note = 2'-O-methylguanosine-3'-phosphate
  modified_base 6: mod_base = OTHER; note = 2'-O-methyladenosine-3'-phosphate
  modified_base 7: mod_base = OTHER; note = 2'-O-methylguanosine-3'-phosphate
  modified_base 8: mod_base = OTHER; note = 2'-fluoroadenosine-3'-phosphate
  modified_base 9: mod_base = OTHER; note = 2'-O-methylguanosine-3'-phosphate
  modified_base 10: mod_base = OTHER; note = 2'-fluoroadenosine-3'-phosphate
  modified_base 11: mod_base = OTHER; note = 2'-O-methyladenosine-3'-phosphate
  modified_base 12: mod_base = OTHER; note = 2'-fluoroguanosine-3'-phosphate
  modified_base 13: mod_base = OTHER; note = 2'-O-methyluridine-3'-phosphate
  modified_base 14: mod_base = OTHER; note = 2'-fluorocytidine-3'-phosphate
  modified_base 15: mod_base = OTHER; note = 2'-O-methylcytidine-3'-phosphate
  modified_base 16: mod_base = OTHER; note = 2'-O-methyladenosine-3'-phosphate
  modified_base 17: mod_base = OTHER; note = 2'-O-methylcytidine-3'-phosphate
  modified_base 18: mod_base = OTHER; note = 2'-O-methylcytidine-3'-phosphate
  modified_base 19: mod_base = OTHER; note = 2'-O-methyladenosine-3'-phosphate
  modified_base 20: mod_base = OTHER; note = 2'-O-methylcytidine-3'-phosphate
  modified_base 21: mod_base = OTHER; note = 2'-O-methylguanosine-3'-phosphate
  modified_base 22: mod_base = OTHER; note = 2'-O-methyladenosine-3'-phosphorothioate
  modified_base 23: mod_base = OTHER; note = 2'-O-methylguanosine-3'-phosphate
  misc_feature 1: note = RNA
  misc_feature 2: note = DNA
  misc_feature 3: note = RNA
  misc_feature 4: note = RNA
  misc_feature 5: note = RNA
  misc_feature 6: note = RNA
  misc_feature 7: note = RNA
  misc_feature 8: note = DNA
  misc_feature 9: note = RNA
  misc_feature 10: note = DNA
  misc_feature 11: note = RNA
  misc_feature 12: note = DNA
  misc_feature 13: note = RNA
  misc_feature 14: note = DNA
  misc_feature 15: note = RNA
  misc_feature 16: note = RNA
  misc_feature 17: note = RNA
  misc_feature 18: note = RNA
  misc_feature 19: note = RNA
  misc_feature 20: note = RNA
  misc_feature 21: note = RNA
  misc_feature 22: note = RNA
  misc_feature 23: note = RNA
  source 1..23: mol_type = other RNA
tattgagagaagtccaccacgag

SEQ ID NO: 97 - RNA, 23 nt, synthetic construct
  modified_base 1: mod_base = OTHER; note = 2'-O-methyluridine-3'-phosphorothioate
  modified_base 2: mod_base = OTHER; note = 2'-fluoroadenosine-3'-phosporothioate
  modified_base 3: mod_base = OTHER; note = 2'-O-methyluridine-3'-phosphorothioate
  modified_base 4: mod_base = OTHER; note = 2'-fluorouridine-3'-phosphate
  modified_base 5: mod_base = OTHER; note = 2'-O-methylguanosine-3'-phosphate
  modified_base 6: mod_base = OTHER; note = 2'-fluoroadenosine-3'-phosphate
  modified_base 7: mod_base = OTHER; note = 2'-O-methylguanosine-3'-phosphate
  modified_base 8: mod_base = OTHER; note = 2'-fluoroadenosine-3'-phosphate
  modified_base 9: mod_base = OTHER; note = 2'-O-methylguanosine-3'-phosphate
  modified_base 10: mod_base = OTHER; note = 2'-fluoroadenosine-3'-phosphate
  modified_base 11: mod_base = OTHER; note = 2'-O-methyladenosine-3'-phosphate
  modified_base 12: mod_base = OTHER; note = 2'-fluoroguanosine-3'-phosphate
  modified_base 13: mod_base = OTHER; note = 2'-O-methyluridine-3'-phosphate
  modified_base 14: mod_base = OTHER; note = 2'-fluorocytidine-3'-phosphate
  modified_base 15: mod_base = OTHER; note = 2'-O-methylcytidine-3'-phosphate
  modified_base 16: mod_base = OTHER; note = 2'-fluoroadenosine-3'-phosphate
  modified_base 17: mod_base = OTHER; note = 2'-O-methylcytidine-3'-phosphate
  modified_base 18: mod_base = OTHER; note = 2'-fluorocytidine-3'-phosphate
  modified_base 19: mod_base = OTHER; note = 2'-O-methyladenosine-3'-phosphate
  modified_base 20: mod_base = OTHER; note = 2'-fluorocytidine-3'-phosphate
  modified_base 21: mod_base = OTHER; note = 2'-O-methylguanosine-3'-phosphate
  modified_base 22: mod_base = OTHER; note = 2'-O-methyladenosine-3'-phosphorothioate
  modified_base 23: mod_base = OTHER; note = 2'-O-methylguanosine-3'-phosphate
  misc_feature 1: note = RNA
  misc_feature 2: note = DNA
  misc_feature 3: note = RNA
  misc_feature 4: note = DNA
  misc_feature 5: note = RNA
  misc_feature 6: note = DNA
  misc_feature 7: note = RNA
  misc_feature 8: note = DNA
  misc_feature 9: note = RNA
  misc_feature 10: note = DNA
  misc_feature 11: note = RNA
  misc_feature 12: note = DNA
  misc_feature 13: note = RNA
  misc_feature 14: note = DNA
  misc_feature 15: note = RNA
  misc_feature 16: note = DNA
  misc_feature 17: note = RNA
  misc_feature 18: note = DNA
  misc_feature 19: note = RNA
  misc_feature 20: note = DNA
  misc_feature 21: note = RNA
  misc_feature 22: note = RNA
  misc_feature 23: note = RNA
  source 1..23: mol_type = other RNA
tattgagagaagtccaccacgag

SEQ ID NO: 98 - RNA, 22 nt, synthetic construct
  modified_base 1: mod_base = OTHER; note = 2'-O-methyluridine-3'-phosphorothioate
  modified_base 2: mod_base = OTHER; note = 2'-fluoroadenosine-3'-phosporothioate
  modified_base 3: mod_base = OTHER; note = 2'-O-methyluridine-3'-phosphorothioate
  modified_base 4: mod_base = OTHER; note = 2'-fluorouridine-3'-phosphate
  modified_base 5: mod_base = OTHER; note = 2'-O-methylguanosine-3'-phosphate
  modified_base 6: mod_base = OTHER; note = 2'-fluoroadenosine-3'-phosphate
  modified_base 7: mod_base = OTHER; note = 2'-O-methylguanosine-3'-phosphate
  modified_base 8: mod_base = OTHER; note = 2'-fluoroadenosine-3'-phosphate
  modified_base 9: mod_base = OTHER; note = 2'-O-methylguanosine-3'-phosphate
  modified_base 10: mod_base = OTHER; note = 2'-fluoroadenosine-3'-phosphate
  modified_base 11: mod_base = OTHER; note = 2'-O-methyladenosine-3'-phosphate
  modified_base 12: mod_base = OTHER; note = 2'-fluoroguanosine-3'-phosphate
  modified_base 13: mod_base = OTHER; note = 2'-O-methyluridine-3'-phosphate
  modified_base 14: mod_base = OTHER; note = 2'-fluorocytidine-3'-phosphate
  modified_base 15: mod_base = OTHER; note = 2'-O-methylcytidine-3'-phosphate
  modified_base 16: mod_base = OTHER; note = 2'-fluoroadenosine-3'-phosphate
  modified_base 17: mod_base = OTHER; note = 2'-O-methylcytidine-3'-phosphate
  modified_base 18: mod_base = OTHER; note = 2'-fluorocytidine-3'-phosphate
  modified_base 19: mod_base = OTHER; note = 2'-O-methyladenosine-3'-phosphate
  modified_base 20: mod_base = OTHER; note = 2'-fluorocytidine-3'-phosphate
  modified_base 21: mod_base = OTHER; note = 2'-O-methylguanosine-3'-phosphorothioate
  modified_base 22: mod_base = OTHER; note = 2'-O-methyladenosine-3'-phosphate
  misc_feature 1: note = RNA
  misc_feature 2: note = DNA
  misc_feature 3: note = RNA
  misc_feature 4: note = DNA
  misc_feature 5: note = RNA
  misc_feature 6: note = DNA
  misc_feature 7: note = RNA
  misc_feature 8: note = DNA
  misc_feature 9: note = RNA
  misc_feature 10: note = DNA
  misc_feature 11: note = RNA
  misc_feature 12: note = DNA
  misc_feature 13: note = RNA
  misc_feature 14: note = DNA
  misc_feature 15: note = RNA
  misc_feature 16: note = DNA
  misc_feature 17: note = RNA
  misc_feature 18: note = DNA
  misc_feature 19: note = RNA
  misc_feature 20: note = DNA
  misc_feature 21: note = RNA
  misc_feature 22: note = RNA
  source 1..22: mol_type = other RNA
tattgagagaagtccaccacga

SEQ ID NO: 99 - RNA, 22 nt, synthetic construct
  modified_base 1: mod_base = OTHER; note = 2'-O-methyluridine-3'-phosphorothioate
  modified_base 2: mod_base = OTHER; note = 2'-fluoroadenosine-3'-phosporothioate
  modified_base 3: mod_base = OTHER; note = 2'-O-methyluridine-3'-phosphorothioate
  modified_base 4: mod_base = OTHER; note = 2'-O-methyluridine-3'-phosphate
  modified_base 5: mod_base = OTHER; note = 2'-O-methylguanosine-3'-phosphate
  modified_base 6: mod_base = OTHER; note = 2'-O-methyladenosine-3'-phosphate
  modified_base 7: mod_base = OTHER; note = 2'-O-methylguanosine-3'-phosphate
  modified_base 8: mod_base = OTHER; note = 2'-fluoroadenosine-3'-phosphate
  modified_base 9: mod_base = OTHER; note = 2'-O-methylguanosine-3'-phosphate
  modified_base 10: mod_base = OTHER; note = 2'-fluoroadenosine-3'-phosphate
  modified_base 11: mod_base = OTHER; note = 2'-O-methyladenosine-3'-phosphate
  modified_base 12: mod_base = OTHER; note = 2'-fluoroguanosine-3'-phosphate
  modified_base 13: mod_base = OTHER; note = 2'-O-methyluridine-3'-phosphate
  modified_base 14: mod_base = OTHER; note = 2'-fluorocytidine-3'-phosphate
  modified_base 15: mod_base = OTHER; note = 2'-O-methylcytidine-3'-phosphate
  modified_base 16: mod_base = OTHER; note = 2'-O-methyladenosine-3'-phosphate
  modified_base 17: mod_base = OTHER; note = 2'-O-methylcytidine-3'-phosphate
  modified_base 18: mod_base = OTHER; note = 2'-O-methylcytidine-3'-phosphate
  modified_base 19: mod_base = OTHER; note = 2'-O-methyladenosine-3'-phosphate
  modified_base 20: mod_base = OTHER; note = 2'-O-methylcytidine-3'-phosphate
  modified_base 21: mod_base = OTHER; note = 2'-O-methylguanosine-3'-phosphorothioate
  modified_base 22: mod_base = OTHER; note = 2'-O-methyladenosine-3'-phosphate
  misc_feature 1: note = RNA
  misc_feature 2: note = DNA
  misc_feature 3: note = RNA
  misc_feature 4: note = RNA
  misc_feature 5: note = RNA
  misc_feature 6: note = RNA
  misc_feature 7: note = RNA
  misc_feature 8: note = DNA
  misc_feature 9: note = RNA
  misc_feature 10: note = DNA
  misc_feature 11: note = RNA
  misc_feature 12: note = DNA
  misc_feature 13: note = RNA
  misc_feature 14: note = DNA
  misc_feature 15: note = RNA
  misc_feature 16: note = RNA
  misc_feature 17: note = RNA
  misc_feature 18: note = RNA
  misc_feature 19: note = RNA
  misc_feature 20: note = RNA
  misc_feature 21: note = RNA
  misc_feature 22: note = RNA
  source 1..22: mol_type = other RNA
tattgagagaagtccaccacga

SEQ ID NO: 100 - RNA, 21 nt, synthetic construct
  modified_base 1: mod_base = OTHER; note = 2'-O-methyladenosine-3'-phosphorothioate
  modified_base 2: mod_base = OTHER; note = 2'-fluoroguanosine-3'-phosphorothioate
  modified_base 3: mod_base = OTHER; note = 2'-O-methyladenosine-3'-phosphorothioate
  modified_base 4: mod_base = OTHER; note = 2'-fluoroadenosine-3'-phosphate
  modified_base 5: mod_base = OTHER; note = 2'-O-methyladenosine-3'-phosphate
  modified_base 6: mod_base = OTHER; note = 2'-fluoroadenosine-3'-phosphate
  modified_base 7: mod_base = OTHER; note = 2'-O-methyluridine-3'-phosphate
  modified_base 8: mod_base = OTHER; note = 2'-O-methyluridine-3'-phosphate
  modified_base 9: mod_base = OTHER; note = 2'-O-methylguanosine-3'-phosphate
  modified_base 10: mod_base = OTHER; note = 2'-O-methyladenosine-3'-phosphate
  modified_base 11: mod_base = OTHER; note = 2'-O-methylguanosine-3'-phosphate
  modified_base 12: mod_base = OTHER; note = 2'-fluoroadenosine-3'-phosphate
  modified_base 13: mod_base = OTHER; note = 2'-O-methylguanosine-3'-phosphate
  modified_base 14: mod_base = OTHER; note = 2'-fluoroadenosine-3'-phosphate
  modified_base 15: mod_base = OTHER; note = 2'-O-methyladenosine-3'-phosphate
  modified_base 16: mod_base = OTHER; note = 2'-fluoroguanosine-3'-phosphate
  modified_base 17: mod_base = OTHER; note = 2'-O-methyluridine-3'-phosphate
  modified_base 18: mod_base = OTHER; note = 2'-fluorocytidine-3'-phosphate
  modified_base 19: mod_base = OTHER; note = 2'-O-methylcytidine-3'-phosphate
  modified_base 20: mod_base = OTHER; note = 2'-fluoroadenosine-3'-phosporothioate
  modified_base 21: mod_base = OTHER; note = 2'-O-methylcytidine-3'-phosphate
  misc_feature 1: note = RNA
  misc_feature 2: note = DNA
  misc_feature 3: note = RNA
  misc_feature 4: note = DNA
  misc_feature 5: note = RNA
  misc_feature 6: note = DNA
  misc_feature 7: note = RNA
  misc_feature 8: note = RNA
  misc_feature 9: note = RNA
  misc_feature 10: note = RNA
  misc_feature 11: note = RNA
  misc_feature 12: note = DNA
  misc_feature 13: note = RNA
  misc_feature 14: note = DNA
  misc_feature 15: note = RNA
  misc_feature 16: note = DNA
  misc_feature 17: note = RNA
  misc_feature 18: note = DNA
  misc_feature 19: note = RNA
  misc_feature 20: note = DNA
  misc_feature 21: note = RNA
  source 1..21: mol_type = other RNA
agaaaattgagagaagtccac

SEQ ID NO: 101 - RNA, 21 nt, synthetic construct
  modified_base 1: mod_base = OTHER; note = 2'-O-methyluridine-3'-phosphorothioate
  modified_base 2: mod_base = OTHER; note = 2'-fluoroadenosine-3'-phosporothioate
  modified_base 3: mod_base = OTHER; note = 2'-O-methylcytidine-3'-phosphorothioate
  modified_base 4: mod_base = OTHER; note = 2'-fluorocytidine-3'-phosphate
  modified_base 5: mod_base = OTHER; note = 2'-O-methyladenosine-3'-phosphate
  modified_base 6: mod_base = OTHER; note = 2'-fluoroadenosine-3'-phosphate
  modified_base 7: mod_base = OTHER; note = 2'-O-methyluridine-3'-phosphate
  modified_base 8: mod_base = OTHER; note = 2'-O-methyluridine-3'-phosphate
  modified_base 9: mod_base = OTHER; note = 2'-O-methyluridine-3'-phosphate
  modified_base 10: mod_base = OTHER; note = 2'-O-methyladenosine-3'-phosphate
  modified_base 11: mod_base = OTHER; note = 2'-O-methyluridine-3'-phosphate
  modified_base 12: mod_base = OTHER; note = 2'-fluoroguanosine-3'-phosphate
  modified_base 13: mod_base = OTHER; note = 2'-O-methylcytidine-3'-phosphate
  modified_base 14: mod_base = OTHER; note = 2'-fluorocytidine-3'-phosphate
  modified_base 15: mod_base = OTHER; note = 2'-O-methyluridine-3'-phosphate
  modified_base 16: mod_base = OTHER; note = 2'-fluoroadenosine-3'-phosphate
  modified_base 17: mod_base = OTHER; note = 2'-O-methylcytidine-3'-phosphate
  modified_base 18: mod_base = OTHER; note = 2'-fluoroadenosine-3'-phosphate
  modified_base 19: mod_base = OTHER; note = 2'-O-methylguanosine-3'-phosphate
  modified_base 20: mod_base = OTHER; note = 2'-O-methyluridine-3'-phosphorothioate
  modified_base 21: mod_base = OTHER; note = 2'-O-methyluridine-3'-phosphate
  misc_feature 1: note = RNA
  misc_feature 2: note = DNA
  misc_feature 3: note = RNA
  misc_feature 4: note = DNA
  misc_feature 5: note = RNA
  misc_feature 6: note = DNA
  misc_feature 7: note = RNA
  misc_feature 8: note = RNA
  misc_feature 9: note = RNA
  misc_feature 10: note = RNA
  misc_feature 11: note = RNA
  misc_feature 12: note = DNA
  misc_feature 13: note = RNA
  misc_feature 14: note = DNA
  misc_feature 15: note = RNA
  misc_feature 16: note = DNA
  misc_feature 17: note = RNA
  misc_feature 18: note = DNA
  misc_feature 19: note = RNA
  misc_feature 20: note = RNA
  misc_feature 21: note = RNA
  source 1..21: mol_type = other RNA
taccaatttatgcctacagtt

SEQ ID NO: 102 - RNA, 21 nt, synthetic construct
  modified_base 1: mod_base = OTHER; note = 2'-O-methyluridine-3'-phosphorothioate
  modified_base 2: mod_base = OTHER; note = 2'-fluoroadenosine-3'-phosporothioate
  modified_base 3: mod_base = OTHER; note = 2'-O-methylcytidine-3'-phosphorothioate
  modified_base 4: mod_base = OTHER; note = 2'-fluorocytidine-3'-phosphate
  modified_base 5: mod_base = OTHER; note = 2'-O-methyladenosine-3'-phosphate
  modified_base 6: mod_base = OTHER; note = 2'-fluoroadenosine-3'-phosphate
  modified_base 7: mod_base = OTHER; note = 2'-O-methyluridine-3'-phosphate
  modified_base 8: mod_base = OTHER; note = 2'-O-methyluridine-3'-phosphate
  modified_base 9: mod_base = OTHER; note = 2'-O-methyluridine-3'-phosphate
  modified_base 10: mod_base = OTHER; note = 2'-O-methyladenosine-3'-phosphate
  modified_base 11: mod_base = OTHER; note = 2'-O-methyluridine-3'-phosphate
  modified_base 12: mod_base = OTHER; note = 2'-fluoroguanosine-3'-phosphate
  modified_base 13: mod_base = OTHER; note = 2'-O-methylcytidine-3'-phosphate
  modified_base 14: mod_base = OTHER; note = 2'-fluorocytidine-3'-phosphate
  modified_base 15: mod_base = OTHER; note = 2'-O-methyluridine-3'-phosphate
  modified_base 16: mod_base = OTHER; note = 2'-fluoroadenosine-3'-phosphate
  modified_base 17: mod_base = OTHER; note = 2'-O-methylcytidine-3'-phosphate
  modified_base 18: mod_base = OTHER; note = 2'-fluoroadenosine-3'-phosphate
  modified_base 19: mod_base = OTHER; note = 2'-O-methylguanosine-3'-phosphate
  modified_base 20: mod_base = OTHER; note = 2'-O-methylcytidine-3'-phosphorothioate
  modified_base 21: mod_base = OTHER; note = 2'-O-methylcytidine-3'-phosphate
  misc_feature 1: note = RNA
  misc_feature 2: note = DNA
  misc_feature 3: note = RNA
  misc_feature 4: note = DNA
  misc_feature 5: note = RNA
  misc_feature 6: note = DNA
  misc_feature 7: note = RNA
  misc_feature 8: note = RNA
  misc_feature 9: note = RNA
  misc_feature 10: note = RNA
  misc_feature 11: note = RNA
  misc_feature 12: note = DNA
  misc_feature 13: note = RNA
  misc_feature 14: note = DNA
  misc_feature 15: note = RNA
  misc_feature 16: note = DNA
  misc_feature 17: note = RNA
  misc_feature 18: note = DNA
  misc_feature 19: note = RNA
  misc_feature 20: note = RNA
  misc_feature 21: note = RNA
  source 1..21: mol_type = other RNA
taccaatttatgcctacagcc

SEQ ID NO: 103 - RNA, 22 nt, synthetic construct
  modified_base 1: mod_base = OTHER; note = 2'-O-methyluridine-3'-phosphorothioate
  modified_base 2: mod_base = OTHER; note = 2'-fluoroadenosine-3'-phosporothioate
  modified_base 3: mod_base = OTHER; note = 2'-O-methylcytidine-3'-phosphorothioate
  modified_base 4: mod_base = OTHER; note = 2'-fluorocytidine-3'-phosphate
  modified_base 5: mod_base = OTHER; note = 2'-O-methyladenosine-3'-phosphate
  modified_base 6: mod_base = OTHER; note = 2'-fluoroadenosine-3'-phosphate
  modified_base 7: mod_base = OTHER; note = 2'-O-methyluridine-3'-phosphate
  modified_base 8: mod_base = OTHER; note = 2'-O-methyluridine-3'-phosphate
  modified_base 9: mod_base = OTHER; note = 2'-O-methyluridine-3'-phosphate
  modified_base 10: mod_base = OTHER; note = 2'-O-methyladenosine-3'-phosphate
  modified_base 11: mod_base = OTHER; note = 2'-O-methyluridine-3'-phosphate
  modified_base 12: mod_base = OTHER; note = 2'-fluoroguanosine-3'-phosphate
  modified_base 13: mod_base = OTHER; note = 2'-O-methylcytidine-3'-phosphate
  modified_base 14: mod_base = OTHER; note = 2'-fluorocytidine-3'-phosphate
  modified_base 15: mod_base = OTHER; note = 2'-O-methyluridine-3'-phosphate
  modified_base 16: mod_base = OTHER; note = 2'-fluoroadenosine-3'-phosphate
  modified_base 17: mod_base = OTHER; note = 2'-O-methylcytidine-3'-phosphate
  modified_base 18: mod_base = OTHER; note = 2'-fluoroadenosine-3'-phosphate
  modified_base 19: mod_base = OTHER; note = 2'-O-methylguanosine-3'-phosphate
  modified_base 20: mod_base = OTHER; note = 2'-O-methylcytidine-3'-phosphate
  modified_base 21: mod_base = OTHER; note = 2'-O-methyluridine-3'-phosphorothioate
  modified_base 22: mod_base = OTHER; note = 2'-O-methyluridine-3'-phosphate
  misc_feature 1: note = RNA
  misc_feature 2: note = DNA
  misc_feature 3: note = RNA
  misc_feature 4: note = DNA
  misc_feature 5: note = RNA
  misc_feature 6: note = DNA
  misc_feature 7: note = RNA
  misc_feature 8: note = RNA
  misc_feature 9: note = RNA
  misc_feature 10: note = RNA
  misc_feature 11: note = RNA
  misc_feature 12: note = DNA
  misc_feature 13: note = RNA
  misc_feature 14: note = DNA
  misc_feature 15: note = RNA
  misc_feature 16: note = DNA
  misc_feature 17: note = RNA
  misc_feature 18: note = DNA
  misc_feature 19: note = RNA
  misc_feature 20: note = RNA
  misc_feature 21: note = RNA
  misc_feature 22: note = RNA
  source 1..22: mol_type = other RNA
taccaatttatgcctacagctt

SEQ ID NO: 104 - RNA, 22 nt, synthetic construct
  modified_base 1: mod_base = OTHER; note = 2'-O-methyluridine-3'-phosphorothioate
  modified_base 2: mod_base = OTHER; note = 2'-fluoroadenosine-3'-phosporothioate
  modified_base 3: mod_base = OTHER; note = 2'-O-methylcytidine-3'-phosphorothioate
  modified_base 4: mod_base = OTHER; note = 2'-fluorocytidine-3'-phosphate
  modified_base 5: mod_base = OTHER; note = 2'-O-methyladenosine-3'-phosphate
  modified_base 6: mod_base = OTHER; note = 2'-fluoroadenosine-3'-phosphate
  modified_base 7: mod_base = OTHER; note = 2'-O-methyluridine-3'-phosphate
  modified_base 8: mod_base = OTHER; note = 2'-O-methyluridine-3'-phosphate
  modified_base 9: mod_base = OTHER; note = 2'-O-methyluridine-3'-phosphate
  modified_base 10: mod_base = OTHER; note = 2'-O-methyladenosine-3'-phosphate
  modified_base 11: mod_base = OTHER; note = 2'-O-methyluridine-3'-phosphate
  modified_base 12: mod_base = OTHER; note = 2'-fluoroguanosine-3'-phosphate
  modified_base 13: mod_base = OTHER; note = 2'-O-methylcytidine-3'-phosphate
  modified_base 14: mod_base = OTHER; note = 2'-fluorocytidine-3'-phosphate
  modified_base 15: mod_base = OTHER; note = 2'-O-methyluridine-3'-phosphate
  modified_base 16: mod_base = OTHER; note = 2'-fluoroadenosine-3'-phosphate
  modified_base 17: mod_base = OTHER; note = 2'-O-methylcytidine-3'-phosphate
  modified_base 18: mod_base = OTHER; note = 2'-fluoroadenosine-3'-phosphate
  modified_base 19: mod_base = OTHER; note = 2'-O-methylguanosine-3'-phosphate
  modified_base 20: mod_base = OTHER; note = 2'-O-methylcytidine-3'-phosphate
  modified_base 21: mod_base = OTHER; note = 2'-O-methylcytidine-3'-phosphorothioate
  modified_base 22: mod_base = OTHER; note = 2'-O-methyluridine-3'-phosphate
  misc_feature 1: note = RNA
  misc_feature 2: note = DNA
  misc_feature 3: note = RNA
  misc_feature 4: note = DNA
  misc_feature 5: note = RNA
  misc_feature 6: note = DNA
  misc_feature 7: note = RNA
  misc_feature 8: note = RNA
  misc_feature 9: note = RNA
  misc_feature 10: note = RNA
  misc_feature 11: note = RNA
  misc_feature 12: note = DNA
  misc_feature 13: note = RNA
  misc_feature 14: note = DNA
  misc_feature 15: note = RNA
  misc_feature 16: note = DNA
  misc_feature 17: note = RNA
  misc_feature 18: note = DNA
  misc_feature 19: note = RNA
  misc_feature 20: note = RNA
  misc_feature 21: note = RNA
  misc_feature 22: note = RNA
  source 1..22: mol_type = other RNA
taccaatttatgcctacagcct

SEQ ID NO: 105 - RNA, 23 nt, synthetic construct
  modified_base 1: mod_base = OTHER; note = 2'-O-methyluridine-3'-phosphorothioate
  modified_base 2: mod_base = OTHER; note = 2'-fluoroadenosine-3'-phosporothioate
  modified_base 3: mod_base = OTHER; note = 2'-O-methylcytidine-3'-phosphorothioate
  modified_base 4: mod_base = OTHER; note = 2'-fluorocytidine-3'-phosphate
  modified_base 5: mod_base = OTHER; note = 2'-O-methyladenosine-3'-phosphate
  modified_base 6: mod_base = OTHER; note = 2'-fluoroadenosine-3'-phosphate
  modified_base 7: mod_base = OTHER; note = 2'-O-methyluridine-3'-phosphate
  modified_base 8: mod_base = OTHER; note = 2'-O-methyluridine-3'-phosphate
  modified_base 9: mod_base = OTHER; note = 2'-O-methyluridine-3'-phosphate
  modified_base 10: mod_base = OTHER; note = 2'-O-methyladenosine-3'-phosphate
  modified_base 11: mod_base = OTHER; note = 2'-O-methyluridine-3'-phosphate
  modified_base 12: mod_base = OTHER; note = 2'-fluoroguanosine-3'-phosphate
  modified_base 13: mod_base = OTHER; note = 2'-O-methylcytidine-3'-phosphate
  modified_base 14: mod_base = OTHER; note = 2'-fluorocytidine-3'-phosphate
  modified_base 15: mod_base = OTHER; note = 2'-O-methyluridine-3'-phosphate
  modified_base 16: mod_base = OTHER; note = 2'-fluoroadenosine-3'-phosphate
  modified_base 17: mod_base = OTHER; note = 2'-O-methylcytidine-3'-phosphate
  modified_base 18: mod_base = OTHER; note = 2'-fluoroadenosine-3'-phosphate
  modified_base 19: mod_base = OTHER; note = 2'-O-methylguanosine-3'-phosphate
  modified_base 20: mod_base = OTHER; note = 2'-O-methylcytidine-3'-phosphate
  modified_base 21: mod_base = OTHER; note = 2'-O-methylcytidine-3'-phosphate
  modified_base 22: mod_base = OTHER; note = 2'-O-methyluridine-3'-phosphorothioate
  modified_base 23: mod_base = OTHER; note = 2'-O-methyluridine-3'-phosphate
  misc_feature 1: note = RNA
  misc_feature 2: note = DNA
  misc_feature 3: note = RNA
  misc_feature 4: note = DNA
  misc_feature 5: note = RNA
  misc_feature 6: note = DNA
  misc_feature 7: note = RNA
  misc_feature 8: note = RNA
  misc_feature 9: note = RNA
  misc_feature 10: note = RNA
  misc_feature 11: note = RNA
  misc_feature 12: note = DNA
  misc_feature 13: note = RNA
  misc_feature 14: note = DNA
  misc_feature 15: note = RNA
  misc_feature 16: note = DNA
  misc_feature 17: note = RNA
  misc_feature 18: note = DNA
  misc_feature 19: note = RNA
  misc_feature 20: note = RNA
  misc_feature 21: note = RNA
  misc_feature 22: note = RNA
  misc_feature 23: note = RNA
  source 1..23: mol_type = other RNA
taccaatttatgcctacagcctt

SEQ ID NO: 106 - RNA, 23 nt, synthetic construct
  modified_base 1: mod_base = OTHER; note = 2'-O-methyluridine-3'-phosphorothioate
  modified_base 2: mod_base = OTHER; note = 2'-fluoroadenosine-3'-phosporothioate
  modified_base 3: mod_base = OTHER; note = 2'-O-methylcytidine-3'-phosphorothioate
  modified_base 4: mod_base = OTHER; note = 2'-fluorocytidine-3'-phosphate
  modified_base 5: mod_base = OTHER; note = 2'-O-methyladenosine-3'-phosphate
  modified_base 6: mod_base = OTHER; note = 2'-fluoroadenosine-3'-phosphate
  modified_base 7: mod_base = OTHER; note = 2'-O-methyluridine-3'-phosphate
  modified_base 8: mod_base = OTHER; note = 2'-O-methyluridine-3'-phosphate
  modified_base 9: mod_base = OTHER; note = 2'-O-methyluridine-3'-phosphate
  modified_base 10: mod_base = OTHER; note = 2'-O-methyladenosine-3'-phosphate
  modified_base 11: mod_base = OTHER; note = 2'-O-methyluridine-3'-phosphate
  modified_base 12: mod_base = OTHER; note = 2'-fluoroguanosine-3'-phosphate
  modified_base 13: mod_base = OTHER; note = 2'-O-methylcytidine-3'-phosphate
  modified_base 14: mod_base = OTHER; note = 2'-fluorocytidine-3'-phosphate
  modified_base 15: mod_base = OTHER; note = 2'-O-methyluridine-3'-phosphate
  modified_base 16: mod_base = OTHER; note = 2'-fluoroadenosine-3'-phosphate
  modified_base 17: mod_base = OTHER; note = 2'-O-methylcytidine-3'-phosphate
  modified_base 18: mod_base = OTHER; note = 2'-fluoroadenosine-3'-phosphate
  modified_base 19: mod_base = OTHER; note = 2'-O-methylguanosine-3'-phosphate
  modified_base 20: mod_base = OTHER; note = 2'-O-methylcytidine-3'-phosphate
  modified_base 21: mod_base = OTHER; note = 2'-O-methylcytidine-3'-phosphate
  modified_base 22: mod_base = OTHER; note = 2'-O-methyluridine-3'-phosphorothioate
  modified_base 23: mod_base = OTHER; note = 2'-O-methylcytidine-3'-phosphate
  misc_feature 1: note = RNA
  misc_feature 2: note = DNA
  misc_feature 3: note = RNA
  misc_feature 4: note = DNA
  misc_feature 5: note = RNA
  misc_feature 6: note = DNA
  misc_feature 7: note = RNA
  misc_feature 8: note = RNA
  misc_feature 9: note = RNA
  misc_feature 10: note = RNA
  misc_feature 11: note = RNA
  misc_feature 12: note = DNA
  misc_feature 13: note = RNA
  misc_feature 14: note = DNA
  misc_feature 15: note = RNA
  misc_feature 16: note = DNA
  misc_feature 17: note = RNA
  misc_feature 18: note = DNA
  misc_feature 19: note = RNA
  misc_feature 20: note = RNA
  misc_feature 21: note = RNA
  misc_feature 22: note = RNA
  misc_feature 23: note = RNA
  source 1..23: mol_type = other RNA
taccaatttatgcctacagcctc

SEQ ID NO: 107 - RNA, 21 nt, synthetic construct
  modified_base 1: mod_base = OTHER; note = cyclopropyl phosphonate-2'-O-methyluridine-3'-phosphorothioate
  modified_base 2: mod_base = OTHER; note = 2'-fluoroadenosine-3'-phosporothioate
  modified_base 3: mod_base = OTHER; note = 2'-O-methylcytidine-3'-phosphorothioate
  modified_base 4: mod_base = OTHER; note = 2'-fluorocytidine-3'-phosphate
  modified_base 5: mod_base = OTHER; note = 2'-O-methyladenosine-3'-phosphate
  modified_base 6: mod_base = OTHER; note = 2'-fluoroadenosine-3'-phosphate
  modified_base 7: mod_base = OTHER; note = 2'-O-methyluridine-3'-phosphate
  modified_base 8: mod_base = OTHER; note = 2'-fluorouridine-3'-phosphate
  modified_base 9: mod_base = OTHER; note = 2'-O-methyluridine-3'-phosphate
  modified_base 10: mod_base = OTHER; note = 2'-fluoroadenosine-3'-phosphate
  modified_base 11: mod_base = OTHER; note = 2'-O-methyluridine-3'-phosphate
  modified_base 12: mod_base = OTHER; note = 2'-fluoroguanosine-3'-phosphate
  modified_base 13: mod_base = OTHER; note = 2'-O-methylcytidine-3'-phosphate
  modified_base 14: mod_base = OTHER; note = 2'-fluorocytidine-3'-phosphate
  modified_base 15: mod_base = OTHER; note = 2'-O-methyluridine-3'-phosphate
  modified_base 16: mod_base = OTHER; note = 2'-fluoroadenosine-3'-phosphate
  modified_base 17: mod_base = OTHER; note = 2'-O-methylcytidine-3'-phosphate
  modified_base 18: mod_base = OTHER; note = 2'-fluoroadenosine-3'-phosphate
  modified_base 19: mod_base = OTHER; note = 2'-O-methylguanosine-3'-phosphate
  modified_base 20: mod_base = OTHER; note = 2'-O-methyluridine-3'-phosphorothioate
  modified_base 21: mod_base = OTHER; note = 2'-O-methyluridine-3'-phosphate
  misc_feature 1: note = RNA
  misc_feature 2: note = DNA
  misc_feature 3: note = RNA
  misc_feature 4: note = DNA
  misc_feature 5: note = RNA
  misc_feature 6: note = DNA
  misc_feature 7: note = RNA
  misc_feature 8: note = DNA
  misc_feature 9: note = RNA
  misc_feature 10: note = DNA
  misc_feature 11: note = RNA
  misc_feature 12: note = DNA
  misc_feature 13: note = RNA
  misc_feature 14: note = DNA
  misc_feature 15: note = RNA
  misc_feature 16: note = DNA
  misc_feature 17: note = RNA
  misc_feature 18: note = DNA
  misc_feature 19: note = RNA
  misc_feature 20: note = RNA
  misc_feature 21: note = RNA
  source 1..21: mol_type = other RNA
taccaatttatgcctacagtt

SEQ ID NO: 108 - RNA, 21 nt, synthetic construct
  modified_base 1: mod_base = OTHER; note = cyclopropyl phosphonate-2'-O-methyluridine-3'-phosphorothioate
  modified_base 2: mod_base = OTHER; note = 2'-fluoroadenosine-3'-phosporothioate
  modified_base 3: mod_base = OTHER; note = 2'-O-methyluridine-3'-phosphorothioate
  modified_base 4: mod_base = OTHER; note = 2'-fluorouridine-3'-phosphate
  modified_base 5: mod_base = OTHER; note = 2'-O-methylguanosine-3'-phosphate
  modified_base 6: mod_base = OTHER; note = 2'-fluoroadenosine-3'-phosphate
  modified_base 7: mod_base = OTHER; note = 2'-O-methylguanosine-3'-phosphate
  modified_base 8: mod_base = OTHER; note = 2'-fluoroadenosine-3'-phosphate
  modified_base 9: mod_base = OTHER; note = 2'-O-methylguanosine-3'-phosphate
  modified_base 10: mod_base = OTHER; note = 2'-fluoroadenosine-3'-phosphate
  modified_base 11: mod_base = OTHER; note = 2'-O-methyladenosine-3'-phosphate
  modified_base 12: mod_base = OTHER; note = 2'-fluoroguanosine-3'-phosphate
  modified_base 13: mod_base = OTHER; note = 2'-O-methyluridine-3'-phosphate
  modified_base 14: mod_base = OTHER; note = 2'-fluorocytidine-3'-phosphate
  modified_base 15: mod_base = OTHER; note = 2'-O-methylcytidine-3'-phosphate
  modified_base 16: mod_base = OTHER; note = 2'-fluoroadenosine-3'-phosphate
  modified_base 17: mod_base = OTHER; note = 2'-O-methylcytidine-3'-phosphate
  modified_base 18: mod_base = OTHER; note = 2'-fluorocytidine-3'-phosphate
  modified_base 19: mod_base = OTHER; note = 2'-O-methyladenosine-3'-phosphate
  modified_base 20: mod_base = OTHER; note = 2'-fluorocytidine-3'-phosphorothioate
  modified_base 21: mod_base = OTHER; note = 2'-O-methylguanosine-3'-phosphate
  misc_feature 1: note = RNA
  misc_feature 2: note = DNA
  misc_feature 3: note = RNA
  misc_feature 4: note = DNA
  misc_feature 5: note = RNA
  misc_feature 6: note = DNA
  misc_feature 7: note = RNA
  misc_feature 8: note = DNA
  misc_feature 9: note = RNA
  misc_feature 10: note = DNA
  misc_feature 11: note = RNA
  misc_feature 12: note = DNA
  misc_feature 13: note = RNA
  misc_feature 14: note = DNA
  misc_feature 15: note = RNA
  misc_feature 16: note = DNA
  misc_feature 17: note = RNA
  misc_feature 18: note = DNA
  misc_feature 19: note = RNA
  misc_feature 20: note = DNA
  misc_feature 21: note = RNA
  source 1..21: mol_type = other RNA
tattgagagaagtccaccacg

SEQ ID NO: 109 - RNA, 21 nt, synthetic construct
  modified_base 1: mod_base = OTHER; note = 2'-O-methyluridine-3'-phosphorothioate
  modified_base 2: mod_base = OTHER; note = 2'-fluoroadenosine-3'-phosporothioate
  modified_base 3: mod_base = OTHER; note = 2'-O-methyluridine-3'-phosphorothioate
  modified_base 4: mod_base = OTHER; note = 2'-fluorouridine-3'-phosphate
  modified_base 5: mod_base = OTHER; note = 2'-O-methylguanosine-3'-phosphate
  modified_base 6: mod_base = OTHER; note = 2'-fluoroadenosine-3'-phosphate
  modified_base 7: mod_base = OTHER; note = 2'-O-methylguanosine-3'-phosphate
  modified_base 8: mod_base = OTHER; note = 2'-O-methyladenosine-3'-phosphate
  modified_base 9: mod_base = OTHER; note = 2'-O-methylguanosine-3'-phosphate
  modified_base 10: mod_base = OTHER; note = 2'-O-methyladenosine-3'-phosphate
  modified_base 11: mod_base = OTHER; note = 2'-O-methyladenosine-3'-phosphate
  modified_base 12: mod_base = OTHER; note = 2'-fluoroguanosine-3'-phosphate
  modified_base 13: mod_base = OTHER; note = 2'-O-methyluridine-3'-phosphate
  modified_base 14: mod_base = OTHER; note = 2'-fluorocytidine-3'-phosphate
  modified_base 15: mod_base = OTHER; note = 2'-O-methylcytidine-3'-phosphate
  modified_base 16: mod_base = OTHER; note = 2'-fluoroadenosine-3'-phosphate
  modified_base 17: mod_base = OTHER; note = 2'-O-methylcytidine-3'-phosphate
  modified_base 18: mod_base = OTHER; note = 2'-fluorocytidine-3'-phosphate
  modified_base 19: mod_base = OTHER; note = 2'-O-methyladenosine-3'-phosphate
  modified_base 20: mod_base = OTHER; note = 2'-O-methyluridine-3'-phosphorothioate
  modified_base 21: mod_base = OTHER; note = 2'-O-methyluridine-3'-phosphate
  misc_feature 1: note = RNA
  misc_feature 2: note = DNA
  misc_feature 3: note = RNA
  misc_feature 4: note = DNA
  misc_feature 5: note = RNA
  misc_feature 6: note = DNA
  misc_feature 7: note = RNA
  misc_feature 8: note = RNA
  misc_feature 9: note = RNA
  misc_feature 10: note = RNA
  misc_feature 11: note = RNA
  misc_feature 12: note = DNA
  misc_feature 13: note = RNA
  misc_feature 14: note = DNA
  misc_feature 15: note = RNA
  misc_feature 16: note = DNA
  misc_feature 17: note = RNA
  misc_feature 18: note = DNA
  misc_feature 19: note = RNA
  misc_feature 20: note = RNA
  misc_feature 21: note = RNA
  source 1..21: mol_type = other RNA
tattgagagaagtccaccatt

SEQ ID NO: 110 - RNA, 21 nt, synthetic construct
  modified_base 1: mod_base = OTHER; note = 2'-O-methyluridine-3'-phosphorothioate
  modified_base 2: mod_base = OTHER; note = 2'-fluoroadenosine-3'-phosporothioate
  modified_base 3: mod_base = OTHER; note = 2'-O-methyluridine-3'-phosphorothioate
  modified_base 4: mod_base = OTHER; note = 2'-fluorouridine-3'-phosphate
  modified_base 5: mod_base = OTHER; note = 2'-O-methylguanosine-3'-phosphate
  modified_base 6: mod_base = OTHER; note = 2'-fluoroadenosine-3'-phosphate
  modified_base 7: mod_base = OTHER; note = 2'-O-methylguanosine-3'-phosphate
  modified_base 8: mod_base = OTHER; note = 2'-O-methyladenosine-3'-phosphate
  modified_base 9: mod_base = OTHER; note = 2'-O-methylguanosine-3'-phosphate
  modified_base 10: mod_base = OTHER; note = 2'-O-methyladenosine-3'-phosphate
  modified_base 11: mod_base = OTHER; note = 2'-O-methyladenosine-3'-phosphate
  modified_base 12: mod_base = OTHER; note = 2'-fluoroguanosine-3'-phosphate
  modified_base 13: mod_base = OTHER; note = 2'-O-methyluridine-3'-phosphate
  modified_base 14: mod_base = OTHER; note = 2'-fluorocytidine-3'-phosphate
  modified_base 15: mod_base = OTHER; note = 2'-O-methylcytidine-3'-phosphate
  modified_base 16: mod_base = OTHER; note = 2'-fluoroadenosine-3'-phosphate
  modified_base 17: mod_base = OTHER; note = 2'-O-methylcytidine-3'-phosphate
  modified_base 18: mod_base = OTHER; note = 2'-fluorocytidine-3'-phosphate
  modified_base 19: mod_base = OTHER; note = 2'-O-methyladenosine-3'-phosphate
  modified_base 20: mod_base = OTHER; note = 2'-O-methylcytidine-3'-phosphorothioate
  modified_base 21: mod_base = OTHER; note = 2'-O-methylguanosine-3'-phosphate
  misc_feature 1: note = RNA
  misc_feature 2: note = DNA
  misc_feature 3: note = RNA
  misc_feature 4: note = DNA
  misc_feature 5: note = RNA
  misc_feature 6: note = DNA
  misc_feature 7: note = RNA
  misc_feature 8: note = RNA
  misc_feature 9: note = RNA
  misc_feature 10: note = RNA
  misc_feature 11: note = RNA
  misc_feature 12: note = DNA
  misc_feature 13: note = RNA
  misc_feature 14: note = DNA
  misc_feature 15: note = RNA
  misc_feature 16: note = DNA
  misc_feature 17: note = RNA
  misc_feature 18: note = DNA
  misc_feature 19: note = RNA
  misc_feature 20: note = RNA
  misc_feature 21: note = RNA
  source 1..21: mol_type = other RNA
tattgagagaagtccaccacg

SEQ ID NO: 111 - RNA, 22 nt, synthetic construct
  modified_base 1: mod_base = OTHER; note = 2'-O-methyluridine-3'-phosphorothioate
  modified_base 2: mod_base = OTHER; note = 2'-fluoroadenosine-3'-phosporothioate
  modified_base 3: mod_base = OTHER; note = 2'-O-methyluridine-3'-phosphorothioate
  modified_base 4: mod_base = OTHER; note = 2'-fluorouridine-3'-phosphate
  modified_base 5: mod_base = OTHER; note = 2'-O-methylguanosine-3'-phosphate
  modified_base 6: mod_base = OTHER; note = 2'-fluoroadenosine-3'-phosphate
  modified_base 7: mod_base = OTHER; note = 2'-O-methylguanosine-3'-phosphate
  modified_base 8: mod_base = OTHER; note = 2'-O-methyladenosine-3'-phosphate
  modified_base 9: mod_base = OTHER; note = 2'-O-methylguanosine-3'-phosphate
  modified_base 10: mod_base = OTHER; note = 2'-O-methyladenosine-3'-phosphate
  modified_base 11: mod_base = OTHER; note = 2'-O-methyladenosine-3'-phosphate
  modified_base 12: mod_base = OTHER; note = 2'-fluoroguanosine-3'-phosphate
  modified_base 13: mod_base = OTHER; note = 2'-O-methyluridine-3'-phosphate
  modified_base 14: mod_base = OTHER; note = 2'-fluorocytidine-3'-phosphate
  modified_base 15: mod_base = OTHER; note = 2'-O-methylcytidine-3'-phosphate
  modified_base 16: mod_base = OTHER; note = 2'-fluoroadenosine-3'-phosphate
  modified_base 17: mod_base = OTHER; note = 2'-O-methylcytidine-3'-phosphate
  modified_base 18: mod_base = OTHER; note = 2'-fluorocytidine-3'-phosphate
  modified_base 19: mod_base = OTHER; note = 2'-O-methyladenosine-3'-phosphate
  modified_base 20: mod_base = OTHER; note = 2'-O-methylcytidine-3'-phosphorothioate
  modified_base 21: mod_base = OTHER; note = 2'-O-methyluridine-3'-phosphorothioate
  modified_base 22: mod_base = OTHER; note = 2'-O-methyluridine-3'-phosphate
  misc_feature 1: note = RNA
  misc_feature 2: note = DNA
  misc_feature 3: note = RNA
  misc_feature 4: note = DNA
  misc_feature 5: note = RNA
  misc_feature 6: note = DNA
  misc_feature 7: note = RNA
  misc_feature 8: note = RNA
  misc_feature 9: note = RNA
  misc_feature 10: note = RNA
  misc_feature 11: note = RNA
  misc_feature 12: note = DNA
  misc_feature 13: note = RNA
  misc_feature 14: note = DNA
  misc_feature 15: note = RNA
  misc_feature 16: note = DNA
  misc_feature 17: note = RNA
  misc_feature 18: note = DNA
  misc_feature 19: note = RNA
  misc_feature 20: note = RNA
  misc_feature 21: note = RNA
  misc_feature 22: note = RNA
  source 1..22: mol_type = other RNA
tattgagagaagtccaccactt

SEQ ID NO: 112 - RNA, 22 nt, synthetic construct
  modified_base 1: mod_base = OTHER; note = 2'-O-methyluridine-3'-phosphorothioate
  modified_base 2: mod_base = OTHER; note = 2'-fluoroadenosine-3'-phosporothioate
  modified_base 3: mod_base = OTHER; note = 2'-O-methyluridine-3'-phosphorothioate
  modified_base 4: mod_base = OTHER; note = 2'-fluorouridine-3'-phosphate
  modified_base 5: mod_base = OTHER; note = 2'-O-methylguanosine-3'-phosphate
  modified_base 6: mod_base = OTHER; note = 2'-fluoroadenosine-3'-phosphate
  modified_base 7: mod_base = OTHER; note = 2'-O-methylguanosine-3'-phosphate
  modified_base 8: mod_base = OTHER; note = 2'-O-methyladenosine-3'-phosphate
  modified_base 9: mod_base = OTHER; note = 2'-O-methylguanosine-3'-phosphate
  modified_base 10: mod_base = OTHER; note = 2'-O-methyladenosine-3'-phosphate
  modified_base 11: mod_base = OTHER; note = 2'-O-methyladenosine-3'-phosphate
  modified_base 12: mod_base = OTHER; note = 2'-fluoroguanosine-3'-phosphate
  modified_base 13: mod_base = OTHER; note = 2'-O-methyluridine-3'-phosphate
  modified_base 14: mod_base = OTHER; note = 2'-fluorocytidine-3'-phosphate
  modified_base 15: mod_base = OTHER; note = 2'-O-methylcytidine-3'-phosphate
  modified_base 16: mod_base = OTHER; note = 2'-fluoroadenosine-3'-phosphate
  modified_base 17: mod_base = OTHER; note = 2'-O-methylcytidine-3'-phosphate
  modified_base 18: mod_base = OTHER; note = 2'-fluorocytidine-3'-phosphate
  modified_base 19: mod_base = OTHER; note = 2'-O-methyladenosine-3'-phosphate
  modified_base 20: mod_base = OTHER; note = 2'-O-methylcytidine-3'-phosphorothioate
  modified_base 21: mod_base = OTHER; note = 2'-O-methylguanosine-3'-phosphorothioate
  modified_base 22: mod_base = OTHER; note = 2'-O-methyladenosine-3'-phosphate
  misc_feature 1: note = RNA
  misc_feature 2: note = DNA
  misc_feature 3: note = RNA
  misc_feature 4: note = DNA
  misc_feature 5: note = RNA
  misc_feature 6: note = DNA
  misc_feature 7: note = RNA
  misc_feature 8: note = RNA
  misc_feature 9: note = RNA
  misc_feature 10: note = RNA
  misc_feature 11: note = RNA
  misc_feature 12: note = DNA
  misc_feature 13: note = RNA
  misc_feature 14: note = DNA
  misc_feature 15: note = RNA
  misc_feature 16: note = DNA
  misc_feature 17: note = RNA
  misc_feature 18: note = DNA
  misc_feature 19: note = RNA
  misc_feature 20: note = RNA
  misc_feature 21: note = RNA
  misc_feature 22: note = RNA
  source 1..22: mol_type = other RNA
tattgagagaagtccaccacga

SEQ ID NO: 113 - RNA, 21 nt, synthetic construct
  modified_base 1: mod_base = OTHER; note = vinyl phosphonate-2'-O-methyluridine-3'-phosphorothioate
  modified_base 2: mod_base = OTHER; note = 2'-fluoroadenosine-3'-phosporothioate
  modified_base 3: mod_base = OTHER; note = 2'-O-methyluridine-3'-phosphorothioate
  modified_base 4: mod_base = OTHER; note = 2'-fluorouridine-3'-phosphate
  modified_base 5: mod_base = OTHER; note = 2'-O-methylguanosine-3'-phosphate
  modified_base 6: mod_base = OTHER; note = 2'-fluoroadenosine-3'-phosphate
  modified_base 7: mod_base = OTHER; note = 2'-O-methylguanosine-3'-phosphate
  modified_base 8: mod_base = OTHER; note = 2'-O-methyladenosine-3'-phosphate
  modified_base 9: mod_base = OTHER; note = 2'-O-methylguanosine-3'-phosphate
  modified_base 10: mod_base = OTHER; note = 2'-O-methyladenosine-3'-phosphate
  modified_base 11: mod_base = OTHER; note = 2'-O-methyladenosine-3'-phosphate
  modified_base 12: mod_base = OTHER; note = 2'-fluoroguanosine-3'-phosphate
  modified_base 13: mod_base = OTHER; note = 2'-O-methyluridine-3'-phosphate
  modified_base 14: mod_base = OTHER; note = 2'-fluorocytidine-3'-phosphate
  modified_base 15: mod_base = OTHER; note = 2'-O-methylcytidine-3'-phosphate
  modified_base 16: mod_base = OTHER; note = 2'-fluoroadenosine-3'-phosphate
  modified_base 17: mod_base = OTHER; note = 2'-O-methylcytidine-3'-phosphate
  modified_base 18: mod_base = OTHER; note = 2'-fluorocytidine-3'-phosphate
  modified_base 19: mod_base = OTHER; note = 2'-O-methyladenosine-3'-phosphate
  modified_base 20: mod_base = OTHER; note = 2'-fluorocytidine-3'-phosphorothioate
  modified_base 21: mod_base = OTHER; note = 2'-O-methylguanosine-3'-phosphate
  misc_feature 1: note = RNA
  misc_feature 2: note = DNA
  misc_feature 3: note = RNA
  misc_feature 4: note = DNA
  misc_feature 5: note = RNA
  misc_feature 6: note = DNA
  misc_feature 7: note = RNA
  misc_feature 8: note = RNA
  misc_feature 9: note = RNA
  misc_feature 10: note = RNA
  misc_feature 11: note = RNA
  misc_feature 12: note = DNA
  misc_feature 13: note = RNA
  misc_feature 14: note = DNA
  misc_feature 15: note = RNA
  misc_feature 16: note = DNA
  misc_feature 17: note = RNA
  misc_feature 18: note = DNA
  misc_feature 19: note = RNA
  misc_feature 20: note = DNA
  misc_feature 21: note = RNA
  source 1..21: mol_type = other RNA
tattgagagaagtccaccacg

SEQ ID NO: 114 - RNA, 21 nt, synthetic construct
  modified_base 1: mod_base = OTHER; note = 2'-O-methyluridine-3'-phosphorothioate
  modified_base 2: mod_base = OTHER; note = 2'-fluorouridine-3'-phosphorothioate
  modified_base 3: mod_base = OTHER; note = 2'-O-methyluridine-3'-phosphorothioate
  modified_base 4: mod_base = OTHER; note = 2'-fluoroguanosine-3'-phosphate
  modified_base 5: mod_base = OTHER; note = 2'-O-methyladenosine-3'-phosphate
  modified_base 6: mod_base = OTHER; note = 2'-fluoroguanosine-3'-phosphate
  modified_base 7: mod_base = OTHER; note = 2'-O-methyladenosine-3'-phosphate
  modified_base 8: mod_base = OTHER; note = 2'-O-methylguanosine-3'-phosphate
  modified_base 9: mod_base = OTHER; note = 2'-O-methyladenosine-3'-phosphate
  modified_base 10: mod_base = OTHER; note = 2'-O-methyladenosine-3'-phosphate
  modified_base 11: mod_base = OTHER; note = 2'-O-methylguanosine-3'-phosphate
  modified_base 12: mod_base = OTHER; note = 2'-fluorouridine-3'-phosphate
  modified_base 13: mod_base = OTHER; note = 2'-O-methylcytidine-3'-phosphate
  modified_base 14: mod_base = OTHER; note = 2'-fluorocytidine-3'-phosphate
  modified_base 15: mod_base = OTHER; note = 2'-O-methyladenosine-3'-phosphate
  modified_base 16: mod_base = OTHER; note = 2'-fluorocytidine-3'-phosphate
  modified_base 17: mod_base = OTHER; note = 2'-O-methylcytidine-3'-phosphate
  modified_base 18: mod_base = OTHER; note = 2'-fluoroadenosine-3'-phosphate
  modified_base 19: mod_base = OTHER; note = 2'-O-methylcytidine-3'-phosphate
  modified_base 20: mod_base = OTHER; note = 2'-O-methyluridine-3'-phosphorothioate
  modified_base 21: mod_base = OTHER; note = 2'-O-methyluridine-3'-phosphate
  misc_feature 1: note = RNA
  misc_feature 2: note = DNA
  misc_feature 3: note = RNA
  misc_feature 4: note = DNA
  misc_feature 5: note = RNA
  misc_feature 6: note = DNA
  misc_feature 7: note = RNA
  misc_feature 8: note = RNA
  misc_feature 9: note = RNA
  misc_feature 10: note = RNA
  misc_feature 11: note = RNA
  misc_feature 12: note = DNA
  misc_feature 13: note = RNA
  misc_feature 14: note = DNA
  misc_feature 15: note = RNA
  misc_feature 16: note = DNA
  misc_feature 17: note = RNA
  misc_feature 18: note = DNA
  misc_feature 19: note = RNA
  misc_feature 20: note = RNA
  misc_feature 21: note = RNA
  source 1..21: mol_type = other RNA
tttgagagaagtccaccactt

SEQ ID NO: 115 - RNA, 21 nt, synthetic construct
  modified_base 1: mod_base = OTHER; note = 2'-O-methyluridine-3'-phosphorothioate
  modified_base 2: mod_base = OTHER; note = 2'-fluorouridine-3'-phosphorothioate
  modified_base 3: mod_base = OTHER; note = 2'-O-methyluridine-3'-phosphorothioate
  modified_base 4: mod_base = OTHER; note = 2'-fluoroguanosine-3'-phosphate
  modified_base 5: mod_base = OTHER; note = 2'-O-methyladenosine-3'-phosphate
  modified_base 6: mod_base = OTHER; note = 2'-fluoroguanosine-3'-phosphate
  modified_base 7: mod_base = OTHER; note = 2'-O-methyladenosine-3'-phosphate
  modified_base 8: mod_base = OTHER; note = 2'-O-methylguanosine-3'-phosphate
  modified_base 9: mod_base = OTHER; note = 2'-O-methyladenosine-3'-phosphate
  modified_base 10: mod_base = OTHER; note = 2'-O-methyladenosine-3'-phosphate
  modified_base 11: mod_base = OTHER; note = 2'-O-methylguanosine-3'-phosphate
  modified_base 12: mod_base = OTHER; note = 2'-fluorouridine-3'-phosphate
  modified_base 13: mod_base = OTHER; note = 2'-O-methylcytidine-3'-phosphate
  modified_base 14: mod_base = OTHER; note = 2'-fluorocytidine-3'-phosphate
  modified_base 15: mod_base = OTHER; note = 2'-O-methyladenosine-3'-phosphate
  modified_base 16: mod_base = OTHER; note = 2'-fluorocytidine-3'-phosphate
  modified_base 17: mod_base = OTHER; note = 2'-O-methylcytidine-3'-phosphate
  modified_base 18: mod_base = OTHER; note = 2'-fluoroadenosine-3'-phosphate
  modified_base 19: mod_base = OTHER; note = 2'-O-methylcytidine-3'-phosphate
  modified_base 20: mod_base = OTHER; note = 2'-O-methylguanosine-3'-phosphorothioate
  modified_base 21: mod_base = OTHER; note = 2'-O-methyladenosine-3'-phosphate
  misc_feature 1: note = RNA
  misc_feature 2: note = DNA
  misc_feature 3: note = RNA
  misc_feature 4: note = DNA
  misc_feature 5: note = RNA
  misc_feature 6: note = DNA
  misc_feature 7: note = RNA
  misc_feature 8: note = RNA
  misc_feature 9: note = RNA
  misc_feature 10: note = RNA
  misc_feature 11: note = RNA
  misc_feature 12: note = DNA
  misc_feature 13: note = RNA
  misc_feature 14: note = DNA
  misc_feature 15: note = RNA
  misc_feature 16: note = DNA
  misc_feature 17: note = RNA
  misc_feature 18: note = DNA
  misc_feature 19: note = RNA
  misc_feature 20: note = RNA
  misc_feature 21: note = RNA
  source 1..21: mol_type = other RNA
tttgagagaagtccaccacga

SEQ ID NO: 116 - RNA, 22 nt, synthetic construct
  modified_base 1: mod_base = OTHER; note = 2'-O-methyluridine-3'-phosphorothioate
  modified_base 2: mod_base = OTHER; note = 2'-fluorouridine-3'-phosphorothioate
  modified_base 3: mod_base = OTHER; note = 2'-O-methyluridine-3'-phosphorothioate
  modified_base 4: mod_base = OTHER; note = 2'-fluoroguanosine-3'-phosphate
  modified_base 5: mod_base = OTHER; note = 2'-O-methyladenosine-3'-phosphate
  modified_base 6: mod_base = OTHER; note = 2'-fluoroguanosine-3'-phosphate
  modified_base 7: mod_base = OTHER; note = 2'-O-methyladenosine-3'-phosphate
  modified_base 8: mod_base = OTHER; note = 2'-O-methylguanosine-3'-phosphate
  modified_base 9: mod_base = OTHER; note = 2'-O-methyladenosine-3'-phosphate
  modified_base 10: mod_base = OTHER; note = 2'-O-methyladenosine-3'-phosphate
  modified_base 11: mod_base = OTHER; note = 2'-O-methylguanosine-3'-phosphate
  modified_base 12: mod_base = OTHER; note = 2'-fluorouridine-3'-phosphate
  modified_base 13: mod_base = OTHER; note = 2'-O-methylcytidine-3'-phosphate
  modified_base 14: mod_base = OTHER; note = 2'-fluorocytidine-3'-phosphate
  modified_base 15: mod_base = OTHER; note = 2'-O-methyladenosine-3'-phosphate
  modified_base 16: mod_base = OTHER; note = 2'-fluorocytidine-3'-phosphate
  modified_base 17: mod_base = OTHER; note = 2'-O-methylcytidine-3'-phosphate
  modified_base 18: mod_base = OTHER; note = 2'-fluoroadenosine-3'-phosphate
  modified_base 19: mod_base = OTHER; note = 2'-O-methylcytidine-3'-phosphate
  modified_base 20: mod_base = OTHER; note = 2'-O-methylguanosine-3'-phosphate
  modified_base 21: mod_base = OTHER; note = 2'-O-methyluridine-3'-phosphorothioate
  modified_base 22: mod_base = OTHER; note = 2'-O-methyluridine-3'-phosphate
  misc_feature 1: note = RNA
  misc_feature 2: note = DNA
  misc_feature 3: note = RNA
  misc_feature 4: note = DNA
  misc_feature 5: note = RNA
  misc_feature 6: note = DNA
  misc_feature 7: note = RNA
  misc_feature 8: note = RNA
  misc_feature 9: note = RNA
  misc_feature 10: note = RNA
  misc_feature 11: note = RNA
  misc_feature 12: note = DNA
  misc_feature 13: note = RNA
  misc_feature 14: note = DNA
  misc_feature 15: note = RNA
  misc_feature 16: note = DNA
  misc_feature 17: note = RNA
  misc_feature 18: note = DNA
  misc_feature 19: note = RNA
  misc_feature 20: note = RNA
  misc_feature 21: note = RNA
  misc_feature 22: note = RNA
  source 1..22: mol_type = other RNA
tttgagagaagtccaccacgtt

SEQ ID NO: 117 - RNA, 22 nt, synthetic construct
  modified_base 1: mod_base = OTHER; note = 2'-O-methyluridine-3'-phosphorothioate
  modified_base 2: mod_base = OTHER; note = 2'-fluorouridine-3'-phosphorothioate
  modified_base 3: mod_base = OTHER; note = 2'-O-methyluridine-3'-phosphorothioate
  modified_base 4: mod_base = OTHER; note = 2'-fluoroguanosine-3'-phosphate
  modified_base 5: mod_base = OTHER; note = 2'-O-methyladenosine-3'-phosphate
  modified_base 6: mod_base = OTHER; note = 2'-fluoroguanosine-3'-phosphate
  modified_base 7: mod_base = OTHER; note = 2'-O-methyladenosine-3'-phosphate
  modified_base 8: mod_base = OTHER; note = 2'-O-methylguanosine-3'-phosphate
  modified_base 9: mod_base = OTHER; note = 2'-O-methyladenosine-3'-phosphate
  modified_base 10: mod_base = OTHER; note = 2'-O-methyladenosine-3'-phosphate
  modified_base 11: mod_base = OTHER; note = 2'-O-methylguanosine-3'-phosphate
  modified_base 12: mod_base = OTHER; note = 2'-fluorouridine-3'-phosphate
  modified_base 13: mod_base = OTHER; note = 2'-O-methylcytidine-3'-phosphate
  modified_base 14: mod_base = OTHER; note = 2'-fluorocytidine-3'-phosphate
  modified_base 15: mod_base = OTHER; note = 2'-O-methyladenosine-3'-phosphate
  modified_base 16: mod_base = OTHER; note = 2'-fluorocytidine-3'-phosphate
  modified_base 17: mod_base = OTHER; note = 2'-O-methylcytidine-3'-phosphate
  modified_base 18: mod_base = OTHER; note = 2'-fluoroadenosine-3'-phosphate
  modified_base 19: mod_base = OTHER; note = 2'-O-methylcytidine-3'-phosphate
  modified_base 20: mod_base = OTHER; note = 2'-O-methylguanosine-3'-phosphate
  modified_base 21: mod_base = OTHER; note = 2'-O-methyladenosine-3'-phosphorothioate
  modified_base 22: mod_base = OTHER; note = 2'-O-methylguanosine-3'-phosphate
  misc_feature 1: note = RNA
  misc_feature 2: note = DNA
  misc_feature 3: note = RNA
  misc_feature 4: note = DNA
  misc_feature 5: note = RNA
  misc_feature 6: note = DNA
  misc_feature 7: note = RNA
  misc_feature 8: note = RNA
  misc_feature 9: note = RNA
  misc_feature 10: note = RNA
  misc_feature 11: note = RNA
  misc_feature 12: note = DNA
  misc_feature 13: note = RNA
  misc_feature 14: note = DNA
  misc_feature 15: note = RNA
  misc_feature 16: note = DNA
  misc_feature 17: note = RNA
  misc_feature 18: note = DNA
  misc_feature 19: note = RNA
  misc_feature 20: note = RNA
  misc_feature 21: note = RNA
  misc_feature 22: note = RNA
  source 1..22: mol_type = other RNA
tttgagagaagtccaccacgag

SEQ ID NO: 118 - RNA, 21 nt, synthetic construct
  modified_base 1: mod_base = OTHER; note = cyclopropyl phosphonate-2'-O-methyluridine-3'-phosphorothioate
  modified_base 2: mod_base = OTHER; note = 2'-fluorouridine-3'-phosphorothioate
  modified_base 3: mod_base = OTHER; note = 2'-O-methyluridine-3'-phosphorothioate
  modified_base 4: mod_base = OTHER; note = 2'-fluoroguanosine-3'-phosphate
  modified_base 5: mod_base = OTHER; note = 2'-O-methyladenosine-3'-phosphate
  modified_base 6: mod_base = OTHER; note = 2'-fluoroguanosine-3'-phosphate
  modified_base 7: mod_base = OTHER; note = 2'-O-methyladenosine-3'-phosphate
  modified_base 8: mod_base = OTHER; note = 2'-fluoroguanosine-3'-phosphate
  modified_base 9: mod_base = OTHER; note = 2'-O-methyladenosine-3'-phosphate
  modified_base 10: mod_base = OTHER; note = 2'-fluoroadenosine-3'-phosphate
  modified_base 11: mod_base = OTHER; note = 2'-O-methylguanosine-3'-phosphate
  modified_base 12: mod_base = OTHER; note = 2'-fluorouridine-3'-phosphate
  modified_base 13: mod_base = OTHER; note = 2'-O-methylcytidine-3'-phosphate
  modified_base 14: mod_base = OTHER; note = 2'-fluorocytidine-3'-phosphate
  modified_base 15: mod_base = OTHER; note = 2'-O-methyladenosine-3'-phosphate
  modified_base 16: mod_base = OTHER; note = 2'-fluorocytidine-3'-phosphate
  modified_base 17: mod_base = OTHER; note = 2'-O-methylcytidine-3'-phosphate
  modified_base 18: mod_base = OTHER; note = 2'-fluoroadenosine-3'-phosphate
  modified_base 19: mod_base = OTHER; note = 2'-O-methylcytidine-3'-phosphate
  modified_base 20: mod_base = OTHER; note = 2'-O-methyluridine-3'-phosphorothioate
  modified_base 21: mod_base = OTHER; note = 2'-O-methyluridine-3'-phosphate
  misc_feature 1: note = RNA
  misc_feature 2: note = DNA
  misc_feature 3: note = RNA
  misc_feature 4: note = DNA
  misc_feature 5: note = RNA
  misc_feature 6: note = DNA
  misc_feature 7: note = RNA
  misc_feature 8: note = DNA
  misc_feature 9: note = RNA
  misc_feature 10: note = DNA
  misc_feature 11: note = RNA
  misc_feature 12: note = DNA
  misc_feature 13: note = RNA
  misc_feature 14: note = DNA
  misc_feature 15: note = RNA
  misc_feature 16: note = DNA
  misc_feature 17: note = RNA
  misc_feature 18: note = DNA
  misc_feature 19: note = RNA
  misc_feature 20: note = RNA
  misc_feature 21: note = RNA
  source 1..21: mol_type = other RNA
tttgagagaagtccaccactt

SEQ ID NO: 119 - RNA, 22 nt, synthetic construct
  modified_base 1: mod_base = OTHER; note = cyclopropyl phosphonate-2'-O-methyluridine-3'-phosphorothioate
  modified_base 2: mod_base = OTHER; note = 2'-fluoroadenosine-3'-phosporothioate
  modified_base 3: mod_base = OTHER; note = 2'-O-methyluridine-3'-phosphorothioate
  modified_base 4: mod_base = OTHER; note = 2'-fluorouridine-3'-phosphate
  modified_base 5: mod_base = OTHER; note = 2'-O-methylguanosine-3'-phosphate
  modified_base 6: mod_base = OTHER; note = 2'-fluoroadenosine-3'-phosphate
  modified_base 7: mod_base = OTHER; note = 2'-O-methylguanosine-3'-phosphate
  modified_base 8: mod_base = OTHER; note = 2'-O-methyladenosine-3'-phosphate
  modified_base 9: mod_base = OTHER; note = 2'-O-methylguanosine-3'-phosphate
  modified_base 10: mod_base = OTHER; note = 2'-O-methyladenosine-3'-phosphate
  modified_base 11: mod_base = OTHER; note = 2'-O-methyladenosine-3'-phosphate
  modified_base 12: mod_base = OTHER; note = 2'-fluoroguanosine-3'-phosphate
  modified_base 13: mod_base = OTHER; note = 2'-O-methyluridine-3'-phosphate
  modified_base 14: mod_base = OTHER; note = 2'-fluorocytidine-3'-phosphate
  modified_base 15: mod_base = OTHER; note = 2'-O-methylcytidine-3'-phosphate
  modified_base 16: mod_base = OTHER; note = 2'-fluoroadenosine-3'-phosphate
  modified_base 17: mod_base = OTHER; note = 2'-O-methylcytidine-3'-phosphate
  modified_base 18: mod_base = OTHER; note = 2'-fluorocytidine-3'-phosphate
  modified_base 19: mod_base = OTHER; note = 2'-O-methyladenosine-3'-phosphate
  modified_base 20: mod_base = OTHER; note = 2'-O-methylcytidine-3'-phosphorothioate
  modified_base 21: mod_base = OTHER; note = 2'-O-methyluridine-3'-phosphorothioate
  modified_base 22: mod_base = OTHER; note = 2'-O-methyluridine-3'-phosphate
  misc_feature 1: note = RNA
  misc_feature 2: note = DNA
  misc_feature 3: note = RNA
  misc_feature 4: note = DNA
  misc_feature 5: note = RNA
  misc_feature 6: note = DNA
  misc_feature 7: note = RNA
  misc_feature 8: note = RNA
  misc_feature 9: note = RNA
  misc_feature 10: note = RNA
  misc_feature 11: note = RNA
  misc_feature 12: note = DNA
  misc_feature 13: note = RNA
  misc_feature 14: note = DNA
  misc_feature 15: note = RNA
  misc_feature 16: note = DNA
  misc_feature 17: note = RNA
  misc_feature 18: note = DNA
  misc_feature 19: note = RNA
  misc_feature 20: note = RNA
  misc_feature 21: note = RNA
  misc_feature 22: note = RNA
  source 1..22: mol_type = other RNA
tattgagagaagtccaccactt

SEQ ID NO: 120 - RNA, 22 nt, synthetic construct
  modified_base 1: mod_base = OTHER; note = 2'-O-methyluridine-3'-phosphorothioate
  modified_base 2: mod_base = OTHER; note = 2'-fluoroadenosine-3'-phosporothioate
  modified_base 3: mod_base = OTHER; note = 2'-O-methyluridine-3'-phosphorothioate
  modified_base 4: mod_base = OTHER; note = 2'-fluorouridine-3'-phosphate
  modified_base 5: mod_base = OTHER; note = 2'-O-methylguanosine-3'-phosphate
  modified_base 6: mod_base = OTHER; note = 2'-fluoroadenosine-3'-phosphate
  modified_base 7: mod_base = OTHER; note = 2'-O-methylguanosine-3'-phosphate
  modified_base 8: mod_base = OTHER; note = 2'-O-methyladenosine-3'-phosphate
  modified_base 9: mod_base = OTHER; note = 2'-O-methylguanosine-3'-phosphate
  modified_base 10: mod_base = OTHER; note = 2'-O-methyladenosine-3'-phosphate
  modified_base 11: mod_base = OTHER; note = 2'-O-methyladenosine-3'-phosphate
  modified_base 12: mod_base = OTHER; note = 2'-fluoroguanosine-3'-phosphate
  modified_base 13: mod_base = OTHER; note = 2'-O-methyluridine-3'-phosphate
  modified_base 14: mod_base = OTHER; note = 2'-fluorocytidine-3'-phosphate
  modified_base 15: mod_base = OTHER; note = 2'-O-methylcytidine-3'-phosphate
  modified_base 16: mod_base = OTHER; note = 2'-fluoroadenosine-3'-phosphate
  modified_base 17: mod_base = OTHER; note = 2'-O-methylcytidine-3'-phosphate
  modified_base 18: mod_base = OTHER; note = 2'-fluorocytidine-3'-phosphate
  modified_base 19: mod_base = OTHER; note = 2'-O-methyladenosine-3'-phosphate
  modified_base 20: mod_base = OTHER; note = 2'-O-methylcytidine-3'-phosphate
  modified_base 21: mod_base = OTHER; note = 2'-O-methyluridine-3'-phosphorothioate
  modified_base 22: mod_base = OTHER; note = 2'-O-methyluridine-3'-phosphate
  misc_feature 1: note = RNA
  misc_feature 2: note = DNA
  misc_feature 3: note = RNA
  misc_feature 4: note = DNA
  misc_feature 5: note = RNA
  misc_feature 6: note = DNA
  misc_feature 7: note = RNA
  misc_feature 8: note = RNA
  misc_feature 9: note = RNA
  misc_feature 10: note = RNA
  misc_feature 11: note = RNA
  misc_feature 12: note = DNA
  misc_feature 13: note = RNA
  misc_feature 14: note = DNA
  misc_feature 15: note = RNA
  misc_feature 16: note = DNA
  misc_feature 17: note = RNA
  misc_feature 18: note = DNA
  misc_feature 19: note = RNA
  misc_feature 20: note = RNA
  misc_feature 21: note = RNA
  misc_feature 22: note = RNA
  source 1..22: mol_type = other RNA
tattgagagaagtccaccactt

SEQ ID NO: 121 - RNA, 23 nt, synthetic construct
  modified_base 1: mod_base = OTHER; note = 2'-O-methyluridine-3'-phosphorothioate
  modified_base 2: mod_base = OTHER; note = 2'-fluoroadenosine-3'-phosporothioate
  modified_base 3: mod_base = OTHER; note = 2'-O-methyluridine-3'-phosphorothioate
  modified_base 4: mod_base = OTHER; note = 2'-fluorouridine-3'-phosphate
  modified_base 5: mod_base = OTHER; note = 2'-O-methylguanosine-3'-phosphate
  modified_base 6: mod_base = OTHER; note = 2'-fluoroadenosine-3'-phosphate
  modified_base 7: mod_base = OTHER; note = 2'-O-methylguanosine-3'-phosphate
  modified_base 8: mod_base = OTHER; note = 2'-O-methyladenosine-3'-phosphate
  modified_base 9: mod_base = OTHER; note = 2'-O-methylguanosine-3'-phosphate
  modified_base 10: mod_base = OTHER; note = 2'-O-methyladenosine-3'-phosphate
  modified_base 11: mod_base = OTHER; note = 2'-O-methyladenosine-3'-phosphate
  modified_base 12: mod_base = OTHER; note = 2'-fluoroguanosine-3'-phosphate
  modified_base 13: mod_base = OTHER; note = 2'-O-methyluridine-3'-phosphate
  modified_base 14: mod_base = OTHER; note = 2'-fluorocytidine-3'-phosphate
  modified_base 15: mod_base = OTHER; note = 2'-O-methylcytidine-3'-phosphate
  modified_base 16: mod_base = OTHER; note = 2'-fluoroadenosine-3'-phosphate
  modified_base 17: mod_base = OTHER; note = 2'-O-methylcytidine-3'-phosphate
  modified_base 18: mod_base = OTHER; note = 2'-fluorocytidine-3'-phosphate
  modified_base 19: mod_base = OTHER; note = 2'-O-methyladenosine-3'-phosphate
  modified_base 20: mod_base = OTHER; note = 2'-O-methylcytidine-3'-phosphate
  modified_base 21: mod_base = OTHER; note = 2'-O-methylguanosine-3'-phosphate
  modified_base 22: mod_base = OTHER; note = 2'-O-methyluridine-3'-phosphorothioate
  modified_base 23: mod_base = OTHER; note = 2'-O-methyluridine-3'-phosphate
  misc_feature 1: note = RNA
  misc_feature 2: note = DNA
  misc_feature 3: note = RNA
  misc_feature 4: note = DNA
  misc_feature 5: note = RNA
  misc_feature 6: note = DNA
  misc_feature 7: note = RNA
  misc_feature 8: note = RNA
  misc_feature 9: note = RNA
  misc_feature 10: note = RNA
  misc_feature 11: note = RNA
  misc_feature 12: note = DNA
  misc_feature 13: note = RNA
  misc_feature 14: note = DNA
  misc_feature 15: note = RNA
  misc_feature 16: note = DNA
  misc_feature 17: note = RNA
  misc_feature 18: note = DNA
  misc_feature 19: note = RNA
  misc_feature 20: note = RNA
  misc_feature 21: note = RNA
  misc_feature 22: note = RNA
  misc_feature 23: note = RNA
  source 1..23: mol_type = other RNA
tattgagagaagtccaccacgtt

SEQ ID NO: 122 - RNA, 23 nt, synthetic construct
  modified_base 1: mod_base = OTHER; note = 2'-O-methyluridine-3'-phosphorothioate
  modified_base 2: mod_base = OTHER; note = 2'-fluoroadenosine-3'-phosporothioate
  modified_base 3: mod_base = OTHER; note = 2'-O-methyluridine-3'-phosphorothioate
  modified_base 4: mod_base = OTHER; note = 2'-fluorouridine-3'-phosphate
  modified_base 5: mod_base = OTHER; note = 2'-O-methylguanosine-3'-phosphate
  modified_base 6: mod_base = OTHER; note = 2'-fluoroadenosine-3'-phosphate
  modified_base 7: mod_base = OTHER; note = 2'-O-methylguanosine-3'-phosphate
  modified_base 8: mod_base = OTHER; note = 2'-O-methyladenosine-3'-phosphate
  modified_base 9: mod_base = OTHER; note = 2'-O-methylguanosine-3'-phosphate
  modified_base 10: mod_base = OTHER; note = 2'-O-methyladenosine-3'-phosphate
  modified_base 11: mod_base = OTHER; note = 2'-O-methyladenosine-3'-phosphate
  modified_base 12: mod_base = OTHER; note = 2'-fluoroguanosine-3'-phosphate
  modified_base 13: mod_base = OTHER; note = 2'-O-methyluridine-3'-phosphate
  modified_base 14: mod_base = OTHER; note = 2'-fluorocytidine-3'-phosphate
  modified_base 15: mod_base = OTHER; note = 2'-O-methylcytidine-3'-phosphate
  modified_base 16: mod_base = OTHER; note = 2'-fluoroadenosine-3'-phosphate
  modified_base 17: mod_base = OTHER; note = 2'-O-methylcytidine-3'-phosphate
  modified_base 18: mod_base = OTHER; note = 2'-fluorocytidine-3'-phosphate
  modified_base 19: mod_base = OTHER; note = 2'-O-methyladenosine-3'-phosphate
  modified_base 20: mod_base = OTHER; note = 2'-O-methylcytidine-3'-phosphate
  modified_base 21: mod_base = OTHER; note = 2'-O-methyluridine-3'-phosphate
  modified_base 22: mod_base = OTHER; note = 2'-O-methyluridine-3'-phosphorothioate
  modified_base 23: mod_base = OTHER; note = inverted (3'-3' linked) abasic deoxyribonucleotide
  misc_feature 1: note = RNA
  misc_feature 2: note = DNA
  misc_feature 3: note = RNA
  misc_feature 4: note = DNA
  misc_feature 5: note = RNA
  misc_feature 6: note = DNA
  misc_feature 7: note = RNA
  misc_feature 8: note = RNA
  misc_feature 9: note = RNA
  misc_feature 10: note = RNA
  misc_feature 11: note = RNA
  misc_feature 12: note = DNA
  misc_feature 13: note = RNA
  misc_feature 14: note = DNA
  misc_feature 15: note = RNA
  misc_feature 16: note = DNA
  misc_feature 17: note = RNA
  misc_feature 18: note = DNA
  misc_feature 19: note = RNA
  misc_feature 20: note = RNA
  misc_feature 21: note = RNA
  misc_feature 22: note = RNA
  misc_feature 23: note = DNA
  source 1..23: mol_type = other RNA
tattgagagaagtccaccacttn

SEQ ID NO: 123 - RNA, 23 nt, synthetic construct
  modified_base 1: mod_base = OTHER; note = 2'-O-methyluridine-3'-phosphorothioate
  modified_base 2: mod_base = OTHER; note = 2'-fluoroadenosine-3'-phosporothioate
  modified_base 3: mod_base = OTHER; note = 2'-O-methyluridine-3'-phosphorothioate
  modified_base 4: mod_base = OTHER; note = 2'-fluorouridine-3'-phosphate
  modified_base 5: mod_base = OTHER; note = 2'-O-methylguanosine-3'-phosphate
  modified_base 6: mod_base = OTHER; note = 2'-fluoroadenosine-3'-phosphate
  modified_base 7: mod_base = OTHER; note = 2'-O-methylguanosine-3'-phosphate
  modified_base 8: mod_base = OTHER; note = 2'-O-methyladenosine-3'-phosphate
  modified_base 9: mod_base = OTHER; note = 2'-O-methylguanosine-3'-phosphate
  modified_base 10: mod_base = OTHER; note = 2'-O-methyladenosine-3'-phosphate
  modified_base 11: mod_base = OTHER; note = 2'-O-methyladenosine-3'-phosphate
  modified_base 12: mod_base = OTHER; note = 2'-fluoroguanosine-3'-phosphate
  modified_base 13: mod_base = OTHER; note = 2'-O-methyluridine-3'-phosphate
  modified_base 14: mod_base = OTHER; note = 2'-fluorocytidine-3'-phosphate
  modified_base 15: mod_base = OTHER; note = 2'-O-methylcytidine-3'-phosphate
  modified_base 16: mod_base = OTHER; note = 2'-fluoroadenosine-3'-phosphate
  modified_base 17: mod_base = OTHER; note = 2'-O-methylcytidine-3'-phosphate
  modified_base 18: mod_base = OTHER; note = 2'-fluorocytidine-3'-phosphate
  modified_base 19: mod_base = OTHER; note = 2'-O-methyladenosine-3'-phosphate
  modified_base 20: mod_base = OTHER; note = 2'-O-methylcytidine-3'-phosphate
  modified_base 21: mod_base = OTHER; note = 2'-O-methylguanosine-3'-phosphate
  modified_base 22: mod_base = OTHER; note = 2'-O-methyladenosine-3'-phosphorothioate
  modified_base 23: mod_base = OTHER; note = 2'-O-methylguanosine-3'-phosphate
  misc_feature 1: note = RNA
  misc_feature 2: note = DNA
  misc_feature 3: note = RNA
  misc_feature 4: note = DNA
  misc_feature 5: note = RNA
  misc_feature 6: note = DNA
  misc_feature 7: note = RNA
  misc_feature 8: note = RNA
  misc_feature 9: note = RNA
  misc_feature 10: note = RNA
  misc_feature 11: note = RNA
  misc_feature 12: note = DNA
  misc_feature 13: note = RNA
  misc_feature 14: note = DNA
  misc_feature 15: note = RNA
  misc_feature 16: note = DNA
  misc_feature 17: note = RNA
  misc_feature 18: note = DNA
  misc_feature 19: note = RNA
  misc_feature 20: note = RNA
  misc_feature 21: note = RNA
  misc_feature 22: note = RNA
  misc_feature 23: note = RNA
  source 1..23: mol_type = other RNA
tattgagagaagtccaccacgag

SEQ ID NO: 124 - RNA, 22 nt, synthetic construct
  modified_base 1: mod_base = OTHER; note = 2'-O-methyluridine-3'-phosphorothioate
  modified_base 2: mod_base = OTHER; note = 2'-fluoroadenosine-3'-phosporothioate
  modified_base 3: mod_base = OTHER; note = 2'-O-methyluridine-3'-phosphorothioate
  modified_base 4: mod_base = OTHER; note = 2'-fluorouridine-3'-phosphate
  modified_base 5: mod_base = OTHER; note = 2'-O-methylguanosine-3'-phosphate
  modified_base 6: mod_base = OTHER; note = 2'-fluoroadenosine-3'-phosphate
  modified_base 7: mod_base = OTHER; note = 2'-O-methylguanosine-3'-phosphate
  modified_base 8: mod_base = OTHER; note = 2'-fluoroadenosine-3'-phosphate
  modified_base 9: mod_base = OTHER; note = 2'-O-methylguanosine-3'-phosphate
  modified_base 10: mod_base = OTHER; note = 2'-fluoroadenosine-3'-phosphate
  modified_base 11: mod_base = OTHER; note = 2'-O-methyladenosine-3'-phosphate
  modified_base 12: mod_base = OTHER; note = 2'-fluoroguanosine-3'-phosphate
  modified_base 13: mod_base = OTHER; note = 2'-O-methyluridine-3'-phosphate
  modified_base 14: mod_base = OTHER; note = 2'-fluorocytidine-3'-phosphate
  modified_base 15: mod_base = OTHER; note = 2'-O-methylcytidine-3'-phosphate
  modified_base 16: mod_base = OTHER; note = 2'-fluoroadenosine-3'-phosphate
  modified_base 17: mod_base = OTHER; note = 2'-O-methylcytidine-3'-phosphate
  modified_base 18: mod_base = OTHER; note = 2'-fluorocytidine-3'-phosphate
  modified_base 19: mod_base = OTHER; note = 2'-O-methyladenosine-3'-phosphate
  modified_base 20: mod_base = OTHER; note = 2'-O-methylcytidine-3'-phosphate
  modified_base 21: mod_base = OTHER; note = 2'-O-methyluridine-3'-phosphorothioate
  modified_base 22: mod_base = OTHER; note = 2'-O-methyluridine-3'-phosphate
  misc_feature 1: note = RNA
  misc_feature 2: note = DNA
  misc_feature 3: note = RNA
  misc_feature 4: note = DNA
  misc_feature 5: note = RNA
  misc_feature 6: note = DNA
  misc_feature 7: note = RNA
  misc_feature 8: note = DNA
  misc_feature 9: note = RNA
  misc_feature 10: note = DNA
  misc_feature 11: note = RNA
  misc_feature 12: note = DNA
  misc_feature 13: note = RNA
  misc_feature 14: note = DNA
  misc_feature 15: note = RNA
  misc_feature 16: note = DNA
  misc_feature 17: note = RNA
  misc_feature 18: note = DNA
  misc_feature 19: note = RNA
  misc_feature 20: note = RNA
  misc_feature 21: note = RNA
  misc_feature 22: note = RNA
  source 1..22: mol_type = other RNA
tattgagagaagtccaccactt

SEQ ID NO: 125 - RNA, 21 nt, synthetic construct
  modified_base 1: mod_base = OTHER; note = 2'-O-methyladenosine-3'-phosphorothioate
  modified_base 2: mod_base = OTHER; note = 2'-fluoroguanosine-3'-phosphorothioate
  modified_base 3: mod_base = OTHER; note = 2'-O-methyladenosine-3'-phosphorothioate
  modified_base 4: mod_base = OTHER; note = 2'-fluoroadenosine-3'-phosphate
  modified_base 5: mod_base = OTHER; note = 2'-O-methyladenosine-3'-phosphate
  modified_base 6: mod_base = OTHER; note = 2'-fluoroadenosine-3'-phosphate
  modified_base 7: mod_base = OTHER; note = 2'-O-methyluridine-3'-phosphate
  modified_base 8: mod_base = OTHER; note = 2'-fluorouridine-3'-phosphate
  modified_base 9: mod_base = OTHER; note = 2'-O-methylguanosine-3'-phosphate
  modified_base 10: mod_base = OTHER; note = 2'-fluoroadenosine-3'-phosphate
  modified_base 11: mod_base = OTHER; note = 2'-O-methylguanosine-3'-phosphate
  modified_base 12: mod_base = OTHER; note = 2'-fluoroadenosine-3'-phosphate
  modified_base 13: mod_base = OTHER; note = 2'-O-methylguanosine-3'-phosphate
  modified_base 14: mod_base = OTHER; note = 2'-fluoroadenosine-3'-phosphate
  modified_base 15: mod_base = OTHER; note = 2'-O-methyladenosine-3'-phosphate
  modified_base 16: mod_base = OTHER; note = 2'-fluoroguanosine-3'-phosphate
  modified_base 17: mod_base = OTHER; note = 2'-O-methyluridine-3'-phosphate
  modified_base 18: mod_base = OTHER; note = 2'-fluorocytidine-3'-phosphate
  modified_base 19: mod_base = OTHER; note = 2'-O-methylcytidine-3'-phosphate
  modified_base 20: mod_base = OTHER; note = 2'-O-methyluridine-3'-phosphorothioate
  modified_base 21: mod_base = OTHER; note = 2'-O-methyluridine-3'-phosphate
  misc_feature 1: note = RNA
  misc_feature 2: note = DNA
  misc_feature 3: note = RNA
  misc_feature 4: note = DNA
  misc_feature 5: note = RNA
  misc_feature 6: note = DNA
  misc_feature 7: note = RNA
  misc_feature 8: note = DNA
  misc_feature 9: note = RNA
  misc_feature 10: note = DNA
  misc_feature 11: note = RNA
  misc_feature 12: note = DNA
  misc_feature 13: note = RNA
  misc_feature 14: note = DNA
  misc_feature 15: note = RNA
  misc_feature 16: note = DNA
  misc_feature 17: note = RNA
  misc_feature 18: note = DNA
  misc_feature 19: note = RNA
  misc_feature 20: note = RNA
  misc_feature 21: note = RNA
  source 1..21: mol_type = other RNA
agaaaattgagagaagtcctt

SEQ ID NO: 126 - RNA, 21 nt, synthetic construct
  modified_base 1: mod_base = OTHER; note = 2'-O-methyladenosine-3'-phosphorothioate
  modified_base 2: mod_base = OTHER; note = 2'-fluoroguanosine-3'-phosphorothioate
  modified_base 3: mod_base = OTHER; note = 2'-O-methyladenosine-3'-phosphorothioate
  modified_base 4: mod_base = OTHER; note = 2'-fluoroadenosine-3'-phosphate
  modified_base 5: mod_base = OTHER; note = 2'-O-methyladenosine-3'-phosphate
  modified_base 6: mod_base = OTHER; note = 2'-fluoroadenosine-3'-phosphate
  modified_base 7: mod_base = OTHER; note = 2'-O-methyluridine-3'-phosphate
  modified_base 8: mod_base = OTHER; note = 2'-fluorouridine-3'-phosphate
  modified_base 9: mod_base = OTHER; note = 2'-O-methylguanosine-3'-phosphate
  modified_base 10: mod_base = OTHER; note = 2'-fluoroadenosine-3'-phosphate
  modified_base 11: mod_base = OTHER; note = 2'-O-methylguanosine-3'-phosphate
  modified_base 12: mod_base = OTHER; note = 2'-fluoroadenosine-3'-phosphate
  modified_base 13: mod_base = OTHER; note = 2'-O-methylguanosine-3'-phosphate
  modified_base 14: mod_base = OTHER; note = 2'-fluoroadenosine-3'-phosphate
  modified_base 15: mod_base = OTHER; note = 2'-O-methyladenosine-3'-phosphate
  modified_base 16: mod_base = OTHER; note = 2'-fluoroguanosine-3'-phosphate
  modified_base 17: mod_base = OTHER; note = 2'-O-methyluridine-3'-phosphate
  modified_base 18: mod_base = OTHER; note = 2'-fluorocytidine-3'-phosphate
  modified_base 19: mod_base = OTHER; note = 2'-O-methylcytidine-3'-phosphate
  modified_base 20: mod_base = OTHER; note = 2'-O-methyladenosine-3'-phosphorothioate
  modified_base 21: mod_base = OTHER; note = 2'-O-methylcytidine-3'-phosphate
  misc_feature 1: note = RNA
  misc_feature 2: note = DNA
  misc_feature 3: note = RNA
  misc_feature 4: note = DNA
  misc_feature 5: note = RNA
  misc_feature 6: note = DNA
  misc_feature 7: note = RNA
  misc_feature 8: note = DNA
  misc_feature 9: note = RNA
  misc_feature 10: note = DNA
  misc_feature 11: note = RNA
  misc_feature 12: note = DNA
  misc_feature 13: note = RNA
  misc_feature 14: note = DNA
  misc_feature 15: note = RNA
  misc_feature 16: note = DNA
  misc_feature 17: note = RNA
  misc_feature 18: note = DNA
  misc_feature 19: note = RNA
  misc_feature 20: note = RNA
  misc_feature 21: note = RNA
  source 1..21: mol_type = other RNA
agaaaattgagagaagtccac

SEQ ID NO: 127 - RNA, 23 nt, synthetic construct
  modified_base 1: mod_base = OTHER; note = 2'-O-methyladenosine-3'-phosphorothioate
  modified_base 2: mod_base = OTHER; note = 2'-fluoroguanosine-3'-phosphorothioate
  modified_base 3: mod_base = OTHER; note = 2'-O-methyladenosine-3'-phosphorothioate
  modified_base 4: mod_base = OTHER; note = 2'-fluoroadenosine-3'-phosphate
  modified_base 5: mod_base = OTHER; note = 2'-O-methyladenosine-3'-phosphate
  modified_base 6: mod_base = OTHER; note = 2'-fluoroadenosine-3'-phosphate
  modified_base 7: mod_base = OTHER; note = 2'-O-methyluridine-3'-phosphate
  modified_base 8: mod_base = OTHER; note = 2'-fluorouridine-3'-phosphate
  modified_base 9: mod_base = OTHER; note = 2'-O-methylguanosine-3'-phosphate
  modified_base 10: mod_base = OTHER; note = 2'-fluoroadenosine-3'-phosphate
  modified_base 11: mod_base = OTHER; note = 2'-O-methylguanosine-3'-phosphate
  modified_base 12: mod_base = OTHER; note = 2'-fluoroadenosine-3'-phosphate
  modified_base 13: mod_base = OTHER; note = 2'-O-methylguanosine-3'-phosphate
  modified_base 14: mod_base = OTHER; note = 2'-fluoroadenosine-3'-phosphate
  modified_base 15: mod_base = OTHER; note = 2'-O-methyladenosine-3'-phosphate
  modified_base 16: mod_base = OTHER; note = 2'-fluoroguanosine-3'-phosphate
  modified_base 17: mod_base = OTHER; note = 2'-O-methyluridine-3'-phosphate
  modified_base 18: mod_base = OTHER; note = 2'-fluorocytidine-3'-phosphate
  modified_base 19: mod_base = OTHER; note = 2'-O-methylcytidine-3'-phosphate
  modified_base 20: mod_base = OTHER; note = 2'-O-methyladenosine-3'-phosphate
  modified_base 21: mod_base = OTHER; note = 2'-O-methylcytidine-3'-phosphate
  modified_base 22: mod_base = OTHER; note = 2'-O-methyluridine-3'-phosphorothioate
  modified_base 23: mod_base = OTHER; note = 2'-O-methyluridine-3'-phosphate
  misc_feature 1: note = RNA
  misc_feature 2: note = DNA
  misc_feature 3: note = RNA
  misc_feature 4: note = DNA
  misc_feature 5: note = RNA
  misc_feature 6: note = DNA
  misc_feature 7: note = RNA
  misc_feature 8: note = DNA
  misc_feature 9: note = RNA
  misc_feature 10: note = DNA
  misc_feature 11: note = RNA
  misc_feature 12: note = DNA
  misc_feature 13: note = RNA
  misc_feature 14: note = DNA
  misc_feature 15: note = RNA
  misc_feature 16: note = DNA
  misc_feature 17: note = RNA
  misc_feature 18: note = DNA
  misc_feature 19: note = RNA
  misc_feature 20: note = RNA
  misc_feature 21: note = RNA
  misc_feature 22: note = RNA
  misc_feature 23: note = RNA
  source 1..23: mol_type = other RNA
agaaaattgagagaagtccactt

SEQ ID NO: 128 - RNA, 22 nt, synthetic construct
  modified_base 1: mod_base = OTHER; note = 2'-O-methyladenosine-3'-phosphorothioate
  modified_base 2: mod_base = OTHER; note = 2'-fluoroguanosine-3'-phosphorothioate
  modified_base 3: mod_base = OTHER; note = 2'-O-methyladenosine-3'-phosphorothioate
  modified_base 4: mod_base = OTHER; note = 2'-fluoroadenosine-3'-phosphate
  modified_base 5: mod_base = OTHER; note = 2'-O-methyladenosine-3'-phosphate
  modified_base 6: mod_base = OTHER; note = 2'-fluoroadenosine-3'-phosphate
  modified_base 7: mod_base = OTHER; note = 2'-O-methyluridine-3'-phosphate
  modified_base 8: mod_base = OTHER; note = 2'-fluorouridine-3'-phosphate
  modified_base 9: mod_base = OTHER; note = 2'-O-methylguanosine-3'-phosphate
  modified_base 10: mod_base = OTHER; note = 2'-fluoroadenosine-3'-phosphate
  modified_base 11: mod_base = OTHER; note = 2'-O-methylguanosine-3'-phosphate
  modified_base 12: mod_base = OTHER; note = 2'-fluoroadenosine-3'-phosphate
  modified_base 13: mod_base = OTHER; note = 2'-O-methylguanosine-3'-phosphate
  modified_base 14: mod_base = OTHER; note = 2'-fluoroadenosine-3'-phosphate
  modified_base 15: mod_base = OTHER; note = 2'-O-methyladenosine-3'-phosphate
  modified_base 16: mod_base = OTHER; note = 2'-fluoroguanosine-3'-phosphate
  modified_base 17: mod_base = OTHER; note = 2'-O-methyluridine-3'-phosphate
  modified_base 18: mod_base = OTHER; note = 2'-fluorocytidine-3'-phosphate
  modified_base 19: mod_base = OTHER; note = 2'-O-methylcytidine-3'-phosphate
  modified_base 20: mod_base = OTHER; note = 2'-O-methyladenosine-3'-phosphate
  modified_base 21: mod_base = OTHER; note = 2'-O-methylcytidine-3'-phosphorothioate
  modified_base 22: mod_base = OTHER; note = 2'-O-methylcytidine-3'-phosphate
  misc_feature 1: note = RNA
  misc_feature 2: note = DNA
  misc_feature 3: note = RNA
  misc_feature 4: note = DNA
  misc_feature 5: note = RNA
  misc_feature 6: note = DNA
  misc_feature 7: note = RNA
  misc_feature 8: note = DNA
  misc_feature 9: note = RNA
  misc_feature 10: note = DNA
  misc_feature 11: note = RNA
  misc_feature 12: note = DNA
  misc_feature 13: note = RNA
  misc_feature 14: note = DNA
  misc_feature 15: note = RNA
  misc_feature 16: note = DNA
  misc_feature 17: note = RNA
  misc_feature 18: note = DNA
  misc_feature 19: note = RNA
  misc_feature 20: note = RNA
  misc_feature 21: note = RNA
  misc_feature 22: note = RNA
  source 1..22: mol_type = other RNA
agaaaattgagagaagtccacc

SEQ ID NO: 129 - RNA, 21 nt, synthetic construct
  modified_base 1: mod_base = OTHER; note = 2'-O-methyluridine-3'-phosphorothioate
  modified_base 2: mod_base = OTHER; note = 2'-fluoroguanosine-3'-phosphorothioate
  modified_base 3: mod_base = OTHER; note = 2'-O-methyladenosine-3'-phosphorothioate
  modified_base 4: mod_base = OTHER; note = 2'-fluoroadenosine-3'-phosphate
  modified_base 5: mod_base = OTHER; note = 2'-O-methyladenosine-3'-phosphate
  modified_base 6: mod_base = OTHER; note = 2'-fluoroadenosine-3'-phosphate
  modified_base 7: mod_base = OTHER; note = 2'-O-methyluridine-3'-phosphate
  modified_base 8: mod_base = OTHER; note = 2'-fluorouridine-3'-phosphate
  modified_base 9: mod_base = OTHER; note = 2'-O-methylguanosine-3'-phosphate
  modified_base 10: mod_base = OTHER; note = 2'-fluoroadenosine-3'-phosphate
  modified_base 11: mod_base = OTHER; note = 2'-O-methylguanosine-3'-phosphate
  modified_base 12: mod_base = OTHER; note = 2'-fluoroadenosine-3'-phosphate
  modified_base 13: mod_base = OTHER; note = 2'-O-methylguanosine-3'-phosphate
  modified_base 14: mod_base = OTHER; note = 2'-fluoroadenosine-3'-phosphate
  modified_base 15: mod_base = OTHER; note = 2'-O-methyladenosine-3'-phosphate
  modified_base 16: mod_base = OTHER; note = 2'-fluoroguanosine-3'-phosphate
  modified_base 17: mod_base = OTHER; note = 2'-O-methyluridine-3'-phosphate
  modified_base 18: mod_base = OTHER; note = 2'-fluorocytidine-3'-phosphate
  modified_base 19: mod_base = OTHER; note = 2'-O-methylcytidine-3'-phosphate
  modified_base 20: mod_base = OTHER; note = 2'-O-methyluridine-3'-phosphorothioate
  modified_base 21: mod_base = OTHER; note = 2'-O-methyluridine-3'-phosphate
  misc_feature 1: note = RNA
  misc_feature 2: note = DNA
  misc_feature 3: note = RNA
  misc_feature 4: note = DNA
  misc_feature 5: note = RNA
  misc_feature 6: note = DNA
  misc_feature 7: note = RNA
  misc_feature 8: note = DNA
  misc_feature 9: note = RNA
  misc_feature 10: note = DNA
  misc_feature 11: note = RNA
  misc_feature 12: note = DNA
  misc_feature 13: note = RNA
  misc_feature 14: note = DNA
  misc_feature 15: note = RNA
  misc_feature 16: note = DNA
  misc_feature 17: note = RNA
  misc_feature 18: note = DNA
  misc_feature 19: note = RNA
  misc_feature 20: note = RNA
  misc_feature 21: note = RNA
  source 1..21: mol_type = other RNA
tgaaaattgagagaagtcctt

SEQ ID NO: 130 - RNA, 21 nt, synthetic construct
  modified_base 1: mod_base = OTHER; note = 2'-O-methyluridine-3'-phosphorothioate
  modified_base 2: mod_base = OTHER; note = 2'-fluoroguanosine-3'-phosphorothioate
  modified_base 3: mod_base = OTHER; note = 2'-O-methyladenosine-3'-phosphorothioate
  modified_base 4: mod_base = OTHER; note = 2'-fluoroadenosine-3'-phosphate
  modified_base 5: mod_base = OTHER; note = 2'-O-methyladenosine-3'-phosphate
  modified_base 6: mod_base = OTHER; note = 2'-fluoroadenosine-3'-phosphate
  modified_base 7: mod_base = OTHER; note = 2'-O-methyluridine-3'-phosphate
  modified_base 8: mod_base = OTHER; note = 2'-fluorouridine-3'-phosphate
  modified_base 9: mod_base = OTHER; note = 2'-O-methylguanosine-3'-phosphate
  modified_base 10: mod_base = OTHER; note = 2'-fluoroadenosine-3'-phosphate
  modified_base 11: mod_base = OTHER; note = 2'-O-methylguanosine-3'-phosphate
  modified_base 12: mod_base = OTHER; note = 2'-fluoroadenosine-3'-phosphate
  modified_base 13: mod_base = OTHER; note = 2'-O-methylguanosine-3'-phosphate
  modified_base 14: mod_base = OTHER; note = 2'-fluoroadenosine-3'-phosphate
  modified_base 15: mod_base = OTHER; note = 2'-O-methyladenosine-3'-phosphate
  modified_base 16: mod_base = OTHER; note = 2'-fluoroguanosine-3'-phosphate
  modified_base 17: mod_base = OTHER; note = 2'-O-methyluridine-3'-phosphate
  modified_base 18: mod_base = OTHER; note = 2'-fluorocytidine-3'-phosphate
  modified_base 19: mod_base = OTHER; note = 2'-O-methylcytidine-3'-phosphate
  modified_base 20: mod_base = OTHER; note = 2'-O-methyladenosine-3'-phosphorothioate
  modified_base 21: mod_base = OTHER; note = 2'-O-methylcytidine-3'-phosphate
  misc_feature 1: note = RNA
  misc_feature 2: note = DNA
  misc_feature 3: note = RNA
  misc_feature 4: note = DNA
  misc_feature 5: note = RNA
  misc_feature 6: note = DNA
  misc_feature 7: note = RNA
  misc_feature 8: note = DNA
  misc_feature 9: note = RNA
  misc_feature 10: note = DNA
  misc_feature 11: note = RNA
  misc_feature 12: note = DNA
  misc_feature 13: note = RNA
  misc_feature 14: note = DNA
  misc_feature 15: note = RNA
  misc_feature 16: note = DNA
  misc_feature 17: note = RNA
  misc_feature 18: note = DNA
  misc_feature 19: note = RNA
  misc_feature 20: note = RNA
  misc_feature 21: note = RNA
  source 1..21: mol_type = other RNA
tgaaaattgagagaagtccac

SEQ ID NO: 131 - RNA, 21 nt, synthetic construct
  modified_base 1: mod_base = OTHER; note = 2'-O-methyladenosine-3'-phosphorothioate
  modified_base 2: mod_base = OTHER; note = 2'-fluorocytidine-3'-phosphorothioate
  modified_base 3: mod_base = OTHER; note = 2'-O-methylcytidine-3'-phosphorothioate
  modified_base 4: mod_base = OTHER; note = 2'-fluoroadenosine-3'-phosphate
  modified_base 5: mod_base = OTHER; note = 2'-O-methyladenosine-3'-phosphate
  modified_base 6: mod_base = OTHER; note = 2'-fluorouridine-3'-phosphate
  modified_base 7: mod_base = OTHER; note = 2'-O-methyluridine-3'-phosphate
  modified_base 8: mod_base = OTHER; note = 2'-fluorouridine-3'-phosphate
  modified_base 9: mod_base = OTHER; note = 2'-O-methyladenosine-3'-phosphate
  modified_base 10: mod_base = OTHER; note = 2'-fluorouridine-3'-phosphate
  modified_base 11: mod_base = OTHER; note = 2'-O-methylguanosine-3'-phosphate
  modified_base 12: mod_base = OTHER; note = 2'-fluorocytidine-3'-phosphate
  modified_base 13: mod_base = OTHER; note = 2'-O-methylcytidine-3'-phosphate
  modified_base 14: mod_base = OTHER; note = 2'-fluorouridine-3'-phosphate
  modified_base 15: mod_base = OTHER; note = 2'-O-methyladenosine-3'-phosphate
  modified_base 16: mod_base = OTHER; note = 2'-fluorocytidine-3'-phosphate
  modified_base 17: mod_base = OTHER; note = 2'-O-methyladenosine-3'-phosphate
  modified_base 18: mod_base = OTHER; note = 2'-fluoroguanosine-3'-phosphate
  modified_base 19: mod_base = OTHER; note = 2'-O-methylcytidine-3'-phosphate
  modified_base 20: mod_base = OTHER; note = 2'-O-methyluridine-3'-phosphorothioate
  modified_base 21: mod_base = OTHER; note = 2'-O-methyluridine-3'-phosphate
  misc_feature 1: note = RNA
  misc_feature 2: note = DNA
  misc_feature 3: note = RNA
  misc_feature 4: note = DNA
  misc_feature 5: note = RNA
  misc_feature 6: note = DNA
  misc_feature 7: note = RNA
  misc_feature 8: note = DNA
  misc_feature 9: note = RNA
  misc_feature 10: note = DNA
  misc_feature 11: note = RNA
  misc_feature 12: note = DNA
  misc_feature 13: note = RNA
  misc_feature 14: note = DNA
  misc_feature 15: note = RNA
  misc_feature 16: note = DNA
  misc_feature 17: note = RNA
  misc_feature 18: note = DNA
  misc_feature 19: note = RNA
  misc_feature 20: note = RNA
  misc_feature 21: note = RNA
  source 1..21: mol_type = other RNA
accaatttatgcctacagctt

SEQ ID NO: 132 - RNA, 22 nt, synthetic construct
  modified_base 1: mod_base = OTHER; note = 2'-O-methyladenosine-3'-phosphorothioate
  modified_base 2: mod_base = OTHER; note = 2'-fluorocytidine-3'-phosphorothioate
  modified_base 3: mod_base = OTHER; note = 2'-O-methylcytidine-3'-phosphorothioate
  modified_base 4: mod_base = OTHER; note = 2'-fluoroadenosine-3'-phosphate
  modified_base 5: mod_base = OTHER; note = 2'-O-methyladenosine-3'-phosphate
  modified_base 6: mod_base = OTHER; note = 2'-fluorouridine-3'-phosphate
  modified_base 7: mod_base = OTHER; note = 2'-O-methyluridine-3'-phosphate
  modified_base 8: mod_base = OTHER; note = 2'-fluorouridine-3'-phosphate
  modified_base 9: mod_base = OTHER; note = 2'-O-methyladenosine-3'-phosphate
  modified_base 10: mod_base = OTHER; note = 2'-fluorouridine-3'-phosphate
  modified_base 11: mod_base = OTHER; note = 2'-O-methylguanosine-3'-phosphate
  modified_base 12: mod_base = OTHER; note = 2'-fluorocytidine-3'-phosphate
  modified_base 13: mod_base = OTHER; note = 2'-O-methylcytidine-3'-phosphate
  modified_base 14: mod_base = OTHER; note = 2'-fluorouridine-3'-phosphate
  modified_base 15: mod_base = OTHER; note = 2'-O-methyladenosine-3'-phosphate
  modified_base 16: mod_base = OTHER; note = 2'-fluorocytidine-3'-phosphate
  modified_base 17: mod_base = OTHER; note = 2'-O-methyladenosine-3'-phosphate
  modified_base 18: mod_base = OTHER; note = 2'-fluoroguanosine-3'-phosphate
  modified_base 19: mod_base = OTHER; note = 2'-O-methylcytidine-3'-phosphate
  modified_base 20: mod_base = OTHER; note = 2'-O-methylcytidine-3'-phosphate
  modified_base 21: mod_base = OTHER; note = 2'-O-methyluridine-3'-phosphorothioate
  modified_base 22: mod_base = OTHER; note = 2'-O-methyluridine-3'-phosphate
  misc_feature 1: note = RNA
  misc_feature 2: note = DNA
  misc_feature 3: note = RNA
  misc_feature 4: note = DNA
  misc_feature 5: note = RNA
  misc_feature 6: note = DNA
  misc_feature 7: note = RNA
  misc_feature 8: note = DNA
  misc_feature 9: note = RNA
  misc_feature 10: note = DNA
  misc_feature 11: note = RNA
  misc_feature 12: note = DNA
  misc_feature 13: note = RNA
  misc_feature 14: note = DNA
  misc_feature 15: note = RNA
  misc_feature 16: note = DNA
  misc_feature 17: note = RNA
  misc_feature 18: note = DNA
  misc_feature 19: note = RNA
  misc_feature 20: note = RNA
  misc_feature 21: note = RNA
  misc_feature 22: note = RNA
  source 1..22: mol_type = other RNA
accaatttatgcctacagcctt

SEQ ID NO: 133 - RNA, 22 nt, synthetic construct
  modified_base 1: mod_base = OTHER; note = 2'-O-methyladenosine-3'-phosphorothioate
  modified_base 2: mod_base = OTHER; note = 2'-fluorocytidine-3'-phosphorothioate
  modified_base 3: mod_base = OTHER; note = 2'-O-methylcytidine-3'-phosphorothioate
  modified_base 4: mod_base = OTHER; note = 2'-fluoroadenosine-3'-phosphate
  modified_base 5: mod_base = OTHER; note = 2'-O-methyladenosine-3'-phosphate
  modified_base 6: mod_base = OTHER; note = 2'-fluorouridine-3'-phosphate
  modified_base 7: mod_base = OTHER; note = 2'-O-methyluridine-3'-phosphate
  modified_base 8: mod_base = OTHER; note = 2'-fluorouridine-3'-phosphate
  modified_base 9: mod_base = OTHER; note = 2'-O-methyladenosine-3'-phosphate
  modified_base 10: mod_base = OTHER; note = 2'-fluorouridine-3'-phosphate
  modified_base 11: mod_base = OTHER; note = 2'-O-methylguanosine-3'-phosphate
  modified_base 12: mod_base = OTHER; note = 2'-fluorocytidine-3'-phosphate
  modified_base 13: mod_base = OTHER; note = 2'-O-methylcytidine-3'-phosphate
  modified_base 14: mod_base = OTHER; note = 2'-fluorouridine-3'-phosphate
  modified_base 15: mod_base = OTHER; note = 2'-O-methyladenosine-3'-phosphate
  modified_base 16: mod_base = OTHER; note = 2'-fluorocytidine-3'-phosphate
  modified_base 17: mod_base = OTHER; note = 2'-O-methyladenosine-3'-phosphate
  modified_base 18: mod_base = OTHER; note = 2'-fluoroguanosine-3'-phosphate
  modified_base 19: mod_base = OTHER; note = 2'-O-methylcytidine-3'-phosphate
  modified_base 20: mod_base = OTHER; note = 2'-O-methylcytidine-3'-phosphate
  modified_base 21: mod_base = OTHER; note = 2'-O-methyluridine-3'-phosphorothioate
  modified_base 22: mod_base = OTHER; note = 2'-O-methylcytidine-3'-phosphate
  misc_feature 1: note = RNA
  misc_feature 2: note = DNA
  misc_feature 3: note = RNA
  misc_feature 4: note = DNA
  misc_feature 5: note = RNA
  misc_feature 6: note = DNA
  misc_feature 7: note = RNA
  misc_feature 8: note = DNA
  misc_feature 9: note = RNA
  misc_feature 10: note = DNA
  misc_feature 11: note = RNA
  misc_feature 12: note = DNA
  misc_feature 13: note = RNA
  misc_feature 14: note = DNA
  misc_feature 15: note = RNA
  misc_feature 16: note = DNA
  misc_feature 17: note = RNA
  misc_feature 18: note = DNA
  misc_feature 19: note = RNA
  misc_feature 20: note = RNA
  misc_feature 21: note = RNA
  misc_feature 22: note = RNA
  source 1..22: mol_type = other RNA
accaatttatgcctacagcctc

SEQ ID NO: 134 - RNA, 21 nt, synthetic construct
  modified_base 1: mod_base = OTHER; note = 2'-O-methyluridine-3'-phosphorothioate
  modified_base 2: mod_base = OTHER; note = 2'-fluorocytidine-3'-phosphorothioate
  modified_base 3: mod_base = OTHER; note = 2'-O-methylcytidine-3'-phosphorothioate
  modified_base 4: mod_base = OTHER; note = 2'-fluoroadenosine-3'-phosphate
  modified_base 5: mod_base = OTHER; note = 2'-O-methyladenosine-3'-phosphate
  modified_base 6: mod_base = OTHER; note = 2'-fluorouridine-3'-phosphate
  modified_base 7: mod_base = OTHER; note = 2'-O-methyluridine-3'-phosphate
  modified_base 8: mod_base = OTHER; note = 2'-fluorouridine-3'-phosphate
  modified_base 9: mod_base = OTHER; note = 2'-O-methyladenosine-3'-phosphate
  modified_base 10: mod_base = OTHER; note = 2'-fluorouridine-3'-phosphate
  modified_base 11: mod_base = OTHER; note = 2'-O-methylguanosine-3'-phosphate
  modified_base 12: mod_base = OTHER; note = 2'-fluorocytidine-3'-phosphate
  modified_base 13: mod_base = OTHER; note = 2'-O-methylcytidine-3'-phosphate
  modified_base 14: mod_base = OTHER; note = 2'-fluorouridine-3'-phosphate
  modified_base 15: mod_base = OTHER; note = 2'-O-methyladenosine-3'-phosphate
  modified_base 16: mod_base = OTHER; note = 2'-fluorocytidine-3'-phosphate
  modified_base 17: mod_base = OTHER; note = 2'-O-methyladenosine-3'-phosphate
  modified_base 18: mod_base = OTHER; note = 2'-fluoroguanosine-3'-phosphate
  modified_base 19: mod_base = OTHER; note = 2'-O-methylcytidine-3'-phosphate
  modified_base 20: mod_base = OTHER; note = 2'-O-methyluridine-3'-phosphorothioate
  modified_base 21: mod_base = OTHER; note = 2'-O-methyluridine-3'-phosphate
  misc_feature 1: note = RNA
  misc_feature 2: note = DNA
  misc_feature 3: note = RNA
  misc_feature 4: note = DNA
  misc_feature 5: note = RNA
  misc_feature 6: note = DNA
  misc_feature 7: note = RNA
  misc_feature 8: note = DNA
  misc_feature 9: note = RNA
  misc_feature 10: note = DNA
  misc_feature 11: note = RNA
  misc_feature 12: note = DNA
  misc_feature 13: note = RNA
  misc_feature 14: note = DNA
  misc_feature 15: note = RNA
  misc_feature 16: note = DNA
  misc_feature 17: note = RNA
  misc_feature 18: note = DNA
  misc_feature 19: note = RNA
  misc_feature 20: note = RNA
  misc_feature 21: note = RNA
  source 1..21: mol_type = other RNA
tccaatttatgcctacagctt

SEQ ID NO: 135 - RNA, 22 nt, synthetic construct
  modified_base 1: mod_base = OTHER; note = 2'-O-methyluridine-3'-phosphorothioate
  modified_base 2: mod_base = OTHER; note = 2'-fluorocytidine-3'-phosphorothioate
  modified_base 3: mod_base = OTHER; note = 2'-O-methylcytidine-3'-phosphorothioate
  modified_base 4: mod_base = OTHER; note = 2'-fluoroadenosine-3'-phosphate
  modified_base 5: mod_base = OTHER; note = 2'-O-methyladenosine-3'-phosphate
  modified_base 6: mod_base = OTHER; note = 2'-fluorouridine-3'-phosphate
  modified_base 7: mod_base = OTHER; note = 2'-O-methyluridine-3'-phosphate
  modified_base 8: mod_base = OTHER; note = 2'-fluorouridine-3'-phosphate
  modified_base 9: mod_base = OTHER; note = 2'-O-methyladenosine-3'-phosphate
  modified_base 10: mod_base = OTHER; note = 2'-fluorouridine-3'-phosphate
  modified_base 11: mod_base = OTHER; note = 2'-O-methylguanosine-3'-phosphate
  modified_base 12: mod_base = OTHER; note = 2'-fluorocytidine-3'-phosphate
  modified_base 13: mod_base = OTHER; note = 2'-O-methylcytidine-3'-phosphate
  modified_base 14: mod_base = OTHER; note = 2'-fluorouridine-3'-phosphate
  modified_base 15: mod_base = OTHER; note = 2'-O-methyladenosine-3'-phosphate
  modified_base 16: mod_base = OTHER; note = 2'-fluorocytidine-3'-phosphate
  modified_base 17: mod_base = OTHER; note = 2'-O-methyladenosine-3'-phosphate
  modified_base 18: mod_base = OTHER; note = 2'-fluoroguanosine-3'-phosphate
  modified_base 19: mod_base = OTHER; note = 2'-O-methylcytidine-3'-phosphate
  modified_base 20: mod_base = OTHER; note = 2'-O-methylcytidine-3'-phosphate
  modified_base 21: mod_base = OTHER; note = 2'-O-methyluridine-3'-phosphorothioate
  modified_base 22: mod_base = OTHER; note = 2'-O-methyluridine-3'-phosphate
  misc_feature 1: note = RNA
  misc_feature 2: note = DNA
  misc_feature 3: note = RNA
  misc_feature 4: note = DNA
  misc_feature 5: note = RNA
  misc_feature 6: note = DNA
  misc_feature 7: note = RNA
  misc_feature 8: note = DNA
  misc_feature 9: note = RNA
  misc_feature 10: note = DNA
  misc_feature 11: note = RNA
  misc_feature 12: note = DNA
  misc_feature 13: note = RNA
  misc_feature 14: note = DNA
  misc_feature 15: note = RNA
  misc_feature 16: note = DNA
  misc_feature 17: note = RNA
  misc_feature 18: note = DNA
  misc_feature 19: note = RNA
  misc_feature 20: note = RNA
  misc_feature 21: note = RNA
  misc_feature 22: note = RNA
  source 1..22: mol_type = other RNA
tccaatttatgcctacagcctt

SEQ ID NO: 136 - RNA, 21 nt, synthetic construct
  modified_base 1: mod_base = OTHER; note = cyclopropyl phosphonate-2'-O-methyluridine-3'-phosphorothioate
  modified_base 2: mod_base = OTHER; note = 2'-fluoroadenosine-3'-phosporothioate
  modified_base 3: mod_base = OTHER; note = 2'-O-methylcytidine-3'-phosphorothioate
  modified_base 4: mod_base = OTHER; note = 2'-fluorocytidine-3'-phosphate
  modified_base 5: mod_base = OTHER; note = 2'-O-methyladenosine-3'-phosphate
  modified_base 6: mod_base = OTHER; note = 2'-fluoroadenosine-3'-phosphate
  modified_base 7: mod_base = OTHER; note = 2'-O-methyluridine-3'-phosphate
  modified_base 8: mod_base = OTHER; note = 2'-fluorouridine-3'-phosphate
  modified_base 9: mod_base = OTHER; note = 2'-O-methyluridine-3'-phosphate
  modified_base 10: mod_base = OTHER; note = 2'-fluoroadenosine-3'-phosphate
  modified_base 11: mod_base = OTHER; note = 2'-O-methyluridine-3'-phosphate
  modified_base 12: mod_base = OTHER; note = 2'-fluoroguanosine-3'-phosphate
  modified_base 13: mod_base = OTHER; note = 2'-O-methylcytidine-3'-phosphate
  modified_base 14: mod_base = OTHER; note = 2'-fluorocytidine-3'-phosphate
  modified_base 15: mod_base = OTHER; note = 2'-O-methyluridine-3'-phosphate
  modified_base 16: mod_base = OTHER; note = 2'-fluoroadenosine-3'-phosphate
  modified_base 17: mod_base = OTHER; note = 2'-O-methylcytidine-3'-phosphate
  modified_base 18: mod_base = OTHER; note = 2'-fluoroadenosine-3'-phosphate
  modified_base 19: mod_base = OTHER; note = 2'-O-methylguanosine-3'-phosphate
  modified_base 20: mod_base = OTHER; note = 2'-O-methylcytidine-3'-phosphorothioate
  modified_base 21: mod_base = OTHER; note = 2'-O-methylcytidine-3'-phosphate
  misc_feature 1: note = RNA
  misc_feature 2: note = DNA
  misc_feature 3: note = RNA
  misc_feature 4: note = DNA
  misc_feature 5: note = RNA
  misc_feature 6: note = DNA
  misc_feature 7: note = RNA
  misc_feature 8: note = DNA
  misc_feature 9: note = RNA
  misc_feature 10: note = DNA
  misc_feature 11: note = RNA
  misc_feature 12: note = DNA
  misc_feature 13: note = RNA
  misc_feature 14: note = DNA
  misc_feature 15: note = RNA
  misc_feature 16: note = DNA
  misc_feature 17: note = RNA
  misc_feature 18: note = DNA
  misc_feature 19: note = RNA
  misc_feature 20: note = RNA
  misc_feature 21: note = RNA
  source 1..21: mol_type = other RNA
taccaatttatgcctacagcc

SEQ ID NO: 137 - RNA, 21 nt, synthetic construct
  modified_base 1: mod_base = OTHER; note = 2'-O-methyluridine-3'-phosphorothioate
  modified_base 2: mod_base = OTHER; note = 2'-fluoroadenosine-3'-phosporothioate
  modified_base 3: mod_base = OTHER; note = 2'-O-methylcytidine-3'-phosphorothioate
  modified_base 4: mod_base = OTHER; note = 2'-fluorocytidine-3'-phosphate
  modified_base 5: mod_base = OTHER; note = 2'-O-methyladenosine-3'-phosphate
  modified_base 6: mod_base = OTHER; note = 2'-fluoroadenosine-3'-phosphate
  modified_base 7: mod_base = OTHER; note = 2'-O-methyluridine-3'-phosphate
  modified_base 8: mod_base = OTHER; note = 2'-fluorouridine-3'-phosphate
  modified_base 9: mod_base = OTHER; note = 2'-O-methyluridine-3'-phosphate
  modified_base 10: mod_base = OTHER; note = 2'-fluoroadenosine-3'-phosphate
  modified_base 11: mod_base = OTHER; note = 2'-O-methyluridine-3'-phosphate
  modified_base 12: mod_base = OTHER; note = 2'-fluoroguanosine-3'-phosphate
  modified_base 13: mod_base = OTHER; note = 2'-O-methylcytidine-3'-phosphate
  modified_base 14: mod_base = OTHER; note = 2'-fluorocytidine-3'-phosphate
  modified_base 15: mod_base = OTHER; note = 2'-O-methyluridine-3'-phosphate
  modified_base 16: mod_base = OTHER; note = 2'-fluoroadenosine-3'-phosphate
  modified_base 17: mod_base = OTHER; note = 2'-O-methylcytidine-3'-phosphate
  modified_base 18: mod_base = OTHER; note = 2'-fluoroadenosine-3'-phosphate
  modified_base 19: mod_base = OTHER; note = 2'-O-methylguanosine-3'-phosphorothioate
  modified_base 20: mod_base = OTHER; note = 2'-O-methylcytidine-3'-phosphorothioate
  modified_base 21: mod_base = OTHER; note = 2'-O-methylcytidine-3'-phosphate
  misc_feature 1: note = RNA
  misc_feature 2: note = DNA
  misc_feature 3: note = RNA
  misc_feature 4: note = DNA
  misc_feature 5: note = RNA
  misc_feature 6: note = DNA
  misc_feature 7: note = RNA
  misc_feature 8: note = DNA
  misc_feature 9: note = RNA
  misc_feature 10: note = DNA
  misc_feature 11: note = RNA
  misc_feature 12: note = DNA
  misc_feature 13: note = RNA
  misc_feature 14: note = DNA
  misc_feature 15: note = RNA
  misc_feature 16: note = DNA
  misc_feature 17: note = RNA
  misc_feature 18: note = DNA
  misc_feature 19: note = RNA
  misc_feature 20: note = RNA
  misc_feature 21: note = RNA
  source 1..21: mol_type = other RNA
taccaatttatgcctacagcc

SEQ ID NO: 138 - RNA, 21 nt, synthetic construct
  modified_base 1: mod_base = OTHER; note = cyclopropyl phosphonate-2'-O-methyluridine-3'-phosphorothioate
  modified_base 2: mod_base = OTHER; note = 2'-fluoroadenosine-3'-phosporothioate
  modified_base 3: mod_base = OTHER; note = 2'-O-methylcytidine-3'-phosphorothioate
  modified_base 4: mod_base = OTHER; note = 2'-fluorocytidine-3'-phosphate
  modified_base 5: mod_base = OTHER; note = 2'-O-methyladenosine-3'-phosphate
  modified_base 6: mod_base = OTHER; note = 2'-fluoroadenosine-3'-phosphate
  modified_base 7: mod_base = OTHER; note = 2'-O-methyluridine-3'-phosphate
  modified_base 8: mod_base = OTHER; note = 2'-fluorouridine-3'-phosphate
  modified_base 9: mod_base = OTHER; note = 2'-O-methyluridine-3'-phosphate
  modified_base 10: mod_base = OTHER; note = 2'-fluoroadenosine-3'-phosphate
  modified_base 11: mod_base = OTHER; note = 2'-O-methyluridine-3'-phosphate
  modified_base 12: mod_base = OTHER; note = 2'-fluoroguanosine-3'-phosphate
  modified_base 13: mod_base = OTHER; note = 2'-O-methylcytidine-3'-phosphate
  modified_base 14: mod_base = OTHER; note = 2'-fluorocytidine-3'-phosphate
  modified_base 15: mod_base = OTHER; note = 2'-O-methyluridine-3'-phosphate
  modified_base 16: mod_base = OTHER; note = 2'-fluoroadenosine-3'-phosphate
  modified_base 17: mod_base = OTHER; note = 2'-O-methylcytidine-3'-phosphate
  modified_base 18: mod_base = OTHER; note = 2'-fluoroadenosine-3'-phosphate
  modified_base 19: mod_base = OTHER; note = 2'-O-methylguanosine-3'-phosphorothioate
  modified_base 20: mod_base = OTHER; note = 2'-O-methylcytidine-3'-phosphorothioate
  modified_base 21: mod_base = OTHER; note = 2'-O-methylcytidine-3'-phosphate
  misc_feature 1: note = RNA
  misc_feature 2: note = DNA
  misc_feature 3: note = RNA
  misc_feature 4: note = DNA
  misc_feature 5: note = RNA
  misc_feature 6: note = DNA
  misc_feature 7: note = RNA
  misc_feature 8: note = DNA
  misc_feature 9: note = RNA
  misc_feature 10: note = DNA
  misc_feature 11: note = RNA
  misc_feature 12: note = DNA
  misc_feature 13: note = RNA
  misc_feature 14: note = DNA
  misc_feature 15: note = RNA
  misc_feature 16: note = DNA
  misc_feature 17: note = RNA
  misc_feature 18: note = DNA
  misc_feature 19: note = RNA
  misc_feature 20: note = RNA
  misc_feature 21: note = RNA
  source 1..21: mol_type = other RNA
taccaatttatgcctacagcc

SEQ ID NO: 139 - RNA, 21 nt, synthetic construct
  modified_base 1: mod_base = OTHER; note = 2'-O-methyluridine-3'-phosphorothioate
  modified_base 2: mod_base = OTHER; note = 2'-fluoroadenosine-3'-phosporothioate
  modified_base 3: mod_base = OTHER; note = 2'-O-methylcytidine-3'-phosphorothioate
  modified_base 4: mod_base = OTHER; note = 2'-fluorocytidine-3'-phosphate
  modified_base 5: mod_base = OTHER; note = 2'-O-methyladenosine-3'-phosphate
  modified_base 6: mod_base = OTHER; note = 2'-fluoroadenosine-3'-phosphate
  modified_base 7: mod_base = OTHER; note = 2'-O-methyluridine-3'-phosphate
  modified_base 8: mod_base = OTHER; note = 2'-fluorouridine-3'-phosphate
  modified_base 9: mod_base = OTHER; note = 2'-O-methyluridine-3'-phosphate
  modified_base 10: mod_base = OTHER; note = 2'-fluoroadenosine-3'-phosphate
  modified_base 11: mod_base = OTHER; note = 2'-O-methyluridine-3'-phosphate
  modified_base 12: mod_base = OTHER; note = 2'-fluoroguanosine-3'-phosphate
  modified_base 13: mod_base = OTHER; note = 2'-O-methylcytidine-3'-phosphate
  modified_base 14: mod_base = OTHER; note = 2'-fluorocytidine-3'-phosphate
  modified_base 15: mod_base = OTHER; note = 2'-O-methyluridine-3'-phosphate
  modified_base 16: mod_base = OTHER; note = 2'-fluoroadenosine-3'-phosphate
  modified_base 17: mod_base = OTHER; note = 2'-O-methylcytidine-3'-phosphate
  modified_base 18: mod_base = OTHER; note = 2'-fluoroadenosine-3'-phosphate
  modified_base 19: mod_base = OTHER; note = 2'-O-methylguanosine-3'-phosphate
  modified_base 20: mod_base = OTHER; note = 2'-O-methylcytidine-3'-phosphorothioate
  modified_base 21: mod_base = OTHER; note = 2'-O-methyluridine-3'-phosphate
  misc_feature 1: note = RNA
  misc_feature 2: note = DNA
  misc_feature 3: note = RNA
  misc_feature 4: note = DNA
  misc_feature 5: note = RNA
  misc_feature 6: note = DNA
  misc_feature 7: note = RNA
  misc_feature 8: note = DNA
  misc_feature 9: note = RNA
  misc_feature 10: note = DNA
  misc_feature 11: note = RNA
  misc_feature 12: note = DNA
  misc_feature 13: note = RNA
  misc_feature 14: note = DNA
  misc_feature 15: note = RNA
  misc_feature 16: note = DNA
  misc_feature 17: note = RNA
  misc_feature 18: note = DNA
  misc_feature 19: note = RNA
  misc_feature 20: note = RNA
  misc_feature 21: note = RNA
  source 1..21: mol_type = other RNA
taccaatttatgcctacagct

SEQ ID NO: 140 - RNA, 21 nt, synthetic construct
  modified_base 1: mod_base = OTHER; note = 2'-O-methyluridine-3'-phosphorothioate
  modified_base 2: mod_base = OTHER; note = 2'-fluoroadenosine-3'-phosporothioate
  modified_base 3: mod_base = OTHER; note = 2'-O-methylcytidine-3'-phosphorothioate
  modified_base 4: mod_base = OTHER; note = 2'-fluorocytidine-3'-phosphate
  modified_base 5: mod_base = OTHER; note = 2'-O-methyladenosine-3'-phosphate
  modified_base 6: mod_base = OTHER; note = 2'-fluoroadenosine-3'-phosphate
  modified_base 7: mod_base = OTHER; note = 2'-O-methyluridine-3'-phosphate
  modified_base 8: mod_base = OTHER; note = 2'-fluorouridine-3'-phosphate
  modified_base 9: mod_base = OTHER; note = 2'-O-methyluridine-3'-phosphate
  modified_base 10: mod_base = OTHER; note = 2'-fluoroadenosine-3'-phosphate
  modified_base 11: mod_base = OTHER; note = 2'-O-methyluridine-3'-phosphate
  modified_base 12: mod_base = OTHER; note = 2'-fluoroguanosine-3'-phosphate
  modified_base 13: mod_base = OTHER; note = 2'-O-methylcytidine-3'-phosphate
  modified_base 14: mod_base = OTHER; note = 2'-fluorocytidine-3'-phosphate
  modified_base 15: mod_base = OTHER; note = 2'-O-methyluridine-3'-phosphate
  modified_base 16: mod_base = OTHER; note = 2'-fluoroadenosine-3'-phosphate
  modified_base 17: mod_base = OTHER; note = 2'-O-methylcytidine-3'-phosphate
  modified_base 18: mod_base = OTHER; note = 2'-fluoroadenosine-3'-phosphate
  modified_base 19: mod_base = OTHER; note = 2'-O-methylguanosine-3'-phosphate
  modified_base 20: mod_base = OTHER; note = 2'-O-methylcytidine-3'-phosphorothioate
  modified_base 21: mod_base = OTHER; note = 2'-O-methylguanosine-3'-phosphate
  misc_feature 1: note = RNA
  misc_feature 2: note = DNA
  misc_feature 3: note = RNA
  misc_feature 4: note = DNA
  misc_feature 5: note = RNA
  misc_feature 6: note = DNA
  misc_feature 7: note = RNA
  misc_feature 8: note = DNA
  misc_feature 9: note = RNA
  misc_feature 10: note = DNA
  misc_feature 11: note = RNA
  misc_feature 12: note = DNA
  misc_feature 13: note = RNA
  misc_feature 14: note = DNA
  misc_feature 15: note = RNA
  misc_feature 16: note = DNA
  misc_feature 17: note = RNA
  misc_feature 18: note = DNA
  misc_feature 19: note = RNA
  misc_feature 20: note = RNA
  misc_feature 21: note = RNA
  source 1..21: mol_type = other RNA
taccaatttatgcctacagcg

SEQ ID NO: 141 - RNA, 21 nt, synthetic construct
  modified_base 1: mod_base = OTHER; note = 2'-O-methyladenosine-3'-phosphorothioate
  modified_base 2: mod_base = OTHER; note = 2'-fluoroadenosine-3'-phosporothioate
  modified_base 3: mod_base = OTHER; note = 2'-O-methylcytidine-3'-phosphorothioate
  modified_base 4: mod_base = OTHER; note = 2'-fluorocytidine-3'-phosphate
  modified_base 5: mod_base = OTHER; note = 2'-O-methyladenosine-3'-phosphate
  modified_base 6: mod_base = OTHER; note = 2'-fluoroadenosine-3'-phosphate
  modified_base 7: mod_base = OTHER; note = 2'-O-methyluridine-3'-phosphate
  modified_base 8: mod_base = OTHER; note = 2'-fluorouridine-3'-phosphate
  modified_base 9: mod_base = OTHER; note = 2'-O-methyluridine-3'-phosphate
  modified_base 10: mod_base = OTHER; note = 2'-fluoroadenosine-3'-phosphate
  modified_base 11: mod_base = OTHER; note = 2'-O-methyluridine-3'-phosphate
  modified_base 12: mod_base = OTHER; note = 2'-fluoroguanosine-3'-phosphate
  modified_base 13: mod_base = OTHER; note = 2'-O-methylcytidine-3'-phosphate
  modified_base 14: mod_base = OTHER; note = 2'-fluorocytidine-3'-phosphate
  modified_base 15: mod_base = OTHER; note = 2'-O-methyluridine-3'-phosphate
  modified_base 16: mod_base = OTHER; note = 2'-fluoroadenosine-3'-phosphate
  modified_base 17: mod_base = OTHER; note = 2'-O-methylcytidine-3'-phosphate
  modified_base 18: mod_base = OTHER; note = 2'-fluoroadenosine-3'-phosphate
  modified_base 19: mod_base = OTHER; note = 2'-O-methylguanosine-3'-phosphate
  modified_base 20: mod_base = OTHER; note = 2'-O-methylcytidine-3'-phosphorothioate
  modified_base 21: mod_base = OTHER; note = 2'-O-methylcytidine-3'-phosphate
  misc_feature 1: note = RNA
  misc_feature 2: note = DNA
  misc_feature 3: note = RNA
  misc_feature 4: note = DNA
  misc_feature 5: note = RNA
  misc_feature 6: note = DNA
  misc_feature 7: note = RNA
  misc_feature 8: note = DNA
  misc_feature 9: note = RNA
  misc_feature 10: note = DNA
  misc_feature 11: note = RNA
  misc_feature 12: note = DNA
  misc_feature 13: note = RNA
  misc_feature 14: note = DNA
  misc_feature 15: note = RNA
  misc_feature 16: note = DNA
  misc_feature 17: note = RNA
  misc_feature 18: note = DNA
  misc_feature 19: note = RNA
  misc_feature 20: note = RNA
  misc_feature 21: note = RNA
  source 1..21: mol_type = other RNA
aaccaatttatgcctacagcc

SEQ ID NO: 142 - RNA, 21 nt, synthetic construct
  modified_base 1: mod_base = OTHER; note = 2'-O-methyluridine-3'-phosphorothioate
  modified_base 2: mod_base = OTHER; note = 2'-fluoroadenosine-3'-phosporothioate
  modified_base 3: mod_base = OTHER; note = 2'-O-methylcytidine-3'-phosphorothioate
  modified_base 4: mod_base = OTHER; note = 2'-fluorocytidine-3'-phosphate
  modified_base 5: mod_base = OTHER; note = 2'-O-methyladenosine-3'-phosphate
  modified_base 6: mod_base = OTHER; note = 2'-fluoroadenosine-3'-phosphate
  modified_base 7: mod_base = OTHER; note = 2'-O-methyluridine-3'-phosphate
  modified_base 8: mod_base = OTHER; note = 2'-fluorouridine-3'-phosphate
  modified_base 9: mod_base = OTHER; note = 2'-fluorouridine-3'-phosphate
  modified_base 10: mod_base = OTHER; note = 2'-fluoroadenosine-3'-phosphate
  modified_base 11: mod_base = OTHER; note = 2'-O-methyluridine-3'-phosphate
  modified_base 12: mod_base = OTHER; note = 2'-fluoroguanosine-3'-phosphate
  modified_base 13: mod_base = OTHER; note = 2'-O-methylcytidine-3'-phosphate
  modified_base 14: mod_base = OTHER; note = 2'-fluorocytidine-3'-phosphate
  modified_base 15: mod_base = OTHER; note = 2'-O-methyluridine-3'-phosphate
  modified_base 16: mod_base = OTHER; note = 2'-fluoroadenosine-3'-phosphate
  modified_base 17: mod_base = OTHER; note = 2'-O-methylcytidine-3'-phosphate
  modified_base 18: mod_base = OTHER; note = 2'-fluoroadenosine-3'-phosphate
  modified_base 19: mod_base = OTHER; note = 2'-O-methylguanosine-3'-phosphate
  modified_base 20: mod_base = OTHER; note = 2'-O-methyluridine-3'-phosphorothioate
  modified_base 21: mod_base = OTHER; note = 2'-O-methyluridine-3'-phosphate
  misc_feature 1: note = RNA
  misc_feature 2: note = DNA
  misc_feature 3: note = RNA
  misc_feature 4: note = DNA
  misc_feature 5: note = RNA
  misc_feature 6: note = DNA
  misc_feature 7: note = RNA
  misc_feature 8: note = DNA
  misc_feature 9: note = DNA
  misc_feature 10: note = DNA
  misc_feature 11: note = RNA
  misc_feature 12: note = DNA
  misc_feature 13: note = RNA
  misc_feature 14: note = DNA
  misc_feature 15: note = RNA
  misc_feature 16: note = DNA
  misc_feature 17: note = RNA
  misc_feature 18: note = DNA
  misc_feature 19: note = RNA
  misc_feature 20: note = RNA
  misc_feature 21: note = RNA
  source 1..21: mol_type = other RNA
taccaatttatgcctacagtt

SEQ ID NO: 143 - RNA, 21 nt, synthetic construct
  modified_base 1: mod_base = OTHER; note = 2'-O-methyluridine-3'-phosphorothioate
  modified_base 2: mod_base = OTHER; note = 2'-fluoroadenosine-3'-phosporothioate
  modified_base 3: mod_base = OTHER; note = 2'-O-methylcytidine-3'-phosphorothioate
  modified_base 4: mod_base = OTHER; note = 2'-fluorocytidine-3'-phosphate
  modified_base 5: mod_base = OTHER; note = 2'-O-methyladenosine-3'-phosphate
  modified_base 6: mod_base = OTHER; note = 2'-fluoroadenosine-3'-phosphate
  modified_base 7: mod_base = OTHER; note = 2'-O-methyluridine-3'-phosphate
  modified_base 8: mod_base = OTHER; note = 2'-fluorouridine-3'-phosphate
  modified_base 9: mod_base = OTHER; note = 2'-O-methyluridine-3'-phosphate
  modified_base 10: mod_base = OTHER; note = 2'-fluoroadenosine-3'-phosphate
  modified_base 11: mod_base = OTHER; note = 2'-O-methyluridine-3'-phosphate
  modified_base 12: mod_base = OTHER; note = 2'-fluoroguanosine-3'-phosphate
  modified_base 13: mod_base = OTHER; note = 2'-O-methylcytidine-3'-phosphate
  modified_base 14: mod_base = OTHER; note = 2'-fluorocytidine-3'-phosphate
  modified_base 15: mod_base = OTHER; note = 2'-O-methyluridine-3'-phosphate
  modified_base 16: mod_base = OTHER; note = 2'-fluoroadenosine-3'-phosphate
  modified_base 17: mod_base = OTHER; note = 2'-O-methylcytidine-3'-phosphate
  modified_base 18: mod_base = OTHER; note = 2'-fluoroadenosine-3'-phosphate
  modified_base 19: mod_base = OTHER; note = 2'-O-methylguanosine-3'-phosphate
  modified_base 20: mod_base = OTHER; note = 2'-fluorocytidine-3'-phosphorothioate
  modified_base 21: mod_base = OTHER; note = 2'-O-methylcytidine-3'-phosphate
  misc_feature 1: note = RNA
  misc_feature 2: note = DNA
  misc_feature 3: note = RNA
  misc_feature 4: note = DNA
  misc_feature 5: note = RNA
  misc_feature 6: note = DNA
  misc_feature 7: note = RNA
  misc_feature 8: note = DNA
  misc_feature 9: note = RNA
  misc_feature 10: note = DNA
  misc_feature 11: note = RNA
  misc_feature 12: note = DNA
  misc_feature 13: note = RNA
  misc_feature 14: note = DNA
  misc_feature 15: note = RNA
  misc_feature 16: note = DNA
  misc_feature 17: note = RNA
  misc_feature 18: note = DNA
  misc_feature 19: note = RNA
  misc_feature 20: note = DNA
  misc_feature 21: note = RNA
  source 1..21: mol_type = other RNA
taccaatttatgcctacagcc

SEQ ID NO: 144 - RNA, 21 nt, synthetic construct
  modified_base 1: mod_base = OTHER; note = 2'-O-methyladenosine-3'-phosphorothioate
  modified_base 2: mod_base = OTHER; note = 2'-fluorocytidine-3'-phosphorothioate
  modified_base 3: mod_base = OTHER; note = 2'-O-methylcytidine-3'-phosphate
  modified_base 4: mod_base = OTHER; note = 2'-fluoroadenosine-3'-phosphate
  modified_base 5: mod_base = OTHER; note = 2'-O-methyladenosine-3'-phosphate
  modified_base 6: mod_base = OTHER; note = 2'-fluorouridine-3'-phosphate
  modified_base 7: mod_base = OTHER; note = 2'-O-methyluridine-3'-phosphate
  modified_base 8: mod_base = OTHER; note = 2'-fluorouridine-3'-phosphate
  modified_base 9: mod_base = OTHER; note = 2'-O-methyladenosine-3'-phosphate
  modified_base 10: mod_base = OTHER; note = 2'-fluorouridine-3'-phosphate
  modified_base 11: mod_base = OTHER; note = 2'-O-methylguanosine-3'-phosphate
  modified_base 12: mod_base = OTHER; note = 2'-fluorocytidine-3'-phosphate
  modified_base 13: mod_base = OTHER; note = 2'-O-methylcytidine-3'-phosphate
  modified_base 14: mod_base = OTHER; note = 2'-fluorouridine-3'-phosphate
  modified_base 15: mod_base = OTHER; note = 2'-O-methyladenosine-3'-phosphate
  modified_base 16: mod_base = OTHER; note = 2'-fluorocytidine-3'-phosphate
  modified_base 17: mod_base = OTHER; note = 2'-O-methyladenosine-3'-phosphate
  modified_base 18: mod_base = OTHER; note = 2'-fluoroguanosine-3'-phosphate
  modified_base 19: mod_base = OTHER; note = 2'-O-methylcytidine-3'-phosphate
  modified_base 20: mod_base = OTHER; note = 2'-fluorocytidine-3'-phosphorothioate
  modified_base 21: mod_base = OTHER; note = 2'-O-methyluridine-3'-phosphate
  misc_feature 1: note = RNA
  misc_feature 2: note = DNA
  misc_feature 3: note = RNA
  misc_feature 4: note = DNA
  misc_feature 5: note = RNA
  misc_feature 6: note = DNA
  misc_feature 7: note = RNA
  misc_feature 8: note = DNA
  misc_feature 9: note = RNA
  misc_feature 10: note = DNA
  misc_feature 11: note = RNA
  misc_feature 12: note = DNA
  misc_feature 13: note = RNA
  misc_feature 14: note = DNA
  misc_feature 15: note = RNA
  misc_feature 16: note = DNA
  misc_feature 17: note = RNA
  misc_feature 18: note = DNA
  misc_feature 19: note = RNA
  misc_feature 20: note = DNA
  misc_feature 21: note = RNA
  source 1..21: mol_type = other RNA
accaatttatgcctacagcct

SEQ ID NO: 145 - RNA, 21 nt, synthetic construct
  modified_base 1: mod_base = OTHER; note = 2'-O-methyluridine-3'-phosphorothioate
  modified_base 2: mod_base = OTHER; note = 2'-fluorocytidine-3'-phosphorothioate
  modified_base 3: mod_base = OTHER; note = 2'-O-methylcytidine-3'-phosphate
  modified_base 4: mod_base = OTHER; note = 2'-fluoroadenosine-3'-phosphate
  modified_base 5: mod_base = OTHER; note = 2'-O-methyladenosine-3'-phosphate
  modified_base 6: mod_base = OTHER; note = 2'-fluorouridine-3'-phosphate
  modified_base 7: mod_base = OTHER; note = 2'-O-methyluridine-3'-phosphate
  modified_base 8: mod_base = OTHER; note = 2'-fluorouridine-3'-phosphate
  modified_base 9: mod_base = OTHER; note = 2'-O-methyladenosine-3'-phosphate
  modified_base 10: mod_base = OTHER; note = 2'-fluorouridine-3'-phosphate
  modified_base 11: mod_base = OTHER; note = 2'-O-methylguanosine-3'-phosphate
  modified_base 12: mod_base = OTHER; note = 2'-fluorocytidine-3'-phosphate
  modified_base 13: mod_base = OTHER; note = 2'-O-methylcytidine-3'-phosphate
  modified_base 14: mod_base = OTHER; note = 2'-fluorouridine-3'-phosphate
  modified_base 15: mod_base = OTHER; note = 2'-O-methyladenosine-3'-phosphate
  modified_base 16: mod_base = OTHER; note = 2'-fluorocytidine-3'-phosphate
  modified_base 17: mod_base = OTHER; note = 2'-O-methyladenosine-3'-phosphate
  modified_base 18: mod_base = OTHER; note = 2'-fluoroguanosine-3'-phosphate
  modified_base 19: mod_base = OTHER; note = 2'-O-methylcytidine-3'-phosphate
  modified_base 20: mod_base = OTHER; note = 2'-fluorocytidine-3'-phosphorothioate
  modified_base 21: mod_base = OTHER; note = 2'-O-methyluridine-3'-phosphate
  misc_feature 1: note = RNA
  misc_feature 2: note = DNA
  misc_feature 3: note = RNA
  misc_feature 4: note = DNA
  misc_feature 5: note = RNA
  misc_feature 6: note = DNA
  misc_feature 7: note = RNA
  misc_feature 8: note = DNA
  misc_feature 9: note = RNA
  misc_feature 10: note = DNA
  misc_feature 11: note = RNA
  misc_feature 12: note = DNA
  misc_feature 13: note = RNA
  misc_feature 14: note = DNA
  misc_feature 15: note = RNA
  misc_feature 16: note = DNA
  misc_feature 17: note = RNA
  misc_feature 18: note = DNA
  misc_feature 19: note = RNA
  misc_feature 20: note = DNA
  misc_feature 21: note = RNA
  source 1..21: mol_type = other RNA
tccaatttatgcctacagcct

SEQ ID NO: 146 - RNA, 21 nt, synthetic construct
  modified_base 1: mod_base = OTHER; note = 2'-O-methyladenosine-3'-phosphorothioate
  modified_base 2: mod_base = OTHER; note = 2'-fluorocytidine-3'-phosphorothioate
  modified_base 3: mod_base = OTHER; note = 2'-O-methylcytidine-3'-phosphate
  modified_base 4: mod_base = OTHER; note = 2'-fluoroadenosine-3'-phosphate
  modified_base 5: mod_base = OTHER; note = 2'-O-methyladenosine-3'-phosphate
  modified_base 6: mod_base = OTHER; note = 2'-fluorouridine-3'-phosphate
  modified_base 7: mod_base = OTHER; note = 2'-O-methyluridine-3'-phosphate
  modified_base 8: mod_base = OTHER; note = 2'-fluorouridine-3'-phosphate
  modified_base 9: mod_base = OTHER; note = 2'-O-methyladenosine-3'-phosphate
  modified_base 10: mod_base = OTHER; note = 2'-fluorouridine-3'-phosphate
  modified_base 11: mod_base = OTHER; note = 2'-O-methylguanosine-3'-phosphate
  modified_base 12: mod_base = OTHER; note = 2'-fluorocytidine-3'-phosphate
  modified_base 13: mod_base = OTHER; note = 2'-O-methylcytidine-3'-phosphate
  modified_base 14: mod_base = OTHER; note = 2'-fluorouridine-3'-phosphate
  modified_base 15: mod_base = OTHER; note = 2'-O-methyladenosine-3'-phosphate
  modified_base 16: mod_base = OTHER; note = 2'-fluorocytidine-3'-phosphate
  modified_base 17: mod_base = OTHER; note = 2'-O-methyladenosine-3'-phosphate
  modified_base 18: mod_base = OTHER; note = 2'-fluoroguanosine-3'-phosphate
  modified_base 19: mod_base = OTHER; note = 2'-O-methylcytidine-3'-phosphate
  modified_base 20: mod_base = OTHER; note = 2'-O-methylcytidine-3'-phosphorothioate
  modified_base 21: mod_base = OTHER; note = 2'-O-methylguanosine-3'-phosphate
  misc_feature 1: note = RNA
  misc_feature 2: note = DNA
  misc_feature 3: note = RNA
  misc_feature 4: note = DNA
  misc_feature 5: note = RNA
  misc_feature 6: note = DNA
  misc_feature 7: note = RNA
  misc_feature 8: note = DNA
  misc_feature 9: note = RNA
  misc_feature 10: note = DNA
  misc_feature 11: note = RNA
  misc_feature 12: note = DNA
  misc_feature 13: note = RNA
  misc_feature 14: note = DNA
  misc_feature 15: note = RNA
  misc_feature 16: note = DNA
  misc_feature 17: note = RNA
  misc_feature 18: note = DNA
  misc_feature 19: note = RNA
  misc_feature 20: note = RNA
  misc_feature 21: note = RNA
  source 1..21: mol_type = other RNA
accaatttatgcctacagccg

SEQ ID NO: 147 - RNA, 21 nt, synthetic construct
  modified_base 1: mod_base = OTHER; note = 2'-O-methyluridine-3'-phosphorothioate
  modified_base 2: mod_base = OTHER; note = 2'-fluorocytidine-3'-phosphorothioate
  modified_base 3: mod_base = OTHER; note = 2'-O-methylcytidine-3'-phosphate
  modified_base 4: mod_base = OTHER; note = 2'-fluoroadenosine-3'-phosphate
  modified_base 5: mod_base = OTHER; note = 2'-O-methyladenosine-3'-phosphate
  modified_base 6: mod_base = OTHER; note = 2'-fluorouridine-3'-phosphate
  modified_base 7: mod_base = OTHER; note = 2'-O-methyluridine-3'-phosphate
  modified_base 8: mod_base = OTHER; note = 2'-fluorouridine-3'-phosphate
  modified_base 9: mod_base = OTHER; note = 2'-O-methyladenosine-3'-phosphate
  modified_base 10: mod_base = OTHER; note = 2'-fluorouridine-3'-phosphate
  modified_base 11: mod_base = OTHER; note = 2'-O-methylguanosine-3'-phosphate
  modified_base 12: mod_base = OTHER; note = 2'-fluorocytidine-3'-phosphate
  modified_base 13: mod_base = OTHER; note = 2'-O-methylcytidine-3'-phosphate
  modified_base 14: mod_base = OTHER; note = 2'-fluorouridine-3'-phosphate
  modified_base 15: mod_base = OTHER; note = 2'-O-methyladenosine-3'-phosphate
  modified_base 16: mod_base = OTHER; note = 2'-fluorocytidine-3'-phosphate
  modified_base 17: mod_base = OTHER; note = 2'-O-methyladenosine-3'-phosphate
  modified_base 18: mod_base = OTHER; note = 2'-fluoroguanosine-3'-phosphate
  modified_base 19: mod_base = OTHER; note = 2'-O-methylcytidine-3'-phosphate
  modified_base 20: mod_base = OTHER; note = 2'-O-methylcytidine-3'-phosphorothioate
  modified_base 21: mod_base = OTHER; note = 2'-O-methylguanosine-3'-phosphate
  misc_feature 1: note = RNA
  misc_feature 2: note = DNA
  misc_feature 3: note = RNA
  misc_feature 4: note = DNA
  misc_feature 5: note = RNA
  misc_feature 6: note = DNA
  misc_feature 7: note = RNA
  misc_feature 8: note = DNA
  misc_feature 9: note = RNA
  misc_feature 10: note = DNA
  misc_feature 11: note = RNA
  misc_feature 12: note = DNA
  misc_feature 13: note = RNA
  misc_feature 14: note = DNA
  misc_feature 15: note = RNA
  misc_feature 16: note = DNA
  misc_feature 17: note = RNA
  misc_feature 18: note = DNA
  misc_feature 19: note = RNA
  misc_feature 20: note = RNA
  misc_feature 21: note = RNA
  source 1..21: mol_type = other RNA
tccaatttatgcctacagccg

SEQ ID NO: 148 - RNA, 21 nt, synthetic construct
  modified_base 1: mod_base = OTHER; note = 2'-O-methyluridine-3'-phosphorothioate
  modified_base 2: mod_base = OTHER; note = 2'-fluoroadenosine-3'-phosporothioate
  modified_base 3: mod_base = OTHER; note = 2'-O-methylcytidine-3'-phosphorothioate
  modified_base 4: mod_base = OTHER; note = 2'-fluorocytidine-3'-phosphate
  modified_base 5: mod_base = OTHER; note = 2'-O-methyladenosine-3'-phosphate
  modified_base 6: mod_base = OTHER; note = 2'-fluoroadenosine-3'-phosphate
  modified_base 7: mod_base = OTHER; note = 2'-O-methyluridine-3'-phosphate
  modified_base 8: mod_base = OTHER; note = 2'-fluorouridine-3'-phosphate
  modified_base 9: mod_base = OTHER; note = 2'-O-methyluridine-3'-phosphate
  modified_base 10: mod_base = OTHER; note = 2'-fluoroadenosine-3'-phosphate
  modified_base 11: mod_base = OTHER; note = 2'-O-methyluridine-3'-phosphate
  modified_base 12: mod_base = OTHER; note = 2'-fluoroguanosine-3'-phosphate
  modified_base 13: mod_base = OTHER; note = 2'-O-methylcytidine-3'-phosphate
  modified_base 14: mod_base = OTHER; note = 2'-fluorocytidine-3'-phosphate
  modified_base 15: mod_base = OTHER; note = 2'-O-methyluridine-3'-phosphate
  modified_base 16: mod_base = OTHER; note = 2'-fluoroadenosine-3'-phosphate
  modified_base 17: mod_base = OTHER; note = 2'-O-methylcytidine-3'-phosphate
  modified_base 18: mod_base = OTHER; note = 2'-fluoroadenosine-3'-phosphate
  modified_base 19: mod_base = OTHER; note = 2'-O-methylguanosine-3'-phosphate
  modified_base 20: mod_base = OTHER; note = 2'-O-methylguanosine-3'-phosphorothioate
  modified_base 21: mod_base = OTHER; note = 2'-O-methylguanosine-3'-phosphate
  misc_feature 1: note = RNA
  misc_feature 2: note = DNA
  misc_feature 3: note = RNA
  misc_feature 4: note = DNA
  misc_feature 5: note = RNA
  misc_feature 6: note = DNA
  misc_feature 7: note = RNA
  misc_feature 8: note = DNA
  misc_feature 9: note = RNA
  misc_feature 10: note = DNA
  misc_feature 11: note = RNA
  misc_feature 12: note = DNA
  misc_feature 13: note = RNA
  misc_feature 14: note = DNA
  misc_feature 15: note = RNA
  misc_feature 16: note = DNA
  misc_feature 17: note = RNA
  misc_feature 18: note = DNA
  misc_feature 19: note = RNA
  misc_feature 20: note = RNA
  misc_feature 21: note = RNA
  source 1..21: mol_type = other RNA
taccaatttatgcctacaggg

SEQ ID NO: 149 - RNA, 26 nt, synthetic construct
  source 1..26: mol_type = other RNA
taccaatttatgcctacaggccttat

SEQ ID NO: 150 - RNA, 23 nt, synthetic construct
  source 1..23: mol_type = other RNA
taccaatttatgcctacaggcct

SEQ ID NO: 151 - RNA, 21 nt, synthetic construct
  source 1..21: mol_type = other RNA
taccaatttatgcctacaggc

SEQ ID NO: 152 - RNA, 21 nt, synthetic construct
  source 1..21: mol_type = other RNA
tgtgaagcgaagtgcacactt

SEQ ID NO: 153 - RNA, 26 nt, synthetic construct
  source 1..26: mol_type = other RNA
taccaatttatgcctacagcctccgc

SEQ ID NO: 154 - RNA, 21 nt, synthetic construct
  source 1..21: mol_type = other RNA
taccaatttatgcctacagtt

SEQ ID NO: 155 - RNA, 21 nt, synthetic construct
  source 1..21: mol_type = other RNA
attgagagaagtccaccacga

SEQ ID NO: 156 - RNA, 21 nt, synthetic construct
  source 1..21: mol_type = other RNA
attgagagaagtccaccactt

SEQ ID NO: 157 - RNA, 21 nt, synthetic construct
  source 1..21: mol_type = other RNA
tttgagagaagtccaccacga

SEQ ID NO: 158 - RNA, 21 nt, synthetic construct
  source 1..21: mol_type = other RNA
aattgagagaagtccaccacg

SEQ ID NO: 159 - RNA, 21 nt, synthetic construct
  source 1..21: mol_type = other RNA
aattgagagaagtccaccatt

SEQ ID NO: 160 - RNA, 21 nt, synthetic construct
  source 1..21: mol_type = other RNA
tattgagagaagtccaccacg

SEQ ID NO: 161 - RNA, 21 nt, synthetic construct
  source 1..21: mol_type = other RNA
taccaatttatgcctacaggt

SEQ ID NO: 162 - RNA, 21 nt, synthetic construct
  source 1..21: mol_type = other RNA
taccaatttatgcctacagcc

SEQ ID NO: 163 - RNA, 23 nt, synthetic construct
  source 1..23: mol_type = other RNA
taccaatttatgcctacagcctt

SEQ ID NO: 164 - RNA, 23 nt, synthetic construct
  source 1..23: mol_type = other RNA
taccaatttatgcctacagcctc

SEQ ID NO: 165 - RNA, 21 nt, synthetic construct
  source 1..21: mol_type = other RNA
tttgagagaagtccaccactt

SEQ ID NO: 166 - RNA, 23 nt, synthetic construct
  source 1..23: mol_type = other RNA
attgagagaagtccaccacggtt

SEQ ID NO: 167 - RNA, 23 nt, synthetic construct
  source 1..23: mol_type = other RNA
attgagagaagtccaccacgagt

SEQ ID NO: 168 - RNA, 23 nt, synthetic construct
  source 1..23: mol_type = other RNA
tattgagagaagtccaccacgtt

SEQ ID NO: 169 - RNA, 23 nt, synthetic construct
  source 1..23: mol_type = other RNA
tattgagagaagtccaccacgag

SEQ ID NO: 170 - RNA, 22 nt, synthetic construct
  source 1..22: mol_type = other RNA
tattgagagaagtccaccacga

SEQ ID NO: 171 - RNA, 21 nt, synthetic construct
  source 1..21: mol_type = other RNA
agaaaattgagagaagtccac

SEQ ID NO: 172 - RNA, 22 nt, synthetic construct
  source 1..22: mol_type = other RNA
taccaatttatgcctacagctt

SEQ ID NO: 173 - RNA, 22 nt, synthetic construct
  source 1..22: mol_type = other RNA
taccaatttatgcctacagcct

SEQ ID NO: 174 - RNA, 21 nt, synthetic construct
  source 1..21: mol_type = other RNA
tattgagagaagtccaccatt

SEQ ID NO: 175 - RNA, 22 nt, synthetic construct
  source 1..22: mol_type = other RNA
tattgagagaagtccaccactt

SEQ ID NO: 176 - RNA, 22 nt, synthetic construct
  source 1..22: mol_type = other RNA
tttgagagaagtccaccacgtt

SEQ ID NO: 177 - RNA, 22 nt, synthetic construct
  source 1..22: mol_type = other RNA
tttgagagaagtccaccacgag

SEQ ID NO: 178 - RNA, 21 nt, synthetic construct
  source 1..21: mol_type = other RNA
agaaaattgagagaagtcctt

SEQ ID NO: 179 - RNA, 23 nt, synthetic construct
  source 1..23: mol_type = other RNA
agaaaattgagagaagtccactt

SEQ ID NO: 180 - RNA, 22 nt, synthetic construct
  source 1..22: mol_type = other RNA
agaaaattgagagaagtccacc

SEQ ID NO: 181 - RNA, 21 nt, synthetic construct
  source 1..21: mol_type = other RNA
tgaaaattgagagaagtccac

SEQ ID NO: 182 - RNA, 21 nt, synthetic construct
  source 1..21: mol_type = other RNA
accaatttatgcctacagctt

SEQ ID NO: 183 - RNA, 22 nt, synthetic construct
  source 1..22: mol_type = other RNA
accaatttatgcctacagcctt

SEQ ID NO: 184 - RNA, 22 nt, synthetic construct
  source 1..22: mol_type = other RNA
accaatttatgcctacagcctc

SEQ ID NO: 185 - RNA, 21 nt, synthetic construct
  source 1..21: mol_type = other RNA
tccaatttatgcctacagctt

SEQ ID NO: 186 - RNA, 22 nt, synthetic construct
  source 1..22: mol_type = other RNA
tccaatttatgcctacagcctt

SEQ ID NO: 187 - RNA, 21 nt, synthetic construct
  source 1..21: mol_type = other RNA
taccaatttatgcctacagct

SEQ ID NO: 188 - RNA, 21 nt, synthetic construct
  source 1..21: mol_type = other RNA
taccaatttatgcctacagcg

SEQ ID NO: 189 - RNA, 21 nt, synthetic construct
  source 1..21: mol_type = other RNA
aaccaatttatgcctacagcc

SEQ ID NO: 190 - RNA, 21 nt, synthetic construct
  source 1..21: mol_type = other RNA
accaatttatgcctacagcct

SEQ ID NO: 191 - RNA, 21 nt, synthetic construct
  source 1..21: mol_type = other RNA
tccaatttatgcctacagcct

SEQ ID NO: 192 - RNA, 21 nt, synthetic construct
  source 1..21: mol_type = other RNA
accaatttatgcctacagccg

SEQ ID NO: 193 - RNA, 21 nt, synthetic construct
  source 1..21: mol_type = other RNA
tccaatttatgcctacagccg

SEQ ID NO: 194 - RNA, 21 nt, synthetic construct
  source 1..21: mol_type = other RNA
taccaatttatgcctacaggg

SEQ ID NO: 195 - RNA, 25 nt, synthetic construct
  modified_base 1: mod_base = OTHER; note = (NAG25)-2'-O-methyluridine-3'-phosphate
  modified_base 2: mod_base = OTHER; note = 2'-O-methyluridine-3'-phosphorothioate
  modified_base 3: mod_base = OTHER; note = 2'-O-methylguanosine-3'-phosphorothioate
  modified_base 4: mod_base = OTHER; note = 2'-O-methylcytidine-3'-phosphate
  modified_base 5: mod_base = OTHER; note = 2'-O-methylcytidine-3'-phosphate
  modified_base 6: mod_base = OTHER; note = 2'-O-methyluridine-3'-phosphate
  modified_base 7: mod_base = OTHER; note = 2'-O-methylguanosine-3'-phosphate
  modified_base 8: mod_base = OTHER; note = 2'-O-methyluridine-3'-phosphate
  modified_base 9: mod_base = OTHER; note = 2'-O-methyladenosine-3'-phosphate
  modified_base 10: mod_base = OTHER; note = 2'-O-methylguanosine-3'-phosphate
  modified_base 11: mod_base = OTHER; note = 2'-fluoroguanosine-3'-phosphate
  modified_base 12: mod_base = OTHER; note = 2'-fluorocytidine-3'-phosphate
  modified_base 13: mod_base = OTHER; note = 2'-fluoroadenosine-3'-phosphate
  modified_base 14: mod_base = OTHER; note = 2'-O-methyluridine-3'-phosphate
  modified_base 15: mod_base = OTHER; note = 2'-O-methyladenosine-3'-phosphate
  modified_base 16: mod_base = OTHER; note = 2'-O-methyladenosine-3'-phosphate
  modified_base 17: mod_base = OTHER; note = 2'-O-methyladenosine-3'-phosphate
  modified_base 18: mod_base = OTHER; note = 2'-O-methyluridine-3'-phosphate
  modified_base 19: mod_base = OTHER; note = 2'-O-methyluridine-3'-phosphate
  modified_base 20: mod_base = OTHER; note = 2'-O-methylguanosine-3'-phosphate
  modified_base 21: mod_base = OTHER; note = 2'-O-methylguanosine-3'-phosphate
  modified_base 22: mod_base = OTHER; note = 2'-O-methyluridine-3'-phosphate
  modified_base 23: mod_base = OTHER; note = 2'-O-methyladenosine-3'-phosphate
  modified_base 24: mod_base = OTHER; note = 2'-O-methyluridine-3'-phosphorothioate
  modified_base 25: mod_base = OTHER; note = inverted 2'-deoxythymidine-3'-phosphate
  misc_feature 1: note = RNA
  misc_feature 2: note = RNA
  misc_feature 3: note = RNA
  misc_feature 4: note = RNA
  misc_feature 5: note = RNA
  misc_feature 6: note = RNA
  misc_feature 7: note = RNA
  misc_feature 8: note = RNA
  misc_feature 9: note = RNA
  misc_feature 10: note = RNA
  misc_feature 11: note = DNA
  misc_feature 12: note = DNA
  misc_feature 13: note = DNA
  misc_feature 14: note = RNA
  misc_feature 15: note = RNA
  misc_feature 16: note = RNA
  misc_feature 17: note = RNA
  misc_feature 18: note = RNA
  misc_feature 19: note = RNA
  misc_feature 20: note = RNA
  misc_feature 21: note = RNA
  misc_feature 22: note = RNA
  misc_feature 23: note = RNA
  misc_feature 24: note = RNA
  misc_feature 25: note = DNA
  source 1..25: mol_type = other RNA
ttgcctgtaggcataaattggtatt

SEQ ID NO: 196 - RNA, 26 nt, synthetic construct
  modified_base 1: mod_base = OTHER; note = (NAG25)-2'-O-methyluridine-3'-phosphate
  modified_base 2: mod_base = OTHER; note = 2'-O-methyladenosine-3'-phosphate
  modified_base 3: mod_base = OTHER; note = 2'-O-methyluridine-3'-phosphate
  modified_base 4: mod_base = OTHER; note = 2'-O-methyladenosine-3'-phosphate
  modified_base 5: mod_base = OTHER; note = 2'-O-methyluridine-3'-phosphorothioate
  modified_base 6: mod_base = OTHER; note = 2'-O-methylguanosine-3'-phosphorothioate
  modified_base 7: mod_base = OTHER; note = 2'-O-methylcytidine-3'-phosphate
  modified_base 8: mod_base = OTHER; note = 2'-O-methylcytidine-3'-phosphate
  modified_base 9: mod_base = OTHER; note = 2'-O-methyluridine-3'-phosphate
  modified_base 10: mod_base = OTHER; note = 2'-O-methylguanosine-3'-phosphate
  modified_base 11: mod_base = OTHER; note = 2'-O-methyluridine-3'-phosphate
  modified_base 12: mod_base = OTHER; note = 2'-O-methyladenosine-3'-phosphate
  modified_base 13: mod_base = OTHER; note = 2'-O-methylguanosine-3'-phosphate
  modified_base 14: mod_base = OTHER; note = 2'-fluoroguanosine-3'-phosphate
  modified_base 15: mod_base = OTHER; note = 2'-fluorocytidine-3'-phosphate
  modified_base 16: mod_base = OTHER; note = 2'-fluoroadenosine-3'-phosphate
  modified_base 17: mod_base = OTHER; note = 2'-O-methyluridine-3'-phosphate
  modified_base 18: mod_base = OTHER; note = 2'-O-methyladenosine-3'-phosphate
  modified_base 19: mod_base = OTHER; note = 2'-O-methyladenosine-3'-phosphate
  modified_base 20: mod_base = OTHER; note = 2'-O-methyladenosine-3'-phosphate
  modified_base 21: mod_base = OTHER; note = 2'-O-methyluridine-3'-phosphate
  modified_base 22: mod_base = OTHER; note = 2'-O-methyluridine-3'-phosphate
  modified_base 23: mod_base = OTHER; note = 2'-O-methylguanosine-3'-phosphate
  modified_base 24: mod_base = OTHER; note = 2'-O-methylguanosine-3'-phosphate
  modified_base 25: mod_base = OTHER; note = 2'-O-methyluridine-3'-phosphate
  modified_base 26: mod_base = OTHER; note = inverted 2'-deoxyadenosine-3'-phosphate
  misc_feature 1: note = RNA
  misc_feature 2: note = RNA
  misc_feature 3: note = RNA
  misc_feature 4: note = RNA
  misc_feature 5: note = RNA
  misc_feature 6: note = RNA
  misc_feature 7: note = RNA
  misc_feature 8: note = RNA
  misc_feature 9: note = RNA
  misc_feature 10: note = RNA
  misc_feature 11: note = RNA
  misc_feature 12: note = RNA
  misc_feature 13: note = RNA
  misc_feature 14: note = DNA
  misc_feature 15: note = DNA
  misc_feature 16: note = DNA
  misc_feature 17: note = RNA
  misc_feature 18: note = RNA
  misc_feature 19: note = RNA
  misc_feature 20: note = RNA
  misc_feature 21: note = RNA
  misc_feature 22: note = RNA
  misc_feature 23: note = RNA
  misc_feature 24: note = RNA
  misc_feature 25: note = RNA
  misc_feature 26: note = DNA
  source 1..26: mol_type = other RNA
tatatgcctgtaggcataaattggta

SEQ ID NO: 197 - RNA, 26 nt, synthetic construct
  modified_base 1: mod_base = OTHER; note = (NAG25)-2'-O-methylguanosine-3'-phosphate
  modified_base 2: mod_base = OTHER; note = 2'-O-methylcytidine-3'-phosphate
  modified_base 3: mod_base = OTHER; note = 2'-O-methylguanosine-3'-phosphate
  modified_base 4: mod_base = OTHER; note = 2'-O-methylguanosine-3'-phosphate
  modified_base 5: mod_base = OTHER; note = 2'-O-methyladenosine-3'-phosphate
  modified_base 6: mod_base = OTHER; note = 2'-O-methylguanosine-3'-phosphorothioate
  modified_base 7: mod_base = OTHER; note = 2'-O-methylguanosine-3'-phosphate
  modified_base 8: mod_base = OTHER; note = 2'-O-methylcytidine-3'-phosphate
  modified_base 9: mod_base = OTHER; note = 2'-O-methyluridine-3'-phosphate
  modified_base 10: mod_base = OTHER; note = 2'-O-methylguanosine-3'-phosphate
  modified_base 11: mod_base = OTHER; note = 2'-O-methyluridine-3'-phosphate
  modified_base 12: mod_base = OTHER; note = 2'-O-methyladenosine-3'-phosphate
  modified_base 13: mod_base = OTHER; note = 2'-O-methylguanosine-3'-phosphate
  modified_base 14: mod_base = OTHER; note = 2'-fluoroguanosine-3'-phosphate
  modified_base 15: mod_base = OTHER; note = 2'-fluorocytidine-3'-phosphate
  modified_base 16: mod_base = OTHER; note = 2'-fluoroadenosine-3'-phosphate
  modified_base 17: mod_base = OTHER; note = 2'-O-methyluridine-3'-phosphate
  modified_base 18: mod_base = OTHER; note = 2'-O-methyladenosine-3'-phosphate
  modified_base 19: mod_base = OTHER; note = 2'-O-methyladenosine-3'-phosphate
  modified_base 20: mod_base = OTHER; note = 2'-O-methyladenosine-3'-phosphate
  modified_base 21: mod_base = OTHER; note = 2'-O-methyluridine-3'-phosphate
  modified_base 22: mod_base = OTHER; note = 2'-O-methyluridine-3'-phosphate
  modified_base 23: mod_base = OTHER; note = 2'-O-methylguanosine-3'-phosphate
  modified_base 24: mod_base = OTHER; note = 2'-O-methylguanosine-3'-phosphate
  modified_base 25: mod_base = OTHER; note = 2'-methoxyethylthymidine-3'-phosphate
  modified_base 26: mod_base = OTHER; note = inverted 2'-deoxyadenosine-3'-phosphate
  misc_feature 1: note = RNA
  misc_feature 2: note = RNA
  misc_feature 3: note = RNA
  misc_feature 4: note = RNA
  misc_feature 5: note = RNA
  misc_feature 6: note = RNA
  misc_feature 7: note = RNA
  misc_feature 8: note = RNA
  misc_feature 9: note = RNA
  misc_feature 10: note = RNA
  misc_feature 11: note = RNA
  misc_feature 12: note = RNA
  misc_feature 13: note = RNA
  misc_feature 14: note = DNA
  misc_feature 15: note = DNA
  misc_feature 16: note = DNA
  misc_feature 17: note = RNA
  misc_feature 18: note = RNA
  misc_feature 19: note = RNA
  misc_feature 20: note = RNA
  misc_feature 21: note = RNA
  misc_feature 22: note = RNA
  misc_feature 23: note = RNA
  misc_feature 24: note = RNA
  misc_feature 25: note = RNA
  misc_feature 26: note = DNA
  source 1..26: mol_type = other RNA
gcggaggctgtaggcataaattggta

SEQ ID NO: 198 - RNA, 22 nt, synthetic construct
  modified_base 1: mod_base = OTHER; note = (NAG25)s-2'-O-methylcytidine-3'-phosphorothioate
  modified_base 2: mod_base = OTHER; note = 2'-O-methyluridine-3'-phosphate
  modified_base 3: mod_base = OTHER; note = 2'-O-methylguanosine-3'-phosphate
  modified_base 4: mod_base = OTHER; note = 2'-O-methyluridine-3'-phosphate
  modified_base 5: mod_base = OTHER; note = 2'-O-methyladenosine-3'-phosphate
  modified_base 6: mod_base = OTHER; note = 2'-O-methylguanosine-3'-phosphate
  modified_base 7: mod_base = OTHER; note = 2'-fluoroguanosine-3'-phosphate
  modified_base 8: mod_base = OTHER; note = 2'-fluorocytidine-3'-phosphate
  modified_base 9: mod_base = OTHER; note = 2'-fluoroadenosine-3'-phosphate
  modified_base 10: mod_base = OTHER; note = 2'-O-methyluridine-3'-phosphate
  modified_base 11: mod_base = OTHER; note = 2'-O-methyladenosine-3'-phosphate
  modified_base 12: mod_base = OTHER; note = 2'-O-methyladenosine-3'-phosphate
  modified_base 13: mod_base = OTHER; note = 2'-O-methyladenosine-3'-phosphate
  modified_base 14: mod_base = OTHER; note = 2'-O-methyluridine-3'-phosphate
  modified_base 15: mod_base = OTHER; note = 2'-O-methyluridine-3'-phosphate
  modified_base 16: mod_base = OTHER; note = 2'-O-methylguanosine-3'-phosphate
  modified_base 17: mod_base = OTHER; note = 2'-O-methylguanosine-3'-phosphate
  modified_base 18: mod_base = OTHER; note = 2'-O-methyluridine-3'-phosphate
  modified_base 19: mod_base = OTHER; note = 2'-O-methyladenosine-3'-phosphate
  modified_base 20: mod_base = OTHER; note = 2'-O-methyluridine-3'-phosphate
  modified_base 21: mod_base = OTHER; note = 2'-O-methyluridine-3'-phosphorothioate
  modified_base 22: mod_base = OTHER; note = inverted (3'-3' linked) abasic deoxyribonucleotide
  misc_feature 1: note = RNA
  misc_feature 2: note = RNA
  misc_feature 3: note = RNA
  misc_feature 4: note = RNA
  misc_feature 5: note = RNA
  misc_feature 6: note = RNA
  misc_feature 7: note = DNA
  misc_feature 8: note = DNA
  misc_feature 9: note = DNA
  misc_feature 10: note = RNA
  misc_feature 11: note = RNA
  misc_feature 12: note = RNA
  misc_feature 13: note = RNA
  misc_feature 14: note = RNA
  misc_feature 15: note = RNA
  misc_feature 16: note = RNA
  misc_feature 17: note = RNA
  misc_feature 18: note = RNA
  misc_feature 19: note = RNA
  misc_feature 20: note = RNA
  misc_feature 21: note = RNA
  misc_feature 22: note = DNA
  source 1..22: mol_type = other RNA
ctgtaggcataaattggtattn

SEQ ID NO: 199 - RNA, 22 nt, synthetic construct
  modified_base 1: mod_base = OTHER; note = (NAG25)s-2'-O-methylguanosine-3'-phosphorothioate
  modified_base 2: mod_base = OTHER; note = 2'-O-methylcytidine-3'-phosphate
  modified_base 3: mod_base = OTHER; note = 2'-O-methylcytidine-3'-phosphate
  modified_base 4: mod_base = OTHER; note = 2'-O-methyluridine-3'-phosphate
  modified_base 5: mod_base = OTHER; note = 2'-O-methylguanosine-3'-phosphate
  modified_base 6: mod_base = OTHER; note = 2'-O-methyluridine-3'-phosphate
  modified_base 7: mod_base = OTHER; note = 2'-O-methyladenosine-3'-phosphate
  modified_base 8: mod_base = OTHER; note = 2'-O-methylguanosine-3'-phosphate
  modified_base 9: mod_base = OTHER; note = 2'-fluoroguanosine-3'-phosphate
  modified_base 10: mod_base = OTHER; note = 2'-fluorocytidine-3'-phosphate
  modified_base 11: mod_base = OTHER; note = 2'-fluoroadenosine-3'-phosphate
  modified_base 12: mod_base = OTHER; note = 2'-O-methyluridine-3'-phosphate
  modified_base 13: mod_base = OTHER; note = 2'-O-methyladenosine-3'-phosphate
  modified_base 14: mod_base = OTHER; note = 2'-O-methyladenosine-3'-phosphate
  modified_base 15: mod_base = OTHER; note = 2'-O-methyladenosine-3'-phosphate
  modified_base 16: mod_base = OTHER; note = 2'-O-methyluridine-3'-phosphate
  modified_base 17: mod_base = OTHER; note = 2'-O-methyluridine-3'-phosphate
  modified_base 18: mod_base = OTHER; note = 2'-O-methylguanosine-3'-phosphate
  modified_base 19: mod_base = OTHER; note = 2'-O-methylguanosine-3'-phosphate
  modified_base 20: mod_base = OTHER; note = 2'-O-methyluridine-3'-phosphate
  modified_base 21: mod_base = OTHER; note = 2'-O-methyladenosine-3'-phosphorothioate
  modified_base 22: mod_base = OTHER; note = inverted (3'-3' linked) abasic deoxyribonucleotide
  misc_feature 1: note = RNA
  misc_feature 2: note = RNA
  misc_feature 3: note = RNA
  misc_feature 4: note = RNA
  misc_feature 5: note = RNA
  misc_feature 6: note = RNA
  misc_feature 7: note = RNA
  misc_feature 8: note = RNA
  misc_feature 9: note = DNA
  misc_feature 10: note = DNA
  misc_feature 11: note = DNA
  misc_feature 12: note = RNA
  misc_feature 13: note = RNA
  misc_feature 14: note = RNA
  misc_feature 15: note = RNA
  misc_feature 16: note = RNA
  misc_feature 17: note = RNA
  misc_feature 18: note = RNA
  misc_feature 19: note = RNA
  misc_feature 20: note = RNA
  misc_feature 21: note = RNA
  misc_feature 22: note = DNA
  source 1..22: mol_type = other RNA
gcctgtaggcataaattggtan

SEQ ID NO: 200 - RNA, 21 nt, synthetic construct
  modified_base 1: mod_base = OTHER; note = (NAG25)s-2'-O-methylguanosine-3'-phosphorothioate
  modified_base 2: mod_base = OTHER; note = 2'-O-methylcytidine-3'-phosphate
  modified_base 3: mod_base = OTHER; note = 2'-O-methylcytidine-3'-phosphate
  modified_base 4: mod_base = OTHER; note = 2'-O-methyluridine-3'-phosphate
  modified_base 5: mod_base = OTHER; note = 2'-O-methylguanosine-3'-phosphate
  modified_base 6: mod_base = OTHER; note = 2'-O-methyluridine-3'-phosphate
  modified_base 7: mod_base = OTHER; note = 2'-O-methyladenosine-3'-phosphate
  modified_base 8: mod_base = OTHER; note = 2'-O-methylguanosine-3'-phosphate
  modified_base 9: mod_base = OTHER; note = 2'-fluoroguanosine-3'-phosphate
  modified_base 10: mod_base = OTHER; note = 2'-fluorocytidine-3'-phosphate
  modified_base 11: mod_base = OTHER; note = 2'-fluoroadenosine-3'-phosphate
  modified_base 12: mod_base = OTHER; note = 2'-O-methyluridine-3'-phosphate
  modified_base 13: mod_base = OTHER; note = 2'-O-methyladenosine-3'-phosphate
  modified_base 14: mod_base = OTHER; note = 2'-O-methyladenosine-3'-phosphate
  modified_base 15: mod_base = OTHER; note = 2'-O-methyladenosine-3'-phosphate
  modified_base 16: mod_base = OTHER; note = 2'-O-methyluridine-3'-phosphate
  modified_base 17: mod_base = OTHER; note = 2'-O-methyluridine-3'-phosphate
  modified_base 18: mod_base = OTHER; note = 2'-O-methylguanosine-3'-phosphate
  modified_base 19: mod_base = OTHER; note = 2'-O-methylguanosine-3'-phosphate
  modified_base 20: mod_base = OTHER; note = 2'-O-methyluridine-3'-phosphorothioate
  modified_base 21: mod_base = OTHER; note = inverted 2'-deoxyadenosine-3'-phosphate
  misc_feature 1: note = RNA
  misc_feature 2: note = RNA
  misc_feature 3: note = RNA
  misc_feature 4: note = RNA
  misc_feature 5: note = RNA
  misc_feature 6: note = RNA
  misc_feature 7: note = RNA
  misc_feature 8: note = RNA
  misc_feature 9: note = DNA
  misc_feature 10: note = DNA
  misc_feature 11: note = DNA
  misc_feature 12: note = RNA
  misc_feature 13: note = RNA
  misc_feature 14: note = RNA
  misc_feature 15: note = RNA
  misc_feature 16: note = RNA
  misc_feature 17: note = RNA
  misc_feature 18: note = RNA
  misc_feature 19: note = RNA
  misc_feature 20: note = RNA
  misc_feature 21: note = DNA
  source 1..21: mol_type = other RNA
gcctgtaggcataaattggta

SEQ ID NO: 201 - RNA, 22 nt, synthetic construct
  modified_base 1: mod_base = OTHER; note = (NAG25)s-2'-O-methylguanosine-3'-phosphorothioate
  modified_base 2: mod_base = OTHER; note = 2'-O-methylcytidine-3'-phosphate
  modified_base 3: mod_base = OTHER; note = 2'-O-methylcytidine-3'-phosphate
  modified_base 4: mod_base = OTHER; note = 2'-O-methyluridine-3'-phosphate
  modified_base 5: mod_base = OTHER; note = 2'-O-methylguanosine-3'-phosphate
  modified_base 6: mod_base = OTHER; note = 2'-O-methyluridine-3'-phosphate
  modified_base 7: mod_base = OTHER; note = 2'-O-methyladenosine-3'-phosphate
  modified_base 8: mod_base = OTHER; note = 2'-O-methylguanosine-3'-phosphate
  modified_base 9: mod_base = OTHER; note = 2'-fluoroguanosine-3'-phosphate
  modified_base 10: mod_base = OTHER; note = 2'-fluorocytidine-3'-phosphate
  modified_base 11: mod_base = OTHER; note = 2'-fluoroadenosine-3'-phosphate
  modified_base 12: mod_base = OTHER; note = 2'-O-methyluridine-3'-phosphate
  modified_base 13: mod_base = OTHER; note = 2'-O-methyladenosine-3'-phosphate
  modified_base 14: mod_base = OTHER; note = 2'-O-methyladenosine-3'-phosphate
  modified_base 15: mod_base = OTHER; note = 2'-O-methyladenosine-3'-phosphate
  modified_base 16: mod_base = OTHER; note = 2'-O-methyluridine-3'-phosphate
  modified_base 17: mod_base = OTHER; note = 2'-O-methyluridine-3'-phosphate
  modified_base 18: mod_base = OTHER; note = 2'-O-methylguanosine-3'-phosphate
  modified_base 19: mod_base = OTHER; note = 2'-O-methylguanosine-3'-phosphate
  modified_base 20: mod_base = OTHER; note = 2'-O-methyluridine-3'-phosphate
  modified_base 21: mod_base = OTHER; note = 2'-methoxyethyladenosine-3'-phosphorothioate
  modified_base 22: mod_base = OTHER; note = inverted (3'-3' linked) abasic deoxyribonucleotide
  misc_feature 1: note = RNA
  misc_feature 2: note = RNA
  misc_feature 3: note = RNA
  misc_feature 4: note = RNA
  misc_feature 5: note = RNA
  misc_feature 6: note = RNA
  misc_feature 7: note = RNA
  misc_feature 8: note = RNA
  misc_feature 9: note = DNA
  misc_feature 10: note = DNA
  misc_feature 11: note = DNA
  misc_feature 12: note = RNA
  misc_feature 13: note = RNA
  misc_feature 14: note = RNA
  misc_feature 15: note = RNA
  misc_feature 16: note = RNA
  misc_feature 17: note = RNA
  misc_feature 18: note = RNA
  misc_feature 19: note = RNA
  misc_feature 20: note = RNA
  misc_feature 21: note = RNA
  misc_feature 22: note = DNA
  source 1..22: mol_type = other RNA
gcctgtaggcataaattggtan

SEQ ID NO: 202 - RNA, 22 nt, synthetic construct
  modified_base 1: mod_base = OTHER; note = (NAG25)s-2'-O-methylguanosine-3'-phosphorothioate
  modified_base 2: mod_base = OTHER; note = 2'-O-methylcytidine-3'-phosphate
  modified_base 3: mod_base = OTHER; note = 2'-O-methylcytidine-3'-phosphate
  modified_base 4: mod_base = OTHER; note = 2'-O-methyluridine-3'-phosphate
  modified_base 5: mod_base = OTHER; note = 2'-O-methylguanosine-3'-phosphate
  modified_base 6: mod_base = OTHER; note = 2'-O-methyluridine-3'-phosphate
  modified_base 7: mod_base = OTHER; note = 2'-O-methyladenosine-3'-phosphate
  modified_base 8: mod_base = OTHER; note = 2'-O-methylguanosine-3'-phosphate
  modified_base 9: mod_base = OTHER; note = 2'-fluoroguanosine-3'-phosphate
  modified_base 10: mod_base = OTHER; note = 2'-fluorocytidine-3'-phosphate
  modified_base 11: mod_base = OTHER; note = 2'-fluoroadenosine-3'-phosphate
  modified_base 12: mod_base = OTHER; note = 2'-O-methyluridine-3'-phosphate
  modified_base 13: mod_base = OTHER; note = 2'-O-methyladenosine-3'-phosphate
  modified_base 14: mod_base = OTHER; note = 2'-O-methyladenosine-3'-phosphate
  modified_base 15: mod_base = OTHER; note = 2'-O-methyladenosine-3'-phosphate
  modified_base 16: mod_base = OTHER; note = 2'-O-methyluridine-3'-phosphate
  modified_base 17: mod_base = OTHER; note = 2'-O-methyluridine-3'-phosphate
  modified_base 18: mod_base = OTHER; note = 2'-O-methylguanosine-3'-phosphate
  modified_base 19: mod_base = OTHER; note = 2'-O-methylguanosine-3'-phosphate
  modified_base 20: mod_base = OTHER; note = 2'-methoxyethylthymidine-3'-phosphate
  modified_base 21: mod_base = OTHER; note = 2'-methoxyethyladenosine-3'-phosphorothioate
  modified_base 22: mod_base = OTHER; note = inverted (3'-3' linked) abasic deoxyribonucleotide
  misc_feature 1: note = RNA
  misc_feature 2: note = RNA
  misc_feature 3: note = RNA
  misc_feature 4: note = RNA
  misc_feature 5: note = RNA
  misc_feature 6: note = RNA
  misc_feature 7: note = RNA
  misc_feature 8: note = RNA
  misc_feature 9: note = DNA
  misc_feature 10: note = DNA
  misc_feature 11: note = DNA
  misc_feature 12: note = RNA
  misc_feature 13: note = RNA
  misc_feature 14: note = RNA
  misc_feature 15: note = RNA
  misc_feature 16: note = RNA
  misc_feature 17: note = RNA
  misc_feature 18: note = RNA
  misc_feature 19: note = RNA
  misc_feature 20: note = RNA
  misc_feature 21: note = RNA
  misc_feature 22: note = DNA
  source 1..22: mol_type = other RNA
gcctgtaggcataaattggtan

SEQ ID NO: 203 - RNA, 22 nt, synthetic construct
  modified_base 1: mod_base = OTHER; note = (NAG25)s-2'-O-methyladenosine-3'-phosphorothioate
  modified_base 2: mod_base = OTHER; note = 2'-O-methyladenosine-3'-phosphate
  modified_base 3: mod_base = OTHER; note = 2'-O-methylcytidine-3'-phosphate
  modified_base 4: mod_base = OTHER; note = 2'-O-methyluridine-3'-phosphate
  modified_base 5: mod_base = OTHER; note = 2'-O-methylguanosine-3'-phosphate
  modified_base 6: mod_base = OTHER; note = 2'-O-methyluridine-3'-phosphate
  modified_base 7: mod_base = OTHER; note = 2'-O-methyladenosine-3'-phosphate
  modified_base 8: mod_base = OTHER; note = 2'-O-methylguanosine-3'-phosphate
  modified_base 9: mod_base = OTHER; note = 2'-fluoroguanosine-3'-phosphate
  modified_base 10: mod_base = OTHER; note = 2'-fluorocytidine-3'-phosphate
  modified_base 11: mod_base = OTHER; note = 2'-fluoroadenosine-3'-phosphate
  modified_base 12: mod_base = OTHER; note = 2'-O-methyluridine-3'-phosphate
  modified_base 13: mod_base = OTHER; note = 2'-O-methyladenosine-3'-phosphate
  modified_base 14: mod_base = OTHER; note = 2'-O-methyladenosine-3'-phosphate
  modified_base 15: mod_base = OTHER; note = 2'-O-methyladenosine-3'-phosphate
  modified_base 16: mod_base = OTHER; note = 2'-O-methyluridine-3'-phosphate
  modified_base 17: mod_base = OTHER; note = 2'-O-methyluridine-3'-phosphate
  modified_base 18: mod_base = OTHER; note = 2'-O-methylguanosine-3'-phosphate
  modified_base 19: mod_base = OTHER; note = 2'-O-methylguanosine-3'-phosphate
  modified_base 20: mod_base = OTHER; note = 2'-O-methyluridine-3'-phosphate
  modified_base 21: mod_base = OTHER; note = 2'-O-methyladenosine-3'-phosphorothioate
  modified_base 22: mod_base = OTHER; note = inverted (3'-3' linked) abasic deoxyribonucleotide
  misc_feature 1: note = RNA
  misc_feature 2: note = RNA
  misc_feature 3: note = RNA
  misc_feature 4: note = RNA
  misc_feature 5: note = RNA
  misc_feature 6: note = RNA
  misc_feature 7: note = RNA
  misc_feature 8: note = RNA
  misc_feature 9: note = DNA
  misc_feature 10: note = DNA
  misc_feature 11: note = DNA
  misc_feature 12: note = RNA
  misc_feature 13: note = RNA
  misc_feature 14: note = RNA
  misc_feature 15: note = RNA
  misc_feature 16: note = RNA
  misc_feature 17: note = RNA
  misc_feature 18: note = RNA
  misc_feature 19: note = RNA
  misc_feature 20: note = RNA
  misc_feature 21: note = RNA
  misc_feature 22: note = DNA
  source 1..22: mol_type = other RNA
aactgtaggcataaattggtan

SEQ ID NO: 204 - RNA, 22 nt, synthetic construct
  modified_base 1: mod_base = OTHER; note = (NAG25)s-2'-O-methyluridine-3'-phosphorothioate
  modified_base 2: mod_base = OTHER; note = 2'-O-methylcytidine-3'-phosphate
  modified_base 3: mod_base = OTHER; note = 2'-O-methylguanosine-3'-phosphate
  modified_base 4: mod_base = OTHER; note = 2'-O-methyluridine-3'-phosphate
  modified_base 5: mod_base = OTHER; note = 2'-O-methylguanosine-3'-phosphate
  modified_base 6: mod_base = OTHER; note = 2'-O-methylguanosine-3'-phosphate
  modified_base 7: mod_base = OTHER; note = 2'-O-methyluridine-3'-phosphate
  modified_base 8: mod_base = OTHER; note = 2'-O-methylguanosine-3'-phosphate
  modified_base 9: mod_base = OTHER; note = 2'-fluoroguanosine-3'-phosphate
  modified_base 10: mod_base = OTHER; note = 2'-fluoroadenosine-3'-phosphate
  modified_base 11: mod_base = OTHER; note = 2'-fluorocytidine-3'-phosphate
  modified_base 12: mod_base = OTHER; note = 2'-O-methyluridine-3'-phosphate
  modified_base 13: mod_base = OTHER; note = 2'-O-methyluridine-3'-phosphate
  modified_base 14: mod_base = OTHER; note = 2'-O-methylcytidine-3'-phosphate
  modified_base 15: mod_base = OTHER; note = 2'-O-methyluridine-3'-phosphate
  modified_base 16: mod_base = OTHER; note = 2'-O-methylcytidine-3'-phosphate
  modified_base 17: mod_base = OTHER; note = 2'-O-methyluridine-3'-phosphate
  modified_base 18: mod_base = OTHER; note = 2'-O-methylcytidine-3'-phosphate
  modified_base 19: mod_base = OTHER; note = 2'-O-methyladenosine-3'-phosphate
  modified_base 20: mod_base = OTHER; note = 2'-O-methyladenosine-3'-phosphate
  modified_base 21: mod_base = OTHER; note = 2'-O-methyluridine-3'-phosphorothioate
  modified_base 22: mod_base = OTHER; note = inverted (3'-3' linked) abasic deoxyribonucleotide
  misc_feature 1: note = RNA
  misc_feature 2: note = RNA
  misc_feature 3: note = RNA
  misc_feature 4: note = RNA
  misc_feature 5: note = RNA
  misc_feature 6: note = RNA
  misc_feature 7: note = RNA
  misc_feature 8: note = RNA
  misc_feature 9: note = DNA
  misc_feature 10: note = DNA
  misc_feature 11: note = DNA
  misc_feature 12: note = RNA
  misc_feature 13: note = RNA
  misc_feature 14: note = RNA
  misc_feature 15: note = RNA
  misc_feature 16: note = RNA
  misc_feature 17: note = RNA
  misc_feature 18: note = RNA
  misc_feature 19: note = RNA
  misc_feature 20: note = RNA
  misc_feature 21: note = RNA
  misc_feature 22: note = DNA
  source 1..22: mol_type = other RNA
tcgtggtggacttctctcaatn

SEQ ID NO: 205 - RNA, 22 nt, synthetic construct
  modified_base 1: mod_base = OTHER; note = (NAG25)s-2'-O-methyladenosine-3'-phosphorothioate
  modified_base 2: mod_base = OTHER; note = 2'-O-methyladenosine-3'-phosphate
  modified_base 3: mod_base = OTHER; note = 2'-O-methylguanosine-3'-phosphate
  modified_base 4: mod_base = OTHER; note = 2'-O-methyluridine-3'-phosphate
  modified_base 5: mod_base = OTHER; note = 2'-O-methylguanosine-3'-phosphate
  modified_base 6: mod_base = OTHER; note = 2'-O-methylguanosine-3'-phosphate
  modified_base 7: mod_base = OTHER; note = 2'-O-methyluridine-3'-phosphate
  modified_base 8: mod_base = OTHER; note = 2'-O-methylguanosine-3'-phosphate
  modified_base 9: mod_base = OTHER; note = 2'-fluoroguanosine-3'-phosphate
  modified_base 10: mod_base = OTHER; note = 2'-fluoroadenosine-3'-phosphate
  modified_base 11: mod_base = OTHER; note = 2'-fluorocytidine-3'-phosphate
  modified_base 12: mod_base = OTHER; note = 2'-O-methyluridine-3'-phosphate
  modified_base 13: mod_base = OTHER; note = 2'-O-methyluridine-3'-phosphate
  modified_base 14: mod_base = OTHER; note = 2'-O-methylcytidine-3'-phosphate
  modified_base 15: mod_base = OTHER; note = 2'-O-methyluridine-3'-phosphate
  modified_base 16: mod_base = OTHER; note = 2'-O-methylcytidine-3'-phosphate
  modified_base 17: mod_base = OTHER; note = 2'-O-methyluridine-3'-phosphate
  modified_base 18: mod_base = OTHER; note = 2'-O-methylcytidine-3'-phosphate
  modified_base 19: mod_base = OTHER; note = 2'-O-methyladenosine-3'-phosphate
  modified_base 20: mod_base = OTHER; note = 2'-O-methyladenosine-3'-phosphate
  modified_base 21: mod_base = OTHER; note = 2'-O-methyluridine-3'-phosphorothioate
  modified_base 22: mod_base = OTHER; note = inverted (3'-3' linked) abasic deoxyribonucleotide
  misc_feature 1: note = RNA
  misc_feature 2: note = RNA
  misc_feature 3: note = RNA
  misc_feature 4: note = RNA
  misc_feature 5: note = RNA
  misc_feature 6: note = RNA
  misc_feature 7: note = RNA
  misc_feature 8: note = RNA
  misc_feature 9: note = DNA
  misc_feature 10: note = DNA
  misc_feature 11: note = DNA
  misc_feature 12: note = RNA
  misc_feature 13: note = RNA
  misc_feature 14: note = RNA
  misc_feature 15: note = RNA
  misc_feature 16: note = RNA
  misc_feature 17: note = RNA
  misc_feature 18: note = RNA
  misc_feature 19: note = RNA
  misc_feature 20: note = RNA
  misc_feature 21: note = RNA
  misc_feature 22: note = DNA
  source 1..22: mol_type = other RNA
aagtggtggacttctctcaatn

SEQ ID NO: 206 - RNA, 22 nt, synthetic construct
  modified_base 1: mod_base = OTHER; note = (NAG25)s-2'-O-methyluridine-3'-phosphorothioate
  modified_base 2: mod_base = OTHER; note = 2'-O-methylcytidine-3'-phosphate
  modified_base 3: mod_base = OTHER; note = 2'-O-methylguanosine-3'-phosphate
  modified_base 4: mod_base = OTHER; note = 2'-O-methyluridine-3'-phosphate
  modified_base 5: mod_base = OTHER; note = 2'-O-methylguanosine-3'-phosphate
  modified_base 6: mod_base = OTHER; note = 2'-O-methylguanosine-3'-phosphate
  modified_base 7: mod_base = OTHER; note = 2'-O-methyluridine-3'-phosphate
  modified_base 8: mod_base = OTHER; note = 2'-O-methylguanosine-3'-phosphate
  modified_base 9: mod_base = OTHER; note = 2'-fluoroguanosine-3'-phosphate
  modified_base 10: mod_base = OTHER; note = 2'-fluoroadenosine-3'-phosphate
  modified_base 11: mod_base = OTHER; note = 2'-fluorocytidine-3'-phosphate
  modified_base 12: mod_base = OTHER; note = 2'-O-methyluridine-3'-phosphate
  modified_base 13: mod_base = OTHER; note = 2'-O-methyluridine-3'-phosphate
  modified_base 14: mod_base = OTHER; note = 2'-O-methylcytidine-3'-phosphate
  modified_base 15: mod_base = OTHER; note = 2'-O-methyluridine-3'-phosphate
  modified_base 16: mod_base = OTHER; note = 2'-O-methylcytidine-3'-phosphate
  modified_base 17: mod_base = OTHER; note = 2'-O-methyluridine-3'-phosphate
  modified_base 18: mod_base = OTHER; note = 2'-O-methylcytidine-3'-phosphate
  modified_base 19: mod_base = OTHER; note = 2'-O-methyladenosine-3'-phosphate
  modified_base 20: mod_base = OTHER; note = 2'-methoxyethyladenosine-3'-phosphate
  modified_base 21: mod_base = OTHER; note = 2'-methoxyethylthymidine-3'-phosphorothioate
  modified_base 22: mod_base = OTHER; note = inverted (3'-3' linked) abasic deoxyribonucleotide
  misc_feature 1: note = RNA
  misc_feature 2: note = RNA
  misc_feature 3: note = RNA
  misc_feature 4: note = RNA
  misc_feature 5: note = RNA
  misc_feature 6: note = RNA
  misc_feature 7: note = RNA
  misc_feature 8: note = RNA
  misc_feature 9: note = DNA
  misc_feature 10: note = DNA
  misc_feature 11: note = DNA
  misc_feature 12: note = RNA
  misc_feature 13: note = RNA
  misc_feature 14: note = RNA
  misc_feature 15: note = RNA
  misc_feature 16: note = RNA
  misc_feature 17: note = RNA
  misc_feature 18: note = RNA
  misc_feature 19: note = RNA
  misc_feature 20: note = RNA
  misc_feature 21: note = RNA
  misc_feature 22: note = DNA
  source 1..22: mol_type = other RNA
tcgtggtggacttctctcaatn

SEQ ID NO: 207 - RNA, 22 nt, synthetic construct
  modified_base 1: mod_base = OTHER; note = (NAG25)s-2'-O-methylcytidine-3'-phosphorothioate
  modified_base 2: mod_base = OTHER; note = 2'-O-methylguanosine-3'-phosphate
  modified_base 3: mod_base = OTHER; note = 2'-O-methyluridine-3'-phosphate
  modified_base 4: mod_base = OTHER; note = 2'-O-methylguanosine-3'-phosphate
  modified_base 5: mod_base = OTHER; note = 2'-O-methylguanosine-3'-phosphate
  modified_base 6: mod_base = OTHER; note = 2'-O-methyluridine-3'-phosphate
  modified_base 7: mod_base = OTHER; note = 2'-O-methylguanosine-3'-phosphate
  modified_base 8: mod_base = OTHER; note = 2'-O-methylguanosine-3'-phosphate
  modified_base 9: mod_base = OTHER; note = 2'-fluoroadenosine-3'-phosphate
  modified_base 10: mod_base = OTHER; note = 2'-fluorocytidine-3'-phosphate
  modified_base 11: mod_base = OTHER; note = 2'-fluorouridine-3'-phosphate
  modified_base 12: mod_base = OTHER; note = 2'-O-methyluridine-3'-phosphate
  modified_base 13: mod_base = OTHER; note = 2'-O-methylcytidine-3'-phosphate
  modified_base 14: mod_base = OTHER; note = 2'-O-methyluridine-3'-phosphate
  modified_base 15: mod_base = OTHER; note = 2'-O-methylcytidine-3'-phosphate
  modified_base 16: mod_base = OTHER; note = 2'-O-methyluridine-3'-phosphate
  modified_base 17: mod_base = OTHER; note = 2'-O-methylcytidine-3'-phosphate
  modified_base 18: mod_base = OTHER; note = 2'-O-methyladenosine-3'-phosphate
  modified_base 19: mod_base = OTHER; note = 2'-O-methyladenosine-3'-phosphate
  modified_base 20: mod_base = OTHER; note = 2'-O-methyluridine-3'-phosphate
  modified_base 21: mod_base = OTHER; note = 2'-O-methyluridine-3'-phosphorothioate
  modified_base 22: mod_base = OTHER; note = inverted (3'-3' linked) abasic deoxyribonucleotide
  misc_feature 1: note = RNA
  misc_feature 2: note = RNA
  misc_feature 3: note = RNA
  misc_feature 4: note = RNA
  misc_feature 5: note = RNA
  misc_feature 6: note = RNA
  misc_feature 7: note = RNA
  misc_feature 8: note = RNA
  misc_feature 9: note = DNA
  misc_feature 10: note = DNA
  misc_feature 11: note = DNA
  misc_feature 12: note = RNA
  misc_feature 13: note = RNA
  misc_feature 14: note = RNA
  misc_feature 15: note = RNA
  misc_feature 16: note = RNA
  misc_feature 17: note = RNA
  misc_feature 18: note = RNA
  misc_feature 19: note = RNA
  misc_feature 20: note = RNA
  misc_feature 21: note = RNA
  misc_feature 22: note = DNA
  source 1..22: mol_type = other RNA
cgtggtggacttctctcaattn

SEQ ID NO: 208 - RNA, 22 nt, synthetic construct
  modified_base 1: mod_base = OTHER; note = (NAG25)s-2'-O-methyladenosine-3'-phosphorothioate
  modified_base 2: mod_base = OTHER; note = 2'-O-methyladenosine-3'-phosphate
  modified_base 3: mod_base = OTHER; note = 2'-O-methyluridine-3'-phosphate
  modified_base 4: mod_base = OTHER; note = 2'-O-methylguanosine-3'-phosphate
  modified_base 5: mod_base = OTHER; note = 2'-O-methylguanosine-3'-phosphate
  modified_base 6: mod_base = OTHER; note = 2'-O-methyluridine-3'-phosphate
  modified_base 7: mod_base = OTHER; note = 2'-O-methylguanosine-3'-phosphate
  modified_base 8: mod_base = OTHER; note = 2'-O-methylguanosine-3'-phosphate
  modified_base 9: mod_base = OTHER; note = 2'-fluoroadenosine-3'-phosphate
  modified_base 10: mod_base = OTHER; note = 2'-fluorocytidine-3'-phosphate
  modified_base 11: mod_base = OTHER; note = 2'-fluorouridine-3'-phosphate
  modified_base 12: mod_base = OTHER; note = 2'-O-methyluridine-3'-phosphate
  modified_base 13: mod_base = OTHER; note = 2'-O-methylcytidine-3'-phosphate
  modified_base 14: mod_base = OTHER; note = 2'-O-methyluridine-3'-phosphate
  modified_base 15: mod_base = OTHER; note = 2'-O-methylcytidine-3'-phosphate
  modified_base 16: mod_base = OTHER; note = 2'-O-methyluridine-3'-phosphate
  modified_base 17: mod_base = OTHER; note = 2'-O-methylcytidine-3'-phosphate
  modified_base 18: mod_base = OTHER; note = 2'-O-methyladenosine-3'-phosphate
  modified_base 19: mod_base = OTHER; note = 2'-O-methyladenosine-3'-phosphate
  modified_base 20: mod_base = OTHER; note = 2'-O-methyluridine-3'-phosphate
  modified_base 21: mod_base = OTHER; note = 2'-O-methyluridine-3'-phosphorothioate
  modified_base 22: mod_base = OTHER; note = inverted (3'-3' linked) abasic deoxyribonucleotide
  misc_feature 1: note = RNA
  misc_feature 2: note = RNA
  misc_feature 3: note = RNA
  misc_feature 4: note = RNA
  misc_feature 5: note = RNA
  misc_feature 6: note = RNA
  misc_feature 7: note = RNA
  misc_feature 8: note = RNA
  misc_feature 9: note = DNA
  misc_feature 10: note = DNA
  misc_feature 11: note = DNA
  misc_feature 12: note = RNA
  misc_feature 13: note = RNA
  misc_feature 14: note = RNA
  misc_feature 15: note = RNA
  misc_feature 16: note = RNA
  misc_feature 17: note = RNA
  misc_feature 18: note = RNA
  misc_feature 19: note = RNA
  misc_feature 20: note = RNA
  misc_feature 21: note = RNA
  misc_feature 22: note = DNA
  source 1..22: mol_type = other RNA
aatggtggacttctctcaattn

SEQ ID NO: 209 - RNA, 22 nt, synthetic construct
  modified_base 1: mod_base = OTHER; note = (NAG25)s-2'-O-methylcytidine-3'-phosphorothioate
  modified_base 2: mod_base = OTHER; note = 2'-O-methylguanosine-3'-phosphate
  modified_base 3: mod_base = OTHER; note = 2'-O-methyluridine-3'-phosphate
  modified_base 4: mod_base = OTHER; note = 2'-O-methylguanosine-3'-phosphate
  modified_base 5: mod_base = OTHER; note = 2'-O-methylguanosine-3'-phosphate
  modified_base 6: mod_base = OTHER; note = 2'-O-methyluridine-3'-phosphate
  modified_base 7: mod_base = OTHER; note = 2'-O-methylguanosine-3'-phosphate
  modified_base 8: mod_base = OTHER; note = 2'-O-methylguanosine-3'-phosphate
  modified_base 9: mod_base = OTHER; note = 2'-fluoroadenosine-3'-phosphate
  modified_base 10: mod_base = OTHER; note = 2'-fluorocytidine-3'-phosphate
  modified_base 11: mod_base = OTHER; note = 2'-fluorouridine-3'-phosphate
  modified_base 12: mod_base = OTHER; note = 2'-O-methyluridine-3'-phosphate
  modified_base 13: mod_base = OTHER; note = 2'-O-methylcytidine-3'-phosphate
  modified_base 14: mod_base = OTHER; note = 2'-O-methyluridine-3'-phosphate
  modified_base 15: mod_base = OTHER; note = 2'-O-methylcytidine-3'-phosphate
  modified_base 16: mod_base = OTHER; note = 2'-O-methyluridine-3'-phosphate
  modified_base 17: mod_base = OTHER; note = 2'-O-methylcytidine-3'-phosphate
  modified_base 18: mod_base = OTHER; note = 2'-O-methyladenosine-3'-phosphate
  modified_base 19: mod_base = OTHER; note = 2'-O-methyladenosine-3'-phosphate
  modified_base 20: mod_base = OTHER; note = 2'-methoxyethylthymidine-3'-phosphate
  modified_base 21: mod_base = OTHER; note = 2'-methoxyethylthymidine-3'-phosphorothioate
  modified_base 22: mod_base = OTHER; note = inverted (3'-3' linked) abasic deoxyribonucleotide
  misc_feature 1: note = RNA
  misc_feature 2: note = RNA
  misc_feature 3: note = RNA
  misc_feature 4: note = RNA
  misc_feature 5: note = RNA
  misc_feature 6: note = RNA
  misc_feature 7: note = RNA
  misc_feature 8: note = RNA
  misc_feature 9: note = DNA
  misc_feature 10: note = DNA
  misc_feature 11: note = DNA
  misc_feature 12: note = RNA
  misc_feature 13: note = RNA
  misc_feature 14: note = RNA
  misc_feature 15: note = RNA
  misc_feature 16: note = RNA
  misc_feature 17: note = RNA
  misc_feature 18: note = RNA
  misc_feature 19: note = RNA
  misc_feature 20: note = RNA
  misc_feature 21: note = RNA
  misc_feature 22: note = DNA
  source 1..22: mol_type = other RNA
cgtggtggacttctctcaattn

SEQ ID NO: 210 - RNA, 22 nt, synthetic construct
  modified_base 1: mod_base = OTHER; note = (NAG25)s-2'-O-methylguanosine-3'-phosphorothioate
  modified_base 2: mod_base = OTHER; note = 2'-O-methylguanosine-3'-phosphate
  modified_base 3: mod_base = OTHER; note = 2'-O-methyladenosine-3'-phosphate
  modified_base 4: mod_base = OTHER; note = 2'-O-methylcytidine-3'-phosphate
  modified_base 5: mod_base = OTHER; note = 2'-O-methyluridine-3'-phosphate
  modified_base 6: mod_base = OTHER; note = 2'-O-methyluridine-3'-phosphate
  modified_base 7: mod_base = OTHER; note = 2'-O-methylcytidine-3'-phosphate
  modified_base 8: mod_base = OTHER; note = 2'-O-methyluridine-3'-phosphate
  modified_base 9: mod_base = OTHER; note = 2'-fluorocytidine-3'-phosphate
  modified_base 10: mod_base = OTHER; note = 2'-fluorouridine-3'-phosphate
  modified_base 11: mod_base = OTHER; note = 2'-fluorocytidine-3'-phosphate
  modified_base 12: mod_base = OTHER; note = 2'-O-methyladenosine-3'-phosphate
  modified_base 13: mod_base = OTHER; note = 2'-O-methyladenosine-3'-phosphate
  modified_base 14: mod_base = OTHER; note = 2'-O-methyluridine-3'-phosphate
  modified_base 15: mod_base = OTHER; note = 2'-O-methyluridine-3'-phosphate
  modified_base 16: mod_base = OTHER; note = 2'-O-methyluridine-3'-phosphate
  modified_base 17: mod_base = OTHER; note = 2'-O-methyluridine-3'-phosphate
  modified_base 18: mod_base = OTHER; note = 2'-O-methylcytidine-3'-phosphate
  modified_base 19: mod_base = OTHER; note = 2'-O-methyluridine-3'-phosphate
  modified_base 20: mod_base = OTHER; note = 2'-O-methyladenosine-3'-phosphate
  modified_base 21: mod_base = OTHER; note = 2'-O-methyladenosine-3'-phosphorothioate
  modified_base 22: mod_base = OTHER; note = inverted (3'-3' linked) abasic deoxyribonucleotide
  misc_feature 1: note = RNA
  misc_feature 2: note = RNA
  misc_feature 3: note = RNA
  misc_feature 4: note = RNA
  misc_feature 5: note = RNA
  misc_feature 6: note = RNA
  misc_feature 7: note = RNA
  misc_feature 8: note = RNA
  misc_feature 9: note = DNA
  misc_feature 10: note = DNA
  misc_feature 11: note = DNA
  misc_feature 12: note = RNA
  misc_feature 13: note = RNA
  misc_feature 14: note = RNA
  misc_feature 15: note = RNA
  misc_feature 16: note = RNA
  misc_feature 17: note = RNA
  misc_feature 18: note = RNA
  misc_feature 19: note = RNA
  misc_feature 20: note = RNA
  misc_feature 21: note = RNA
  misc_feature 22: note = DNA
  source 1..22: mol_type = other RNA
ggacttctctcaattttctaan

SEQ ID NO: 211 - RNA, 22 nt, synthetic construct
  modified_base 1: mod_base = OTHER; note = (NAG25)s-2'-O-methylcytidine-3'-phosphorothioate
  modified_base 2: mod_base = OTHER; note = 2'-O-methylguanosine-3'-phosphate
  modified_base 3: mod_base = OTHER; note = 2'-O-methyluridine-3'-phosphate
  modified_base 4: mod_base = OTHER; note = 2'-O-methylguanosine-3'-phosphate
  modified_base 5: mod_base = OTHER; note = 2'-O-methylguanosine-3'-phosphate
  modified_base 6: mod_base = OTHER; note = 2'-O-methyluridine-3'-phosphate
  modified_base 7: mod_base = OTHER; note = 2'-O-methylguanosine-3'-phosphate
  modified_base 8: mod_base = OTHER; note = 2'-O-methylguanosine-3'-phosphate
  modified_base 9: mod_base = OTHER; note = 2'-fluoroadenosine-3'-phosphate
  modified_base 10: mod_base = OTHER; note = 2'-fluorocytidine-3'-phosphate
  modified_base 11: mod_base = OTHER; note = 2'-fluorouridine-3'-phosphate
  modified_base 12: mod_base = OTHER; note = 2'-O-methyluridine-3'-phosphate
  modified_base 13: mod_base = OTHER; note = 2'-O-methylcytidine-3'-phosphate
  modified_base 14: mod_base = OTHER; note = 2'-O-methyluridine-3'-phosphate
  modified_base 15: mod_base = OTHER; note = 2'-O-methylcytidine-3'-phosphate
  modified_base 16: mod_base = OTHER; note = 2'-O-methyluridine-3'-phosphate
  modified_base 17: mod_base = OTHER; note = 2'-O-methylcytidine-3'-phosphate
  modified_base 18: mod_base = OTHER; note = 2'-O-methyladenosine-3'-phosphate
  modified_base 19: mod_base = OTHER; note = 2'-O-methyladenosine-3'-phosphate
  modified_base 20: mod_base = OTHER; note = 2'-O-methyluridine-3'-phosphate
  modified_base 21: mod_base = OTHER; note = 2'-O-methyladenosine-3'-phosphorothioate
  modified_base 22: mod_base = OTHER; note = inverted (3'-3' linked) abasic deoxyribonucleotide
  misc_feature 1: note = RNA
  misc_feature 2: note = RNA
  misc_feature 3: note = RNA
  misc_feature 4: note = RNA
  misc_feature 5: note = RNA
  misc_feature 6: note = RNA
  misc_feature 7: note = RNA
  misc_feature 8: note = RNA
  misc_feature 9: note = DNA
  misc_feature 10: note = DNA
  misc_feature 11: note = DNA
  misc_feature 12: note = RNA
  misc_feature 13: note = RNA
  misc_feature 14: note = RNA
  misc_feature 15: note = RNA
  misc_feature 16: note = RNA
  misc_feature 17: note = RNA
  misc_feature 18: note = RNA
  misc_feature 19: note = RNA
  misc_feature 20: note = RNA
  misc_feature 21: note = RNA
  misc_feature 22: note = DNA
  source 1..22: mol_type = other RNA
cgtggtggacttctctcaatan

SEQ ID NO: 212 - RNA, 22 nt, synthetic construct
  modified_base 1: mod_base = OTHER; note = (NAG25)s-2'-O-methyluridine-3'-phosphorothioate
  modified_base 2: mod_base = OTHER; note = 2'-O-methylcytidine-3'-phosphate
  modified_base 3: mod_base = OTHER; note = 2'-O-methylguanosine-3'-phosphate
  modified_base 4: mod_base = OTHER; note = 2'-O-methyluridine-3'-phosphate
  modified_base 5: mod_base = OTHER; note = 2'-O-methylguanosine-3'-phosphate
  modified_base 6: mod_base = OTHER; note = 2'-O-methylguanosine-3'-phosphate
  modified_base 7: mod_base = OTHER; note = 2'-O-methyluridine-3'-phosphate
  modified_base 8: mod_base = OTHER; note = 2'-O-methylguanosine-3'-phosphate
  modified_base 9: mod_base = OTHER; note = 2'-fluoroguanosine-3'-phosphate
  modified_base 10: mod_base = OTHER; note = 2'-fluoroadenosine-3'-phosphate
  modified_base 11: mod_base = OTHER; note = 2'-fluorocytidine-3'-phosphate
  modified_base 12: mod_base = OTHER; note = 2'-O-methyluridine-3'-phosphate
  modified_base 13: mod_base = OTHER; note = 2'-O-methyluridine-3'-phosphate
  modified_base 14: mod_base = OTHER; note = 2'-O-methylcytidine-3'-phosphate
  modified_base 15: mod_base = OTHER; note = 2'-O-methyluridine-3'-phosphate
  modified_base 16: mod_base = OTHER; note = 2'-O-methylcytidine-3'-phosphate
  modified_base 17: mod_base = OTHER; note = 2'-O-methyluridine-3'-phosphate
  modified_base 18: mod_base = OTHER; note = 2'-O-methylcytidine-3'-phosphate
  modified_base 19: mod_base = OTHER; note = 2'-O-methyladenosine-3'-phosphate
  modified_base 20: mod_base = OTHER; note = 2'-O-methyladenosine-3'-phosphate
  modified_base 21: mod_base = OTHER; note = 2'-O-methyladenosine-3'-phosphorothioate
  modified_base 22: mod_base = OTHER; note = inverted (3'-3' linked) abasic deoxyribonucleotide
  misc_feature 1: note = RNA
  misc_feature 2: note = RNA
  misc_feature 3: note = RNA
  misc_feature 4: note = RNA
  misc_feature 5: note = RNA
  misc_feature 6: note = RNA
  misc_feature 7: note = RNA
  misc_feature 8: note = RNA
  misc_feature 9: note = DNA
  misc_feature 10: note = DNA
  misc_feature 11: note = DNA
  misc_feature 12: note = RNA
  misc_feature 13: note = RNA
  misc_feature 14: note = RNA
  misc_feature 15: note = RNA
  misc_feature 16: note = RNA
  misc_feature 17: note = RNA
  misc_feature 18: note = RNA
  misc_feature 19: note = RNA
  misc_feature 20: note = RNA
  misc_feature 21: note = RNA
  misc_feature 22: note = DNA
  source 1..22: mol_type = other RNA
tcgtggtggacttctctcaaan

SEQ ID NO: 213 - RNA, 22 nt, synthetic construct
  modified_base 1: mod_base = OTHER; note = (NAG31)s-2'-O-methyladenosine-3'-phosphorothioate
  modified_base 2: mod_base = OTHER; note = 2'-O-methylcytidine-3'-phosphate
  modified_base 3: mod_base = OTHER; note = 2'-O-methylcytidine-3'-phosphate
  modified_base 4: mod_base = OTHER; note = 2'-O-methyluridine-3'-phosphate
  modified_base 5: mod_base = OTHER; note = 2'-O-methylguanosine-3'-phosphate
  modified_base 6: mod_base = OTHER; note = 2'-O-methyluridine-3'-phosphate
  modified_base 7: mod_base = OTHER; note = 2'-O-methyladenosine-3'-phosphate
  modified_base 8: mod_base = OTHER; note = 2'-O-methylguanosine-3'-phosphate
  modified_base 9: mod_base = OTHER; note = 2'-fluoroguanosine-3'-phosphate
  modified_base 10: mod_base = OTHER; note = 2'-fluorocytidine-3'-phosphate
  modified_base 11: mod_base = OTHER; note = 2'-fluoroadenosine-3'-phosphate
  modified_base 12: mod_base = OTHER; note = 2'-O-methyluridine-3'-phosphate
  modified_base 13: mod_base = OTHER; note = 2'-O-methyladenosine-3'-phosphate
  modified_base 14: mod_base = OTHER; note = 2'-O-methyladenosine-3'-phosphate
  modified_base 15: mod_base = OTHER; note = 2'-O-methyladenosine-3'-phosphate
  modified_base 16: mod_base = OTHER; note = 2'-O-methyluridine-3'-phosphate
  modified_base 17: mod_base = OTHER; note = 2'-O-methyluridine-3'-phosphate
  modified_base 18: mod_base = OTHER; note = 2'-O-methylguanosine-3'-phosphate
  modified_base 19: mod_base = OTHER; note = 2'-O-methylguanosine-3'-phosphate
  modified_base 20: mod_base = OTHER; note = 2'-O-methyluridine-3'-phosphate
  modified_base 21: mod_base = OTHER; note = 2'-O-methyladenosine-3'-phosphorothioate
  modified_base 22: mod_base = OTHER; note = inverted (3'-3' linked) abasic deoxyribonucleotide
  misc_feature 1: note = RNA
  misc_feature 2: note = RNA
  misc_feature 3: note = RNA
  misc_feature 4: note = RNA
  misc_feature 5: note = RNA
  misc_feature 6: note = RNA
  misc_feature 7: note = RNA
  misc_feature 8: note = RNA
  misc_feature 9: note = DNA
  misc_feature 10: note = DNA
  misc_feature 11: note = DNA
  misc_feature 12: note = RNA
  misc_feature 13: note = RNA
  misc_feature 14: note = RNA
  misc_feature 15: note = RNA
  misc_feature 16: note = RNA
  misc_feature 17: note = RNA
  misc_feature 18: note = RNA
  misc_feature 19: note = RNA
  misc_feature 20: note = RNA
  misc_feature 21: note = RNA
  misc_feature 22: note = DNA
  source 1..22: mol_type = other RNA
acctgtaggcataaattggtan

SEQ ID NO: 214 - RNA, 21 nt, synthetic construct
  modified_base 1: mod_base = OTHER; note = (NAG31)s-inverted (3'-3' linked) abasic deoxyribonucleotide-5'-phosphorothioate
  modified_base 2: mod_base = OTHER; note = 2'-O-methylcytidine-3'-phosphate
  modified_base 3: mod_base = OTHER; note = 2'-O-methyluridine-3'-phosphate
  modified_base 4: mod_base = OTHER; note = 2'-O-methylguanosine-3'-phosphate
  modified_base 5: mod_base = OTHER; note = 2'-O-methyluridine-3'-phosphate
  modified_base 6: mod_base = OTHER; note = 2'-O-methyladenosine-3'-phosphate
  modified_base 7: mod_base = OTHER; note = 2'-O-methylguanosine-3'-phosphate
  modified_base 8: mod_base = OTHER; note = 2'-fluoroguanosine-3'-phosphate
  modified_base 9: mod_base = OTHER; note = 2'-fluorocytidine-3'-phosphate
  modified_base 10: mod_base = OTHER; note = 2'-fluoroadenosine-3'-phosphate
  modified_base 11: mod_base = OTHER; note = 2'-O-methyluridine-3'-phosphate
  modified_base 12: mod_base = OTHER; note = 2'-O-methyladenosine-3'-phosphate
  modified_base 13: mod_base = OTHER; note = 2'-O-methyladenosine-3'-phosphate
  modified_base 14: mod_base = OTHER; note = 2'-O-methyladenosine-3'-phosphate
  modified_base 15: mod_base = OTHER; note = 2'-O-methyluridine-3'-phosphate
  modified_base 16: mod_base = OTHER; note = 2'-O-methyluridine-3'-phosphate
  modified_base 17: mod_base = OTHER; note = 2'-O-methylguanosine-3'-phosphate
  modified_base 18: mod_base = OTHER; note = 2'-O-methylguanosine-3'-phosphate
  modified_base 19: mod_base = OTHER; note = 2'-O-methyluridine-3'-phosphate
  modified_base 20: mod_base = OTHER; note = 2'-O-methyladenosine-3'-phosphorothioate
  modified_base 21: mod_base = OTHER; note = inverted (3'-3' linked) abasic deoxyribonucleotide
  misc_feature 1: note = DNA
  misc_feature 2: note = RNA
  misc_feature 3: note = RNA
  misc_feature 4: note = RNA
  misc_feature 5: note = RNA
  misc_feature 6: note = RNA
  misc_feature 7: note = RNA
  misc_feature 8: note = DNA
  misc_feature 9: note = DNA
  misc_feature 10: note = DNA
  misc_feature 11: note = RNA
  misc_feature 12: note = RNA
  misc_feature 13: note = RNA
  misc_feature 14: note = RNA
  misc_feature 15: note = RNA
  misc_feature 16: note = RNA
  misc_feature 17: note = RNA
  misc_feature 18: note = RNA
  misc_feature 19: note = RNA
  misc_feature 20: note = RNA
  misc_feature 21: note = DNA
  source 1..21: mol_type = other RNA
nctgtaggcataaattggtan

SEQ ID NO: 215 - RNA, 21 nt, synthetic construct
  modified_base 1: mod_base = OTHER; note = (NAG25)s-inverted (3'-3' linked) abasic deoxyribonucleotide-5'-phosphorothioate
  modified_base 2: mod_base = OTHER; note = 2'-O-methylcytidine-3'-phosphate
  modified_base 3: mod_base = OTHER; note = 2'-O-methyluridine-3'-phosphate
  modified_base 4: mod_base = OTHER; note = 2'-O-methylguanosine-3'-phosphate
  modified_base 5: mod_base = OTHER; note = 2'-O-methyluridine-3'-phosphate
  modified_base 6: mod_base = OTHER; note = 2'-O-methyladenosine-3'-phosphate
  modified_base 7: mod_base = OTHER; note = 2'-O-methylguanosine-3'-phosphate
  modified_base 8: mod_base = OTHER; note = 2'-fluoroguanosine-3'-phosphate
  modified_base 9: mod_base = OTHER; note = 2'-fluorocytidine-3'-phosphate
  modified_base 10: mod_base = OTHER; note = 2'-fluoroadenosine-3'-phosphate
  modified_base 11: mod_base = OTHER; note = 2'-O-methyluridine-3'-phosphate
  modified_base 12: mod_base = OTHER; note = 2'-O-methyladenosine-3'-phosphate
  modified_base 13: mod_base = OTHER; note = 2'-O-methyladenosine-3'-phosphate
  modified_base 14: mod_base = OTHER; note = 2'-O-methyladenosine-3'-phosphate
  modified_base 15: mod_base = OTHER; note = 2'-O-methyluridine-3'-phosphate
  modified_base 16: mod_base = OTHER; note = 2'-O-methyluridine-3'-phosphate
  modified_base 17: mod_base = OTHER; note = 2'-O-methylguanosine-3'-phosphate
  modified_base 18: mod_base = OTHER; note = 2'-O-methylguanosine-3'-phosphate
  modified_base 19: mod_base = OTHER; note = 2'-O-methyluridine-3'-phosphate
  modified_base 20: mod_base = OTHER; note = 2'-O-methyladenosine-3'-phosphorothioate
  modified_base 21: mod_base = OTHER; note = inverted (3'-3' linked) abasic deoxyribonucleotide
  misc_feature 1: note = DNA
  misc_feature 2: note = RNA
  misc_feature 3: note = RNA
  misc_feature 4: note = RNA
  misc_feature 5: note = RNA
  misc_feature 6: note = RNA
  misc_feature 7: note = RNA
  misc_feature 8: note = DNA
  misc_feature 9: note = DNA
  misc_feature 10: note = DNA
  misc_feature 11: note = RNA
  misc_feature 12: note = RNA
  misc_feature 13: note = RNA
  misc_feature 14: note = RNA
  misc_feature 15: note = RNA
  misc_feature 16: note = RNA
  misc_feature 17: note = RNA
  misc_feature 18: note = RNA
  misc_feature 19: note = RNA
  misc_feature 20: note = RNA
  misc_feature 21: note = DNA
  source 1..21: mol_type = other RNA
nctgtaggcataaattggtan

SEQ ID NO: 216 - RNA, 21 nt, synthetic construct
  modified_base 1: mod_base = OTHER; note = (NAG37)s-inverted (3'-3' linked) abasic deoxyribonucleotide-5'-phosphorothioate
  modified_base 2: mod_base = OTHER; note = 2'-O-methylcytidine-3'-phosphate
  modified_base 3: mod_base = OTHER; note = 2'-O-methyluridine-3'-phosphate
  modified_base 4: mod_base = OTHER; note = 2'-O-methylguanosine-3'-phosphate
  modified_base 5: mod_base = OTHER; note = 2'-O-methyluridine-3'-phosphate
  modified_base 6: mod_base = OTHER; note = 2'-O-methyladenosine-3'-phosphate
  modified_base 7: mod_base = OTHER; note = 2'-O-methylguanosine-3'-phosphate
  modified_base 8: mod_base = OTHER; note = 2'-fluoroguanosine-3'-phosphate
  modified_base 9: mod_base = OTHER; note = 2'-fluorocytidine-3'-phosphate
  modified_base 10: mod_base = OTHER; note = 2'-fluoroadenosine-3'-phosphate
  modified_base 11: mod_base = OTHER; note = 2'-O-methyluridine-3'-phosphate
  modified_base 12: mod_base = OTHER; note = 2'-O-methyladenosine-3'-phosphate
  modified_base 13: mod_base = OTHER; note = 2'-O-methyladenosine-3'-phosphate
  modified_base 14: mod_base = OTHER; note = 2'-O-methyladenosine-3'-phosphate
  modified_base 15: mod_base = OTHER; note = 2'-O-methyluridine-3'-phosphate
  modified_base 16: mod_base = OTHER; note = 2'-O-methyluridine-3'-phosphate
  modified_base 17: mod_base = OTHER; note = 2'-O-methylguanosine-3'-phosphate
  modified_base 18: mod_base = OTHER; note = 2'-O-methylguanosine-3'-phosphate
  modified_base 19: mod_base = OTHER; note = 2'-O-methyluridine-3'-phosphate
  modified_base 20: mod_base = OTHER; note = 2'-O-methyladenosine-3'-phosphorothioate
  modified_base 21: mod_base = OTHER; note = inverted (3'-3' linked) abasic deoxyribonucleotide
  misc_feature 1: note = DNA
  misc_feature 2: note = RNA
  misc_feature 3: note = RNA
  misc_feature 4: note = RNA
  misc_feature 5: note = RNA
  misc_feature 6: note = RNA
  misc_feature 7: note = RNA
  misc_feature 8: note = DNA
  misc_feature 9: note = DNA
  misc_feature 10: note = DNA
  misc_feature 11: note = RNA
  misc_feature 12: note = RNA
  misc_feature 13: note = RNA
  misc_feature 14: note = RNA
  misc_feature 15: note = RNA
  misc_feature 16: note = RNA
  misc_feature 17: note = RNA
  misc_feature 18: note = RNA
  misc_feature 19: note = RNA
  misc_feature 20: note = RNA
  misc_feature 21: note = DNA
  source 1..21: mol_type = other RNA
nctgtaggcataaattggtan

SEQ ID NO: 217 - RNA, 22 nt, synthetic construct
  modified_base 1: mod_base = OTHER; note = (NAG25)s-inverted (3'-3' linked) abasic deoxyribonucleotide-5'-phosphorothioate
  modified_base 2: mod_base = OTHER; note = 2'-O-methyladenosine-3'-phosphate
  modified_base 3: mod_base = OTHER; note = 2'-O-methylcytidine-3'-phosphate
  modified_base 4: mod_base = OTHER; note = 2'-O-methyluridine-3'-phosphate
  modified_base 5: mod_base = OTHER; note = 2'-O-methylguanosine-3'-phosphate
  modified_base 6: mod_base = OTHER; note = 2'-O-methyluridine-3'-phosphate
  modified_base 7: mod_base = OTHER; note = 2'-O-methyladenosine-3'-phosphate
  modified_base 8: mod_base = OTHER; note = 2'-O-methylguanosine-3'-phosphate
  modified_base 9: mod_base = OTHER; note = 2'-fluoroguanosine-3'-phosphate
  modified_base 10: mod_base = OTHER; note = 2'-fluorocytidine-3'-phosphate
  modified_base 11: mod_base = OTHER; note = 2'-fluoroadenosine-3'-phosphate
  modified_base 12: mod_base = OTHER; note = 2'-O-methyluridine-3'-phosphate
  modified_base 13: mod_base = OTHER; note = 2'-O-methyladenosine-3'-phosphate
  modified_base 14: mod_base = OTHER; note = 2'-O-methyladenosine-3'-phosphate
  modified_base 15: mod_base = OTHER; note = 2'-O-methyladenosine-3'-phosphate
  modified_base 16: mod_base = OTHER; note = 2'-O-methyluridine-3'-phosphate
  modified_base 17: mod_base = OTHER; note = 2'-O-methyluridine-3'-phosphate
  modified_base 18: mod_base = OTHER; note = 2'-O-methylguanosine-3'-phosphate
  modified_base 19: mod_base = OTHER; note = 2'-O-methylguanosine-3'-phosphate
  modified_base 20: mod_base = OTHER; note = 2'-O-methyluridine-3'-phosphate
  modified_base 21: mod_base = OTHER; note = 2'-O-methyladenosine-3'-phosphorothioate
  modified_base 22: mod_base = OTHER; note = inverted (3'-3' linked) abasic deoxyribonucleotide
  misc_feature 1: note = DNA
  misc_feature 2: note = RNA
  misc_feature 3: note = RNA
  misc_feature 4: note = RNA
  misc_feature 5: note = RNA
  misc_feature 6: note = RNA
  misc_feature 7: note = RNA
  misc_feature 8: note = RNA
  misc_feature 9: note = DNA
  misc_feature 10: note = DNA
  misc_feature 11: note = DNA
  misc_feature 12: note = RNA
  misc_feature 13: note = RNA
  misc_feature 14: note = RNA
  misc_feature 15: note = RNA
  misc_feature 16: note = RNA
  misc_feature 17: note = RNA
  misc_feature 18: note = RNA
  misc_feature 19: note = RNA
  misc_feature 20: note = RNA
  misc_feature 21: note = RNA
  misc_feature 22: note = DNA
  source 1..22: mol_type = other RNA
nactgtaggcataaattggtan

SEQ ID NO: 218 - RNA, 22 nt, synthetic construct
  modified_base 1: mod_base = OTHER; note = (NAG25)s-2'-O-methylguanosine-3'-phosphorothioate
  modified_base 2: mod_base = OTHER; note = 2'-O-methylguanosine-3'-phosphate
  modified_base 3: mod_base = OTHER; note = 2'-O-methylcytidine-3'-phosphate
  modified_base 4: mod_base = OTHER; note = 2'-O-methyluridine-3'-phosphate
  modified_base 5: mod_base = OTHER; note = 2'-O-methylguanosine-3'-phosphate
  modified_base 6: mod_base = OTHER; note = 2'-O-methyluridine-3'-phosphate
  modified_base 7: mod_base = OTHER; note = 2'-O-methyladenosine-3'-phosphate
  modified_base 8: mod_base = OTHER; note = 2'-O-methylguanosine-3'-phosphate
  modified_base 9: mod_base = OTHER; note = 2'-fluoroguanosine-3'-phosphate
  modified_base 10: mod_base = OTHER; note = 2'-fluorocytidine-3'-phosphate
  modified_base 11: mod_base = OTHER; note = 2'-fluoroadenosine-3'-phosphate
  modified_base 12: mod_base = OTHER; note = 2'-O-methyluridine-3'-phosphate
  modified_base 13: mod_base = OTHER; note = 2'-O-methyladenosine-3'-phosphate
  modified_base 14: mod_base = OTHER; note = 2'-O-methyladenosine-3'-phosphate
  modified_base 15: mod_base = OTHER; note = 2'-O-methyladenosine-3'-phosphate
  modified_base 16: mod_base = OTHER; note = 2'-O-methyluridine-3'-phosphate
  modified_base 17: mod_base = OTHER; note = 2'-O-methyluridine-3'-phosphate
  modified_base 18: mod_base = OTHER; note = 2'-O-methylguanosine-3'-phosphate
  modified_base 19: mod_base = OTHER; note = 2'-O-methylguanosine-3'-phosphate
  modified_base 20: mod_base = OTHER; note = 2'-O-methyluridine-3'-phosphate
  modified_base 21: mod_base = OTHER; note = 2'-O-methyladenosine-3'-phosphorothioate
  modified_base 22: mod_base = OTHER; note = inverted (3'-3' linked) abasic deoxyribonucleotide
  misc_feature 1: note = RNA
  misc_feature 2: note = RNA
  misc_feature 3: note = RNA
  misc_feature 4: note = RNA
  misc_feature 5: note = RNA
  misc_feature 6: note = RNA
  misc_feature 7: note = RNA
  misc_feature 8: note = RNA
  misc_feature 9: note = DNA
  misc_feature 10: note = DNA
  misc_feature 11: note = DNA
  misc_feature 12: note = RNA
  misc_feature 13: note = RNA
  misc_feature 14: note = RNA
  misc_feature 15: note = RNA
  misc_feature 16: note = RNA
  misc_feature 17: note = RNA
  misc_feature 18: note = RNA
  misc_feature 19: note = RNA
  misc_feature 20: note = RNA
  misc_feature 21: note = RNA
  misc_feature 22: note = DNA
  source 1..22: mol_type = other RNA
ggctgtaggcataaattggtan

SEQ ID NO: 219 - RNA, 22 nt, synthetic construct
  modified_base 1: mod_base = OTHER; note = (NAG37)s-2'-O-methyladenosine-3'-phosphorothioate
  modified_base 2: mod_base = OTHER; note = 2'-O-methyladenosine-3'-phosphate
  modified_base 3: mod_base = OTHER; note = 2'-O-methylguanosine-3'-phosphate
  modified_base 4: mod_base = OTHER; note = 2'-O-methyluridine-3'-phosphate
  modified_base 5: mod_base = OTHER; note = 2'-O-methylguanosine-3'-phosphate
  modified_base 6: mod_base = OTHER; note = 2'-O-methylguanosine-3'-phosphate
  modified_base 7: mod_base = OTHER; note = 2'-O-methyluridine-3'-phosphate
  modified_base 8: mod_base = OTHER; note = 2'-O-methylguanosine-3'-phosphate
  modified_base 9: mod_base = OTHER; note = 2'-fluoroguanosine-3'-phosphate
  modified_base 10: mod_base = OTHER; note = 2'-fluoroadenosine-3'-phosphate
  modified_base 11: mod_base = OTHER; note = 2'-fluorocytidine-3'-phosphate
  modified_base 12: mod_base = OTHER; note = 2'-O-methyluridine-3'-phosphate
  modified_base 13: mod_base = OTHER; note = 2'-O-methyluridine-3'-phosphate
  modified_base 14: mod_base = OTHER; note = 2'-O-methylcytidine-3'-phosphate
  modified_base 15: mod_base = OTHER; note = 2'-O-methyluridine-3'-phosphate
  modified_base 16: mod_base = OTHER; note = 2'-O-methylcytidine-3'-phosphate
  modified_base 17: mod_base = OTHER; note = 2'-O-methyluridine-3'-phosphate
  modified_base 18: mod_base = OTHER; note = 2'-O-methylcytidine-3'-phosphate
  modified_base 19: mod_base = OTHER; note = 2'-O-methyladenosine-3'-phosphate
  modified_base 20: mod_base = OTHER; note = 2'-O-methyladenosine-3'-phosphate
  modified_base 21: mod_base = OTHER; note = 2'-O-methyluridine-3'-phosphorothioate
  modified_base 22: mod_base = OTHER; note = inverted (3'-3' linked) abasic deoxyribonucleotide
  misc_feature 1: note = RNA
  misc_feature 2: note = RNA
  misc_feature 3: note = RNA
  misc_feature 4: note = RNA
  misc_feature 5: note = RNA
  misc_feature 6: note = RNA
  misc_feature 7: note = RNA
  misc_feature 8: note = RNA
  misc_feature 9: note = DNA
  misc_feature 10: note = DNA
  misc_feature 11: note = DNA
  misc_feature 12: note = RNA
  misc_feature 13: note = RNA
  misc_feature 14: note = RNA
  misc_feature 15: note = RNA
  misc_feature 16: note = RNA
  misc_feature 17: note = RNA
  misc_feature 18: note = RNA
  misc_feature 19: note = RNA
  misc_feature 20: note = RNA
  misc_feature 21: note = RNA
  misc_feature 22: note = DNA
  source 1..22: mol_type = other RNA
aagtggtggacttctctcaatn

SEQ ID NO: 220 - RNA, 22 nt, synthetic construct
  modified_base 1: mod_base = OTHER; note = (NAG25)s-2'-O-methyladenosine-3'-phosphorothioate
  modified_base 2: mod_base = OTHER; note = 2'-O-methyladenosine-3'-phosphate
  modified_base 3: mod_base = OTHER; note = 2'-O-methylguanosine-3'-phosphate
  modified_base 4: mod_base = OTHER; note = 2'-O-methyluridine-3'-phosphate
  modified_base 5: mod_base = OTHER; note = 2'-O-methylguanosine-3'-phosphate
  modified_base 6: mod_base = OTHER; note = 2'-O-methylguanosine-3'-phosphate
  modified_base 7: mod_base = OTHER; note = 2'-O-methyluridine-3'-phosphate
  modified_base 8: mod_base = OTHER; note = 2'-O-methylguanosine-3'-phosphate
  modified_base 9: mod_base = OTHER; note = 2'-fluoroguanosine-3'-phosphate
  modified_base 10: mod_base = OTHER; note = 2'-fluoroadenosine-3'-phosphate
  modified_base 11: mod_base = OTHER; note = 2'-fluorocytidine-3'-phosphate
  modified_base 12: mod_base = OTHER; note = 2'-O-methyluridine-3'-phosphate
  modified_base 13: mod_base = OTHER; note = 2'-O-methyluridine-3'-phosphate
  modified_base 14: mod_base = OTHER; note = 2'-O-methylcytidine-3'-phosphate
  modified_base 15: mod_base = OTHER; note = 2'-O-methyluridine-3'-phosphate
  modified_base 16: mod_base = OTHER; note = 2'-O-methylcytidine-3'-phosphate
  modified_base 17: mod_base = OTHER; note = 2'-O-methyluridine-3'-phosphate
  modified_base 18: mod_base = OTHER; note = 2'-O-methylcytidine-3'-phosphate
  modified_base 19: mod_base = OTHER; note = 2'-O-methyladenosine-3'-phosphate
  modified_base 20: mod_base = OTHER; note = 2'-O-methyladenosine-3'-phosphate
  modified_base 21: mod_base = OTHER; note = 2'-O-methyladenosine-3'-phosphorothioate
  modified_base 22: mod_base = OTHER; note = inverted (3'-3' linked) abasic deoxyribonucleotide
  misc_feature 1: note = RNA
  misc_feature 2: note = RNA
  misc_feature 3: note = RNA
  misc_feature 4: note = RNA
  misc_feature 5: note = RNA
  misc_feature 6: note = RNA
  misc_feature 7: note = RNA
  misc_feature 8: note = RNA
  misc_feature 9: note = DNA
  misc_feature 10: note = DNA
  misc_feature 11: note = DNA
  misc_feature 12: note = RNA
  misc_feature 13: note = RNA
  misc_feature 14: note = RNA
  misc_feature 15: note = RNA
  misc_feature 16: note = RNA
  misc_feature 17: note = RNA
  misc_feature 18: note = RNA
  misc_feature 19: note = RNA
  misc_feature 20: note = RNA
  misc_feature 21: note = RNA
  misc_feature 22: note = DNA
  source 1..22: mol_type = other RNA
aagtggtggacttctctcaaan

SEQ ID NO: 221 - RNA, 22 nt, synthetic construct
  modified_base 1: mod_base = OTHER; note = (NAG25)s-2'-O-methylcytidine-3'-phosphorothioate
  modified_base 2: mod_base = OTHER; note = 2'-O-methylcytidine-3'-phosphate
  modified_base 3: mod_base = OTHER; note = 2'-O-methylguanosine-3'-phosphate
  modified_base 4: mod_base = OTHER; note = 2'-O-methyluridine-3'-phosphate
  modified_base 5: mod_base = OTHER; note = 2'-O-methylguanosine-3'-phosphate
  modified_base 6: mod_base = OTHER; note = 2'-O-methylguanosine-3'-phosphate
  modified_base 7: mod_base = OTHER; note = 2'-O-methyluridine-3'-phosphate
  modified_base 8: mod_base = OTHER; note = 2'-O-methylguanosine-3'-phosphate
  modified_base 9: mod_base = OTHER; note = 2'-fluoroguanosine-3'-phosphate
  modified_base 10: mod_base = OTHER; note = 2'-fluoroadenosine-3'-phosphate
  modified_base 11: mod_base = OTHER; note = 2'-fluorocytidine-3'-phosphate
  modified_base 12: mod_base = OTHER; note = 2'-O-methyluridine-3'-phosphate
  modified_base 13: mod_base = OTHER; note = 2'-O-methyluridine-3'-phosphate
  modified_base 14: mod_base = OTHER; note = 2'-O-methylcytidine-3'-phosphate
  modified_base 15: mod_base = OTHER; note = 2'-O-methyluridine-3'-phosphate
  modified_base 16: mod_base = OTHER; note = 2'-O-methylcytidine-3'-phosphate
  modified_base 17: mod_base = OTHER; note = 2'-O-methyluridine-3'-phosphate
  modified_base 18: mod_base = OTHER; note = 2'-O-methylcytidine-3'-phosphate
  modified_base 19: mod_base = OTHER; note = 2'-O-methyladenosine-3'-phosphate
  modified_base 20: mod_base = OTHER; note = 2'-O-methyladenosine-3'-phosphate
  modified_base 21: mod_base = OTHER; note = 2'-O-methyluridine-3'-phosphorothioate
  modified_base 22: mod_base = OTHER; note = inverted (3'-3' linked) abasic deoxyribonucleotide
  misc_feature 1: note = RNA
  misc_feature 2: note = RNA
  misc_feature 3: note = RNA
  misc_feature 4: note = RNA
  misc_feature 5: note = RNA
  misc_feature 6: note = RNA
  misc_feature 7: note = RNA
  misc_feature 8: note = RNA
  misc_feature 9: note = DNA
  misc_feature 10: note = DNA
  misc_feature 11: note = DNA
  misc_feature 12: note = RNA
  misc_feature 13: note = RNA
  misc_feature 14: note = RNA
  misc_feature 15: note = RNA
  misc_feature 16: note = RNA
  misc_feature 17: note = RNA
  misc_feature 18: note = RNA
  misc_feature 19: note = RNA
  misc_feature 20: note = RNA
  misc_feature 21: note = RNA
  misc_feature 22: note = DNA
  source 1..22: mol_type = other RNA
ccgtggtggacttctctcaatn

SEQ ID NO: 222 - RNA, 23 nt, synthetic construct
  modified_base 1: mod_base = OTHER; note = (NAG25)s-inverted (3'-3' linked) abasic deoxyribonucleotide-5'-phosphorothioate
  modified_base 2: mod_base = OTHER; note = 2'-O-methylcytidine-3'-phosphate
  modified_base 3: mod_base = OTHER; note = 2'-O-methylcytidine-3'-phosphate
  modified_base 4: mod_base = OTHER; note = 2'-O-methylguanosine-3'-phosphate
  modified_base 5: mod_base = OTHER; note = 2'-O-methyluridine-3'-phosphate
  modified_base 6: mod_base = OTHER; note = 2'-O-methylguanosine-3'-phosphate
  modified_base 7: mod_base = OTHER; note = 2'-O-methylguanosine-3'-phosphate
  modified_base 8: mod_base = OTHER; note = 2'-O-methyluridine-3'-phosphate
  modified_base 9: mod_base = OTHER; note = 2'-O-methylguanosine-3'-phosphate
  modified_base 10: mod_base = OTHER; note = 2'-fluoroguanosine-3'-phosphate
  modified_base 11: mod_base = OTHER; note = 2'-fluoroadenosine-3'-phosphate
  modified_base 12: mod_base = OTHER; note = 2'-fluorocytidine-3'-phosphate
  modified_base 13: mod_base = OTHER; note = 2'-O-methyluridine-3'-phosphate
  modified_base 14: mod_base = OTHER; note = 2'-O-methyluridine-3'-phosphate
  modified_base 15: mod_base = OTHER; note = 2'-O-methylcytidine-3'-phosphate
  modified_base 16: mod_base = OTHER; note = 2'-O-methyluridine-3'-phosphate
  modified_base 17: mod_base = OTHER; note = 2'-O-methylcytidine-3'-phosphate
  modified_base 18: mod_base = OTHER; note = 2'-O-methyluridine-3'-phosphate
  modified_base 19: mod_base = OTHER; note = 2'-O-methylcytidine-3'-phosphate
  modified_base 20: mod_base = OTHER; note = 2'-O-methyladenosine-3'-phosphate
  modified_base 21: mod_base = OTHER; note = 2'-O-methyladenosine-3'-phosphate
  modified_base 22: mod_base = OTHER; note = 2'-O-methyluridine-3'-phosphorothioate
  modified_base 23: mod_base = OTHER; note = inverted (3'-3' linked) abasic deoxyribonucleotide
  misc_feature 1: note = DNA
  misc_feature 2: note = RNA
  misc_feature 3: note = RNA
  misc_feature 4: note = RNA
  misc_feature 5: note = RNA
  misc_feature 6: note = RNA
  misc_feature 7: note = RNA
  misc_feature 8: note = RNA
  misc_feature 9: note = RNA
  misc_feature 10: note = DNA
  misc_feature 11: note = DNA
  misc_feature 12: note = DNA
  misc_feature 13: note = RNA
  misc_feature 14: note = RNA
  misc_feature 15: note = RNA
  misc_feature 16: note = RNA
  misc_feature 17: note = RNA
  misc_feature 18: note = RNA
  misc_feature 19: note = RNA
  misc_feature 20: note = RNA
  misc_feature 21: note = RNA
  misc_feature 22: note = RNA
  misc_feature 23: note = DNA
  source 1..23: mol_type = other RNA
nccgtggtggacttctctcaatn

SEQ ID NO: 223 - RNA, 23 nt, synthetic construct
  modified_base 1: mod_base = OTHER; note = (NAG25)s-2'-O-methylcytidine-3'-phosphorothioate
  modified_base 2: mod_base = OTHER; note = 2'-O-methyluridine-3'-phosphate
  modified_base 3: mod_base = OTHER; note = 2'-O-methylcytidine-3'-phosphate
  modified_base 4: mod_base = OTHER; note = 2'-O-methylguanosine-3'-phosphate
  modified_base 5: mod_base = OTHER; note = 2'-O-methyluridine-3'-phosphate
  modified_base 6: mod_base = OTHER; note = 2'-O-methylguanosine-3'-phosphate
  modified_base 7: mod_base = OTHER; note = 2'-O-methylguanosine-3'-phosphate
  modified_base 8: mod_base = OTHER; note = 2'-O-methyluridine-3'-phosphate
  modified_base 9: mod_base = OTHER; note = 2'-O-methylguanosine-3'-phosphate
  modified_base 10: mod_base = OTHER; note = 2'-fluoroguanosine-3'-phosphate
  modified_base 11: mod_base = OTHER; note = 2'-fluoroadenosine-3'-phosphate
  modified_base 12: mod_base = OTHER; note = 2'-fluorocytidine-3'-phosphate
  modified_base 13: mod_base = OTHER; note = 2'-O-methyluridine-3'-phosphate
  modified_base 14: mod_base = OTHER; note = 2'-O-methyluridine-3'-phosphate
  modified_base 15: mod_base = OTHER; note = 2'-O-methylcytidine-3'-phosphate
  modified_base 16: mod_base = OTHER; note = 2'-O-methyluridine-3'-phosphate
  modified_base 17: mod_base = OTHER; note = 2'-O-methylcytidine-3'-phosphate
  modified_base 18: mod_base = OTHER; note = 2'-O-methyluridine-3'-phosphate
  modified_base 19: mod_base = OTHER; note = 2'-O-methylcytidine-3'-phosphate
  modified_base 20: mod_base = OTHER; note = 2'-O-methyladenosine-3'-phosphate
  modified_base 21: mod_base = OTHER; note = 2'-O-methyladenosine-3'-phosphate
  modified_base 22: mod_base = OTHER; note = 2'-O-methyluridine-3'-phosphorothioate
  modified_base 23: mod_base = OTHER; note = inverted (3'-3' linked) abasic deoxyribonucleotide
  misc_feature 1: note = RNA
  misc_feature 2: note = RNA
  misc_feature 3: note = RNA
  misc_feature 4: note = RNA
  misc_feature 5: note = RNA
  misc_feature 6: note = RNA
  misc_feature 7: note = RNA
  misc_feature 8: note = RNA
  misc_feature 9: note = RNA
  misc_feature 10: note = DNA
  misc_feature 11: note = DNA
  misc_feature 12: note = DNA
  misc_feature 13: note = RNA
  misc_feature 14: note = RNA
  misc_feature 15: note = RNA
  misc_feature 16: note = RNA
  misc_feature 17: note = RNA
  misc_feature 18: note = RNA
  misc_feature 19: note = RNA
  misc_feature 20: note = RNA
  misc_feature 21: note = RNA
  misc_feature 22: note = RNA
  misc_feature 23: note = DNA
  source 1..23: mol_type = other RNA
ctcgtggtggacttctctcaatn

SEQ ID NO: 224 - RNA, 21 nt, synthetic construct
  modified_base 1: mod_base = OTHER; note = (NAG25)s-inverted (3'-3' linked) abasic deoxyribonucleotide-5'-phosphorothioate
  modified_base 2: mod_base = OTHER; note = 2'-O-methylguanosine-3'-phosphate
  modified_base 3: mod_base = OTHER; note = 2'-O-methyluridine-3'-phosphate
  modified_base 4: mod_base = OTHER; note = 2'-O-methylguanosine-3'-phosphate
  modified_base 5: mod_base = OTHER; note = 2'-O-methylguanosine-3'-phosphate
  modified_base 6: mod_base = OTHER; note = 2'-O-methyluridine-3'-phosphate
  modified_base 7: mod_base = OTHER; note = 2'-O-methylguanosine-3'-phosphate
  modified_base 8: mod_base = OTHER; note = 2'-fluoroguanosine-3'-phosphate
  modified_base 9: mod_base = OTHER; note = 2'-fluoroadenosine-3'-phosphate
  modified_base 10: mod_base = OTHER; note = 2'-fluorocytidine-3'-phosphate
  modified_base 11: mod_base = OTHER; note = 2'-O-methyluridine-3'-phosphate
  modified_base 12: mod_base = OTHER; note = 2'-O-methyluridine-3'-phosphate
  modified_base 13: mod_base = OTHER; note = 2'-O-methylcytidine-3'-phosphate
  modified_base 14: mod_base = OTHER; note = 2'-O-methyluridine-3'-phosphate
  modified_base 15: mod_base = OTHER; note = 2'-O-methylcytidine-3'-phosphate
  modified_base 16: mod_base = OTHER; note = 2'-O-methyluridine-3'-phosphate
  modified_base 17: mod_base = OTHER; note = 2'-O-methylcytidine-3'-phosphate
  modified_base 18: mod_base = OTHER; note = 2'-O-methyladenosine-3'-phosphate
  modified_base 19: mod_base = OTHER; note = 2'-O-methyladenosine-3'-phosphate
  modified_base 20: mod_base = OTHER; note = 2'-O-methyluridine-3'-phosphorothioate
  modified_base 21: mod_base = OTHER; note = inverted (3'-3' linked) abasic deoxyribonucleotide
  misc_feature 1: note = DNA
  misc_feature 2: note = RNA
  misc_feature 3: note = RNA
  misc_feature 4: note = RNA
  misc_feature 5: note = RNA
  misc_feature 6: note = RNA
  misc_feature 7: note = RNA
  misc_feature 8: note = DNA
  misc_feature 9: note = DNA
  misc_feature 10: note = DNA
  misc_feature 11: note = RNA
  misc_feature 12: note = RNA
  misc_feature 13: note = RNA
  misc_feature 14: note = RNA
  misc_feature 15: note = RNA
  misc_feature 16: note = RNA
  misc_feature 17: note = RNA
  misc_feature 18: note = RNA
  misc_feature 19: note = RNA
  misc_feature 20: note = RNA
  misc_feature 21: note = DNA
  source 1..21: mol_type = other RNA
ngtggtggacttctctcaatn

SEQ ID NO: 225 - RNA, 23 nt, synthetic construct
  modified_base 1: mod_base = OTHER; note = (NAG25)s-inverted (3'-3' linked) abasic deoxyribonucleotide-5'-phosphorothioate
  modified_base 2: mod_base = OTHER; note = 2'-O-methylguanosine-3'-phosphate
  modified_base 3: mod_base = OTHER; note = 2'-O-methyluridine-3'-phosphate
  modified_base 4: mod_base = OTHER; note = 2'-O-methylguanosine-3'-phosphate
  modified_base 5: mod_base = OTHER; note = 2'-O-methylguanosine-3'-phosphate
  modified_base 6: mod_base = OTHER; note = 2'-O-methyluridine-3'-phosphate
  modified_base 7: mod_base = OTHER; note = 2'-O-methylguanosine-3'-phosphate
  modified_base 8: mod_base = OTHER; note = 2'-fluoroguanosine-3'-phosphate
  modified_base 9: mod_base = OTHER; note = 2'-fluoroadenosine-3'-phosphate
  modified_base 10: mod_base = OTHER; note = 2'-fluorocytidine-3'-phosphate
  modified_base 11: mod_base = OTHER; note = 2'-O-methyluridine-3'-phosphate
  modified_base 12: mod_base = OTHER; note = 2'-O-methyluridine-3'-phosphate
  modified_base 13: mod_base = OTHER; note = 2'-O-methylcytidine-3'-phosphate
  modified_base 14: mod_base = OTHER; note = 2'-O-methyluridine-3'-phosphate
  modified_base 15: mod_base = OTHER; note = 2'-O-methylcytidine-3'-phosphate
  modified_base 16: mod_base = OTHER; note = 2'-O-methyluridine-3'-phosphate
  modified_base 17: mod_base = OTHER; note = 2'-O-methylcytidine-3'-phosphate
  modified_base 18: mod_base = OTHER; note = 2'-O-methyladenosine-3'-phosphate
  modified_base 19: mod_base = OTHER; note = 2'-O-methyladenosine-3'-phosphate
  modified_base 20: mod_base = OTHER; note = 2'-O-methyluridine-3'-phosphate
  modified_base 21: mod_base = OTHER; note = 2'-O-methyluridine-3'-phosphorothioate
  modified_base 22: mod_base = OTHER; note = 2'-O-methyluridine-3'-phosphate
  modified_base 23: mod_base = OTHER; note = inverted (3'-3' linked) abasic deoxyribonucleotide
  misc_feature 1: note = DNA
  misc_feature 2: note = RNA
  misc_feature 3: note = RNA
  misc_feature 4: note = RNA
  misc_feature 5: note = RNA
  misc_feature 6: note = RNA
  misc_feature 7: note = RNA
  misc_feature 8: note = DNA
  misc_feature 9: note = DNA
  misc_feature 10: note = DNA
  misc_feature 11: note = RNA
  misc_feature 12: note = RNA
  misc_feature 13: note = RNA
  misc_feature 14: note = RNA
  misc_feature 15: note = RNA
  misc_feature 16: note = RNA
  misc_feature 17: note = RNA
  misc_feature 18: note = RNA
  misc_feature 19: note = RNA
  misc_feature 20: note = RNA
  misc_feature 21: note = RNA
  misc_feature 22: note = RNA
  misc_feature 23: note = DNA
  source 1..23: mol_type = other RNA
ngtggtggacttctctcaatttn

SEQ ID NO: 226 - RNA, 23 nt, synthetic construct
  modified_base 1: mod_base = OTHER; note = (NAG25)s-2'-O-methyluridine-3'-phosphorothioate
  modified_base 2: mod_base = OTHER; note = 2'-O-methylcytidine-3'-phosphate
  modified_base 3: mod_base = OTHER; note = 2'-O-methylguanosine-3'-phosphate
  modified_base 4: mod_base = OTHER; note = 2'-O-methyluridine-3'-phosphate
  modified_base 5: mod_base = OTHER; note = 2'-O-methylguanosine-3'-phosphate
  modified_base 6: mod_base = OTHER; note = 2'-O-methylguanosine-3'-phosphate
  modified_base 7: mod_base = OTHER; note = 2'-O-methyluridine-3'-phosphate
  modified_base 8: mod_base = OTHER; note = 2'-O-methylguanosine-3'-phosphate
  modified_base 9: mod_base = OTHER; note = 2'-O-methylguanosine-3'-phosphate
  modified_base 10: mod_base = OTHER; note = 2'-fluoroadenosine-3'-phosphate
  modified_base 11: mod_base = OTHER; note = 2'-fluorocytidine-3'-phosphate
  modified_base 12: mod_base = OTHER; note = 2'-fluorouridine-3'-phosphate
  modified_base 13: mod_base = OTHER; note = 2'-O-methyluridine-3'-phosphate
  modified_base 14: mod_base = OTHER; note = 2'-O-methylcytidine-3'-phosphate
  modified_base 15: mod_base = OTHER; note = 2'-O-methyluridine-3'-phosphate
  modified_base 16: mod_base = OTHER; note = 2'-O-methylcytidine-3'-phosphate
  modified_base 17: mod_base = OTHER; note = 2'-O-methyluridine-3'-phosphate
  modified_base 18: mod_base = OTHER; note = 2'-O-methylcytidine-3'-phosphate
  modified_base 19: mod_base = OTHER; note = 2'-O-methyladenosine-3'-phosphate
  modified_base 20: mod_base = OTHER; note = 2'-O-methyladenosine-3'-phosphate
  modified_base 21: mod_base = OTHER; note = 2'-O-methyluridine-3'-phosphate
  modified_base 22: mod_base = OTHER; note = 2'-O-methyluridine-3'-phosphorothioate
  modified_base 23: mod_base = OTHER; note = inverted (3'-3' linked) abasic deoxyribonucleotide
  misc_feature 1: note = RNA
  misc_feature 2: note = RNA
  misc_feature 3: note = RNA
  misc_feature 4: note = RNA
  misc_feature 5: note = RNA
  misc_feature 6: note = RNA
  misc_feature 7: note = RNA
  misc_feature 8: note = RNA
  misc_feature 9: note = RNA
  misc_feature 10: note = DNA
  misc_feature 11: note = DNA
  misc_feature 12: note = DNA
  misc_feature 13: note = RNA
  misc_feature 14: note = RNA
  misc_feature 15: note = RNA
  misc_feature 16: note = RNA
  misc_feature 17: note = RNA
  misc_feature 18: note = RNA
  misc_feature 19: note = RNA
  misc_feature 20: note = RNA
  misc_feature 21: note = RNA
  misc_feature 22: note = RNA
  misc_feature 23: note = DNA
  source 1..23: mol_type = other RNA
tcgtggtggacttctctcaattn

SEQ ID NO: 227 - RNA, 21 nt, synthetic construct
  modified_base 1: mod_base = OTHER; note = (NAG25)s-inverted (3'-3' linked) abasic deoxyribonucleotide-5'-phosphorothioate
  modified_base 2: mod_base = OTHER; note = 2'-O-methyluridine-3'-phosphate
  modified_base 3: mod_base = OTHER; note = 2'-O-methylguanosine-3'-phosphate
  modified_base 4: mod_base = OTHER; note = 2'-O-methylguanosine-3'-phosphate
  modified_base 5: mod_base = OTHER; note = 2'-O-methyluridine-3'-phosphate
  modified_base 6: mod_base = OTHER; note = 2'-O-methylguanosine-3'-phosphate
  modified_base 7: mod_base = OTHER; note = 2'-O-methylguanosine-3'-phosphate
  modified_base 8: mod_base = OTHER; note = 2'-fluoroadenosine-3'-phosphate
  modified_base 9: mod_base = OTHER; note = 2'-fluorocytidine-3'-phosphate
  modified_base 10: mod_base = OTHER; note = 2'-fluorouridine-3'-phosphate
  modified_base 11: mod_base = OTHER; note = 2'-O-methyluridine-3'-phosphate
  modified_base 12: mod_base = OTHER; note = 2'-O-methylcytidine-3'-phosphate
  modified_base 13: mod_base = OTHER; note = 2'-O-methyluridine-3'-phosphate
  modified_base 14: mod_base = OTHER; note = 2'-O-methylcytidine-3'-phosphate
  modified_base 15: mod_base = OTHER; note = 2'-O-methyluridine-3'-phosphate
  modified_base 16: mod_base = OTHER; note = 2'-O-methylcytidine-3'-phosphate
  modified_base 17: mod_base = OTHER; note = 2'-O-methyladenosine-3'-phosphate
  modified_base 18: mod_base = OTHER; note = 2'-O-methyladenosine-3'-phosphate
  modified_base 19: mod_base = OTHER; note = 2'-O-methyluridine-3'-phosphate
  modified_base 20: mod_base = OTHER; note = 2'-O-methyluridine-3'-phosphorothioate
  modified_base 21: mod_base = OTHER; note = inverted (3'-3' linked) abasic deoxyribonucleotide
  misc_feature 1: note = DNA
  misc_feature 2: note = RNA
  misc_feature 3: note = RNA
  misc_feature 4: note = RNA
  misc_feature 5: note = RNA
  misc_feature 6: note = RNA
  misc_feature 7: note = RNA
  misc_feature 8: note = DNA
  misc_feature 9: note = DNA
  misc_feature 10: note = DNA
  misc_feature 11: note = RNA
  misc_feature 12: note = RNA
  misc_feature 13: note = RNA
  misc_feature 14: note = RNA
  misc_feature 15: note = RNA
  misc_feature 16: note = RNA
  misc_feature 17: note = RNA
  misc_feature 18: note = RNA
  misc_feature 19: note = RNA
  misc_feature 20: note = RNA
  misc_feature 21: note = DNA
  source 1..21: mol_type = other RNA
ntggtggacttctctcaattn

SEQ ID NO: 228 - RNA, 21 nt, synthetic construct
  modified_base 1: mod_base = OTHER; note = (NAG37)s-inverted (3'-3' linked) abasic deoxyribonucleotide-5'-phosphorothioate
  modified_base 2: mod_base = OTHER; note = 2'-O-methyluridine-3'-phosphate
  modified_base 3: mod_base = OTHER; note = 2'-O-methylguanosine-3'-phosphate
  modified_base 4: mod_base = OTHER; note = 2'-O-methylguanosine-3'-phosphate
  modified_base 5: mod_base = OTHER; note = 2'-O-methyluridine-3'-phosphate
  modified_base 6: mod_base = OTHER; note = 2'-O-methylguanosine-3'-phosphate
  modified_base 7: mod_base = OTHER; note = 2'-O-methylguanosine-3'-phosphate
  modified_base 8: mod_base = OTHER; note = 2'-fluoroadenosine-3'-phosphate
  modified_base 9: mod_base = OTHER; note = 2'-fluorocytidine-3'-phosphate
  modified_base 10: mod_base = OTHER; note = 2'-fluorouridine-3'-phosphate
  modified_base 11: mod_base = OTHER; note = 2'-O-methyluridine-3'-phosphate
  modified_base 12: mod_base = OTHER; note = 2'-O-methylcytidine-3'-phosphate
  modified_base 13: mod_base = OTHER; note = 2'-O-methyluridine-3'-phosphate
  modified_base 14: mod_base = OTHER; note = 2'-O-methylcytidine-3'-phosphate
  modified_base 15: mod_base = OTHER; note = 2'-O-methyluridine-3'-phosphate
  modified_base 16: mod_base = OTHER; note = 2'-O-methylcytidine-3'-phosphate
  modified_base 17: mod_base = OTHER; note = 2'-O-methyladenosine-3'-phosphate
  modified_base 18: mod_base = OTHER; note = 2'-O-methyladenosine-3'-phosphate
  modified_base 19: mod_base = OTHER; note = 2'-O-methyluridine-3'-phosphate
  modified_base 20: mod_base = OTHER; note = 2'-O-methyluridine-3'-phosphorothioate
  modified_base 21: mod_base = OTHER; note = inverted (3'-3' linked) abasic deoxyribonucleotide
  misc_feature 1: note = DNA
  misc_feature 2: note = RNA
  misc_feature 3: note = RNA
  misc_feature 4: note = RNA
  misc_feature 5: note = RNA
  misc_feature 6: note = RNA
  misc_feature 7: note = RNA
  misc_feature 8: note = DNA
  misc_feature 9: note = DNA
  misc_feature 10: note = DNA
  misc_feature 11: note = RNA
  misc_feature 12: note = RNA
  misc_feature 13: note = RNA
  misc_feature 14: note = RNA
  misc_feature 15: note = RNA
  misc_feature 16: note = RNA
  misc_feature 17: note = RNA
  misc_feature 18: note = RNA
  misc_feature 19: note = RNA
  misc_feature 20: note = RNA
  misc_feature 21: note = DNA
  source 1..21: mol_type = other RNA
ntggtggacttctctcaattn

SEQ ID NO: 229 - RNA, 22 nt, synthetic construct
  modified_base 1: mod_base = OTHER; note = (NAG25)s-2'-O-methylguanosine-3'-phosphorothioate
  modified_base 2: mod_base = OTHER; note = 2'-O-methyluridine-3'-phosphate
  modified_base 3..4: mod_base = OTHER; note = 2'-O-methylguanosine-3'-phosphate
  modified_base 5: mod_base = OTHER; note = 2'-O-methyladenosine-3'-phosphate
  modified_base 6: mod_base = OTHER; note = 2'-O-methylcytidine-3'-phosphate
  modified_base 7..8: mod_base = OTHER; note = 2'-O-methyluridine-3'-phosphate
  modified_base 9: mod_base = OTHER; note = 2'-fluorocytidine-3'-phosphate
  modified_base 10: mod_base = OTHER; note = 2'-fluorouridine-3'-phosphate
  modified_base 11: mod_base = OTHER; note = 2'-fluorocytidine-3'-phosphate
  modified_base 12: mod_base = OTHER; note = 2'-O-methyluridine-3'-phosphate
  modified_base 13: mod_base = OTHER; note = 2'-O-methylcytidine-3'-phosphate
  modified_base 14..15: mod_base = OTHER; note = 2'-O-methyladenosine-3'-phosphate
  modified_base 16..19: mod_base = OTHER; note = 2'-O-methyluridine-3'-phosphate
  modified_base 20: mod_base = OTHER; note = 2'-O-methylcytidine-3'-phosphate
  modified_base 21: mod_base = OTHER; note = 2'-O-methyluridine-3'-phosphorothioate
  modified_base 22: mod_base = OTHER; note = inverted (3'-3' linked) abasic deoxyribonucleotide
  misc_feature 1: note = RNA
  misc_feature 2: note = RNA
  misc_feature 3..4: note = RNA
  misc_feature 5: note = RNA
  misc_feature 6: note = RNA
  misc_feature 7..8: note = RNA
  misc_feature 9: note = DNA
  misc_feature 10: note = DNA
  misc_feature 11: note = DNA
  misc_feature 12: note = RNA
  misc_feature 13: note = RNA
  misc_feature 14..15: note = RNA
  misc_feature 16..19: note = RNA
  misc_feature 20: note = RNA
  misc_feature 21: note = RNA
  misc_feature 22: note = DNA
  source 1..22: mol_type = other RNA
gtggacttctctcaattttctn

SEQ ID NO: 230 - RNA, 23 nt, synthetic construct
  modified_base 1: mod_base = OTHER; note = (NAG25)s-inverted (3'-3' linked) abasic deoxyribonucleotide-5'-phosphorothioate
  modified_base 2: mod_base = OTHER; note = 2'-O-methylcytidine-3'-phosphate
  modified_base 3: mod_base = OTHER; note = 2'-O-methyluridine-3'-phosphate
  modified_base 4: mod_base = OTHER; note = 2'-O-methylguanosine-3'-phosphate
  modified_base 5: mod_base = OTHER; note = 2'-O-methyluridine-3'-phosphate
  modified_base 6: mod_base = OTHER; note = 2'-O-methyladenosine-3'-phosphate
  modified_base 7: mod_base = OTHER; note = 2'-O-methylguanosine-3'-phosphate
  modified_base 8: mod_base = OTHER; note = 2'-fluoroguanosine-3'-phosphate
  modified_base 9: mod_base = OTHER; note = 2'-fluorocytidine-3'-phosphate
  modified_base 10: mod_base = OTHER; note = 2'-fluoroadenosine-3'-phosphate
  modified_base 11: mod_base = OTHER; note = 2'-O-methyluridine-3'-phosphate
  modified_base 12: mod_base = OTHER; note = 2'-O-methyladenosine-3'-phosphate
  modified_base 13: mod_base = OTHER; note = 2'-O-methyladenosine-3'-phosphate
  modified_base 14: mod_base = OTHER; note = 2'-O-methyladenosine-3'-phosphate
  modified_base 15: mod_base = OTHER; note = 2'-O-methyluridine-3'-phosphate
  modified_base 16: mod_base = OTHER; note = 2'-O-methyluridine-3'-phosphate
  modified_base 17: mod_base = OTHER; note = 2'-O-methylguanosine-3'-phosphate
  modified_base 18: mod_base = OTHER; note = 2'-O-methylguanosine-3'-phosphate
  modified_base 19: mod_base = OTHER; note = 2'-O-methyluridine-3'-phosphate
  modified_base 20: mod_base = OTHER; note = 2'-O-methyladenosine-3'-phosphate
  modified_base 21: mod_base = OTHER; note = 2'-O-methyluridine-3'-phosphorothioate
  modified_base 22: mod_base = OTHER; note = 2'-O-methyluridine-3'-phosphate
  modified_base 23: mod_base = OTHER; note = inverted (3'-3' linked) abasic deoxyribonucleotide
  misc_feature 1: note = DNA
  misc_feature 2: note = RNA
  misc_feature 3: note = RNA
  misc_feature 4: note = RNA
  misc_feature 5: note = RNA
  misc_feature 6: note = RNA
  misc_feature 7: note = RNA
  misc_feature 8: note = DNA
  misc_feature 9: note = DNA
  misc_feature 10: note = DNA
  misc_feature 11: note = RNA
  misc_feature 12: note = RNA
  misc_feature 13: note = RNA
  misc_feature 14: note = RNA
  misc_feature 15: note = RNA
  misc_feature 16: note = RNA
  misc_feature 17: note = RNA
  misc_feature 18: note = RNA
  misc_feature 19: note = RNA
  misc_feature 20: note = RNA
  misc_feature 21: note = RNA
  misc_feature 22: note = RNA
  misc_feature 23: note = DNA
  source 1..23: mol_type = other RNA
nctgtaggcataaattggtattn

SEQ ID NO: 231 - RNA, 24 nt, synthetic construct
  modified_base 1: mod_base = OTHER; note = (NAG25)s-inverted (3'-3' linked) abasic deoxyribonucleotide-5'-phosphorothioate
  modified_base 2: mod_base = OTHER; note = 2'-O-methylguanosine-3'-phosphate
  modified_base 3: mod_base = OTHER; note = 2'-O-methylcytidine-3'-phosphate
  modified_base 4: mod_base = OTHER; note = 2'-O-methyluridine-3'-phosphate
  modified_base 5: mod_base = OTHER; note = 2'-O-methylguanosine-3'-phosphate
  modified_base 6: mod_base = OTHER; note = 2'-O-methyluridine-3'-phosphate
  modified_base 7: mod_base = OTHER; note = 2'-O-methyladenosine-3'-phosphate
  modified_base 8: mod_base = OTHER; note = 2'-O-methylguanosine-3'-phosphate
  modified_base 9: mod_base = OTHER; note = 2'-fluoroguanosine-3'-phosphate
  modified_base 10: mod_base = OTHER; note = 2'-fluorocytidine-3'-phosphate
  modified_base 11: mod_base = OTHER; note = 2'-fluoroadenosine-3'-phosphate
  modified_base 12: mod_base = OTHER; note = 2'-O-methyluridine-3'-phosphate
  modified_base 13: mod_base = OTHER; note = 2'-O-methyladenosine-3'-phosphate
  modified_base 14: mod_base = OTHER; note = 2'-O-methyladenosine-3'-phosphate
  modified_base 15: mod_base = OTHER; note = 2'-O-methyladenosine-3'-phosphate
  modified_base 16: mod_base = OTHER; note = 2'-O-methyluridine-3'-phosphate
  modified_base 17: mod_base = OTHER; note = 2'-O-methyluridine-3'-phosphate
  modified_base 18: mod_base = OTHER; note = 2'-O-methylguanosine-3'-phosphate
  modified_base 19: mod_base = OTHER; note = 2'-O-methylguanosine-3'-phosphate
  modified_base 20: mod_base = OTHER; note = 2'-O-methyluridine-3'-phosphate
  modified_base 21: mod_base = OTHER; note = 2'-O-methyladenosine-3'-phosphate
  modified_base 22: mod_base = OTHER; note = 2'-O-methyluridine-3'-phosphorothioate
  modified_base 23: mod_base = OTHER; note = 2'-O-methyluridine-3'-phosphate
  modified_base 24: mod_base = OTHER; note = inverted (3'-3' linked) abasic deoxyribonucleotide
  misc_feature 1: note = DNA
  misc_feature 2: note = RNA
  misc_feature 3: note = RNA
  misc_feature 4: note = RNA
  misc_feature 5: note = RNA
  misc_feature 6: note = RNA
  misc_feature 7: note = RNA
  misc_feature 8: note = RNA
  misc_feature 9: note = DNA
  misc_feature 10: note = DNA
  misc_feature 11: note = DNA
  misc_feature 12: note = RNA
  misc_feature 13: note = RNA
  misc_feature 14: note = RNA
  misc_feature 15: note = RNA
  misc_feature 16: note = RNA
  misc_feature 17: note = RNA
  misc_feature 18: note = RNA
  misc_feature 19: note = RNA
  misc_feature 20: note = RNA
  misc_feature 21: note = RNA
  misc_feature 22: note = RNA
  misc_feature 23: note = RNA
  misc_feature 24: note = DNA
  source 1..24: mol_type = other RNA
ngctgtaggcataaattggtattn

SEQ ID NO: 232 - RNA, 25 nt, synthetic construct
  modified_base 1: mod_base = OTHER; note = (NAG25)s-inverted (3'-3' linked) abasic deoxyribonucleotide-5'-phosphorothioate
  modified_base 2: mod_base = OTHER; note = 2'-O-methylguanosine-3'-phosphate
  modified_base 3: mod_base = OTHER; note = 2'-O-methylguanosine-3'-phosphate
  modified_base 4: mod_base = OTHER; note = 2'-O-methylcytidine-3'-phosphate
  modified_base 5: mod_base = OTHER; note = 2'-O-methyluridine-3'-phosphate
  modified_base 6: mod_base = OTHER; note = 2'-O-methylguanosine-3'-phosphate
  modified_base 7: mod_base = OTHER; note = 2'-O-methyluridine-3'-phosphate
  modified_base 8: mod_base = OTHER; note = 2'-O-methyladenosine-3'-phosphate
  modified_base 9: mod_base = OTHER; note = 2'-O-methylguanosine-3'-phosphate
  modified_base 10: mod_base = OTHER; note = 2'-fluoroguanosine-3'-phosphate
  modified_base 11: mod_base = OTHER; note = 2'-fluorocytidine-3'-phosphate
  modified_base 12: mod_base = OTHER; note = 2'-fluoroadenosine-3'-phosphate
  modified_base 13: mod_base = OTHER; note = 2'-O-methyluridine-3'-phosphate
  modified_base 14: mod_base = OTHER; note = 2'-O-methyladenosine-3'-phosphate
  modified_base 15: mod_base = OTHER; note = 2'-O-methyladenosine-3'-phosphate
  modified_base 16: mod_base = OTHER; note = 2'-O-methyladenosine-3'-phosphate
  modified_base 17: mod_base = OTHER; note = 2'-O-methyluridine-3'-phosphate
  modified_base 18: mod_base = OTHER; note = 2'-O-methyluridine-3'-phosphate
  modified_base 19: mod_base = OTHER; note = 2'-O-methylguanosine-3'-phosphate
  modified_base 20: mod_base = OTHER; note = 2'-O-methylguanosine-3'-phosphate
  modified_base 21: mod_base = OTHER; note = 2'-O-methyluridine-3'-phosphate
  modified_base 22: mod_base = OTHER; note = 2'-O-methyladenosine-3'-phosphate
  modified_base 23: mod_base = OTHER; note = 2'-O-methyluridine-3'-phosphorothioate
  modified_base 24: mod_base = OTHER; note = 2'-O-methyluridine-3'-phosphate
  modified_base 25: mod_base = OTHER; note = inverted (3'-3' linked) abasic deoxyribonucleotide
  misc_feature 1: note = DNA
  misc_feature 2: note = RNA
  misc_feature 3: note = RNA
  misc_feature 4: note = RNA
  misc_feature 5: note = RNA
  misc_feature 6: note = RNA
  misc_feature 7: note = RNA
  misc_feature 8: note = RNA
  misc_feature 9: note = RNA
  misc_feature 10: note = DNA
  misc_feature 11: note = DNA
  misc_feature 12: note = DNA
  misc_feature 13: note = RNA
  misc_feature 14: note = RNA
  misc_feature 15: note = RNA
  misc_feature 16: note = RNA
  misc_feature 17: note = RNA
  misc_feature 18: note = RNA
  misc_feature 19: note = RNA
  misc_feature 20: note = RNA
  misc_feature 21: note = RNA
  misc_feature 22: note = RNA
  misc_feature 23: note = RNA
  misc_feature 24: note = RNA
  misc_feature 25: note = DNA
  source 1..25: mol_type = other RNA
nggctgtaggcataaattggtattn

SEQ ID NO: 233 - RNA, 25 nt, synthetic construct
  modified_base 1: mod_base = OTHER; note = (NAG25)s-inverted (3'-3' linked) abasic deoxyribonucleotide-5'-phosphorothioate
  modified_base 2: mod_base = OTHER; note = 2'-O-methyladenosine-3'-phosphate
  modified_base 3: mod_base = OTHER; note = 2'-O-methyladenosine-3'-phosphate
  modified_base 4: mod_base = OTHER; note = 2'-O-methylcytidine-3'-phosphate
  modified_base 5: mod_base = OTHER; note = 2'-O-methyluridine-3'-phosphate
  modified_base 6: mod_base = OTHER; note = 2'-O-methylguanosine-3'-phosphate
  modified_base 7: mod_base = OTHER; note = 2'-O-methyluridine-3'-phosphate
  modified_base 8: mod_base = OTHER; note = 2'-O-methyladenosine-3'-phosphate
  modified_base 9: mod_base = OTHER; note = 2'-O-methylguanosine-3'-phosphate
  modified_base 10: mod_base = OTHER; note = 2'-fluoroguanosine-3'-phosphate
  modified_base 11: mod_base = OTHER; note = 2'-fluorocytidine-3'-phosphate
  modified_base 12: mod_base = OTHER; note = 2'-fluoroadenosine-3'-phosphate
  modified_base 13: mod_base = OTHER; note = 2'-O-methyluridine-3'-phosphate
  modified_base 14: mod_base = OTHER; note = 2'-O-methyladenosine-3'-phosphate
  modified_base 15: mod_base = OTHER; note = 2'-O-methyladenosine-3'-phosphate
  modified_base 16: mod_base = OTHER; note = 2'-O-methyladenosine-3'-phosphate
  modified_base 17: mod_base = OTHER; note = 2'-O-methyluridine-3'-phosphate
  modified_base 18: mod_base = OTHER; note = 2'-O-methyluridine-3'-phosphate
  modified_base 19: mod_base = OTHER; note = 2'-O-methylguanosine-3'-phosphate
  modified_base 20: mod_base = OTHER; note = 2'-O-methylguanosine-3'-phosphate
  modified_base 21: mod_base = OTHER; note = 2'-O-methyluridine-3'-phosphate
  modified_base 22: mod_base = OTHER; note = 2'-O-methyladenosine-3'-phosphate
  modified_base 23: mod_base = OTHER; note = 2'-O-methyluridine-3'-phosphorothioate
  modified_base 24: mod_base = OTHER; note = 2'-O-methyluridine-3'-phosphate
  modified_base 25: mod_base = OTHER; note = inverted (3'-3' linked) abasic deoxyribonucleotide
  misc_feature 1: note = DNA
  misc_feature 2: note = RNA
  misc_feature 3: note = RNA
  misc_feature 4: note = RNA
  misc_feature 5: note = RNA
  misc_feature 6: note = RNA
  misc_feature 7: note = RNA
  misc_feature 8: note = RNA
  misc_feature 9: note = RNA
  misc_feature 10: note = DNA
  misc_feature 11: note = DNA
  misc_feature 12: note = DNA
  misc_feature 13: note = RNA
  misc_feature 14: note = RNA
  misc_feature 15: note = RNA
  misc_feature 16: note = RNA
  misc_feature 17: note = RNA
  misc_feature 18: note = RNA
  misc_feature 19: note = RNA
  misc_feature 20: note = RNA
  misc_feature 21: note = RNA
  misc_feature 22: note = RNA
  misc_feature 23: note = RNA
  misc_feature 24: note = RNA
  misc_feature 25: note = DNA
  source 1..25: mol_type = other RNA
naactgtaggcataaattggtattn

SEQ ID NO: 234 - RNA, 23 nt, synthetic construct
  modified_base 1: mod_base = OTHER; note = (NAG25)s-inverted (3'-3' linked) abasic deoxyribonucleotide
  modified_base 2: mod_base = OTHER; note = 2'-O-methyluridine-3'-phosphate
  modified_base 3: mod_base = OTHER; note = 2'-O-methylguanosine-3'-phosphate
  modified_base 4: mod_base = OTHER; note = 2'-O-methylguanosine-3'-phosphate
  modified_base 5: mod_base = OTHER; note = 2'-O-methyluridine-3'-phosphate
  modified_base 6: mod_base = OTHER; note = 2'-O-methylguanosine-3'-phosphate
  modified_base 7: mod_base = OTHER; note = 2'-O-methylguanosine-3'-phosphate
  modified_base 8: mod_base = OTHER; note = 2'-fluoroadenosine-3'-phosphate
  modified_base 9: mod_base = OTHER; note = 2'-fluorocytidine-3'-phosphate
  modified_base 10: mod_base = OTHER; note = 2'-fluorouridine-3'-phosphate
  modified_base 11: mod_base = OTHER; note = 2'-O-methyluridine-3'-phosphate
  modified_base 12: mod_base = OTHER; note = 2'-O-methylcytidine-3'-phosphate
  modified_base 13: mod_base = OTHER; note = 2'-O-methyluridine-3'-phosphate
  modified_base 14: mod_base = OTHER; note = 2'-O-methylcytidine-3'-phosphate
  modified_base 15: mod_base = OTHER; note = 2'-O-methyluridine-3'-phosphate
  modified_base 16: mod_base = OTHER; note = 2'-O-methylcytidine-3'-phosphate
  modified_base 17: mod_base = OTHER; note = 2'-O-methyladenosine-3'-phosphate
  modified_base 18: mod_base = OTHER; note = 2'-O-methyladenosine-3'-phosphate
  modified_base 19: mod_base = OTHER; note = 2'-O-methyluridine-3'-phosphate
  modified_base 20: mod_base = OTHER; note = 2'-O-methyladenosine-3'-phosphate
  modified_base 21: mod_base = OTHER; note = 2'-O-methyluridine-3'-phosphorothioate
  modified_base 22: mod_base = OTHER; note = 2'-O-methyluridine-3'-phosphate
  modified_base 23: mod_base = OTHER; note = inverted (3'-3' linked) abasic deoxyribonucleotide
  misc_feature 1: note = DNA
  misc_feature 2: note = RNA
  misc_feature 3: note = RNA
  misc_feature 4: note = RNA
  misc_feature 5: note = RNA
  misc_feature 6: note = RNA
  misc_feature 7: note = RNA
  misc_feature 8: note = DNA
  misc_feature 9: note = DNA
  misc_feature 10: note = DNA
  misc_feature 11: note = RNA
  misc_feature 12: note = RNA
  misc_feature 13: note = RNA
  misc_feature 14: note = RNA
  misc_feature 15: note = RNA
  misc_feature 16: note = RNA
  misc_feature 17: note = RNA
  misc_feature 18: note = RNA
  misc_feature 19: note = RNA
  misc_feature 20: note = RNA
  misc_feature 21: note = RNA
  misc_feature 22: note = RNA
  misc_feature 23: note = DNA
  source 1..23: mol_type = other RNA
ntggtggacttctctcaatattn

SEQ ID NO: 235 - RNA, 24 nt, synthetic construct
  modified_base 1: mod_base = OTHER; note = (NAG25)s-inverted (3'-3' linked) abasic deoxyribonucleotide-5'-phosphorothioate
  modified_base 2: mod_base = OTHER; note = 2'-O-methylguanosine-3'-phosphate
  modified_base 3: mod_base = OTHER; note = 2'-O-methyluridine-3'-phosphate
  modified_base 4: mod_base = OTHER; note = 2'-O-methylguanosine-3'-phosphate
  modified_base 5: mod_base = OTHER; note = 2'-O-methylguanosine-3'-phosphate
  modified_base 6: mod_base = OTHER; note = 2'-O-methyluridine-3'-phosphate
  modified_base 7: mod_base = OTHER; note = 2'-O-methylguanosine-3'-phosphate
  modified_base 8: mod_base = OTHER; note = 2'-O-methylguanosine-3'-phosphate
  modified_base 9: mod_base = OTHER; note = 2'-fluoroadenosine-3'-phosphate
  modified_base 10: mod_base = OTHER; note = 2'-fluorocytidine-3'-phosphate
  modified_base 11: mod_base = OTHER; note = 2'-fluorouridine-3'-phosphate
  modified_base 12: mod_base = OTHER; note = 2'-O-methyluridine-3'-phosphate
  modified_base 13: mod_base = OTHER; note = 2'-O-methylcytidine-3'-phosphate
  modified_base 14: mod_base = OTHER; note = 2'-O-methyluridine-3'-phosphate
  modified_base 15: mod_base = OTHER; note = 2'-O-methylcytidine-3'-phosphate
  modified_base 16: mod_base = OTHER; note = 2'-O-methyluridine-3'-phosphate
  modified_base 17: mod_base = OTHER; note = 2'-O-methylcytidine-3'-phosphate
  modified_base 18: mod_base = OTHER; note = 2'-O-methyladenosine-3'-phosphate
  modified_base 19: mod_base = OTHER; note = 2'-O-methyladenosine-3'-phosphate
  modified_base 20: mod_base = OTHER; note = 2'-O-methyluridine-3'-phosphate
  modified_base 21: mod_base = OTHER; note = 2'-O-methyladenosine-3'-phosphate
  modified_base 22: mod_base = OTHER; note = 2'-O-methyluridine-3'-phosphorothioate
  modified_base 23: mod_base = OTHER; note = 2'-O-methyluridine-3'-phosphate
  modified_base 24: mod_base = OTHER; note = inverted (3'-3' linked) abasic deoxyribonucleotide
  misc_feature 1: note = DNA
  misc_feature 2: note = RNA
  misc_feature 3: note = RNA
  misc_feature 4: note = RNA
  misc_feature 5: note = RNA
  misc_feature 6: note = RNA
  misc_feature 7: note = RNA
  misc_feature 8: note = RNA
  misc_feature 9: note = DNA
  misc_feature 10: note = DNA
  misc_feature 11: note = DNA
  misc_feature 12: note = RNA
  misc_feature 13: note = RNA
  misc_feature 14: note = RNA
  misc_feature 15: note = RNA
  misc_feature 16: note = RNA
  misc_feature 17: note = RNA
  misc_feature 18: note = RNA
  misc_feature 19: note = RNA
  misc_feature 20: note = RNA
  misc_feature 21: note = RNA
  misc_feature 22: note = RNA
  misc_feature 23: note = RNA
  misc_feature 24: note = DNA
  source 1..24: mol_type = other RNA
ngtggtggacttctctcaatattn

SEQ ID NO: 236 - RNA, 24 nt, synthetic construct
  modified_base 1: mod_base = OTHER; note = (NAG25)s-2'-O-methyladenosine-3'-phosphorothioate
  modified_base 2: mod_base = OTHER; note = 2'-O-methyladenosine-3'-phosphate
  modified_base 3: mod_base = OTHER; note = 2'-O-methyluridine-3'-phosphate
  modified_base 4: mod_base = OTHER; note = 2'-O-methylguanosine-3'-phosphate
  modified_base 5: mod_base = OTHER; note = 2'-O-methylguanosine-3'-phosphate
  modified_base 6: mod_base = OTHER; note = 2'-O-methyluridine-3'-phosphate
  modified_base 7: mod_base = OTHER; note = 2'-O-methylguanosine-3'-phosphate
  modified_base 8: mod_base = OTHER; note = 2'-O-methylguanosine-3'-phosphate
  modified_base 9: mod_base = OTHER; note = 2'-fluoroadenosine-3'-phosphate
  modified_base 10: mod_base = OTHER; note = 2'-fluorocytidine-3'-phosphate
  modified_base 11: mod_base = OTHER; note = 2'-fluorouridine-3'-phosphate
  modified_base 12: mod_base = OTHER; note = 2'-O-methyluridine-3'-phosphate
  modified_base 13: mod_base = OTHER; note = 2'-O-methylcytidine-3'-phosphate
  modified_base 14: mod_base = OTHER; note = 2'-O-methyluridine-3'-phosphate
  modified_base 15: mod_base = OTHER; note = 2'-O-methylcytidine-3'-phosphate
  modified_base 16: mod_base = OTHER; note = 2'-O-methyluridine-3'-phosphate
  modified_base 17: mod_base = OTHER; note = 2'-O-methylcytidine-3'-phosphate
  modified_base 18: mod_base = OTHER; note = 2'-O-methyladenosine-3'-phosphate
  modified_base 19: mod_base = OTHER; note = 2'-O-methyladenosine-3'-phosphate
  modified_base 20: mod_base = OTHER; note = 2'-O-methyluridine-3'-phosphate
  modified_base 21: mod_base = OTHER; note = 2'-O-methyladenosine-3'-phosphate
  modified_base 22: mod_base = OTHER; note = 2'-O-methyluridine-3'-phosphorothioate
  modified_base 23: mod_base = OTHER; note = 2'-O-methyluridine-3'-phosphate
  modified_base 24: mod_base = OTHER; note = inverted (3'-3' linked) abasic deoxyribonucleotide
  misc_feature 1: note = RNA
  misc_feature 2: note = RNA
  misc_feature 3: note = RNA
  misc_feature 4: note = RNA
  misc_feature 5: note = RNA
  misc_feature 6: note = RNA
  misc_feature 7: note = RNA
  misc_feature 8: note = RNA
  misc_feature 9: note = DNA
  misc_feature 10: note = DNA
  misc_feature 11: note = DNA
  misc_feature 12: note = RNA
  misc_feature 13: note = RNA
  misc_feature 14: note = RNA
  misc_feature 15: note = RNA
  misc_feature 16: note = RNA
  misc_feature 17: note = RNA
  misc_feature 18: note = RNA
  misc_feature 19: note = RNA
  misc_feature 20: note = RNA
  misc_feature 21: note = RNA
  misc_feature 22: note = RNA
  misc_feature 23: note = RNA
  misc_feature 24: note = DNA
  source 1..24: mol_type = other RNA
aatggtggacttctctcaatattn

SEQ ID NO: 237 - RNA, 24 nt, synthetic construct
  modified_base 1: mod_base = OTHER; note = (NAG25)s-2'-O-methylcytidine-3'-phosphorothioate
  modified_base 2: mod_base = OTHER; note = 2'-O-methylguanosine-3'-phosphate
  modified_base 3: mod_base = OTHER; note = 2'-O-methyluridine-3'-phosphate
  modified_base 4: mod_base = OTHER; note = 2'-O-methylguanosine-3'-phosphate
  modified_base 5: mod_base = OTHER; note = 2'-O-methylguanosine-3'-phosphate
  modified_base 6: mod_base = OTHER; note = 2'-O-methyluridine-3'-phosphate
  modified_base 7: mod_base = OTHER; note = 2'-O-methylguanosine-3'-phosphate
  modified_base 8: mod_base = OTHER; note = 2'-O-methylguanosine-3'-phosphate
  modified_base 9: mod_base = OTHER; note = 2'-fluoroadenosine-3'-phosphate
  modified_base 10: mod_base = OTHER; note = 2'-fluorocytidine-3'-phosphate
  modified_base 11: mod_base = OTHER; note = 2'-fluorouridine-3'-phosphate
  modified_base 12: mod_base = OTHER; note = 2'-O-methyluridine-3'-phosphate
  modified_base 13: mod_base = OTHER; note = 2'-O-methylcytidine-3'-phosphate
  modified_base 14: mod_base = OTHER; note = 2'-O-methyluridine-3'-phosphate
  modified_base 15: mod_base = OTHER; note = 2'-O-methylcytidine-3'-phosphate
  modified_base 16: mod_base = OTHER; note = 2'-O-methyluridine-3'-phosphate
  modified_base 17: mod_base = OTHER; note = 2'-O-methylcytidine-3'-phosphate
  modified_base 18: mod_base = OTHER; note = 2'-O-methyladenosine-3'-phosphate
  modified_base 19: mod_base = OTHER; note = 2'-O-methyladenosine-3'-phosphate
  modified_base 20: mod_base = OTHER; note = 2'-O-methyluridine-3'-phosphate
  modified_base 21: mod_base = OTHER; note = 2'-O-methyladenosine-3'-phosphate
  modified_base 22: mod_base = OTHER; note = 2'-O-methyluridine-3'-phosphorothioate
  modified_base 23: mod_base = OTHER; note = 2'-O-methyluridine-3'-phosphate
  modified_base 24: mod_base = OTHER; note = inverted (3'-3' linked) abasic deoxyribonucleotide
  misc_feature 1: note = RNA
  misc_feature 2: note = RNA
  misc_feature 3: note = RNA
  misc_feature 4: note = RNA
  misc_feature 5: note = RNA
  misc_feature 6: note = RNA
  misc_feature 7: note = RNA
  misc_feature 8: note = RNA
  misc_feature 9: note = DNA
  misc_feature 10: note = DNA
  misc_feature 11: note = DNA
  misc_feature 12: note = RNA
  misc_feature 13: note = RNA
  misc_feature 14: note = RNA
  misc_feature 15: note = RNA
  misc_feature 16: note = RNA
  misc_feature 17: note = RNA
  misc_feature 18: note = RNA
  misc_feature 19: note = RNA
  misc_feature 20: note = RNA
  misc_feature 21: note = RNA
  misc_feature 22: note = RNA
  misc_feature 23: note = RNA
  misc_feature 24: note = DNA
  source 1..24: mol_type = other RNA
cgtggtggacttctctcaatattn

SEQ ID NO: 238 - RNA, 22 nt, synthetic construct
  modified_base 1: mod_base = OTHER; note = (NAG31)s-2'-O-methylcytidine-3'-phosphorothioate
  modified_base 2: mod_base = OTHER; note = 2'-O-methylguanosine-3'-phosphate
  modified_base 3: mod_base = OTHER; note = 2'-O-methyluridine-3'-phosphate
  modified_base 4: mod_base = OTHER; note = 2'-O-methylguanosine-3'-phosphate
  modified_base 5: mod_base = OTHER; note = 2'-O-methylguanosine-3'-phosphate
  modified_base 6: mod_base = OTHER; note = 2'-O-methyluridine-3'-phosphate
  modified_base 7: mod_base = OTHER; note = 2'-O-methylguanosine-3'-phosphate
  modified_base 8: mod_base = OTHER; note = 2'-O-methylguanosine-3'-phosphate
  modified_base 9: mod_base = OTHER; note = 2'-fluoroadenosine-3'-phosphate
  modified_base 10: mod_base = OTHER; note = 2'-fluorocytidine-3'-phosphate
  modified_base 11: mod_base = OTHER; note = 2'-fluorouridine-3'-phosphate
  modified_base 12: mod_base = OTHER; note = 2'-O-methyluridine-3'-phosphate
  modified_base 13: mod_base = OTHER; note = 2'-O-methylcytidine-3'-phosphate
  modified_base 14: mod_base = OTHER; note = 2'-O-methyluridine-3'-phosphate
  modified_base 15: mod_base = OTHER; note = 2'-O-methylcytidine-3'-phosphate
  modified_base 16: mod_base = OTHER; note = 2'-O-methyluridine-3'-phosphate
  modified_base 17: mod_base = OTHER; note = 2'-O-methylcytidine-3'-phosphate
  modified_base 18: mod_base = OTHER; note = 2'-O-methyladenosine-3'-phosphate
  modified_base 19: mod_base = OTHER; note = 2'-O-methyladenosine-3'-phosphate
  modified_base 20: mod_base = OTHER; note = 2'-O-methyluridine-3'-phosphate
  modified_base 21: mod_base = OTHER; note = 2'-O-methyladenosine-3'-phosphorothioate
  modified_base 22: mod_base = OTHER; note = inverted (3'-3' linked) abasic deoxyribonucleotide
  misc_feature 1: note = RNA
  misc_feature 2: note = RNA
  misc_feature 3: note = RNA
  misc_feature 4: note = RNA
  misc_feature 5: note = RNA
  misc_feature 6: note = RNA
  misc_feature 7: note = RNA
  misc_feature 8: note = RNA
  misc_feature 9: note = DNA
  misc_feature 10: note = DNA
  misc_feature 11: note = DNA
  misc_feature 12: note = RNA
  misc_feature 13: note = RNA
  misc_feature 14: note = RNA
  misc_feature 15: note = RNA
  misc_feature 16: note = RNA
  misc_feature 17: note = RNA
  misc_feature 18: note = RNA
  misc_feature 19: note = RNA
  misc_feature 20: note = RNA
  misc_feature 21: note = RNA
  misc_feature 22: note = DNA
  source 1..22: mol_type = other RNA
cgtggtggacttctctcaatan

SEQ ID NO: 239 - RNA, 23 nt, synthetic construct
  modified_base 1: mod_base = OTHER; note = (NAG25)s-inverted (3'-3' linked) abasic deoxyribonucleotide-5'-phosphorothioate
  modified_base 2: mod_base = OTHER; note = 2'-O-methyladenosine-3'-phosphate
  modified_base 3: mod_base = OTHER; note = 2'-O-methyladenosine-3'-phosphate
  modified_base 4: mod_base = OTHER; note = 2'-O-methylguanosine-3'-phosphate
  modified_base 5: mod_base = OTHER; note = 2'-O-methyluridine-3'-phosphate
  modified_base 6: mod_base = OTHER; note = 2'-O-methylguanosine-3'-phosphate
  modified_base 7: mod_base = OTHER; note = 2'-O-methylguanosine-3'-phosphate
  modified_base 8: mod_base = OTHER; note = 2'-O-methyluridine-3'-phosphate
  modified_base 9: mod_base = OTHER; note = 2'-O-methylguanosine-3'-phosphate
  modified_base 10: mod_base = OTHER; note = 2'-fluoroguanosine-3'-phosphate
  modified_base 11: mod_base = OTHER; note = 2'-fluoroadenosine-3'-phosphate
  modified_base 12: mod_base = OTHER; note = 2'-fluorocytidine-3'-phosphate
  modified_base 13: mod_base = OTHER; note = 2'-O-methyluridine-3'-phosphate
  modified_base 14: mod_base = OTHER; note = 2'-O-methyluridine-3'-phosphate
  modified_base 15: mod_base = OTHER; note = 2'-O-methylcytidine-3'-phosphate
  modified_base 16: mod_base = OTHER; note = 2'-O-methyluridine-3'-phosphate
  modified_base 17: mod_base = OTHER; note = 2'-O-methylcytidine-3'-phosphate
  modified_base 18: mod_base = OTHER; note = 2'-O-methyluridine-3'-phosphate
  modified_base 19: mod_base = OTHER; note = 2'-O-methylcytidine-3'-phosphate
  modified_base 20: mod_base = OTHER; note = 2'-O-methyladenosine-3'-phosphate
  modified_base 21: mod_base = OTHER; note = 2'-O-methyladenosine-3'-phosphate
  modified_base 22: mod_base = OTHER; note = 2'-O-methyluridine-3'-phosphorothioate
  modified_base 23: mod_base = OTHER; note = inverted (3'-3' linked) abasic deoxyribonucleotide
  misc_feature 1: note = DNA
  misc_feature 2: note = RNA
  misc_feature 3: note = RNA
  misc_feature 4: note = RNA
  misc_feature 5: note = RNA
  misc_feature 6: note = RNA
  misc_feature 7: note = RNA
  misc_feature 8: note = RNA
  misc_feature 9: note = RNA
  misc_feature 10: note = DNA
  misc_feature 11: note = DNA
  misc_feature 12: note = DNA
  misc_feature 13: note = RNA
  misc_feature 14: note = RNA
  misc_feature 15: note = RNA
  misc_feature 16: note = RNA
  misc_feature 17: note = RNA
  misc_feature 18: note = RNA
  misc_feature 19: note = RNA
  misc_feature 20: note = RNA
  misc_feature 21: note = RNA
  misc_feature 22: note = RNA
  misc_feature 23: note = DNA
  source 1..23: mol_type = other RNA
naagtggtggacttctctcaatn

SEQ ID NO: 240 - RNA, 23 nt, synthetic construct
  modified_base 1: mod_base = OTHER; note = (NAG25)s-inverted (3'-3' linked) abasic deoxyribonucleotide-5'-phosphorothioate
  modified_base 2: mod_base = OTHER; note = 2'-O-methylguanosine-3'-phosphate
  modified_base 3: mod_base = OTHER; note = 2'-O-methyluridine-3'-phosphate
  modified_base 4: mod_base = OTHER; note = 2'-O-methylguanosine-3'-phosphate
  modified_base 5: mod_base = OTHER; note = 2'-O-methylguanosine-3'-phosphate
  modified_base 6: mod_base = OTHER; note = 2'-O-methyluridine-3'-phosphate
  modified_base 7: mod_base = OTHER; note = 2'-O-methylguanosine-3'-phosphate
  modified_base 8: mod_base = OTHER; note = 2'-fluoroguanosine-3'-phosphate
  modified_base 9: mod_base = OTHER; note = 2'-fluoroadenosine-3'-phosphate
  modified_base 10: mod_base = OTHER; note = 2'-fluorocytidine-3'-phosphate
  modified_base 11: mod_base = OTHER; note = 2'-O-methyluridine-3'-phosphate
  modified_base 12: mod_base = OTHER; note = 2'-O-methyluridine-3'-phosphate
  modified_base 13: mod_base = OTHER; note = 2'-O-methylcytidine-3'-phosphate
  modified_base 14: mod_base = OTHER; note = 2'-O-methyluridine-3'-phosphate
  modified_base 15: mod_base = OTHER; note = 2'-O-methylcytidine-3'-phosphate
  modified_base 16: mod_base = OTHER; note = 2'-O-methyluridine-3'-phosphate
  modified_base 17: mod_base = OTHER; note = 2'-O-methylcytidine-3'-phosphate
  modified_base 18: mod_base = OTHER; note = 2'-O-methyladenosine-3'-phosphate
  modified_base 19: mod_base = OTHER; note = 2'-O-methyladenosine-3'-phosphate
  modified_base 20: mod_base = OTHER; note = 2'-O-methyladenosine-3'-phosphate
  modified_base 21: mod_base = OTHER; note = 2'-O-methyluridine-3'-phosphorothioate
  modified_base 22: mod_base = OTHER; note = 2'-O-methyluridine-3'-phosphate
  modified_base 23: mod_base = OTHER; note = inverted (3'-3' linked) abasic deoxyribonucleotide
  misc_feature 1: note = DNA
  misc_feature 2: note = RNA
  misc_feature 3: note = RNA
  misc_feature 4: note = RNA
  misc_feature 5: note = RNA
  misc_feature 6: note = RNA
  misc_feature 7: note = RNA
  misc_feature 8: note = DNA
  misc_feature 9: note = DNA
  misc_feature 10: note = DNA
  misc_feature 11: note = RNA
  misc_feature 12: note = RNA
  misc_feature 13: note = RNA
  misc_feature 14: note = RNA
  misc_feature 15: note = RNA
  misc_feature 16: note = RNA
  misc_feature 17: note = RNA
  misc_feature 18: note = RNA
  misc_feature 19: note = RNA
  misc_feature 20: note = RNA
  misc_feature 21: note = RNA
  misc_feature 22: note = RNA
  misc_feature 23: note = DNA
  source 1..23: mol_type = other RNA
ngtggtggacttctctcaaattn

SEQ ID NO: 241 - RNA, 24 nt, synthetic construct
  modified_base 1: mod_base = OTHER; note = (NAG25)s-inverted (3'-3' linked) abasic deoxyribonucleotide-5'-phosphorothioate
  modified_base 2: mod_base = OTHER; note = 2'-O-methylcytidine-3'-phosphate
  modified_base 3: mod_base = OTHER; note = 2'-O-methylguanosine-3'-phosphate
  modified_base 4: mod_base = OTHER; note = 2'-O-methyluridine-3'-phosphate
  modified_base 5: mod_base = OTHER; note = 2'-O-methylguanosine-3'-phosphate
  modified_base 6: mod_base = OTHER; note = 2'-O-methylguanosine-3'-phosphate
  modified_base 7: mod_base = OTHER; note = 2'-O-methyluridine-3'-phosphate
  modified_base 8: mod_base = OTHER; note = 2'-O-methylguanosine-3'-phosphate
  modified_base 9: mod_base = OTHER; note = 2'-fluoroguanosine-3'-phosphate
  modified_base 10: mod_base = OTHER; note = 2'-fluoroadenosine-3'-phosphate
  modified_base 11: mod_base = OTHER; note = 2'-fluorocytidine-3'-phosphate
  modified_base 12: mod_base = OTHER; note = 2'-O-methyluridine-3'-phosphate
  modified_base 13: mod_base = OTHER; note = 2'-O-methyluridine-3'-phosphate
  modified_base 14: mod_base = OTHER; note = 2'-O-methylcytidine-3'-phosphate
  modified_base 15: mod_base = OTHER; note = 2'-O-methyluridine-3'-phosphate
  modified_base 16: mod_base = OTHER; note = 2'-O-methylcytidine-3'-phosphate
  modified_base 17: mod_base = OTHER; note = 2'-O-methyluridine-3'-phosphate
  modified_base 18: mod_base = OTHER; note = 2'-O-methylcytidine-3'-phosphate
  modified_base 19: mod_base = OTHER; note = 2'-O-methyladenosine-3'-phosphate
  modified_base 20: mod_base = OTHER; note = 2'-O-methyladenosine-3'-phosphate
  modified_base 21: mod_base = OTHER; note = 2'-O-methyladenosine-3'-phosphate
  modified_base 22: mod_base = OTHER; note = 2'-O-methyluridine-3'-phosphorothioate
  modified_base 23: mod_base = OTHER; note = 2'-O-methyluridine-3'-phosphate
  modified_base 24: mod_base = OTHER; note = inverted (3'-3' linked) abasic deoxyribonucleotide
  misc_feature 1: note = DNA
  misc_feature 2: note = RNA
  misc_feature 3: note = RNA
  misc_feature 4: note = RNA
  misc_feature 5: note = RNA
  misc_feature 6: note = RNA
  misc_feature 7: note = RNA
  misc_feature 8: note = RNA
  misc_feature 9: note = DNA
  misc_feature 10: note = DNA
  misc_feature 11: note = DNA
  misc_feature 12: note = RNA
  misc_feature 13: note = RNA
  misc_feature 14: note = RNA
  misc_feature 15: note = RNA
  misc_feature 16: note = RNA
  misc_feature 17: note = RNA
  misc_feature 18: note = RNA
  misc_feature 19: note = RNA
  misc_feature 20: note = RNA
  misc_feature 21: note = RNA
  misc_feature 22: note = RNA
  misc_feature 23: note = RNA
  misc_feature 24: note = DNA
  source 1..24: mol_type = other RNA
ncgtggtggacttctctcaaattn

SEQ ID NO: 242 - RNA, 24 nt, synthetic construct
  modified_base 1: mod_base = OTHER; note = (NAG25)s-2'-O-methyladenosine-3'-phosphorothioate
  modified_base 2: mod_base = OTHER; note = 2'-O-methyladenosine-3'-phosphate
  modified_base 3: mod_base = OTHER; note = 2'-O-methylguanosine-3'-phosphate
  modified_base 4: mod_base = OTHER; note = 2'-O-methyluridine-3'-phosphate
  modified_base 5: mod_base = OTHER; note = 2'-O-methylguanosine-3'-phosphate
  modified_base 6: mod_base = OTHER; note = 2'-O-methylguanosine-3'-phosphate
  modified_base 7: mod_base = OTHER; note = 2'-O-methyluridine-3'-phosphate
  modified_base 8: mod_base = OTHER; note = 2'-O-methylguanosine-3'-phosphate
  modified_base 9: mod_base = OTHER; note = 2'-fluoroguanosine-3'-phosphate
  modified_base 10: mod_base = OTHER; note = 2'-fluoroadenosine-3'-phosphate
  modified_base 11: mod_base = OTHER; note = 2'-fluorocytidine-3'-phosphate
  modified_base 12: mod_base = OTHER; note = 2'-O-methyluridine-3'-phosphate
  modified_base 13: mod_base = OTHER; note = 2'-O-methyluridine-3'-phosphate
  modified_base 14: mod_base = OTHER; note = 2'-O-methylcytidine-3'-phosphate
  modified_base 15: mod_base = OTHER; note = 2'-O-methyluridine-3'-phosphate
  modified_base 16: mod_base = OTHER; note = 2'-O-methylcytidine-3'-phosphate
  modified_base 17: mod_base = OTHER; note = 2'-O-methyluridine-3'-phosphate
  modified_base 18: mod_base = OTHER; note = 2'-O-methylcytidine-3'-phosphate
  modified_base 19: mod_base = OTHER; note = 2'-O-methyladenosine-3'-phosphate
  modified_base 20: mod_base = OTHER; note = 2'-O-methyladenosine-3'-phosphate
  modified_base 21: mod_base = OTHER; note = 2'-O-methyladenosine-3'-phosphate
  modified_base 22: mod_base = OTHER; note = 2'-O-methyluridine-3'-phosphorothioate
  modified_base 23: mod_base = OTHER; note = 2'-O-methyluridine-3'-phosphate
  modified_base 24: mod_base = OTHER; note = inverted (3'-3' linked) abasic deoxyribonucleotide
  misc_feature 1: note = RNA
  misc_feature 2: note = RNA
  misc_feature 3: note = RNA
  misc_feature 4: note = RNA
  misc_feature 5: note = RNA
  misc_feature 6: note = RNA
  misc_feature 7: note = RNA
  misc_feature 8: note = RNA
  misc_feature 9: note = DNA
  misc_feature 10: note = DNA
  misc_feature 11: note = DNA
  misc_feature 12: note = RNA
  misc_feature 13: note = RNA
  misc_feature 14: note = RNA
  misc_feature 15: note = RNA
  misc_feature 16: note = RNA
  misc_feature 17: note = RNA
  misc_feature 18: note = RNA
  misc_feature 19: note = RNA
  misc_feature 20: note = RNA
  misc_feature 21: note = RNA
  misc_feature 22: note = RNA
  misc_feature 23: note = RNA
  misc_feature 24: note = DNA
  source 1..24: mol_type = other RNA
aagtggtggacttctctcaaattn

SEQ ID NO: 243 - RNA, 24 nt, synthetic construct
  modified_base 1: mod_base = OTHER; note = (NAG25)s-2'-O-methyluridine-3'-phosphorothioate
  modified_base 2: mod_base = OTHER; note = 2'-O-methylcytidine-3'-phosphate
  modified_base 3: mod_base = OTHER; note = 2'-O-methylguanosine-3'-phosphate
  modified_base 4: mod_base = OTHER; note = 2'-O-methyluridine-3'-phosphate
  modified_base 5: mod_base = OTHER; note = 2'-O-methylguanosine-3'-phosphate
  modified_base 6: mod_base = OTHER; note = 2'-O-methylguanosine-3'-phosphate
  modified_base 7: mod_base = OTHER; note = 2'-O-methyluridine-3'-phosphate
  modified_base 8: mod_base = OTHER; note = 2'-O-methylguanosine-3'-phosphate
  modified_base 9: mod_base = OTHER; note = 2'-fluoroguanosine-3'-phosphate
  modified_base 10: mod_base = OTHER; note = 2'-fluoroadenosine-3'-phosphate
  modified_base 11: mod_base = OTHER; note = 2'-fluorocytidine-3'-phosphate
  modified_base 12: mod_base = OTHER; note = 2'-O-methyluridine-3'-phosphate
  modified_base 13: mod_base = OTHER; note = 2'-O-methyluridine-3'-phosphate
  modified_base 14: mod_base = OTHER; note = 2'-O-methylcytidine-3'-phosphate
  modified_base 15: mod_base = OTHER; note = 2'-O-methyluridine-3'-phosphate
  modified_base 16: mod_base = OTHER; note = 2'-O-methylcytidine-3'-phosphate
  modified_base 17: mod_base = OTHER; note = 2'-O-methyluridine-3'-phosphate
  modified_base 18: mod_base = OTHER; note = 2'-O-methylcytidine-3'-phosphate
  modified_base 19: mod_base = OTHER; note = 2'-O-methyladenosine-3'-phosphate
  modified_base 20: mod_base = OTHER; note = 2'-O-methyladenosine-3'-phosphate
  modified_base 21: mod_base = OTHER; note = 2'-O-methyladenosine-3'-phosphate
  modified_base 22: mod_base = OTHER; note = 2'-O-methyluridine-3'-phosphorothioate
  modified_base 23: mod_base = OTHER; note = 2'-O-methyluridine-3'-phosphate
  modified_base 24: mod_base = OTHER; note = inverted (3'-3' linked) abasic deoxyribonucleotide
  misc_feature 1: note = RNA
  misc_feature 2: note = RNA
  misc_feature 3: note = RNA
  misc_feature 4: note = RNA
  misc_feature 5: note = RNA
  misc_feature 6: note = RNA
  misc_feature 7: note = RNA
  misc_feature 8: note = RNA
  misc_feature 9: note = DNA
  misc_feature 10: note = DNA
  misc_feature 11: note = DNA
  misc_feature 12: note = RNA
  misc_feature 13: note = RNA
  misc_feature 14: note = RNA
  misc_feature 15: note = RNA
  misc_feature 16: note = RNA
  misc_feature 17: note = RNA
  misc_feature 18: note = RNA
  misc_feature 19: note = RNA
  misc_feature 20: note = RNA
  misc_feature 21: note = RNA
  misc_feature 22: note = RNA
  misc_feature 23: note = RNA
  misc_feature 24: note = DNA
  source 1..24: mol_type = other RNA
tcgtggtggacttctctcaaattn

SEQ ID NO: 244 - RNA, 24 nt, synthetic construct
  modified_base 1: mod_base = OTHER; note = (NAG37)s-inverted (3'-3' linked) abasic deoxyribonucleotide-5'-phosphorothioate
  modified_base 2: mod_base = OTHER; note = 2'-O-methylguanosine-3'-phosphate
  modified_base 3: mod_base = OTHER; note = 2'-O-methyluridine-3'-phosphate
  modified_base 4: mod_base = OTHER; note = 2'-O-methylguanosine-3'-phosphate
  modified_base 5: mod_base = OTHER; note = 2'-O-methylguanosine-3'-phosphate
  modified_base 6: mod_base = OTHER; note = 2'-O-methyluridine-3'-phosphate
  modified_base 7: mod_base = OTHER; note = 2'-O-methylguanosine-3'-phosphate
  modified_base 8: mod_base = OTHER; note = 2'-O-methylguanosine-3'-phosphate
  modified_base 9: mod_base = OTHER; note = 2'-fluoroadenosine-3'-phosphate
  modified_base 10: mod_base = OTHER; note = 2'-fluorocytidine-3'-phosphate
  modified_base 11: mod_base = OTHER; note = 2'-fluorouridine-3'-phosphate
  modified_base 12: mod_base = OTHER; note = 2'-O-methyluridine-3'-phosphate
  modified_base 13: mod_base = OTHER; note = 2'-O-methylcytidine-3'-phosphate
  modified_base 14: mod_base = OTHER; note = 2'-O-methyluridine-3'-phosphate
  modified_base 15: mod_base = OTHER; note = 2'-O-methylcytidine-3'-phosphate
  modified_base 16: mod_base = OTHER; note = 2'-O-methyluridine-3'-phosphate
  modified_base 17: mod_base = OTHER; note = 2'-O-methylcytidine-3'-phosphate
  modified_base 18: mod_base = OTHER; note = 2'-O-methyladenosine-3'-phosphate
  modified_base 19: mod_base = OTHER; note = 2'-O-methyladenosine-3'-phosphate
  modified_base 20: mod_base = OTHER; note = 2'-O-methyluridine-3'-phosphate
  modified_base 21: mod_base = OTHER; note = 2'-O-methyladenosine-3'-phosphate
  modified_base 22: mod_base = OTHER; note = 2'-O-methyluridine-3'-phosphorothioate
  modified_base 23: mod_base = OTHER; note = 2'-O-methyluridine-3'-phosphate
  modified_base 24: mod_base = OTHER; note = inverted (3'-3' linked) abasic deoxyribonucleotide
  misc_feature 1: note = DNA
  misc_feature 2: note = RNA
  misc_feature 3: note = RNA
  misc_feature 4: note = RNA
  misc_feature 5: note = RNA
  misc_feature 6: note = RNA
  misc_feature 7: note = RNA
  misc_feature 8: note = RNA
  misc_feature 9: note = DNA
  misc_feature 10: note = DNA
  misc_feature 11: note = DNA
  misc_feature 12: note = RNA
  misc_feature 13: note = RNA
  misc_feature 14: note = RNA
  misc_feature 15: note = RNA
  misc_feature 16: note = RNA
  misc_feature 17: note = RNA
  misc_feature 18: note = RNA
  misc_feature 19: note = RNA
  misc_feature 20: note = RNA
  misc_feature 21: note = RNA
  misc_feature 22: note = RNA
  misc_feature 23: note = RNA
  misc_feature 24: note = DNA
  source 1..24: mol_type = other RNA
ngtggtggacttctctcaatattn

SEQ ID NO: 245 - RNA, 25 nt, synthetic construct
  modified_base 1: mod_base = OTHER; note = (NAG37)s-inverted (3'-3' linked) abasic deoxyribonucleotide-5'-phosphorothioate
  modified_base 2: mod_base = OTHER; note = 2'-O-methylcytidine-3'-phosphate
  modified_base 3: mod_base = OTHER; note = 2'-O-methylguanosine-3'-phosphate
  modified_base 4: mod_base = OTHER; note = 2'-O-methyluridine-3'-phosphate
  modified_base 5: mod_base = OTHER; note = 2'-O-methylguanosine-3'-phosphate
  modified_base 6: mod_base = OTHER; note = 2'-O-methylguanosine-3'-phosphate
  modified_base 7: mod_base = OTHER; note = 2'-O-methyluridine-3'-phosphate
  modified_base 8: mod_base = OTHER; note = 2'-O-methylguanosine-3'-phosphate
  modified_base 9: mod_base = OTHER; note = 2'-O-methylguanosine-3'-phosphate
  modified_base 10: mod_base = OTHER; note = 2'-fluoroadenosine-3'-phosphate
  modified_base 11: mod_base = OTHER; note = 2'-fluorocytidine-3'-phosphate
  modified_base 12: mod_base = OTHER; note = 2'-fluorouridine-3'-phosphate
  modified_base 13: mod_base = OTHER; note = 2'-O-methyluridine-3'-phosphate
  modified_base 14: mod_base = OTHER; note = 2'-O-methylcytidine-3'-phosphate
  modified_base 15: mod_base = OTHER; note = 2'-O-methyluridine-3'-phosphate
  modified_base 16: mod_base = OTHER; note = 2'-O-methylcytidine-3'-phosphate
  modified_base 17: mod_base = OTHER; note = 2'-O-methyluridine-3'-phosphate
  modified_base 18: mod_base = OTHER; note = 2'-O-methylcytidine-3'-phosphate
  modified_base 19: mod_base = OTHER; note = 2'-O-methyladenosine-3'-phosphate
  modified_base 20: mod_base = OTHER; note = 2'-O-methyladenosine-3'-phosphate
  modified_base 21: mod_base = OTHER; note = 2'-O-methyluridine-3'-phosphate
  modified_base 22: mod_base = OTHER; note = 2'-O-methyladenosine-3'-phosphate
  modified_base 23: mod_base = OTHER; note = 2'-O-methyluridine-3'-phosphorothioate
  modified_base 24: mod_base = OTHER; note = 2'-O-methyluridine-3'-phosphate
  modified_base 25: mod_base = OTHER; note = inverted (3'-3' linked) abasic deoxyribonucleotide
  misc_feature 1: note = DNA
  misc_feature 2: note = RNA
  misc_feature 3: note = RNA
  misc_feature 4: note = RNA
  misc_feature 5: note = RNA
  misc_feature 6: note = RNA
  misc_feature 7: note = RNA
  misc_feature 8: note = RNA
  misc_feature 9: note = RNA
  misc_feature 10: note = DNA
  misc_feature 11: note = DNA
  misc_feature 12: note = DNA
  misc_feature 13: note = RNA
  misc_feature 14: note = RNA
  misc_feature 15: note = RNA
  misc_feature 16: note = RNA
  misc_feature 17: note = RNA
  misc_feature 18: note = RNA
  misc_feature 19: note = RNA
  misc_feature 20: note = RNA
  misc_feature 21: note = RNA
  misc_feature 22: note = RNA
  misc_feature 23: note = RNA
  misc_feature 24: note = RNA
  misc_feature 25: note = DNA
  source 1..25: mol_type = other RNA
ncgtggtggacttctctcaatattn

SEQ ID NO: 246 - RNA, 25 nt, synthetic construct
  modified_base 1: mod_base = OTHER; note = (NAG37)s-inverted (3'-3' linked) abasic deoxyribonucleotide-5'-phosphorothioate
  modified_base 2: mod_base = OTHER; note = 2'-O-methylcytidine-3'-phosphate
  modified_base 3: mod_base = OTHER; note = 2'-O-methyluridine-3'-phosphate
  modified_base 4: mod_base = OTHER; note = 2'-O-methylcytidine-3'-phosphate
  modified_base 5: mod_base = OTHER; note = 2'-O-methylguanosine-3'-phosphate
  modified_base 6: mod_base = OTHER; note = 2'-O-methyluridine-3'-phosphate
  modified_base 7: mod_base = OTHER; note = 2'-O-methylguanosine-3'-phosphate
  modified_base 8: mod_base = OTHER; note = 2'-O-methylguanosine-3'-phosphate
  modified_base 9: mod_base = OTHER; note = 2'-O-methyluridine-3'-phosphate
  modified_base 10: mod_base = OTHER; note = 2'-O-methylguanosine-3'-phosphate
  modified_base 11: mod_base = OTHER; note = 2'-O-methylguanosine-3'-phosphate
  modified_base 12: mod_base = OTHER; note = 2'-fluoroadenosine-3'-phosphate
  modified_base 13: mod_base = OTHER; note = 2'-fluorocytidine-3'-phosphate
  modified_base 14: mod_base = OTHER; note = 2'-fluorouridine-3'-phosphate
  modified_base 15: mod_base = OTHER; note = 2'-O-methyluridine-3'-phosphate
  modified_base 16: mod_base = OTHER; note = 2'-O-methylcytidine-3'-phosphate
  modified_base 17: mod_base = OTHER; note = 2'-O-methyluridine-3'-phosphate
  modified_base 18: mod_base = OTHER; note = 2'-O-methylcytidine-3'-phosphate
  modified_base 19: mod_base = OTHER; note = 2'-O-methyluridine-3'-phosphate
  modified_base 20: mod_base = OTHER; note = 2'-O-methylcytidine-3'-phosphate
  modified_base 21: mod_base = OTHER; note = 2'-O-methyladenosine-3'-phosphate
  modified_base 22: mod_base = OTHER; note = 2'-O-methyladenosine-3'-phosphate
  modified_base 23: mod_base = OTHER; note = 2'-O-methyluridine-3'-phosphate
  modified_base 24: mod_base = OTHER; note = 2'-O-methyladenosine-3'-phosphorothioate
  modified_base 25: mod_base = OTHER; note = inverted (3'-3' linked) abasic deoxyribonucleotide
  misc_feature 1: note = DNA
  misc_feature 2: note = RNA
  misc_feature 3: note = RNA
  misc_feature 4: note = RNA
  misc_feature 5: note = RNA
  misc_feature 6: note = RNA
  misc_feature 7: note = RNA
  misc_feature 8: note = RNA
  misc_feature 9: note = RNA
  misc_feature 10: note = RNA
  misc_feature 11: note = RNA
  misc_feature 12: note = DNA
  misc_feature 13: note = DNA
  misc_feature 14: note = DNA
  misc_feature 15: note = RNA
  misc_feature 16: note = RNA
  misc_feature 17: note = RNA
  misc_feature 18: note = RNA
  misc_feature 19: note = RNA
  misc_feature 20: note = RNA
  misc_feature 21: note = RNA
  misc_feature 22: note = RNA
  misc_feature 23: note = RNA
  misc_feature 24: note = RNA
  misc_feature 25: note = DNA
  source 1..25: mol_type = other RNA
nctcgtggtggacttctctcaatan

SEQ ID NO: 247 - RNA, 27 nt, synthetic construct
  modified_base 1: mod_base = OTHER; note = (NAG37)s-inverted (3'-3' linked) abasic deoxyribonucleotide-5'-phosphorothioate
  modified_base 2: mod_base = OTHER; note = 2'-O-methylcytidine-3'-phosphate
  modified_base 3: mod_base = OTHER; note = 2'-O-methyluridine-3'-phosphate
  modified_base 4: mod_base = OTHER; note = 2'-O-methylcytidine-3'-phosphate
  modified_base 5: mod_base = OTHER; note = 2'-O-methylguanosine-3'-phosphate
  modified_base 6: mod_base = OTHER; note = 2'-O-methyluridine-3'-phosphate
  modified_base 7: mod_base = OTHER; note = 2'-O-methylguanosine-3'-phosphate
  modified_base 8: mod_base = OTHER; note = 2'-O-methylguanosine-3'-phosphate
  modified_base 9: mod_base = OTHER; note = 2'-O-methyluridine-3'-phosphate
  modified_base 10: mod_base = OTHER; note = 2'-O-methylguanosine-3'-phosphate
  modified_base 11: mod_base = OTHER; note = 2'-O-methylguanosine-3'-phosphate
  modified_base 12: mod_base = OTHER; note = 2'-fluoroadenosine-3'-phosphate
  modified_base 13: mod_base = OTHER; note = 2'-fluorocytidine-3'-phosphate
  modified_base 14: mod_base = OTHER; note = 2'-fluorouridine-3'-phosphate
  modified_base 15: mod_base = OTHER; note = 2'-O-methyluridine-3'-phosphate
  modified_base 16: mod_base = OTHER; note = 2'-O-methylcytidine-3'-phosphate
  modified_base 17: mod_base = OTHER; note = 2'-O-methyluridine-3'-phosphate
  modified_base 18: mod_base = OTHER; note = 2'-O-methylcytidine-3'-phosphate
  modified_base 19: mod_base = OTHER; note = 2'-O-methyluridine-3'-phosphate
  modified_base 20: mod_base = OTHER; note = 2'-O-methylcytidine-3'-phosphate
  modified_base 21: mod_base = OTHER; note = 2'-O-methyladenosine-3'-phosphate
  modified_base 22: mod_base = OTHER; note = 2'-O-methyladenosine-3'-phosphate
  modified_base 23: mod_base = OTHER; note = 2'-O-methyluridine-3'-phosphate
  modified_base 24: mod_base = OTHER; note = 2'-O-methyladenosine-3'-phosphate
  modified_base 25: mod_base = OTHER; note = 2'-O-methyluridine-3'-phosphorothioate
  modified_base 26: mod_base = OTHER; note = 2'-O-methyluridine-3'-phosphate
  modified_base 27: mod_base = OTHER; note = inverted (3'-3' linked) abasic deoxyribonucleotide
  misc_feature 1: note = DNA
  misc_feature 2: note = RNA
  misc_feature 3: note = RNA
  misc_feature 4: note = RNA
  misc_feature 5: note = RNA
  misc_feature 6: note = RNA
  misc_feature 7: note = RNA
  misc_feature 8: note = RNA
  misc_feature 9: note = RNA
  misc_feature 10: note = RNA
  misc_feature 11: note = RNA
  misc_feature 12: note = DNA
  misc_feature 13: note = DNA
  misc_feature 14: note = DNA
  misc_feature 15: note = RNA
  misc_feature 16: note = RNA
  misc_feature 17: note = RNA
  misc_feature 18: note = RNA
  misc_feature 19: note = RNA
  misc_feature 20: note = RNA
  misc_feature 21: note = RNA
  misc_feature 22: note = RNA
  misc_feature 23: note = RNA
  misc_feature 24: note = RNA
  misc_feature 25: note = RNA
  misc_feature 26: note = RNA
  misc_feature 27: note = DNA
  source 1..27: mol_type = other RNA
nctcgtggtggacttctctcaatattn

SEQ ID NO: 248 - RNA, 23 nt, synthetic construct
  modified_base 1: mod_base = OTHER; note = (NAG37)s-inverted (3'-3' linked) abasic deoxyribonucleotide-5'-phosphorothioate
  modified_base 2: mod_base = OTHER; note = 2'-O-methylguanosine-3'-phosphate
  modified_base 3: mod_base = OTHER; note = 2'-O-methylguanosine-3'-phosphate
  modified_base 4: mod_base = OTHER; note = 2'-O-methylcytidine-3'-phosphate
  modified_base 5: mod_base = OTHER; note = 2'-O-methyluridine-3'-phosphate
  modified_base 6: mod_base = OTHER; note = 2'-O-methylguanosine-3'-phosphate
  modified_base 7: mod_base = OTHER; note = 2'-O-methyluridine-3'-phosphate
  modified_base 8: mod_base = OTHER; note = 2'-O-methyladenosine-3'-phosphate
  modified_base 9: mod_base = OTHER; note = 2'-O-methylguanosine-3'-phosphate
  modified_base 10: mod_base = OTHER; note = 2'-fluoroguanosine-3'-phosphate
  modified_base 11: mod_base = OTHER; note = 2'-fluorocytidine-3'-phosphate
  modified_base 12: mod_base = OTHER; note = 2'-fluoroadenosine-3'-phosphate
  modified_base 13: mod_base = OTHER; note = 2'-O-methyluridine-3'-phosphate
  modified_base 14: mod_base = OTHER; note = 2'-O-methyladenosine-3'-phosphate
  modified_base 15: mod_base = OTHER; note = 2'-O-methyladenosine-3'-phosphate
  modified_base 16: mod_base = OTHER; note = 2'-O-methyladenosine-3'-phosphate
  modified_base 17: mod_base = OTHER; note = 2'-O-methyluridine-3'-phosphate
  modified_base 18: mod_base = OTHER; note = 2'-O-methyluridine-3'-phosphate
  modified_base 19: mod_base = OTHER; note = 2'-O-methylguanosine-3'-phosphate
  modified_base 20: mod_base = OTHER; note = 2'-O-methylguanosine-3'-phosphate
  modified_base 21: mod_base = OTHER; note = 2'-O-methyluridine-3'-phosphate
  modified_base 22: mod_base = OTHER; note = 2'-O-methyladenosine-3'-phosphorothioate
  modified_base 23: mod_base = OTHER; note = inverted (3'-3' linked) abasic deoxyribonucleotide
  misc_feature 1: note = DNA
  misc_feature 2: note = RNA
  misc_feature 3: note = RNA
  misc_feature 4: note = RNA
  misc_feature 5: note = RNA
  misc_feature 6: note = RNA
  misc_feature 7: note = RNA
  misc_feature 8: note = RNA
  misc_feature 9: note = RNA
  misc_feature 10: note = DNA
  misc_feature 11: note = DNA
  misc_feature 12: note = DNA
  misc_feature 13: note = RNA
  misc_feature 14: note = RNA
  misc_feature 15: note = RNA
  misc_feature 16: note = RNA
  misc_feature 17: note = RNA
  misc_feature 18: note = RNA
  misc_feature 19: note = RNA
  misc_feature 20: note = RNA
  misc_feature 21: note = RNA
  misc_feature 22: note = RNA
  misc_feature 23: note = DNA
  source 1..23: mol_type = other RNA
nggctgtaggcataaattggtan

SEQ ID NO: 249 - RNA, 25 nt, synthetic construct
  modified_base 1: mod_base = OTHER; note = (NAG37)s-inverted (3'-3' linked) abasic deoxyribonucleotide-5'-phosphorothioate
  modified_base 2: mod_base = OTHER; note = 2'-O-methylguanosine-3'-phosphate
  modified_base 3: mod_base = OTHER; note = 2'-O-methyladenosine-3'-phosphate
  modified_base 4: mod_base = OTHER; note = 2'-O-methylguanosine-3'-phosphate
  modified_base 5: mod_base = OTHER; note = 2'-O-methylguanosine-3'-phosphate
  modified_base 6: mod_base = OTHER; note = 2'-O-methylcytidine-3'-phosphate
  modified_base 7: mod_base = OTHER; note = 2'-O-methyluridine-3'-phosphate
  modified_base 8: mod_base = OTHER; note = 2'-O-methylguanosine-3'-phosphate
  modified_base 9: mod_base = OTHER; note = 2'-O-methyluridine-3'-phosphate
  modified_base 10: mod_base = OTHER; note = 2'-O-methyladenosine-3'-phosphate
  modified_base 11: mod_base = OTHER; note = 2'-O-methylguanosine-3'-phosphate
  modified_base 12: mod_base = OTHER; note = 2'-fluoroguanosine-3'-phosphate
  modified_base 13: mod_base = OTHER; note = 2'-fluorocytidine-3'-phosphate
  modified_base 14: mod_base = OTHER; note = 2'-fluoroadenosine-3'-phosphate
  modified_base 15: mod_base = OTHER; note = 2'-O-methyluridine-3'-phosphate
  modified_base 16: mod_base = OTHER; note = 2'-O-methyladenosine-3'-phosphate
  modified_base 17: mod_base = OTHER; note = 2'-O-methyladenosine-3'-phosphate
  modified_base 18: mod_base = OTHER; note = 2'-O-methyladenosine-3'-phosphate
  modified_base 19: mod_base = OTHER; note = 2'-O-methyluridine-3'-phosphate
  modified_base 20: mod_base = OTHER; note = 2'-O-methyluridine-3'-phosphate
  modified_base 21: mod_base = OTHER; note = 2'-O-methylguanosine-3'-phosphate
  modified_base 22: mod_base = OTHER; note = 2'-O-methylguanosine-3'-phosphate
  modified_base 23: mod_base = OTHER; note = 2'-O-methyluridine-3'-phosphate
  modified_base 24: mod_base = OTHER; note = 2'-O-methyladenosine-3'-phosphorothioate
  modified_base 25: mod_base = OTHER; note = inverted (3'-3' linked) abasic deoxyribonucleotide
  misc_feature 1: note = DNA
  misc_feature 2: note = RNA
  misc_feature 3: note = RNA
  misc_feature 4: note = RNA
  misc_feature 5: note = RNA
  misc_feature 6: note = RNA
  misc_feature 7: note = RNA
  misc_feature 8: note = RNA
  misc_feature 9: note = RNA
  misc_feature 10: note = RNA
  misc_feature 11: note = RNA
  misc_feature 12: note = DNA
  misc_feature 13: note = DNA
  misc_feature 14: note = DNA
  misc_feature 15: note = RNA
  misc_feature 16: note = RNA
  misc_feature 17: note = RNA
  misc_feature 18: note = RNA
  misc_feature 19: note = RNA
  misc_feature 20: note = RNA
  misc_feature 21: note = RNA
  misc_feature 22: note = RNA
  misc_feature 23: note = RNA
  misc_feature 24: note = RNA
  misc_feature 25: note = DNA
  source 1..25: mol_type = other RNA
ngaggctgtaggcataaattggtan

SEQ ID NO: 250 - RNA, 27 nt, synthetic construct
  modified_base 1: mod_base = OTHER; note = (NAG37)s-inverted (3'-3' linked) abasic deoxyribonucleotide-5'-phosphorothioate
  modified_base 2: mod_base = OTHER; note = 2'-O-methylguanosine-3'-phosphate
  modified_base 3: mod_base = OTHER; note = 2'-O-methyladenosine-3'-phosphate
  modified_base 4: mod_base = OTHER; note = 2'-O-methylguanosine-3'-phosphate
  modified_base 5: mod_base = OTHER; note = 2'-O-methylguanosine-3'-phosphate
  modified_base 6: mod_base = OTHER; note = 2'-O-methylcytidine-3'-phosphate
  modified_base 7: mod_base = OTHER; note = 2'-O-methyluridine-3'-phosphate
  modified_base 8: mod_base = OTHER; note = 2'-O-methylguanosine-3'-phosphate
  modified_base 9: mod_base = OTHER; note = 2'-O-methyluridine-3'-phosphate
  modified_base 10: mod_base = OTHER; note = 2'-O-methyladenosine-3'-phosphate
  modified_base 11: mod_base = OTHER; note = 2'-O-methylguanosine-3'-phosphate
  modified_base 12: mod_base = OTHER; note = 2'-fluoroguanosine-3'-phosphate
  modified_base 13: mod_base = OTHER; note = 2'-fluorocytidine-3'-phosphate
  modified_base 14: mod_base = OTHER; note = 2'-fluoroadenosine-3'-phosphate
  modified_base 15: mod_base = OTHER; note = 2'-O-methyluridine-3'-phosphate
  modified_base 16: mod_base = OTHER; note = 2'-O-methyladenosine-3'-phosphate
  modified_base 17: mod_base = OTHER; note = 2'-O-methyladenosine-3'-phosphate
  modified_base 18: mod_base = OTHER; note = 2'-O-methyladenosine-3'-phosphate
  modified_base 19: mod_base = OTHER; note = 2'-O-methyluridine-3'-phosphate
  modified_base 20: mod_base = OTHER; note = 2'-O-methyluridine-3'-phosphate
  modified_base 21: mod_base = OTHER; note = 2'-O-methylguanosine-3'-phosphate
  modified_base 22: mod_base = OTHER; note = 2'-O-methylguanosine-3'-phosphate
  modified_base 23: mod_base = OTHER; note = 2'-O-methyluridine-3'-phosphate
  modified_base 24: mod_base = OTHER; note = 2'-O-methyladenosine-3'-phosphate
  modified_base 25: mod_base = OTHER; note = 2'-O-methyluridine-3'-phosphorothioate
  modified_base 26: mod_base = OTHER; note = 2'-O-methyluridine-3'-phosphate
  modified_base 27: mod_base = OTHER; note = inverted (3'-3' linked) abasic deoxyribonucleotide
  misc_feature 1: note = DNA
  misc_feature 2: note = RNA
  misc_feature 3: note = RNA
  misc_feature 4: note = RNA
  misc_feature 5: note = RNA
  misc_feature 6: note = RNA
  misc_feature 7: note = RNA
  misc_feature 8: note = RNA
  misc_feature 9: note = RNA
  misc_feature 10: note = RNA
  misc_feature 11: note = RNA
  misc_feature 12: note = DNA
  misc_feature 13: note = DNA
  misc_feature 14: note = DNA
  misc_feature 15: note = RNA
  misc_feature 16: note = RNA
  misc_feature 17: note = RNA
  misc_feature 18: note = RNA
  misc_feature 19: note = RNA
  misc_feature 20: note = RNA
  misc_feature 21: note = RNA
  misc_feature 22: note = RNA
  misc_feature 23: note = RNA
  misc_feature 24: note = RNA
  misc_feature 25: note = RNA
  misc_feature 26: note = RNA
  misc_feature 27: note = DNA
  source 1..27: mol_type = other RNA
ngaggctgtaggcataaattggtattn

SEQ ID NO: 251 - RNA, 21 nt, synthetic construct
  modified_base 1: mod_base = OTHER; note = (NAG37)s-inverted (3'-3' linked) abasic deoxyribonucleotide-5'-phosphorothioate
  modified_base 2: mod_base = OTHER; note = 2'-O-methylguanosine-3'-phosphate
  modified_base 3: mod_base = OTHER; note = 2'-O-methylguanosine-3'-phosphate
  modified_base 4: mod_base = OTHER; note = 2'-O-methyladenosine-3'-phosphate
  modified_base 5: mod_base = OTHER; note = 2'-O-methylcytidine-3'-phosphate
  modified_base 6: mod_base = OTHER; note = 2'-O-methyluridine-3'-phosphate
  modified_base 7: mod_base = OTHER; note = 2'-O-methyluridine-3'-phosphate
  modified_base 8: mod_base = OTHER; note = 2'-fluorocytidine-3'-phosphate
  modified_base 9: mod_base = OTHER; note = 2'-fluorouridine-3'-phosphate
  modified_base 10: mod_base = OTHER; note = 2'-fluorocytidine-3'-phosphate
  modified_base 11: mod_base = OTHER; note = 2'-O-methyluridine-3'-phosphate
  modified_base 12: mod_base = OTHER; note = 2'-O-methylcytidine-3'-phosphate
  modified_base 13: mod_base = OTHER; note = 2'-O-methyladenosine-3'-phosphate
  modified_base 14: mod_base = OTHER; note = 2'-O-methyladenosine-3'-phosphate
  modified_base 15: mod_base = OTHER; note = 2'-O-methyluridine-3'-phosphate
  modified_base 16: mod_base = OTHER; note = 2'-O-methyluridine-3'-phosphate
  modified_base 17: mod_base = OTHER; note = 2'-O-methyluridine-3'-phosphate
  modified_base 18: mod_base = OTHER; note = 2'-O-methyluridine-3'-phosphate
  modified_base 19: mod_base = OTHER; note = 2'-O-methylcytidine-3'-phosphate
  modified_base 20: mod_base = OTHER; note = 2'-O-methyluridine-3'-phosphorothioate
  modified_base 21: mod_base = OTHER; note = inverted (3'-3' linked) abasic deoxyribonucleotide
  misc_feature 1: note = DNA
  misc_feature 2: note = RNA
  misc_feature 3: note = RNA
  misc_feature 4: note = RNA
  misc_feature 5: note = RNA
  misc_feature 6: note = RNA
  misc_feature 7: note = RNA
  misc_feature 8: note = DNA
  misc_feature 9: note = DNA
  misc_feature 10: note = DNA
  misc_feature 11: note = RNA
  misc_feature 12: note = RNA
  misc_feature 13: note = RNA
  misc_feature 14: note = RNA
  misc_feature 15: note = RNA
  misc_feature 16: note = RNA
  misc_feature 17: note = RNA
  misc_feature 18: note = RNA
  misc_feature 19: note = RNA
  misc_feature 20: note = RNA
  misc_feature 21: note = DNA
  source 1..21: mol_type = other RNA
nggacttctctcaattttctn

SEQ ID NO: 252 - RNA, 23 nt, synthetic construct
  modified_base 1: mod_base = OTHER; note = (NAG37)s-inverted (3'-3' linked) abasic deoxyribonucleotide-5'-phosphorothioate
  modified_base 2: mod_base = OTHER; note = 2'-O-methylguanosine-3'-phosphate
  modified_base 3: mod_base = OTHER; note = 2'-O-methyluridine-3'-phosphate
  modified_base 4..5: mod_base = OTHER; note = 2'-O-methylguanosine-3'-phosphate
  modified_base 6: mod_base = OTHER; note = 2'-O-methyladenosine-3'-phosphate
  modified_base 7: mod_base = OTHER; note = 2'-O-methylcytidine-3'-phosphate
  modified_base 8..9: mod_base = OTHER; note = 2'-O-methyluridine-3'-phosphate
  modified_base 10: mod_base = OTHER; note = 2'-fluorocytidine-3'-phosphate
  modified_base 11: mod_base = OTHER; note = 2'-fluorouridine-3'-phosphate
  modified_base 12: mod_base = OTHER; note = 2'-fluorocytidine-3'-phosphate
  modified_base 13: mod_base = OTHER; note = 2'-O-methyluridine-3'-phosphate
  modified_base 14: mod_base = OTHER; note = 2'-O-methylcytidine-3'-phosphate
  modified_base 15..16: mod_base = OTHER; note = 2'-O-methyladenosine-3'-phosphate
  modified_base 17..20: mod_base = OTHER; note = 2'-O-methyluridine-3'-phosphate
  modified_base 21: mod_base = OTHER; note = 2'-O-methylcytidine-3'-phosphate
  modified_base 22: mod_base = OTHER; note = 2'-O-methyluridine-3'-phosphorothioate
  modified_base 23: mod_base = OTHER; note = inverted (3'-3' linked) abasic deoxyribonucleotide
  misc_feature 1: note = DNA
  misc_feature 2: note = RNA
  misc_feature 3: note = RNA
  misc_feature 4..5: note = RNA
  misc_feature 6: note = RNA
  misc_feature 7: note = RNA
  misc_feature 8..9: note = RNA
  misc_feature 10: note = DNA
  misc_feature 11: note = DNA
  misc_feature 12: note = DNA
  misc_feature 13: note = RNA
  misc_feature 14: note = RNA
  misc_feature 15..16: note = RNA
  misc_feature 17..20: note = RNA
  misc_feature 21: note = RNA
  misc_feature 22: note = RNA
  misc_feature 23: note = DNA
  source 1..23: mol_type = other RNA
ngtggacttctctcaattttctn

SEQ ID NO: 253 - RNA, 24 nt, synthetic construct
  modified_base 1: mod_base = OTHER; note = (NAG37)s-inverted (3'-3' linked) abasic deoxyribonucleotide-5'-phosphorothioate
  modified_base 2..3: mod_base = OTHER; note = 2'-O-methylguanosine-3'-phosphate
  modified_base 4: mod_base = OTHER; note = 2'-O-methyluridine-3'-phosphate
  modified_base 5..6: mod_base = OTHER; note = 2'-O-methylguanosine-3'-phosphate
  modified_base 7: mod_base = OTHER; note = 2'-O-methyladenosine-3'-phosphate
  modified_base 8: mod_base = OTHER; note = 2'-O-methylcytidine-3'-phosphate
  modified_base 9..10: mod_base = OTHER; note = 2'-O-methyluridine-3'-phosphate
  modified_base 11: mod_base = OTHER; note = 2'-fluorocytidine-3'-phosphate
  modified_base 12: mod_base = OTHER; note = 2'-fluorouridine-3'-phosphate
  modified_base 13: mod_base = OTHER; note = 2'-fluorocytidine-3'-phosphate
  modified_base 14: mod_base = OTHER; note = 2'-O-methyluridine-3'-phosphate
  modified_base 15: mod_base = OTHER; note = 2'-O-methylcytidine-3'-phosphate
  modified_base 16..17: mod_base = OTHER; note = 2'-O-methyladenosine-3'-phosphate
  modified_base 18..21: mod_base = OTHER; note = 2'-O-methyluridine-3'-phosphate
  modified_base 22: mod_base = OTHER; note = 2'-O-methylcytidine-3'-phosphate
  modified_base 23: mod_base = OTHER; note = 2'-O-methyluridine-3'-phosphorothioate
  modified_base 24: mod_base = OTHER; note = inverted (3'-3' linked) abasic deoxyribonucleotide
  misc_feature 1: note = DNA
  misc_feature 2..3: note = RNA
  misc_feature 4: note = RNA
  misc_feature 5..6: note = RNA
  misc_feature 7: note = RNA
  misc_feature 8: note = RNA
  misc_feature 9..10: note = RNA
  misc_feature 11: note = DNA
  misc_feature 12: note = DNA
  misc_feature 13: note = DNA
  misc_feature 14: note = RNA
  misc_feature 15: note = RNA
  misc_feature 16..17: note = RNA
  misc_feature 18..21: note = RNA
  misc_feature 22: note = RNA
  misc_feature 23: note = RNA
  misc_feature 24: note = DNA
  source 1..24: mol_type = other RNA
nggtggacttctctcaattttctn

SEQ ID NO: 254 - RNA, 21 nt, synthetic construct
  modified_base 1: mod_base = OTHER; note = (NAG37)s-inverted (3'-3' linked) abasic deoxyribonucleotide-5'-phosphorothioate
  modified_base 2: mod_base = OTHER; note = 2'-O-methylguanosine-3'-phosphate
  modified_base 3: mod_base = OTHER; note = 2'-O-methylguanosine-3'-phosphate
  modified_base 4: mod_base = OTHER; note = 2'-O-methyladenosine-3'-phosphate
  modified_base 5: mod_base = OTHER; note = 2'-O-methylcytidine-3'-phosphate
  modified_base 6: mod_base = OTHER; note = 2'-O-methyluridine-3'-phosphate
  modified_base 7: mod_base = OTHER; note = 2'-O-methyluridine-3'-phosphate
  modified_base 8: mod_base = OTHER; note = 2'-fluorocytidine-3'-phosphate
  modified_base 9: mod_base = OTHER; note = 2'-fluorouridine-3'-phosphate
  modified_base 10: mod_base = OTHER; note = 2'-fluorocytidine-3'-phosphate
  modified_base 11: mod_base = OTHER; note = 2'-O-methyluridine-3'-phosphate
  modified_base 12: mod_base = OTHER; note = 2'-O-methylcytidine-3'-phosphate
  modified_base 13: mod_base = OTHER; note = 2'-O-methyladenosine-3'-phosphate
  modified_base 14: mod_base = OTHER; note = 2'-O-methyladenosine-3'-phosphate
  modified_base 15: mod_base = OTHER; note = 2'-O-methyluridine-3'-phosphate
  modified_base 16: mod_base = OTHER; note = 2'-O-methyluridine-3'-phosphate
  modified_base 17: mod_base = OTHER; note = 2'-O-methyluridine-3'-phosphate
  modified_base 18: mod_base = OTHER; note = 2'-O-methyluridine-3'-phosphate
  modified_base 19: mod_base = OTHER; note = 2'-O-methylcytidine-3'-phosphate
  modified_base 20: mod_base = OTHER; note = 2'-O-methyladenosine-3'-phosphorothioate
  modified_base 21: mod_base = OTHER; note = inverted (3'-3' linked) abasic deoxyribonucleotide
  misc_feature 1: note = DNA
  misc_feature 2: note = RNA
  misc_feature 3: note = RNA
  misc_feature 4: note = RNA
  misc_feature 5: note = RNA
  misc_feature 6: note = RNA
  misc_feature 7: note = RNA
  misc_feature 8: note = DNA
  misc_feature 9: note = DNA
  misc_feature 10: note = DNA
  misc_feature 11: note = RNA
  misc_feature 12: note = RNA
  misc_feature 13: note = RNA
  misc_feature 14: note = RNA
  misc_feature 15: note = RNA
  misc_feature 16: note = RNA
  misc_feature 17: note = RNA
  misc_feature 18: note = RNA
  misc_feature 19: note = RNA
  misc_feature 20: note = RNA
  misc_feature 21: note = DNA
  source 1..21: mol_type = other RNA
nggacttctctcaattttcan

SEQ ID NO: 255 - RNA, 23 nt, synthetic construct
  modified_base 1: mod_base = OTHER; note = (NAG37)s-inverted (3'-3' linked) abasic deoxyribonucleotide-5'-phosphorothioate
  modified_base 2: mod_base = OTHER; note = 2'-O-methylguanosine-3'-phosphate
  modified_base 3: mod_base = OTHER; note = 2'-O-methyluridine-3'-phosphate
  modified_base 4: mod_base = OTHER; note = 2'-O-methylguanosine-3'-phosphate
  modified_base 5: mod_base = OTHER; note = 2'-O-methylguanosine-3'-phosphate
  modified_base 6: mod_base = OTHER; note = 2'-O-methyladenosine-3'-phosphate
  modified_base 7: mod_base = OTHER; note = 2'-O-methylcytidine-3'-phosphate
  modified_base 8: mod_base = OTHER; note = 2'-O-methyluridine-3'-phosphate
  modified_base 9: mod_base = OTHER; note = 2'-O-methyluridine-3'-phosphate
  modified_base 10: mod_base = OTHER; note = 2'-fluorocytidine-3'-phosphate
  modified_base 11: mod_base = OTHER; note = 2'-fluorouridine-3'-phosphate
  modified_base 12: mod_base = OTHER; note = 2'-fluorocytidine-3'-phosphate
  modified_base 13: mod_base = OTHER; note = 2'-O-methyluridine-3'-phosphate
  modified_base 14: mod_base = OTHER; note = 2'-O-methylcytidine-3'-phosphate
  modified_base 15: mod_base = OTHER; note = 2'-O-methyladenosine-3'-phosphate
  modified_base 16: mod_base = OTHER; note = 2'-O-methyladenosine-3'-phosphate
  modified_base 17: mod_base = OTHER; note = 2'-O-methyluridine-3'-phosphate
  modified_base 18: mod_base = OTHER; note = 2'-O-methyluridine-3'-phosphate
  modified_base 19: mod_base = OTHER; note = 2'-O-methyluridine-3'-phosphate
  modified_base 20: mod_base = OTHER; note = 2'-O-methyluridine-3'-phosphate
  modified_base 21: mod_base = OTHER; note = 2'-O-methylcytidine-3'-phosphate
  modified_base 22: mod_base = OTHER; note = 2'-O-methyladenosine-3'-phosphorothioate
  modified_base 23: mod_base = OTHER; note = inverted (3'-3' linked) abasic deoxyribonucleotide
  misc_feature 1: note = DNA
  misc_feature 2: note = RNA
  misc_feature 3: note = RNA
  misc_feature 4: note = RNA
  misc_feature 5: note = RNA
  misc_feature 6: note = RNA
  misc_feature 7: note = RNA
  misc_feature 8: note = RNA
  misc_feature 9: note = RNA
  misc_feature 10: note = DNA
  misc_feature 11: note = DNA
  misc_feature 12: note = DNA
  misc_feature 13: note = RNA
  misc_feature 14: note = RNA
  misc_feature 15: note = RNA
  misc_feature 16: note = RNA
  misc_feature 17: note = RNA
  misc_feature 18: note = RNA
  misc_feature 19: note = RNA
  misc_feature 20: note = RNA
  misc_feature 21: note = RNA
  misc_feature 22: note = RNA
  misc_feature 23: note = DNA
  source 1..23: mol_type = other RNA
ngtggacttctctcaattttcan

SEQ ID NO: 256 - RNA, 21 nt, synthetic construct
  modified_base 1: mod_base = OTHER; note = (NAG37)s-inverted (3'-3' linked) abasic deoxyribonucleotide-5'-phosphorothioate
  modified_base 2: mod_base = OTHER; note = 2'-O-methylguanosine-3'-phosphate
  modified_base 3: mod_base = OTHER; note = 2'-O-methylcytidine-3'-phosphate
  modified_base 4: mod_base = OTHER; note = 2'-O-methyluridine-3'-phosphate
  modified_base 5: mod_base = OTHER; note = 2'-O-methylguanosine-3'-phosphate
  modified_base 6: mod_base = OTHER; note = 2'-O-methyluridine-3'-phosphate
  modified_base 7: mod_base = OTHER; note = 2'-O-methyladenosine-3'-phosphate
  modified_base 8: mod_base = OTHER; note = 2'-fluoroguanosine-3'-phosphate
  modified_base 9: mod_base = OTHER; note = 2'-fluoroguanosine-3'-phosphate
  modified_base 10: mod_base = OTHER; note = 2'-fluorocytidine-3'-phosphate
  modified_base 11: mod_base = OTHER; note = 2'-O-methyladenosine-3'-phosphate
  modified_base 12: mod_base = OTHER; note = 2'-O-methyluridine-3'-phosphate
  modified_base 13: mod_base = OTHER; note = 2'-O-methyladenosine-3'-phosphate
  modified_base 14: mod_base = OTHER; note = 2'-O-methyladenosine-3'-phosphate
  modified_base 15: mod_base = OTHER; note = 2'-O-methyladenosine-3'-phosphate
  modified_base 16: mod_base = OTHER; note = 2'-O-methyluridine-3'-phosphate
  modified_base 17: mod_base = OTHER; note = 2'-O-methyluridine-3'-phosphate
  modified_base 18: mod_base = OTHER; note = 2'-O-methylguanosine-3'-phosphate
  modified_base 19: mod_base = OTHER; note = 2'-O-methylguanosine-3'-phosphate
  modified_base 20: mod_base = OTHER; note = 2'-O-methyluridine-3'-phosphorothioate
  modified_base 21: mod_base = OTHER; note = inverted (3'-3' linked) abasic deoxyribonucleotide
  misc_feature 1: note = DNA
  misc_feature 2: note = RNA
  misc_feature 3: note = RNA
  misc_feature 4: note = RNA
  misc_feature 5: note = RNA
  misc_feature 6: note = RNA
  misc_feature 7: note = RNA
  misc_feature 8: note = DNA
  misc_feature 9: note = DNA
  misc_feature 10: note = DNA
  misc_feature 11: note = RNA
  misc_feature 12: note = RNA
  misc_feature 13: note = RNA
  misc_feature 14: note = RNA
  misc_feature 15: note = RNA
  misc_feature 16: note = RNA
  misc_feature 17: note = RNA
  misc_feature 18: note = RNA
  misc_feature 19: note = RNA
  misc_feature 20: note = RNA
  misc_feature 21: note = DNA
  source 1..21: mol_type = other RNA
ngctgtaggcataaattggtn

SEQ ID NO: 257 - RNA, 22 nt, synthetic construct
  modified_base 1: mod_base = OTHER; note = (NAG37)s-inverted (3'-3' linked) abasic deoxyribonucleotide-5'-phosphorothioate
  modified_base 2: mod_base = OTHER; note = 2'-O-methylguanosine-3'-phosphate
  modified_base 3: mod_base = OTHER; note = 2'-O-methylguanosine-3'-phosphate
  modified_base 4: mod_base = OTHER; note = 2'-O-methylcytidine-3'-phosphate
  modified_base 5: mod_base = OTHER; note = 2'-O-methyluridine-3'-phosphate
  modified_base 6: mod_base = OTHER; note = 2'-O-methylguanosine-3'-phosphate
  modified_base 7: mod_base = OTHER; note = 2'-O-methyluridine-3'-phosphate
  modified_base 8: mod_base = OTHER; note = 2'-O-methyladenosine-3'-phosphate
  modified_base 9: mod_base = OTHER; note = 2'-fluoroguanosine-3'-phosphate
  modified_base 10: mod_base = OTHER; note = 2'-fluoroguanosine-3'-phosphate
  modified_base 11: mod_base = OTHER; note = 2'-fluorocytidine-3'-phosphate
  modified_base 12: mod_base = OTHER; note = 2'-O-methyladenosine-3'-phosphate
  modified_base 13: mod_base = OTHER; note = 2'-O-methyluridine-3'-phosphate
  modified_base 14: mod_base = OTHER; note = 2'-O-methyladenosine-3'-phosphate
  modified_base 15: mod_base = OTHER; note = 2'-O-methyladenosine-3'-phosphate
  modified_base 16: mod_base = OTHER; note = 2'-O-methyladenosine-3'-phosphate
  modified_base 17: mod_base = OTHER; note = 2'-O-methyluridine-3'-phosphate
  modified_base 18: mod_base = OTHER; note = 2'-O-methyluridine-3'-phosphate
  modified_base 19: mod_base = OTHER; note = 2'-O-methylguanosine-3'-phosphate
  modified_base 20: mod_base = OTHER; note = 2'-O-methylguanosine-3'-phosphate
  modified_base 21: mod_base = OTHER; note = 2'-O-methyluridine-3'-phosphorothioate
  modified_base 22: mod_base = OTHER; note = inverted (3'-3' linked) abasic deoxyribonucleotide
  misc_feature 1: note = DNA
  misc_feature 2: note = RNA
  misc_feature 3: note = RNA
  misc_feature 4: note = RNA
  misc_feature 5: note = RNA
  misc_feature 6: note = RNA
  misc_feature 7: note = RNA
  misc_feature 8: note = RNA
  misc_feature 9: note = DNA
  misc_feature 10: note = DNA
  misc_feature 11: note = DNA
  misc_feature 12: note = RNA
  misc_feature 13: note = RNA
  misc_feature 14: note = RNA
  misc_feature 15: note = RNA
  misc_feature 16: note = RNA
  misc_feature 17: note = RNA
  misc_feature 18: note = RNA
  misc_feature 19: note = RNA
  misc_feature 20: note = RNA
  misc_feature 21: note = RNA
  misc_feature 22: note = DNA
  source 1..22: mol_type = other RNA
nggctgtaggcataaattggtn

SEQ ID NO: 258 - RNA, 24 nt, synthetic construct
  modified_base 1: mod_base = OTHER; note = (NAG37)s-inverted (3'-3' linked) abasic deoxyribonucleotide-5'-phosphorothioate
  modified_base 2: mod_base = OTHER; note = 2'-O-methylguanosine-3'-phosphate
  modified_base 3: mod_base = OTHER; note = 2'-O-methyladenosine-3'-phosphate
  modified_base 4: mod_base = OTHER; note = 2'-O-methylguanosine-3'-phosphate
  modified_base 5: mod_base = OTHER; note = 2'-O-methylguanosine-3'-phosphate
  modified_base 6: mod_base = OTHER; note = 2'-O-methylcytidine-3'-phosphate
  modified_base 7: mod_base = OTHER; note = 2'-O-methyluridine-3'-phosphate
  modified_base 8: mod_base = OTHER; note = 2'-O-methylguanosine-3'-phosphate
  modified_base 9: mod_base = OTHER; note = 2'-O-methyluridine-3'-phosphate
  modified_base 10: mod_base = OTHER; note = 2'-O-methyladenosine-3'-phosphate
  modified_base 11: mod_base = OTHER; note = 2'-fluoroguanosine-3'-phosphate
  modified_base 12: mod_base = OTHER; note = 2'-fluoroguanosine-3'-phosphate
  modified_base 13: mod_base = OTHER; note = 2'-fluorocytidine-3'-phosphate
  modified_base 14: mod_base = OTHER; note = 2'-O-methyladenosine-3'-phosphate
  modified_base 15: mod_base = OTHER; note = 2'-O-methyluridine-3'-phosphate
  modified_base 16: mod_base = OTHER; note = 2'-O-methyladenosine-3'-phosphate
  modified_base 17: mod_base = OTHER; note = 2'-O-methyladenosine-3'-phosphate
  modified_base 18: mod_base = OTHER; note = 2'-O-methyladenosine-3'-phosphate
  modified_base 19: mod_base = OTHER; note = 2'-O-methyluridine-3'-phosphate
  modified_base 20: mod_base = OTHER; note = 2'-O-methyluridine-3'-phosphate
  modified_base 21: mod_base = OTHER; note = 2'-O-methylguanosine-3'-phosphate
  modified_base 22: mod_base = OTHER; note = 2'-O-methylguanosine-3'-phosphate
  modified_base 23: mod_base = OTHER; note = 2'-O-methyluridine-3'-phosphorothioate
  modified_base 24: mod_base = OTHER; note = inverted (3'-3' linked) abasic deoxyribonucleotide
  misc_feature 1: note = DNA
  misc_feature 2: note = RNA
  misc_feature 3: note = RNA
  misc_feature 4: note = RNA
  misc_feature 5: note = RNA
  misc_feature 6: note = RNA
  misc_feature 7: note = RNA
  misc_feature 8: note = RNA
  misc_feature 9: note = RNA
  misc_feature 10: note = RNA
  misc_feature 11: note = DNA
  misc_feature 12: note = DNA
  misc_feature 13: note = DNA
  misc_feature 14: note = RNA
  misc_feature 15: note = RNA
  misc_feature 16: note = RNA
  misc_feature 17: note = RNA
  misc_feature 18: note = RNA
  misc_feature 19: note = RNA
  misc_feature 20: note = RNA
  misc_feature 21: note = RNA
  misc_feature 22: note = RNA
  misc_feature 23: note = RNA
  misc_feature 24: note = DNA
  source 1..24: mol_type = other RNA
ngaggctgtaggcataaattggtn

SEQ ID NO: 259 - RNA, 21 nt, synthetic construct
  modified_base 1: mod_base = OTHER; note = (NAG37)s-inverted (3'-3' linked) abasic deoxyribonucleotide-5'-phosphorothioate
  modified_base 2: mod_base = OTHER; note = 2'-O-methylguanosine-3'-phosphate
  modified_base 3: mod_base = OTHER; note = 2'-O-methylcytidine-3'-phosphate
  modified_base 4: mod_base = OTHER; note = 2'-O-methyluridine-3'-phosphate
  modified_base 5: mod_base = OTHER; note = 2'-O-methylguanosine-3'-phosphate
  modified_base 6: mod_base = OTHER; note = 2'-O-methyluridine-3'-phosphate
  modified_base 7: mod_base = OTHER; note = 2'-O-methyladenosine-3'-phosphate
  modified_base 8: mod_base = OTHER; note = 2'-fluoroguanosine-3'-phosphate
  modified_base 9: mod_base = OTHER; note = 2'-fluoroguanosine-3'-phosphate
  modified_base 10: mod_base = OTHER; note = 2'-fluorocytidine-3'-phosphate
  modified_base 11: mod_base = OTHER; note = 2'-O-methyladenosine-3'-phosphate
  modified_base 12: mod_base = OTHER; note = 2'-O-methyluridine-3'-phosphate
  modified_base 13: mod_base = OTHER; note = 2'-O-methyladenosine-3'-phosphate
  modified_base 14: mod_base = OTHER; note = 2'-O-methyladenosine-3'-phosphate
  modified_base 15: mod_base = OTHER; note = 2'-O-methyladenosine-3'-phosphate
  modified_base 16: mod_base = OTHER; note = 2'-O-methyluridine-3'-phosphate
  modified_base 17: mod_base = OTHER; note = 2'-O-methyluridine-3'-phosphate
  modified_base 18: mod_base = OTHER; note = 2'-O-methylguanosine-3'-phosphate
  modified_base 19: mod_base = OTHER; note = 2'-O-methylguanosine-3'-phosphate
  modified_base 20: mod_base = OTHER; note = 2'-O-methyladenosine-3'-phosphorothioate
  modified_base 21: mod_base = OTHER; note = inverted (3'-3' linked) abasic deoxyribonucleotide
  misc_feature 1: note = DNA
  misc_feature 2: note = RNA
  misc_feature 3: note = RNA
  misc_feature 4: note = RNA
  misc_feature 5: note = RNA
  misc_feature 6: note = RNA
  misc_feature 7: note = RNA
  misc_feature 8: note = DNA
  misc_feature 9: note = DNA
  misc_feature 10: note = DNA
  misc_feature 11: note = RNA
  misc_feature 12: note = RNA
  misc_feature 13: note = RNA
  misc_feature 14: note = RNA
  misc_feature 15: note = RNA
  misc_feature 16: note = RNA
  misc_feature 17: note = RNA
  misc_feature 18: note = RNA
  misc_feature 19: note = RNA
  misc_feature 20: note = RNA
  misc_feature 21: note = DNA
  source 1..21: mol_type = other RNA
ngctgtaggcataaattggan

SEQ ID NO: 260 - RNA, 22 nt, synthetic construct
  modified_base 1: mod_base = OTHER; note = (NAG37)s-inverted (3'-3' linked) abasic deoxyribonucleotide-5'-phosphorothioate
  modified_base 2: mod_base = OTHER; note = 2'-O-methylguanosine-3'-phosphate
  modified_base 3: mod_base = OTHER; note = 2'-O-methylguanosine-3'-phosphate
  modified_base 4: mod_base = OTHER; note = 2'-O-methylcytidine-3'-phosphate
  modified_base 5: mod_base = OTHER; note = 2'-O-methyluridine-3'-phosphate
  modified_base 6: mod_base = OTHER; note = 2'-O-methylguanosine-3'-phosphate
  modified_base 7: mod_base = OTHER; note = 2'-O-methyluridine-3'-phosphate
  modified_base 8: mod_base = OTHER; note = 2'-O-methyladenosine-3'-phosphate
  modified_base 9: mod_base = OTHER; note = 2'-fluoroguanosine-3'-phosphate
  modified_base 10: mod_base = OTHER; note = 2'-fluoroguanosine-3'-phosphate
  modified_base 11: mod_base = OTHER; note = 2'-fluorocytidine-3'-phosphate
  modified_base 12: mod_base = OTHER; note = 2'-O-methyladenosine-3'-phosphate
  modified_base 13: mod_base = OTHER; note = 2'-O-methyluridine-3'-phosphate
  modified_base 14: mod_base = OTHER; note = 2'-O-methyladenosine-3'-phosphate
  modified_base 15: mod_base = OTHER; note = 2'-O-methyladenosine-3'-phosphate
  modified_base 16: mod_base = OTHER; note = 2'-O-methyladenosine-3'-phosphate
  modified_base 17: mod_base = OTHER; note = 2'-O-methyluridine-3'-phosphate
  modified_base 18: mod_base = OTHER; note = 2'-O-methyluridine-3'-phosphate
  modified_base 19: mod_base = OTHER; note = 2'-O-methylguanosine-3'-phosphate
  modified_base 20: mod_base = OTHER; note = 2'-O-methylguanosine-3'-phosphate
  modified_base 21: mod_base = OTHER; note = 2'-O-methyladenosine-3'-phosphorothioate
  modified_base 22: mod_base = OTHER; note = inverted (3'-3' linked) abasic deoxyribonucleotide
  misc_feature 1: note = DNA
  misc_feature 2: note = RNA
  misc_feature 3: note = RNA
  misc_feature 4: note = RNA
  misc_feature 5: note = RNA
  misc_feature 6: note = RNA
  misc_feature 7: note = RNA
  misc_feature 8: note = RNA
  misc_feature 9: note = DNA
  misc_feature 10: note = DNA
  misc_feature 11: note = DNA
  misc_feature 12: note = RNA
  misc_feature 13: note = RNA
  misc_feature 14: note = RNA
  misc_feature 15: note = RNA
  misc_feature 16: note = RNA
  misc_feature 17: note = RNA
  misc_feature 18: note = RNA
  misc_feature 19: note = RNA
  misc_feature 20: note = RNA
  misc_feature 21: note = RNA
  misc_feature 22: note = DNA
  source 1..22: mol_type = other RNA
nggctgtaggcataaattggan

SEQ ID NO: 261 - RNA, 23 nt, synthetic construct
  modified_base 1: mod_base = OTHER; note = (NAG37)s-inverted (3'-3' linked) abasic deoxyribonucleotide-5'-phosphorothioate
  modified_base 2: mod_base = OTHER; note = 2'-O-methyladenosine-3'-phosphate
  modified_base 3: mod_base = OTHER; note = 2'-O-methylguanosine-3'-phosphate
  modified_base 4: mod_base = OTHER; note = 2'-O-methylcytidine-3'-phosphate
  modified_base 5: mod_base = OTHER; note = 2'-O-methyluridine-3'-phosphate
  modified_base 6: mod_base = OTHER; note = 2'-O-methylguanosine-3'-phosphate
  modified_base 7: mod_base = OTHER; note = 2'-O-methyluridine-3'-phosphate
  modified_base 8: mod_base = OTHER; note = 2'-O-methyladenosine-3'-phosphate
  modified_base 9: mod_base = OTHER; note = 2'-O-methylguanosine-3'-phosphate
  modified_base 10: mod_base = OTHER; note = 2'-fluoroguanosine-3'-phosphate
  modified_base 11: mod_base = OTHER; note = 2'-fluorocytidine-3'-phosphate
  modified_base 12: mod_base = OTHER; note = 2'-fluoroadenosine-3'-phosphate
  modified_base 13: mod_base = OTHER; note = 2'-O-methyluridine-3'-phosphate
  modified_base 14: mod_base = OTHER; note = 2'-O-methyladenosine-3'-phosphate
  modified_base 15: mod_base = OTHER; note = 2'-O-methyladenosine-3'-phosphate
  modified_base 16: mod_base = OTHER; note = 2'-O-methyladenosine-3'-phosphate
  modified_base 17: mod_base = OTHER; note = 2'-O-methyluridine-3'-phosphate
  modified_base 18: mod_base = OTHER; note = 2'-O-methyluridine-3'-phosphate
  modified_base 19: mod_base = OTHER; note = 2'-O-methylguanosine-3'-phosphate
  modified_base 20: mod_base = OTHER; note = 2'-O-methylguanosine-3'-phosphate
  modified_base 21: mod_base = OTHER; note = 2'-O-methyluridine-3'-phosphate
  modified_base 22: mod_base = OTHER; note = 2'-O-methyladenosine-3'-phosphorothioate
  modified_base 23: mod_base = OTHER; note = inverted (3'-3' linked) abasic deoxyribonucleotide
  misc_feature 1: note = DNA
  misc_feature 2: note = RNA
  misc_feature 3: note = RNA
  misc_feature 4: note = RNA
  misc_feature 5: note = RNA
  misc_feature 6: note = RNA
  misc_feature 7: note = RNA
  misc_feature 8: note = RNA
  misc_feature 9: note = RNA
  misc_feature 10: note = DNA
  misc_feature 11: note = DNA
  misc_feature 12: note = DNA
  misc_feature 13: note = RNA
  misc_feature 14: note = RNA
  misc_feature 15: note = RNA
  misc_feature 16: note = RNA
  misc_feature 17: note = RNA
  misc_feature 18: note = RNA
  misc_feature 19: note = RNA
  misc_feature 20: note = RNA
  misc_feature 21: note = RNA
  misc_feature 22: note = RNA
  misc_feature 23: note = DNA
  source 1..23: mol_type = other RNA
nagctgtaggcataaattggtan

SEQ ID NO: 262 - RNA, 23 nt, synthetic construct
  modified_base 1: mod_base = OTHER; note = (NAG37)s-inverted (3'-3' linked) abasic deoxyribonucleotide-5'-phosphorothioate
  modified_base 2: mod_base = OTHER; note = 2'-O-methylcytidine-3'-phosphate
  modified_base 3: mod_base = OTHER; note = 2'-O-methylguanosine-3'-phosphate
  modified_base 4: mod_base = OTHER; note = 2'-O-methylcytidine-3'-phosphate
  modified_base 5: mod_base = OTHER; note = 2'-O-methyluridine-3'-phosphate
  modified_base 6: mod_base = OTHER; note = 2'-O-methylguanosine-3'-phosphate
  modified_base 7: mod_base = OTHER; note = 2'-O-methyluridine-3'-phosphate
  modified_base 8: mod_base = OTHER; note = 2'-O-methyladenosine-3'-phosphate
  modified_base 9: mod_base = OTHER; note = 2'-O-methylguanosine-3'-phosphate
  modified_base 10: mod_base = OTHER; note = 2'-fluoroguanosine-3'-phosphate
  modified_base 11: mod_base = OTHER; note = 2'-fluorocytidine-3'-phosphate
  modified_base 12: mod_base = OTHER; note = 2'-fluoroadenosine-3'-phosphate
  modified_base 13: mod_base = OTHER; note = 2'-O-methyluridine-3'-phosphate
  modified_base 14..16: mod_base = OTHER; note = 2'-O-methyladenosine-3'-phosphate
  modified_base 17..18: mod_base = OTHER; note = 2'-O-methyluridine-3'-phosphate
  modified_base 19..20: mod_base = OTHER; note = 2'-O-methylguanosine-3'-phosphate
  modified_base 21: mod_base = OTHER; note = 2'-O-methyluridine-3'-phosphate
  modified_base 22: mod_base = OTHER; note = 2'-O-methyladenosine-3'-phosphorothioate
  modified_base 23: mod_base = OTHER; note = inverted (3'-3' linked) abasic deoxyribonucleotide
  misc_feature 1: note = DNA
  misc_feature 2: note = RNA
  misc_feature 3: note = RNA
  misc_feature 4: note = RNA
  misc_feature 5: note = RNA
  misc_feature 6: note = RNA
  misc_feature 7: note = RNA
  misc_feature 8: note = RNA
  misc_feature 9: note = RNA
  misc_feature 10: note = DNA
  misc_feature 11: note = DNA
  misc_feature 12: note = DNA
  misc_feature 13: note = RNA
  misc_feature 14..16: note = RNA
  misc_feature 17..18: note = RNA
  misc_feature 19..20: note = RNA
  misc_feature 21: note = RNA
  misc_feature 22: note = RNA
  misc_feature 23: note = DNA
  source 1..23: mol_type = other RNA
ncgctgtaggcataaattggtan

SEQ ID NO: 263 - RNA, 23 nt, synthetic construct
  modified_base 1: mod_base = OTHER; note = (NAG37)s-inverted (3'-3' linked) abasic deoxyribonucleotide-5'-phosphorothioate
  modified_base 2: mod_base = OTHER; note = 2'-O-methylguanosine-3'-phosphate
  modified_base 3: mod_base = OTHER; note = 2'-O-methylguanosine-3'-phosphate
  modified_base 4: mod_base = OTHER; note = 2'-O-methylcytidine-3'-phosphate
  modified_base 5: mod_base = OTHER; note = 2'-O-methyluridine-3'-phosphate
  modified_base 6: mod_base = OTHER; note = 2'-O-methylguanosine-3'-phosphate
  modified_base 7: mod_base = OTHER; note = 2'-O-methyluridine-3'-phosphate
  modified_base 8: mod_base = OTHER; note = 2'-O-methyladenosine-3'-phosphate
  modified_base 9: mod_base = OTHER; note = 2'-O-methylguanosine-3'-phosphate
  modified_base 10: mod_base = OTHER; note = 2'-fluoroguanosine-3'-phosphate
  modified_base 11: mod_base = OTHER; note = 2'-fluorocytidine-3'-phosphate
  modified_base 12: mod_base = OTHER; note = 2'-fluoroadenosine-3'-phosphate
  modified_base 13: mod_base = OTHER; note = 2'-O-methyluridine-3'-phosphate
  modified_base 14: mod_base = OTHER; note = 2'-O-methyladenosine-3'-phosphate
  modified_base 15: mod_base = OTHER; note = 2'-O-methyladenosine-3'-phosphate
  modified_base 16: mod_base = OTHER; note = 2'-O-methyladenosine-3'-phosphate
  modified_base 17: mod_base = OTHER; note = 2'-O-methyluridine-3'-phosphate
  modified_base 18: mod_base = OTHER; note = 2'-O-methyluridine-3'-phosphate
  modified_base 19: mod_base = OTHER; note = 2'-O-methylguanosine-3'-phosphate
  modified_base 20: mod_base = OTHER; note = 2'-O-methylguanosine-3'-phosphate
  modified_base 21: mod_base = OTHER; note = 2'-O-methyluridine-3'-phosphate
  modified_base 22: mod_base = OTHER; note = 2'-O-methyluridine-3'-phosphorothioate
  modified_base 23: mod_base = OTHER; note = inverted (3'-3' linked) abasic deoxyribonucleotide
  misc_feature 1: note = DNA
  misc_feature 2: note = RNA
  misc_feature 3: note = RNA
  misc_feature 4: note = RNA
  misc_feature 5: note = RNA
  misc_feature 6: note = RNA
  misc_feature 7: note = RNA
  misc_feature 8: note = RNA
  misc_feature 9: note = RNA
  misc_feature 10: note = DNA
  misc_feature 11: note = DNA
  misc_feature 12: note = DNA
  misc_feature 13: note = RNA
  misc_feature 14: note = RNA
  misc_feature 15: note = RNA
  misc_feature 16: note = RNA
  misc_feature 17: note = RNA
  misc_feature 18: note = RNA
  misc_feature 19: note = RNA
  misc_feature 20: note = RNA
  misc_feature 21: note = RNA
  misc_feature 22: note = RNA
  misc_feature 23: note = DNA
  source 1..23: mol_type = other RNA
nggctgtaggcataaattggttn

SEQ ID NO: 264 - RNA, 23 nt, synthetic construct
  modified_base 1: mod_base = OTHER; note = (NAG37)s-inverted (3'-3' linked) abasic deoxyribonucleotide-5'-phosphorothioate
  modified_base 2: mod_base = OTHER; note = 2'-O-methylcytidine-3'-phosphate
  modified_base 3: mod_base = OTHER; note = 2'-O-methyluridine-3'-phosphate
  modified_base 4: mod_base = OTHER; note = 2'-O-methylguanosine-3'-phosphate
  modified_base 5: mod_base = OTHER; note = 2'-O-methyluridine-3'-phosphate
  modified_base 6: mod_base = OTHER; note = 2'-O-methyladenosine-3'-phosphate
  modified_base 7: mod_base = OTHER; note = 2'-O-methylguanosine-3'-phosphate
  modified_base 8: mod_base = OTHER; note = 2'-fluoroguanosine-3'-phosphate
  modified_base 9: mod_base = OTHER; note = 2'-fluorocytidine-3'-phosphate
  modified_base 10: mod_base = OTHER; note = 2'-fluoroadenosine-3'-phosphate
  modified_base 11: mod_base = OTHER; note = 2'-O-methyluridine-3'-phosphate
  modified_base 12: mod_base = OTHER; note = 2'-O-methyladenosine-3'-phosphate
  modified_base 13: mod_base = OTHER; note = 2'-O-methyladenosine-3'-phosphate
  modified_base 14: mod_base = OTHER; note = 2'-O-methyladenosine-3'-phosphate
  modified_base 15: mod_base = OTHER; note = 2'-O-methyluridine-3'-phosphate
  modified_base 16: mod_base = OTHER; note = 2'-O-methyluridine-3'-phosphate
  modified_base 17: mod_base = OTHER; note = 2'-O-methylguanosine-3'-phosphate
  modified_base 18: mod_base = OTHER; note = 2'-O-methylguanosine-3'-phosphate
  modified_base 19: mod_base = OTHER; note = 2'-O-methyluridine-3'-phosphate
  modified_base 20: mod_base = OTHER; note = 2'-O-methyladenosine-3'-phosphorothioate
  modified_base 21: mod_base = OTHER; note = 2'-O-methyluridine-3'-phosphate
  modified_base 22: mod_base = OTHER; note = 2'-O-methyluridine-3'-phosphorothioate
  modified_base 23: mod_base = OTHER; note = inverted (3'-3' linked) abasic deoxyribonucleotide
  misc_feature 1: note = DNA
  misc_feature 2: note = RNA
  misc_feature 3: note = RNA
  misc_feature 4: note = RNA
  misc_feature 5: note = RNA
  misc_feature 6: note = RNA
  misc_feature 7: note = RNA
  misc_feature 8: note = DNA
  misc_feature 9: note = DNA
  misc_feature 10: note = DNA
  misc_feature 11: note = RNA
  misc_feature 12: note = RNA
  misc_feature 13: note = RNA
  misc_feature 14: note = RNA
  misc_feature 15: note = RNA
  misc_feature 16: note = RNA
  misc_feature 17: note = RNA
  misc_feature 18: note = RNA
  misc_feature 19: note = RNA
  misc_feature 20: note = RNA
  misc_feature 21: note = RNA
  misc_feature 22: note = RNA
  misc_feature 23: note = DNA
  source 1..23: mol_type = other RNA
nctgtaggcataaattggtattn

SEQ ID NO: 265 - RNA, 23 nt, synthetic construct
  modified_base 1: mod_base = OTHER; note = (NAG37)s-inverted (3'-3' linked) abasic deoxyribonucleotide-5'-phosphorothioate
  modified_base 2: mod_base = OTHER; note = 2'-O-methylcytidine-3'-phosphate
  modified_base 3: mod_base = OTHER; note = 2'-O-methyluridine-3'-phosphate
  modified_base 4: mod_base = OTHER; note = 2'-fluoroguanosine-3'-phosphate
  modified_base 5: mod_base = OTHER; note = 2'-O-methyluridine-3'-phosphate
  modified_base 6: mod_base = OTHER; note = 2'-fluoroadenosine-3'-phosphate
  modified_base 7: mod_base = OTHER; note = 2'-O-methylguanosine-3'-phosphate
  modified_base 8: mod_base = OTHER; note = 2'-fluoroguanosine-3'-phosphate
  modified_base 9: mod_base = OTHER; note = 2'-fluorocytidine-3'-phosphate
  modified_base 10: mod_base = OTHER; note = 2'-fluoroadenosine-3'-phosphate
  modified_base 11: mod_base = OTHER; note = 2'-O-methyluridine-3'-phosphate
  modified_base 12: mod_base = OTHER; note = 2'-fluoroadenosine-3'-phosphate
  modified_base 13: mod_base = OTHER; note = 2'-O-methyladenosine-3'-phosphate
  modified_base 14: mod_base = OTHER; note = 2'-fluoroadenosine-3'-phosphate
  modified_base 15: mod_base = OTHER; note = 2'-O-methyluridine-3'-phosphate
  modified_base 16: mod_base = OTHER; note = 2'-fluorouridine-3'-phosphate
  modified_base 17: mod_base = OTHER; note = 2'-O-methylguanosine-3'-phosphate
  modified_base 18: mod_base = OTHER; note = 2'-fluoroguanosine-3'-phosphate
  modified_base 19: mod_base = OTHER; note = 2'-O-methyluridine-3'-phosphate
  modified_base 20: mod_base = OTHER; note = 2'-O-methyladenosine-3'-phosphorothioate
  modified_base 21: mod_base = OTHER; note = 2'-O-methyluridine-3'-phosphate
  modified_base 22: mod_base = OTHER; note = 2'-O-methyluridine-3'-phosphorothioate
  modified_base 23: mod_base = OTHER; note = inverted (3'-3' linked) abasic deoxyribonucleotide
  misc_feature 1: note = DNA
  misc_feature 2: note = RNA
  misc_feature 3: note = RNA
  misc_feature 4: note = DNA
  misc_feature 5: note = RNA
  misc_feature 6: note = DNA
  misc_feature 7: note = RNA
  misc_feature 8: note = DNA
  misc_feature 9: note = DNA
  misc_feature 10: note = DNA
  misc_feature 11: note = RNA
  misc_feature 12: note = DNA
  misc_feature 13: note = RNA
  misc_feature 14: note = DNA
  misc_feature 15: note = RNA
  misc_feature 16: note = DNA
  misc_feature 17: note = RNA
  misc_feature 18: note = DNA
  misc_feature 19: note = RNA
  misc_feature 20: note = RNA
  misc_feature 21: note = RNA
  misc_feature 22: note = RNA
  misc_feature 23: note = DNA
  source 1..23: mol_type = other RNA
nctgtaggcataaattggtattn

SEQ ID NO: 266 - RNA, 23 nt, synthetic construct
  modified_base 1: mod_base = OTHER; note = (NAG37)s-inverted (3'-3' linked) abasic deoxyribonucleotide-5'-phosphorothioate
  modified_base 2: mod_base = OTHER; note = 2'-O-methyladenosine-3'-phosphate
  modified_base 3: mod_base = OTHER; note = 2'-O-methylguanosine-3'-phosphate
  modified_base 4: mod_base = OTHER; note = 2'-O-methylguanosine-3'-phosphate
  modified_base 5: mod_base = OTHER; note = 2'-O-methylcytidine-3'-phosphate
  modified_base 6: mod_base = OTHER; note = 2'-O-methyluridine-3'-phosphate
  modified_base 7: mod_base = OTHER; note = 2'-O-methylguanosine-3'-phosphate
  modified_base 8: mod_base = OTHER; note = 2'-O-methyluridine-3'-phosphate
  modified_base 9: mod_base = OTHER; note = 2'-O-methyladenosine-3'-phosphate
  modified_base 10: mod_base = OTHER; note = 2'-fluoroguanosine-3'-phosphate
  modified_base 11: mod_base = OTHER; note = 2'-fluoroguanosine-3'-phosphate
  modified_base 12: mod_base = OTHER; note = 2'-fluorocytidine-3'-phosphate
  modified_base 13: mod_base = OTHER; note = 2'-O-methyladenosine-3'-phosphate
  modified_base 14: mod_base = OTHER; note = 2'-O-methyluridine-3'-phosphate
  modified_base 15: mod_base = OTHER; note = 2'-O-methyladenosine-3'-phosphate
  modified_base 16: mod_base = OTHER; note = 2'-O-methyladenosine-3'-phosphate
  modified_base 17: mod_base = OTHER; note = 2'-O-methyladenosine-3'-phosphate
  modified_base 18: mod_base = OTHER; note = 2'-O-methyluridine-3'-phosphate
  modified_base 19: mod_base = OTHER; note = 2'-O-methyluridine-3'-phosphate
  modified_base 20: mod_base = OTHER; note = 2'-O-methylguanosine-3'-phosphate
  modified_base 21: mod_base = OTHER; note = 2'-O-methylguanosine-3'-phosphate
  modified_base 22: mod_base = OTHER; note = 2'-O-methyluridine-3'-phosphorothioate
  modified_base 23: mod_base = OTHER; note = inverted (3'-3' linked) abasic deoxyribonucleotide
  misc_feature 1: note = DNA
  misc_feature 2: note = RNA
  misc_feature 3: note = RNA
  misc_feature 4: note = RNA
  misc_feature 5: note = RNA
  misc_feature 6: note = RNA
  misc_feature 7: note = RNA
  misc_feature 8: note = RNA
  misc_feature 9: note = RNA
  misc_feature 10: note = DNA
  misc_feature 11: note = DNA
  misc_feature 12: note = DNA
  misc_feature 13: note = RNA
  misc_feature 14: note = RNA
  misc_feature 15: note = RNA
  misc_feature 16: note = RNA
  misc_feature 17: note = RNA
  misc_feature 18: note = RNA
  misc_feature 19: note = RNA
  misc_feature 20: note = RNA
  misc_feature 21: note = RNA
  misc_feature 22: note = RNA
  misc_feature 23: note = DNA
  source 1..23: mol_type = other RNA
naggctgtaggcataaattggtn

SEQ ID NO: 267 - RNA, 23 nt, synthetic construct
  modified_base 1: mod_base = OTHER; note = (NAG37)s-inverted (3'-3' linked) abasic deoxyribonucleotide-5'-phosphorothioate
  modified_base 2: mod_base = OTHER; note = 2'-O-methyladenosine-3'-phosphate
  modified_base 3: mod_base = OTHER; note = 2'-O-methylguanosine-3'-phosphate
  modified_base 4: mod_base = OTHER; note = 2'-O-methylguanosine-3'-phosphate
  modified_base 5: mod_base = OTHER; note = 2'-O-methylcytidine-3'-phosphate
  modified_base 6: mod_base = OTHER; note = 2'-O-methyluridine-3'-phosphate
  modified_base 7: mod_base = OTHER; note = 2'-O-methylguanosine-3'-phosphate
  modified_base 8: mod_base = OTHER; note = 2'-O-methyluridine-3'-phosphate
  modified_base 9: mod_base = OTHER; note = 2'-O-methyladenosine-3'-phosphate
  modified_base 10: mod_base = OTHER; note = 2'-fluoroguanosine-3'-phosphate
  modified_base 11: mod_base = OTHER; note = 2'-fluoroguanosine-3'-phosphate
  modified_base 12: mod_base = OTHER; note = 2'-fluorocytidine-3'-phosphate
  modified_base 13: mod_base = OTHER; note = 2'-O-methyladenosine-3'-phosphate
  modified_base 14: mod_base = OTHER; note = 2'-O-methyluridine-3'-phosphate
  modified_base 15: mod_base = OTHER; note = 2'-O-methyladenosine-3'-phosphate
  modified_base 16: mod_base = OTHER; note = 2'-O-methyladenosine-3'-phosphate
  modified_base 17: mod_base = OTHER; note = 2'-O-methyladenosine-3'-phosphate
  modified_base 18: mod_base = OTHER; note = 2'-O-methyluridine-3'-phosphate
  modified_base 19: mod_base = OTHER; note = 2'-O-methyluridine-3'-phosphate
  modified_base 20: mod_base = OTHER; note = 2'-O-methylguanosine-3'-phosphate
  modified_base 21: mod_base = OTHER; note = 2'-O-methylguanosine-3'-phosphate
  modified_base 22: mod_base = OTHER; note = 2'-O-methyladenosine-3'-phosphorothioate
  modified_base 23: mod_base = OTHER; note = inverted (3'-3' linked) abasic deoxyribonucleotide
  misc_feature 1: note = DNA
  misc_feature 2: note = RNA
  misc_feature 3: note = RNA
  misc_feature 4: note = RNA
  misc_feature 5: note = RNA
  misc_feature 6: note = RNA
  misc_feature 7: note = RNA
  misc_feature 8: note = RNA
  misc_feature 9: note = RNA
  misc_feature 10: note = DNA
  misc_feature 11: note = DNA
  misc_feature 12: note = DNA
  misc_feature 13: note = RNA
  misc_feature 14: note = RNA
  misc_feature 15: note = RNA
  misc_feature 16: note = RNA
  misc_feature 17: note = RNA
  misc_feature 18: note = RNA
  misc_feature 19: note = RNA
  misc_feature 20: note = RNA
  misc_feature 21: note = RNA
  misc_feature 22: note = RNA
  misc_feature 23: note = DNA
  source 1..23: mol_type = other RNA
naggctgtaggcataaattggan

SEQ ID NO: 268 - RNA, 23 nt, synthetic construct
  modified_base 1: mod_base = OTHER; note = (NAG37)s-inverted (3'-3' linked) abasic deoxyribonucleotide-5'-phosphorothioate
  modified_base 2: mod_base = OTHER; note = 2'-O-methylcytidine-3'-phosphate
  modified_base 3: mod_base = OTHER; note = 2'-O-methylguanosine-3'-phosphate
  modified_base 4: mod_base = OTHER; note = 2'-O-methylguanosine-3'-phosphate
  modified_base 5: mod_base = OTHER; note = 2'-O-methylcytidine-3'-phosphate
  modified_base 6: mod_base = OTHER; note = 2'-O-methyluridine-3'-phosphate
  modified_base 7: mod_base = OTHER; note = 2'-O-methylguanosine-3'-phosphate
  modified_base 8: mod_base = OTHER; note = 2'-O-methyluridine-3'-phosphate
  modified_base 9: mod_base = OTHER; note = 2'-O-methyladenosine-3'-phosphate
  modified_base 10: mod_base = OTHER; note = 2'-fluoroguanosine-3'-phosphate
  modified_base 11: mod_base = OTHER; note = 2'-fluoroguanosine-3'-phosphate
  modified_base 12: mod_base = OTHER; note = 2'-fluorocytidine-3'-phosphate
  modified_base 13: mod_base = OTHER; note = 2'-O-methyladenosine-3'-phosphate
  modified_base 14: mod_base = OTHER; note = 2'-O-methyluridine-3'-phosphate
  modified_base 15: mod_base = OTHER; note = 2'-O-methyladenosine-3'-phosphate
  modified_base 16: mod_base = OTHER; note = 2'-O-methyladenosine-3'-phosphate
  modified_base 17: mod_base = OTHER; note = 2'-O-methyladenosine-3'-phosphate
  modified_base 18: mod_base = OTHER; note = 2'-O-methyluridine-3'-phosphate
  modified_base 19: mod_base = OTHER; note = 2'-O-methyluridine-3'-phosphate
  modified_base 20: mod_base = OTHER; note = 2'-O-methylguanosine-3'-phosphate
  modified_base 21: mod_base = OTHER; note = 2'-O-methylguanosine-3'-phosphate
  modified_base 22: mod_base = OTHER; note = 2'-O-methyluridine-3'-phosphorothioate
  modified_base 23: mod_base = OTHER; note = inverted (3'-3' linked) abasic deoxyribonucleotide
  misc_feature 1: note = DNA
  misc_feature 2: note = RNA
  misc_feature 3: note = RNA
  misc_feature 4: note = RNA
  misc_feature 5: note = RNA
  misc_feature 6: note = RNA
  misc_feature 7: note = RNA
  misc_feature 8: note = RNA
  misc_feature 9: note = RNA
  misc_feature 10: note = DNA
  misc_feature 11: note = DNA
  misc_feature 12: note = DNA
  misc_feature 13: note = RNA
  misc_feature 14: note = RNA
  misc_feature 15: note = RNA
  misc_feature 16: note = RNA
  misc_feature 17: note = RNA
  misc_feature 18: note = RNA
  misc_feature 19: note = RNA
  misc_feature 20: note = RNA
  misc_feature 21: note = RNA
  misc_feature 22: note = RNA
  misc_feature 23: note = DNA
  source 1..23: mol_type = other RNA
ncggctgtaggcataaattggtn

SEQ ID NO: 269 - RNA, 23 nt, synthetic construct
  modified_base 1: mod_base = OTHER; note = (NAG37)s-inverted (3'-3' linked) abasic deoxyribonucleotide-5'-phosphorothioate
  modified_base 2: mod_base = OTHER; note = 2'-O-methylcytidine-3'-phosphate
  modified_base 3: mod_base = OTHER; note = 2'-O-methylguanosine-3'-phosphate
  modified_base 4: mod_base = OTHER; note = 2'-O-methylguanosine-3'-phosphate
  modified_base 5: mod_base = OTHER; note = 2'-O-methylcytidine-3'-phosphate
  modified_base 6: mod_base = OTHER; note = 2'-O-methyluridine-3'-phosphate
  modified_base 7: mod_base = OTHER; note = 2'-O-methylguanosine-3'-phosphate
  modified_base 8: mod_base = OTHER; note = 2'-O-methyluridine-3'-phosphate
  modified_base 9: mod_base = OTHER; note = 2'-O-methyladenosine-3'-phosphate
  modified_base 10: mod_base = OTHER; note = 2'-fluoroguanosine-3'-phosphate
  modified_base 11: mod_base = OTHER; note = 2'-fluoroguanosine-3'-phosphate
  modified_base 12: mod_base = OTHER; note = 2'-fluorocytidine-3'-phosphate
  modified_base 13: mod_base = OTHER; note = 2'-O-methyladenosine-3'-phosphate
  modified_base 14: mod_base = OTHER; note = 2'-O-methyluridine-3'-phosphate
  modified_base 15: mod_base = OTHER; note = 2'-O-methyladenosine-3'-phosphate
  modified_base 16: mod_base = OTHER; note = 2'-O-methyladenosine-3'-phosphate
  modified_base 17: mod_base = OTHER; note = 2'-O-methyladenosine-3'-phosphate
  modified_base 18: mod_base = OTHER; note = 2'-O-methyluridine-3'-phosphate
  modified_base 19: mod_base = OTHER; note = 2'-O-methyluridine-3'-phosphate
  modified_base 20: mod_base = OTHER; note = 2'-O-methylguanosine-3'-phosphate
  modified_base 21: mod_base = OTHER; note = 2'-O-methylguanosine-3'-phosphate
  modified_base 22: mod_base = OTHER; note = 2'-O-methyladenosine-3'-phosphorothioate
  modified_base 23: mod_base = OTHER; note = inverted (3'-3' linked) abasic deoxyribonucleotide
  misc_feature 1: note = DNA
  misc_feature 2: note = RNA
  misc_feature 3: note = RNA
  misc_feature 4: note = RNA
  misc_feature 5: note = RNA
  misc_feature 6: note = RNA
  misc_feature 7: note = RNA
  misc_feature 8: note = RNA
  misc_feature 9: note = RNA
  misc_feature 10: note = DNA
  misc_feature 11: note = DNA
  misc_feature 12: note = DNA
  misc_feature 13: note = RNA
  misc_feature 14: note = RNA
  misc_feature 15: note = RNA
  misc_feature 16: note = RNA
  misc_feature 17: note = RNA
  misc_feature 18: note = RNA
  misc_feature 19: note = RNA
  misc_feature 20: note = RNA
  misc_feature 21: note = RNA
  misc_feature 22: note = RNA
  misc_feature 23: note = DNA
  source 1..23: mol_type = other RNA
ncggctgtaggcataaattggan

SEQ ID NO: 270 - RNA, 23 nt, synthetic construct
  modified_base 1: mod_base = OTHER; note = (NAG37)s-inverted (3'-3' linked) abasic deoxyribonucleotide-5'-phosphorothioate
  modified_base 2: mod_base = OTHER; note = 2'-O-methylcytidine-3'-phosphate
  modified_base 3: mod_base = OTHER; note = 2'-O-methylcytidine-3'-phosphate
  modified_base 4: mod_base = OTHER; note = 2'-O-methylcytidine-3'-phosphate
  modified_base 5: mod_base = OTHER; note = 2'-O-methyluridine-3'-phosphate
  modified_base 6: mod_base = OTHER; note = 2'-O-methylguanosine-3'-phosphate
  modified_base 7: mod_base = OTHER; note = 2'-O-methyluridine-3'-phosphate
  modified_base 8: mod_base = OTHER; note = 2'-O-methyladenosine-3'-phosphate
  modified_base 9: mod_base = OTHER; note = 2'-O-methylguanosine-3'-phosphate
  modified_base 10: mod_base = OTHER; note = 2'-fluoroguanosine-3'-phosphate
  modified_base 11: mod_base = OTHER; note = 2'-fluorocytidine-3'-phosphate
  modified_base 12: mod_base = OTHER; note = 2'-fluoroadenosine-3'-phosphate
  modified_base 13: mod_base = OTHER; note = 2'-O-methyluridine-3'-phosphate
  modified_base 14: mod_base = OTHER; note = 2'-O-methyladenosine-3'-phosphate
  modified_base 15: mod_base = OTHER; note = 2'-O-methyladenosine-3'-phosphate
  modified_base 16: mod_base = OTHER; note = 2'-O-methyladenosine-3'-phosphate
  modified_base 17: mod_base = OTHER; note = 2'-O-methyluridine-3'-phosphate
  modified_base 18: mod_base = OTHER; note = 2'-O-methyluridine-3'-phosphate
  modified_base 19: mod_base = OTHER; note = 2'-O-methylguanosine-3'-phosphate
  modified_base 20: mod_base = OTHER; note = 2'-O-methylguanosine-3'-phosphate
  modified_base 21: mod_base = OTHER; note = 2'-O-methyluridine-3'-phosphate
  modified_base 22: mod_base = OTHER; note = 2'-O-methyladenosine-3'-phosphorothioate
  modified_base 23: mod_base = OTHER; note = inverted (3'-3' linked) abasic deoxyribonucleotide
  misc_feature 1: note = DNA
  misc_feature 2: note = RNA
  misc_feature 3: note = RNA
  misc_feature 4: note = RNA
  misc_feature 5: note = RNA
  misc_feature 6: note = RNA
  misc_feature 7: note = RNA
  misc_feature 8: note = RNA
  misc_feature 9: note = RNA
  misc_feature 10: note = DNA
  misc_feature 11: note = DNA
  misc_feature 12: note = DNA
  misc_feature 13: note = RNA
  misc_feature 14: note = RNA
  misc_feature 15: note = RNA
  misc_feature 16: note = RNA
  misc_feature 17: note = RNA
  misc_feature 18: note = RNA
  misc_feature 19: note = RNA
  misc_feature 20: note = RNA
  misc_feature 21: note = RNA
  misc_feature 22: note = RNA
  misc_feature 23: note = DNA
  source 1..23: mol_type = other RNA
nccctgtaggcataaattggtan

SEQ ID NO: 271 - RNA, 22 nt, synthetic construct
  modified_base 1: mod_base = OTHER; note = (NAG37)-2'-O-methylcytidine-3'-phosphorothioate
  modified_base 2: mod_base = OTHER; note = 2'-O-methylguanosine-3'-phosphate
  modified_base 3: mod_base = OTHER; note = 2'-O-methylcytidine-3'-phosphate
  modified_base 4: mod_base = OTHER; note = 2'-O-methyluridine-3'-phosphate
  modified_base 5: mod_base = OTHER; note = 2'-O-methylguanosine-3'-phosphate
  modified_base 6: mod_base = OTHER; note = 2'-O-methyluridine-3'-phosphate
  modified_base 7: mod_base = OTHER; note = 2'-O-methyladenosine-3'-phosphate
  modified_base 8: mod_base = OTHER; note = 2'-O-methylguanosine-3'-phosphate
  modified_base 9: mod_base = OTHER; note = 2'-fluoroguanosine-3'-phosphate
  modified_base 10: mod_base = OTHER; note = 2'-fluorocytidine-3'-phosphate
  modified_base 11: mod_base = OTHER; note = 2'-fluoroadenosine-3'-phosphate
  modified_base 12: mod_base = OTHER; note = 2'-O-methyluridine-3'-phosphate
  modified_base 13..15: mod_base = OTHER; note = 2'-O-methyladenosine-3'-phosphate
  modified_base 16..17: mod_base = OTHER; note = 2'-O-methyluridine-3'-phosphate
  modified_base 18..19: mod_base = OTHER; note = 2'-O-methylguanosine-3'-phosphate
  modified_base 20: mod_base = OTHER; note = 2'-O-methyluridine-3'-phosphate
  modified_base 21: mod_base = OTHER; note = 2'-O-methyladenosine-3'-phosphorothioate
  modified_base 22: mod_base = OTHER; note = inverted (3'-3' linked) abasic deoxyribonucleotide
  misc_feature 1: note = RNA
  misc_feature 2: note = RNA
  misc_feature 3: note = RNA
  misc_feature 4: note = RNA
  misc_feature 5: note = RNA
  misc_feature 6: note = RNA
  misc_feature 7: note = RNA
  misc_feature 8: note = RNA
  misc_feature 9: note = DNA
  misc_feature 10: note = DNA
  misc_feature 11: note = DNA
  misc_feature 12: note = RNA
  misc_feature 13..15: note = RNA
  misc_feature 16..17: note = RNA
  misc_feature 18..19: note = RNA
  misc_feature 20: note = RNA
  misc_feature 21: note = RNA
  misc_feature 22: note = DNA
  source 1..22: mol_type = other RNA
cgctgtaggcataaattggtan

SEQ ID NO: 272 - RNA, 22 nt, synthetic construct
  modified_base 1: mod_base = OTHER; note = (NAG37)-2'-O-methylcytidine-3'-phosphorothioate
  modified_base 2: mod_base = OTHER; note = 2'-O-methylcytidine-3'-phosphate
  modified_base 3: mod_base = OTHER; note = 2'-O-methylcytidine-3'-phosphate
  modified_base 4: mod_base = OTHER; note = 2'-O-methyluridine-3'-phosphate
  modified_base 5: mod_base = OTHER; note = 2'-O-methylguanosine-3'-phosphate
  modified_base 6: mod_base = OTHER; note = 2'-O-methyluridine-3'-phosphate
  modified_base 7: mod_base = OTHER; note = 2'-O-methyladenosine-3'-phosphate
  modified_base 8: mod_base = OTHER; note = 2'-O-methylguanosine-3'-phosphate
  modified_base 9: mod_base = OTHER; note = 2'-fluoroguanosine-3'-phosphate
  modified_base 10: mod_base = OTHER; note = 2'-fluorocytidine-3'-phosphate
  modified_base 11: mod_base = OTHER; note = 2'-fluoroadenosine-3'-phosphate
  modified_base 12: mod_base = OTHER; note = 2'-O-methyluridine-3'-phosphate
  modified_base 13: mod_base = OTHER; note = 2'-O-methyladenosine-3'-phosphate
  modified_base 14: mod_base = OTHER; note = 2'-O-methyladenosine-3'-phosphate
  modified_base 15: mod_base = OTHER; note = 2'-O-methyladenosine-3'-phosphate
  modified_base 16: mod_base = OTHER; note = 2'-O-methyluridine-3'-phosphate
  modified_base 17: mod_base = OTHER; note = 2'-O-methyluridine-3'-phosphate
  modified_base 18: mod_base = OTHER; note = 2'-O-methylguanosine-3'-phosphate
  modified_base 19: mod_base = OTHER; note = 2'-O-methylguanosine-3'-phosphate
  modified_base 20: mod_base = OTHER; note = 2'-O-methyluridine-3'-phosphate
  modified_base 21: mod_base = OTHER; note = 2'-O-methyladenosine-3'-phosphorothioate
  modified_base 22: mod_base = OTHER; note = inverted (3'-3' linked) abasic deoxyribonucleotide
  misc_feature 1: note = RNA
  misc_feature 2: note = RNA
  misc_feature 3: note = RNA
  misc_feature 4: note = RNA
  misc_feature 5: note = RNA
  misc_feature 6: note = RNA
  misc_feature 7: note = RNA
  misc_feature 8: note = RNA
  misc_feature 9: note = DNA
  misc_feature 10: note = DNA
  misc_feature 11: note = DNA
  misc_feature 12: note = RNA
  misc_feature 13: note = RNA
  misc_feature 14: note = RNA
  misc_feature 15: note = RNA
  misc_feature 16: note = RNA
  misc_feature 17: note = RNA
  misc_feature 18: note = RNA
  misc_feature 19: note = RNA
  misc_feature 20: note = RNA
  misc_feature 21: note = RNA
  misc_feature 22: note = DNA
  source 1..22: mol_type = other RNA
ccctgtaggcataaattggtan

SEQ ID NO: 273 - RNA, 23 nt, synthetic construct
  modified_base 1: mod_base = OTHER; note = (NAG25)s-inverted (3'-3' linked) abasic deoxyribonucleotide-5'-phosphorothioate
  modified_base 2: mod_base = OTHER; note = 2'-O-methylguanosine-3'-phosphate
  modified_base 3: mod_base = OTHER; note = 2'-O-methyluridine-3'-phosphate
  modified_base 4..5: mod_base = OTHER; note = 2'-O-methylguanosine-3'-phosphate
  modified_base 6: mod_base = OTHER; note = 2'-O-methyladenosine-3'-phosphate
  modified_base 7: mod_base = OTHER; note = 2'-O-methylcytidine-3'-phosphate
  modified_base 8..9: mod_base = OTHER; note = 2'-O-methyluridine-3'-phosphate
  modified_base 10: mod_base = OTHER; note = 2'-fluorocytidine-3'-phosphate
  modified_base 11: mod_base = OTHER; note = 2'-fluorouridine-3'-phosphate
  modified_base 12: mod_base = OTHER; note = 2'-fluorocytidine-3'-phosphate
  modified_base 13: mod_base = OTHER; note = 2'-O-methyluridine-3'-phosphate
  modified_base 14: mod_base = OTHER; note = 2'-O-methylcytidine-3'-phosphate
  modified_base 15..16: mod_base = OTHER; note = 2'-O-methyladenosine-3'-phosphate
  modified_base 17..20: mod_base = OTHER; note = 2'-O-methyluridine-3'-phosphate
  modified_base 21: mod_base = OTHER; note = 2'-O-methylcytidine-3'-phosphate
  modified_base 22: mod_base = OTHER; note = 2'-O-methyluridine-3'-phosphorothioate
  modified_base 23: mod_base = OTHER; note = inverted (3'-3' linked) abasic deoxyribonucleotide
  misc_feature 1: note = DNA
  misc_feature 2: note = RNA
  misc_feature 3: note = RNA
  misc_feature 4..5: note = RNA
  misc_feature 6: note = RNA
  misc_feature 7: note = RNA
  misc_feature 8..9: note = RNA
  misc_feature 10: note = DNA
  misc_feature 11: note = DNA
  misc_feature 12: note = DNA
  misc_feature 13: note = RNA
  misc_feature 14: note = RNA
  misc_feature 15..16: note = RNA
  misc_feature 17..20: note = RNA
  misc_feature 21: note = RNA
  misc_feature 22: note = RNA
  misc_feature 23: note = DNA
  source 1..23: mol_type = other RNA
ngtggacttctctcaattttctn

SEQ ID NO: 274 - RNA, 23 nt, synthetic construct
  modified_base 1: mod_base = OTHER; note = (NAG25)s-inverted (3'-3' linked) abasic deoxyribonucleotide-5'-phosphorothioate
  modified_base 2: mod_base = OTHER; note = 2'-O-methylcytidine-3'-phosphate
  modified_base 3: mod_base = OTHER; note = 2'-O-methylguanosine-3'-phosphate
  modified_base 4: mod_base = OTHER; note = 2'-O-methylcytidine-3'-phosphate
  modified_base 5: mod_base = OTHER; note = 2'-O-methyluridine-3'-phosphate
  modified_base 6: mod_base = OTHER; note = 2'-O-methylguanosine-3'-phosphate
  modified_base 7: mod_base = OTHER; note = 2'-O-methyluridine-3'-phosphate
  modified_base 8: mod_base = OTHER; note = 2'-O-methyladenosine-3'-phosphate
  modified_base 9: mod_base = OTHER; note = 2'-O-methylguanosine-3'-phosphate
  modified_base 10: mod_base = OTHER; note = 2'-fluoroguanosine-3'-phosphate
  modified_base 11: mod_base = OTHER; note = 2'-fluorocytidine-3'-phosphate
  modified_base 12: mod_base = OTHER; note = 2'-fluoroadenosine-3'-phosphate
  modified_base 13: mod_base = OTHER; note = 2'-O-methyluridine-3'-phosphate
  modified_base 14..16: mod_base = OTHER; note = 2'-O-methyladenosine-3'-phosphate
  modified_base 17..18: mod_base = OTHER; note = 2'-O-methyluridine-3'-phosphate
  modified_base 19..20: mod_base = OTHER; note = 2'-O-methylguanosine-3'-phosphate
  modified_base 21: mod_base = OTHER; note = 2'-O-methyluridine-3'-phosphate
  modified_base 22: mod_base = OTHER; note = 2'-O-methyladenosine-3'-phosphorothioate
  modified_base 23: mod_base = OTHER; note = inverted (3'-3' linked) abasic deoxyribonucleotide
  misc_feature 1: note = DNA
  misc_feature 2: note = RNA
  misc_feature 3: note = RNA
  misc_feature 4: note = RNA
  misc_feature 5: note = RNA
  misc_feature 6: note = RNA
  misc_feature 7: note = RNA
  misc_feature 8: note = RNA
  misc_feature 9: note = RNA
  misc_feature 10: note = DNA
  misc_feature 11: note = DNA
  misc_feature 12: note = DNA
  misc_feature 13: note = RNA
  misc_feature 14..16: note = RNA
  misc_feature 17..18: note = RNA
  misc_feature 19..20: note = RNA
  misc_feature 21: note = RNA
  misc_feature 22: note = RNA
  misc_feature 23: note = DNA
  source 1..23: mol_type = other RNA
ncgctgtaggcataaattggtan

SEQ ID NO: 275 - RNA, 25 nt, synthetic construct
  modified_base 25: mod_base = OTHER; note = thymine
  misc_feature 1..25: note = HBV RNAi Agent sense strand unmodified sequence
  source 1..25: mol_type = other RNA
ttgcctgtaggcataaattggtatt

SEQ ID NO: 276 - RNA, 26 nt, synthetic construct
  misc_feature 1..26: note = HBV RNAi Agent sense strand unmodified sequence
  source 1..26: mol_type = other RNA
tatatgcctgtaggcataaattggta

SEQ ID NO: 277 - RNA, 26 nt, synthetic construct
  modified_base 25: mod_base = OTHER; note = thymine
  misc_feature 1..26: note = HBV RNAi Agent sense strand unmodified sequence
  source 1..26: mol_type = other RNA
gcggaggctgtaggcataaattggta

SEQ ID NO: 278 - RNA, 21 nt, synthetic construct
  misc_feature 1..21: note = HBV RNAi Agent sense strand unmodified sequence
  source 1..21: mol_type = other RNA
ctgtaggcataaattggtatt

SEQ ID NO: 279 - RNA, 21 nt, synthetic construct
  misc_feature 1..21: note = HBV RNAi Agent sense strand unmodified sequence
  source 1..21: mol_type = other RNA
gcctgtaggcataaattggta

SEQ ID NO: 280 - RNA, 21 nt, synthetic construct
  modified_base 20: mod_base = OTHER; note = thymine
  misc_feature 1..21: note = HBV RNAi Agent sense strand unmodified sequence
  source 1..21: mol_type = other RNA
gcctgtaggcataaattggta

SEQ ID NO: 281 - RNA, 21 nt, synthetic construct
  misc_feature 1..21: note = HBV RNAi Agent sense strand unmodified sequence
  source 1..21: mol_type = other RNA
aactgtaggcataaattggta

SEQ ID NO: 282 - RNA, 21 nt, synthetic construct
  misc_feature 1..21: note = HBV RNAi Agent sense strand unmodified sequence
  source 1..21: mol_type = other RNA
tcgtggtggacttctctcaat

SEQ ID NO: 283 - RNA, 21 nt, synthetic construct
  misc_feature 1..21: note = HBV RNAi Agent sense strand unmodified sequence
  source 1..21: mol_type = other RNA
aagtggtggacttctctcaat

SEQ ID NO: 284 - RNA, 21 nt, synthetic construct
  modified_base 21: mod_base = OTHER; note = thymine
  misc_feature 1..21: note = HBV RNAi Agent sense strand unmodified sequence
  source 1..21: mol_type = other RNA
tcgtggtggacttctctcaat

SEQ ID NO: 285 - RNA, 21 nt, synthetic construct
  misc_feature 1..21: note = HBV RNAi Agent sense strand unmodified sequence
  source 1..21: mol_type = other RNA
cgtggtggacttctctcaatt

SEQ ID NO: 286 - RNA, 21 nt, synthetic construct
  misc_feature 1..21: note = HBV RNAi Agent sense strand unmodified sequence
  source 1..21: mol_type = other RNA
aatggtggacttctctcaatt

SEQ ID NO: 287 - RNA, 21 nt, synthetic construct
  modified_base 20..21: mod_base = OTHER; note = thymine
  misc_feature 1..21: note = HBV RNAi Agent sense strand unmodified sequence
  source 1..21: mol_type = other RNA
cgtggtggacttctctcaatt

SEQ ID NO: 288 - RNA, 21 nt, synthetic construct
  misc_feature 1..21: note = HBV RNAi Agent sense strand unmodified sequence
  source 1..21: mol_type = other RNA
ggacttctctcaattttctaa

SEQ ID NO: 289 - RNA, 21 nt, synthetic construct
  misc_feature 1..21: note = HBV RNAi Agent sense strand unmodified sequence
  source 1..21: mol_type = other RNA
cgtggtggacttctctcaata

SEQ ID NO: 290 - RNA, 21 nt, synthetic construct
  misc_feature 1..21: note = HBV RNAi Agent sense strand unmodified sequence
  source 1..21: mol_type = other RNA
tcgtggtggacttctctcaaa

SEQ ID NO: 291 - RNA, 21 nt, synthetic construct
  misc_feature 1..21: note = HBV RNAi Agent sense strand unmodified sequence
  source 1..21: mol_type = other RNA
acctgtaggcataaattggta

SEQ ID NO: 292 - RNA, 19 nt, synthetic construct
  misc_feature 1..19: note = HBV RNAi Agent sense strand unmodified sequence
  source 1..19: mol_type = other RNA
ctgtaggcataaattggta

SEQ ID NO: 293 - RNA, 20 nt, synthetic construct
  misc_feature 1..20: note = HBV RNAi Agent sense strand unmodified sequence
  source 1..20: mol_type = other RNA
actgtaggcataaattggta

SEQ ID NO: 294 - RNA, 21 nt, synthetic construct
  misc_feature 1..21: note = HBV RNAi Agent sense strand unmodified sequence
  source 1..21: mol_type = other RNA
ggctgtaggcataaattggta

SEQ ID NO: 295 - RNA, 21 nt, synthetic construct
  misc_feature 1..21: note = HBV RNAi Agent sense strand unmodified sequence
  source 1..21: mol_type = other RNA
aagtggtggacttctctcaaa

SEQ ID NO: 296 - RNA, 21 nt, synthetic construct
  misc_feature 1..21: note = HBV RNAi Agent sense strand unmodified sequence
  source 1..21: mol_type = other RNA
ccgtggtggacttctctcaat

SEQ ID NO: 297 - RNA, 22 nt, synthetic construct
  misc_feature 1..22: note = HBV RNAi Agent sense strand unmodified sequence
  source 1..22: mol_type = other RNA
ctcgtggtggacttctctcaat

SEQ ID NO: 298 - RNA, 19 nt, synthetic construct
  misc_feature 1..19: note = HBV RNAi Agent sense strand unmodified sequence
  source 1..19: mol_type = other RNA
gtggtggacttctctcaat

SEQ ID NO: 299 - RNA, 21 nt, synthetic construct
  misc_feature 1..21: note = HBV RNAi Agent sense strand unmodified sequence
  source 1..21: mol_type = other RNA
gtggtggacttctctcaattt

SEQ ID NO: 300 - RNA, 22 nt, synthetic construct
  misc_feature 1..22: note = HBV RNAi Agent sense strand unmodified sequence
  source 1..22: mol_type = other RNA
tcgtggtggacttctctcaatt

SEQ ID NO: 301 - RNA, 19 nt, synthetic construct
  misc_feature 1..19: note = HBV RNAi Agent sense strand unmodified sequence
  source 1..19: mol_type = other RNA
tggtggacttctctcaatt

SEQ ID NO: 302 - RNA, 21 nt, synthetic construct
  misc_feature 1..21: note = HBV RNAi Agent sense strand unmodified sequence
  source 1..21: mol_type = other RNA
gtggacttctctcaattttct

SEQ ID NO: 303 - RNA, 22 nt, synthetic construct
  misc_feature 1..22: note = HBV RNAi Agent sense strand unmodified sequence
  source 1..22: mol_type = other RNA
gctgtaggcataaattggtatt

SEQ ID NO: 304 - RNA, 23 nt, synthetic construct
  misc_feature 1..23: note = HBV RNAi Agent sense strand unmodified sequence
  source 1..23: mol_type = other RNA
ggctgtaggcataaattggtatt

SEQ ID NO: 305 - RNA, 23 nt, synthetic construct
  misc_feature 1..23: note = HBV RNAi Agent sense strand unmodified sequence
  source 1..23: mol_type = other RNA
aactgtaggcataaattggtatt

SEQ ID NO: 306 - RNA, 21 nt, synthetic construct
  misc_feature 1..21: note = HBV RNAi Agent sense strand unmodified sequence
  source 1..21: mol_type = other RNA
tggtggacttctctcaatatt

SEQ ID NO: 307 - RNA, 22 nt, synthetic construct
  misc_feature 1..22: note = HBV RNAi Agent sense strand unmodified sequence
  source 1..22: mol_type = other RNA
gtggtggacttctctcaatatt

SEQ ID NO: 308 - RNA, 23 nt, synthetic construct
  misc_feature 1..23: note = HBV RNAi Agent sense strand unmodified sequence
  source 1..23: mol_type = other RNA
aatggtggacttctctcaatatt

SEQ ID NO: 309 - RNA, 23 nt, synthetic construct
  misc_feature 1..23: note = HBV RNAi Agent sense strand unmodified sequence
  source 1..23: mol_type = other RNA
cgtggtggacttctctcaatatt

SEQ ID NO: 310 - RNA, 21 nt, synthetic construct
  misc_feature 1..21: note = HBV RNAi Agent sense strand unmodified sequence
  source 1..21: mol_type = other RNA
gtggtggacttctctcaaatt

SEQ ID NO: 311 - RNA, 22 nt, synthetic construct
  misc_feature 1..22: note = HBV RNAi Agent sense strand unmodified sequence
  source 1..22: mol_type = other RNA
cgtggtggacttctctcaaatt

SEQ ID NO: 312 - RNA, 23 nt, synthetic construct
  misc_feature 1..23: note = HBV RNAi Agent sense strand unmodified sequence
  source 1..23: mol_type = other RNA
aagtggtggacttctctcaaatt

SEQ ID NO: 313 - RNA, 23 nt, synthetic construct
  misc_feature 1..23: note = HBV RNAi Agent sense strand unmodified sequence
  source 1..23: mol_type = other RNA
tcgtggtggacttctctcaaatt

SEQ ID NO: 314 - RNA, 23 nt, synthetic construct
  misc_feature 1..23: note = HBV RNAi Agent sense strand unmodified sequence
  source 1..23: mol_type = other RNA
ctcgtggtggacttctctcaata

SEQ ID NO: 315 - RNA, 25 nt, synthetic construct
  misc_feature 1..25: note = HBV RNAi Agent sense strand unmodified sequence
  source 1..25: mol_type = other RNA
ctcgtggtggacttctctcaatatt

SEQ ID NO: 316 - RNA, 23 nt, synthetic construct
  misc_feature 1..23: note = HBV RNAi Agent sense strand unmodified sequence
  source 1..23: mol_type = other RNA
gaggctgtaggcataaattggta

SEQ ID NO: 317 - RNA, 25 nt, synthetic construct
  misc_feature 1..25: note = HBV RNAi Agent sense strand unmodified sequence
  source 1..25: mol_type = other RNA
gaggctgtaggcataaattggtatt

SEQ ID NO: 318 - RNA, 19 nt, synthetic construct
  misc_feature 1..19: note = HBV RNAi Agent sense strand unmodified sequence
  source 1..19: mol_type = other RNA
ggacttctctcaattttct

SEQ ID NO: 319 - RNA, 22 nt, synthetic construct
  misc_feature 1..22: note = HBV RNAi Agent sense strand unmodified sequence
  source 1..22: mol_type = other RNA
ggtggacttctctcaattttct

SEQ ID NO: 320 - RNA, 19 nt, synthetic construct
  misc_feature 1..19: note = HBV RNAi Agent sense strand unmodified sequence
  source 1..19: mol_type = other RNA
ggacttctctcaattttca

SEQ ID NO: 321 - RNA, 21 nt, synthetic construct
  misc_feature 1..21: note = HBV RNAi Agent sense strand unmodified sequence
  source 1..21: mol_type = other RNA
gtggacttctctcaattttca

SEQ ID NO: 322 - RNA, 19 nt, synthetic construct
  misc_feature 1..19: note = HBV RNAi Agent sense strand unmodified sequence
  source 1..19: mol_type = other RNA
gctgtaggcataaattggt

SEQ ID NO: 323 - RNA, 20 nt, synthetic construct
  misc_feature 1..20: note = HBV RNAi Agent sense strand unmodified sequence
  source 1..20: mol_type = other RNA
ggctgtaggcataaattggt

SEQ ID NO: 324 - RNA, 22 nt, synthetic construct
  misc_feature 1..22: note = HBV RNAi Agent sense strand unmodified sequence
  source 1..22: mol_type = other RNA
gaggctgtaggcataaattggt

SEQ ID NO: 325 - RNA, 19 nt, synthetic construct
  misc_feature 1..19: note = HBV RNAi Agent sense strand unmodified sequence
  source 1..19: mol_type = other RNA
gctgtaggcataaattgga

SEQ ID NO: 326 - RNA, 20 nt, synthetic construct
  misc_feature 1..20: note = HBV RNAi Agent sense strand unmodified sequence
  source 1..20: mol_type = other RNA
ggctgtaggcataaattgga

SEQ ID NO: 327 - RNA, 21 nt, synthetic construct
  misc_feature 1..21: note = HBV RNAi Agent sense strand unmodified sequence
  source 1..21: mol_type = other RNA
agctgtaggcataaattggta

SEQ ID NO: 328 - RNA, 21 nt, synthetic construct
  misc_feature 1..21: note = HBV RNAi Agent sense strand unmodified sequence
  source 1..21: mol_type = other RNA
cgctgtaggcataaattggta

SEQ ID NO: 329 - RNA, 21 nt, synthetic construct
  misc_feature 1..21: note = HBV RNAi Agent sense strand unmodified sequence
  source 1..21: mol_type = other RNA
ggctgtaggcataaattggtt

SEQ ID NO: 330 - RNA, 21 nt, synthetic construct
  misc_feature 1..21: note = HBV RNAi Agent sense strand unmodified sequence
  source 1..21: mol_type = other RNA
aggctgtaggcataaattggt

SEQ ID NO: 331 - RNA, 21 nt, synthetic construct
  misc_feature 1..21: note = HBV RNAi Agent sense strand unmodified sequence
  source 1..21: mol_type = other RNA
aggctgtaggcataaattgga

SEQ ID NO: 332 - RNA, 21 nt, synthetic construct
  misc_feature 1..21: note = HBV RNAi Agent sense strand unmodified sequence
  source 1..21: mol_type = other RNA
cggctgtaggcataaattggt

SEQ ID NO: 333 - RNA, 21 nt, synthetic construct
  misc_feature 1..21: note = HBV RNAi Agent sense strand unmodified sequence
  source 1..21: mol_type = other RNA
cggctgtaggcataaattgga

SEQ ID NO: 334 - RNA, 21 nt, synthetic construct
  misc_feature 1..21: note = HBV RNAi Agent sense strand unmodified sequence
  source 1..21: mol_type = other RNA
ccctgtaggcataaattggta